European Patent Specification EP 4 048 796 B1, published August 27, 2025. Title: Compositions and Methods Comprising Viral Vector Systems for Multiplexed Activation of Endogenous Genes as Immunotherapy and Viral-based Immune-Gene Therapy. Applicant: Yale University Chen, Sidi Wang, Guangchuan Chow, Ryan Zhang, Feifei. The sequence listing filed with the application follows.

SEQUENCE LISTING (411 sequences)

SEQ ID NO: 1 - DNA, 10185 bp, Artificial Sequence
  pGW059
ttaatgtagtcttatgcaatactcttgtagtcttgcaacatggtaacgatgagttagcaacatgccttacaaggagagaaaaagcaccgtgcatgccgattggtggaagtaaggtggtacgatcgtgccttattaggaaggcaacagacgggtctgacatggattggacgaaccactgaattgccgcattgcagagatattgtatttaagtgcctagctcgatacataaacgggtctctctggttagaccagatctgagcctgggagctctctggctaactagggaacccactgcttaagcctcaataaagcttgccttgagtgcttcaagtagtgtgtgcccgtctgttgtgtgactctggtaactagagatccctcagacccttttagtcagtgtggaaaatctctagcagtggcgcccgaacagggacttgaaagcgaaagggaaaccagaggagctctctcgacgcaggactcggcttgctgaagcgcgcacggcaagaggcgaggggcggcgactggtgagtacgccaaaaattttgactagcggaggctagaaggagagagatgggtgcgagagcgtcagtattaagcgggggagaattagatcgcgatgggaaaaaattcggttaaggccagggggaaagaaaaaatataaattaaaacatatagtatgggcaagcagggagctagaacgattcgcagttaatcctggcctgttagaaacatcagaaggctgtagacaaatactgggacagctacaaccatcccttcagacaggatcagaagaacttagatcattatataatacagtagcaaccctctattgtgtgcatcaaaggatagagataaaagacaccaaggaagctttagacaagatagaggaagagcaaaacaaaagtaagaccaccgcacagcaagcggccgctgatcttcagacctggaggaggagatatgagggacaattggagaagtgaattatataaatataaagtagtaaaaattgaaccattaggagtagcacccaccaaggcaaagagaagagtggtgcagagagaaaaaagagcagtgggaataggagctttgttccttgggttcttgggagcagcaggaagcactatgggcgcagcgtcaatgacgctgacggtacaggccagacaattattgtctggtatagtgcagcagcagaacaatttgctgagggctattgaggcgcaacagcatctgttgcaactcacagtctggggcatcaagcagctccaggcaagaatcctggctgtggaaagatacctaaaggatcaacagctcctggggatttggggttgctctggaaaactcatttgcaccactgctgtgccttggaatgctagttggagtaataaatctctggaacagatttggaatcacacgacctggatggagtgggacagagaaattaacaattacacaagcttaatacactccttaattgaagaatcgcaaaaccagcaagaaaagaatgaacaagaattattggaattagataaatgggcaagtttgtggaattggtttaacataacaaattggctgtggtatataaaattattcataatgatagtaggaggcttggtaggtttaagaatagtttttgctgtactttctatagtgaatagagttaggcagggatattcaccattatcgtttcagacccacctcccaaccccgaggggaccctctagagatccgacgcgccatctctaggcccgcgccggccccctcgcacggacttgtgggagaagctcggctactcccctgccccggttaatttgcatataatatttcctagtaactatagaggcttaatgtgcgataaaagacagataatctgttctttttaatactagctacattttacatgataggcttggatttctataacttcgtatagcatacattatacgaagttataaacagcacaaaaggaaactcaccctaactgtaaagtaattgtgtgttttgagactataagtatcccttggagaaccaccttgttgggagacgggataccgtctctgtttaagagctaagctggccaacatgaggatcacccatgtctgcagggccagcttagcaagttaaaataaggctagtccgttatcaacttggccaacatgaggatcacccatgtctgcagggccaagtggcaccgagtcggtgcttttttggatccaagcttggcgtaactagatcttgagacaaatggcagtattcatccacaattttaaaagaaaaggggggattggggggtacagtgcaggggaaagaatagtagacataatagcaacagacatacaaactaaagaattacaaaaacaaattacaaaaattcaaaattttcgggtttattacagggacagcagagatccactttggcgccggctcgagggggcccgggtgcaaagatggataaagttttaaacagagaggaatctttgcagctaatggaccttctaggtcttgaaaggagtgggaattggctccggtgcccgtcagtgggcagagcgcacatcgcccacagtccccgagaagttggggggaggggtcggcaattgatccggtgcctagagaaggtggcgcggggtaaactgggaaagtgatgtcgtgtactggctccgcctttttcccgagggtgggggagaaccgtatataagtgcagtagtcgccgtgaacgttctttttcgcaacgggtttgccgccagaacacaggtaagtgccgtgtgtggttcccgcgggcctggcctctttacgggttatggcccttgcgtgccttgaattacttccactggctgcagtacgtgattcttgatcccgagcttcgggttggaagtgggtgggagagttcgaggccttgcgcttaaggagccccttcgcctcgtgcttgagttgaggcctggcctgggcgctggggccgccgcgtgcgaatctggtggcaccttcgcgcctgtctcgctgctttcgataagtctctagccatttaaaatttttgatgacctgctgcgacgctttttttctggcaagatagtcttgtaaatgcgggccaagatctgcacactggtatttcggtttttggggccgcgggcggcgacggggcccgtgcgtcccagcgcacatgttcggcgaggcggggcctgcgagcgcggccaccgagaatcggacgggggtagtctcaagctggccggcctgctctggtgcctggcctcgcgccgccgtgtatcgccccgccctgggcggcaaggctggcccggtcggcaccagttgcgtgagcggaaagatggccgcttcccggccctgctgcagggagctcaaaatggaggacgcggcgctcgggagagcgggcgggtgagtcacccacacaaaggaaaagggcctttccgtcctcagccgtcgcttcatgtgactccacggagtaccgggcgccgtccaggcacctcgattagttctcgagcttttggagtacgtcgtctttaggttggggggaggggttttatgcgatggagtttccccacactgagtgggtggagactgaagttaggccagcttggcacttgatgtaattctccttggaatttgccctttttgagtttggatcttggttcattctcaagcctcagacagtggttcaaagtttttttcttccatttcaggtgtcgtgacgtacggccaccatgaccgagtacaagcccacggtgcgcctcgccacccgcgacgacgtccccagggccgtacgcaccctcgccgccgcgttcgccgactaccccgccacgcgccacaccgtcgatccggaccgccacatcgagcgggtcaccgagctgcaagaactcttcctcacgcgcgtcgggctcgacatcggcaaggtgtgggtcgcggacgacggcgccgccgtggcggtctggaccacgccggagagcgtcgaagcgggggcggtgttcgccgagatcggcccgcgcatggccgagttgagcggttcccggctggccgcgcagcaacagatggaaggcctcctggcgccgcaccggcccaaggagcccgcgtggttcctggccaccgtcggagtctcgcccgaccaccagggcaagggtctgggcagcgccgtcgtgctccccggagtggaggcggccgagcgcgccggggtgcccgccttcctggagacctccgcgccccgcaacctccccttctacgagcggctcggcttcaccgtcaccgccgacgtcgaggtgcccgaaggaccgcgcacctggtgcatgacccgcaagcccggtgccggatccggcgcaacaaacttctctctgctgaaacaagccggagatgtcgaagagaatcctggaccgatggaagacgccaaaaacataaagaaaggcccggcgccattctatccgctggaagatggaaccgctggagagcaactgcataaggctatgaagagatacgccctggttcctggaacaattgcttttacagatgcacatatcgaggtggacatcacttacgctgagtacttcgaaatgtccgttcggttggcagaagctatgaaacgatatgggctgaatacaaatcacagaatcgtcgtatgcagtgaaaactctcttcaattctttatgccggtgttgggcgcgttatttatcggagttgcagttgcgcccgcgaacgacatttataatgaacgtgaattgctcaacagtatgggcatttcgcagcctaccgtggtgttcgtttccaaaaaggggttgcaaaaaattttgaacgtgcaaaaaaagctcccaatcatccaaaaaattattatcatggattctaaaacggattaccagggatttcagtcgatgtacacgttcgtcacatctcatctacctcccggttttaatgaatacgattttgtgccagagtccttcgatagggacaagacaattgcactgatcatgaactcctctggatctactggtctgcctaaaggtgtcgctctgcctcatagaactgcctgcgtgagattctcgcatgccagagatcctatttttggcaatcaaatcattccggatactgcgattttaagtgttgttccattccatcacggttttggaatgtttactacactcggatatttgatatgtggatttcgagtcgtcttaatgtatagatttgaagaggagctgtttctgaggagccttcaggattacaagattcaaagtgcgctgctggtgccaaccctattctccttcttcgccaaaagcactctgattgacaaatacgatttatctaatttacacgaaattgcttctggtggcgctcccctctctaaggaagtcggggaagcggttgccaagaggttccatctgccaggtatcaggcaaggatatgggctcactgagactacatcagctattctgattacacccgagggggatgataaaccgggcgcggtcggtaaagttgttccattttttgaagcgaaggttgtggatctggataccgggaaaacgctgggcgttaatcaaagaggcgaactgtgtgtgagaggtcctatgattatgtccggttatgtaaacaatccggaagcgaccaacgccttgattgacaaggatggatggctacattctggagacatagcttactgggacgaagacgaacacttcttcatcgttgaccgcctgaagtctctgattaagtacaaaggctatcaggtggctcccgctgaattggaatccatcttgctccaacaccccaacatcttcgacgcaggtgtcgcaggtcttcccgacgatgacgccggtgaacttcccgccgccgttgttgttttggagcacggaaagacgatgacggaaaaagagatcgtggattacgtcgccagtcaagtaacaaccgcgaaaaagttgcgcggaggagttgtgtttgtggacgaagtaccgaaaggtcttaccggaaaactcgacgcaagaaaaatcagagagatcctcataaaggccaagaagggcggaaagatcgccgtgtaagaattcacgcgttaagtcgacaatcaacctctggattacaaaatttgtgaaagattgactggtattcttaactatgttgctccttttacgctatgtggatacgctgctttaatgcctttgtatcatgctattgcttcccgtatggctttcattttctcctccttgtataaatcctggttgctgtctctttatgaggagttgtggcccgttgtcaggcaacgtggcgtggtgtgcactgtgtttgctgacgcaacccccactggttggggcattgccaccacctgtcagctcctttccgggactttcgctttccccctccctattgccacggcggaactcatcgccgcctgccttgcccgctgctggacaggggctcggctgttgggcactgacaattccgtggtgttgtcggggaaatcatcgtcctttccttggctgctcgcctgtgttgccacctggattctgcgcgggacgtccttctgctacgtcccttcggccctcaatccagcggaccttccttcccgcggcctgctgccggctctgcggcctcttccgcgtcttcgccttcgccctcagacgagtcggatctccctttgggccgcctccccgcgtcgactttaagaccaatgacttacaaggcagctgtagatcttagccactttttaaaagaaaaggggggactggaagggctaattcactcccaacgaagacaagatctgctttttgcttgtactgggtctctctggttagaccagatctgagcctgggagctctctggctaactagggaacccactgcttaagcctcaataaagcttgccttgagtgcttcaagtagtgtgtgcccgtctgttgtgtgactctggtaactagagatccctcagacccttttagtcagtgtggaaaatctctagcagtacgtatagtagttcatgtcatcttattattcagtatttataacttgcaaagaaatgaatatcagagagtgagaggaacttgtttattgcagcttataatggttacaaataaagcaatagcatcacaaatttcacaaataaagcatttttttcactgcattctagttgtggtttgtccaaactcatcaatgtatcttatcatgtctggctctagctatcccgcccctaactccgcccatcccgcccctaactccgcccagttccgcccattctccgccccatggctgactaattttttttatttatgcagaggccgaggccgcctcggcctctgagctattccagaagtagtgaggaggcttttttggaggcctagggacgtacccaattcgccctatagtgagtcgtattacgcgcgctcactggccgtcgttttacaacgtcgtgactgggaaaaccctggcgttacccaacttaatcgccttgcagcacatccccctttcgccagctggcgtaatagcgaagaggcccgcaccgatcgcccttcccaacagttgcgcagcctgaatggcgaatgggacgcgccctgtagcggcgcattaagcgcggcgggtgtggtggttacgcgcagcgtgaccgctacacttgccagcgccctagcgcccgctcctttcgctttcttcccttcctttctcgccacgttcgccggctttccccgtcaagctctaaatcgggggctccctttagggttccgatttagtgctttacggcacctcgaccccaaaaaacttgattagggtgatggttcacgtagtgggccatcgccctgatagacggtttttcgccctttgacgttggagtccacgttctttaatagtggactcttgttccaaactggaacaacactcaaccctatctcggtctattcttttgatttataagggattttgccgatttcggcctattggttaaaaaatgagctgatttaacaaaaatttaacgcgaattttaacaaaatattaacgcttacaatttaggtggcacttttcggggaaatgtgcgcggaacccctatttgtttatttttctaaatacattcaaatatgtatccgctcatgagacaataaccctgataaatgcttcaataatattgaaaaaggaagagtatgagtattcaacatttccgtgtcgcccttattcccttttttgcggcattttgccttcctgtttttgctcacccagaaacgctggtgaaagtaaaagatgctgaagatcagttgggtgcacgagtgggttacatcgaactggatctcaacagcggtaagatccttgagagttttcgccccgaagaacgttttccaatgatgagcacttttaaagttctgctatgtggcgcggtattatcccgtattgacgccgggcaagagcaactcggtcgccgcatacactattctcagaatgacttggttgagtactcaccagtcacagaaaagcatcttacggatggcatgacagtaagagaattatgcagtgctgccataaccatgagtgataacactgcggccaacttacttctgacaacgatcggaggaccgaaggagctaaccgcttttttgcacaacatgggggatcatgtaactcgccttgatcgttgggaaccggagctgaatgaagccataccaaacgacgagcgtgacaccacgatgcctgtagcaatggcaacaacgttgcgcaaactattaactggcgaactacttactctagcttcccggcaacaattaatagactggatggaggcggataaagttgcaggaccacttctgcgctcggcccttccggctggctggtttattgctgataaatctggagccggtgagcgtgggtctcgcggtatcattgcagcactggggccagatggtaagccctcccgtatcgtagttatctacacgacggggagtcaggcaactatggatgaacgaaatagacagatcgctgagataggtgcctcactgattaagcattggtaactgtcagaccaagtttactcatatatactttagattgatttaaaacttcatttttaatttaaaaggatctaggtgaagatcctttttgataatctcatgaccaaaatcccttaacgtgagttttcgttccactgagcgtcagaccccgtagaaaagatcaaaggatcttcttgagatcctttttttctgcgcgtaatctgctgcttgcaaacaaaaaaaccaccgctaccagcggtggtttgtttgccggatcaagagctaccaactctttttccgaaggtaactggcttcagcagagcgcagataccaaatactgttcttctagtgtagccgtagttaggccaccacttcaagaactctgtagcaccgcctacatacctcgctctgctaatcctgttaccagtggctgctgccagtggcgataagtcgtgtcttaccgggttggactcaagacgatagttaccggataaggcgcagcggtcgggctgaacggggggttcgtgcacacagcccagcttggagcgaacgacctacaccgaactgagatacctacagcgtgagctatgagaaagcgccacgcttcccgaagggagaaaggcggacaggtatccggtaagcggcagggtcggaacaggagagcgcacgagggagcttccagggggaaacgcctggtatctttatagtcctgtcgggtttcgccacctctgacttgagcgtcgatttttgtgatgctcgtcaggggggcggagcctatggaaaaacgccagcaacgcggcctttttacggttcctggccttttgctggccttttgctcacatgttctttcctgcgttatcccctgattctgtggataaccgtattaccgcctttgagtgagctgataccgctcgccgcagccgaacgaccgagcgcagcgagtcagtgagcgaggaagcggaagagcgcccaatacgcaaaccgcctctccccgcgcgttggccgattcattaatgcagctggcacgacaggtttcccgactggaaagcgggcagtgagcgcaacgcaattaatgtgagttagctcactcattaggcaccccaggctttacactttatgcttccggctcgtatgttgtgtggaattgtgagcggataacaatttcacacaggaaacagctatgaccatgattacgccaagcgcgcaattaaccctcactaaagggaacaaaagctggagctgcaagc

SEQ ID NO: 2 - DNA, 7138 bp, Artificial Sequence
  pGW066
cctgcaggcagctgcgcgctcgctcgctcactgaggccgcccgggcgtcgggcgacctttggtcgcccggcctcagtgagcgagcgagcgcgcagagagggagtggccaactccatcactaggggttcctgcggcctctagaaaggatctgcgatcgctccggtgcccgtcagtgggcagagcgcacatcgcccacagtccccgagaagttggggggaggggtcggcaattgaacgggtgcctagagaaggtggcgcggggtaaactgggaaagtgatgtcgtgtactggctccgcctttttcccgagggtgggggagaaccgtatataagtgcagtagtcgccgtgaacgttctttttcgcaacgggtttgccgccagaacacagctgaagcttcgaggggctcgcatctctccttcacgcgcccgccgccctacctgaggccgccatccacgccggttgagtcgcgttctgccgcctcccgcctgtggtgcctcctgaactgcgtccgccgtctaggtaagtttaaagctcaggtcgagaccgggcctttgtccggcgctcccttggagcctacctagactcagccggctctccacgctttgcctgaccctgcttgctcaactctacgtctttgtttcgttttctgttctgcgccgttacagatctggctaactaccggtgccaccatggcttgcaattgtcagttgatgcaggatacaccactcctcaagtttccatgtccaaggctcattcttctctttgtgctgctgattcgtctttcacaagtgtcttcagatgttgatgaacaactgtccaagtcagtgaaagataaggtattgctgccttgccgttacaactctcctcatgaagatgagtctgaagaccgaatctactggcaaaaacatgacaaagtggtgctgtctgtcattgctgggaaactaaaagtgtggcccgagtataagaaccggactttatatgacaacactacctactctcttatcatcctgggcctggtcctttcagaccggggcacatacagctgtgtcgttcaaaagaaggaaagaggaacgtatgaagttaaacacttggctttagtaaagttgtccatcaaagctgacttctctacccccaacataactgagtctggaaacccatctgcagacactaaaaggattacctgctttgcttccgggggtttcccaaagcctcgcttctcttggttggaaaatggaagagaattacctggcatcaatacgacaatttcccaggatcctgaatctgaattgtacaccattagtagccaactagatttcaatacgactcgcaaccacaccattaagtgtctcattaaatatggagatgctcacgtgtcagaggacttcacctgggaaaaacccccagaagaccctcctgatagcaagaacacacttgtgctctttggggcaggattcggcgcagtaataacagtcgtcgtcatcgttgtcatcatcaaatgcttctgtaagcacagaagctgtttcagaagaaatgaggcaagcagagaaacaaacaacagccttaccttcgggcctgaagaagcattagctgaacagaccgtcttccttcgtacgggcagtggagagggcagaggaagtctgctaacatgcggtgacgtcgaggagaatcctggcccaatggagagtgtggtacagccttcagtgtttgtggtggatggacagacggacatcccattcaggcggctggaacagaaccaccggagacggcgctgtggcactgtccaggtcagcctggccctggtgctgctgctaagtgctgggctggccactcagggctggtttctcctgagactgcatcaacgtcttggagacatagtagctcatctgccagatggaggcaaaggctcctgggagaagctgatacaagatcaacgatctcaccaggccaacccagcagcacatcttacaggagccaacgccagcttgataggtattggtggacctctgttatgggagacacgacttggcctggccttcttgaggggcttgacgtatcatgatggggccctggtgaccatggagcccggttactactatgtgtactccaaagtgcagctgagcggcgtgggctgcccccaggggctggccaatggcctccccatcacccatggactatacaagcgcacatcccgctacccgaaggagttagaactgctggtcagtcggcggtcaccctgtggccgggccaacagctcccgagtctggtgggacagcagcttcctgggcggcgtggtacatctggaggctggggaagaggtggtggtccgcgtgcctggaaaccgcctggtcagaccacgtgacggcaccaggtcctatttcggagctttcatggtcactagtggatccggcgcaacaaacttctctctgctgaaacaagccggagatgtcgaagagaatcctggaccgatgaacccaagtgctgccgtcattttctgcctcatcctgctgggtctgagtgggactcaagggatccctctcgcaaggacggtccgctgcaactgcatccatatcgatgacgggccagtgagaatgagggccatagggaagcttgaaatcatccctgcgagcctatcctgcccacgtgttgagatcattgccacgatgaaaaagaatgatgagcagagatgtctgaatccggaatctaagaccatcaagaatttaatgaaagcgtttagccaaaaaaggtctaaaagggctcctgctagcagcggtacccagtgcaccaactacgccctgctgaagctggccggcgatgtggagagcaaccccgggcccatggaccagcacacacttgatgtggaggataccgcggatgccagacatccagcaggtacttcgtgcccctcggatgcggcgctcctcagagataccgggctcctcgcggacgctgcgctcctctcagatactgtgcgccccacaaatgccgcgctccccacggatgctgcctaccctgcggttaatgttcgggatcgcgaggccgcgtggccgcctgcactgaacttctgttcccgccacccaaagctctatggcctagtcgctttggttttgctgcttctgatcgccgcctgtgttcctatcttcacccgcaccgagcctcggccagcgctcacaatcaccacctcgcccaacctgggtacccgagagaataatgcagaccaggtcacccctgtttcccacattggctgccccaacactacacaacagggctctcctgtgttcgccaagctactggctaaaaaccaagcatcgttgtgcaatacaactctgaactggcacagccaagatggagctgggagctcatacctatctcaaggtctgaggtacgaagaagacaaaaaggagttggtggtagacagtcccgggctctactacgtatttttggaactgaagctcagtccaacattcacaaacacaggccacaaggtgcagggctgggtctctcttgttttgcaagcaaagcctcaggtagatgactttgacaacttggccctgacagtggaactgttcccttgctccatggagaacaagttagtggaccgttcctggagtcaactgttgctcctgaaggctggccaccgcctcagtgtgggtctgagggcttatctgcatggagcccaggatgcatacagagactgggagctgtcttatcccaacaccaccagctttggactctttcttatgaaacccgacaacccatgggaatgagaattcacgcgttaagtcgacaatcaacctctggattacaaaatttgtgaaagattgactggtattcttaactatgttgctccttttacgctatgtggatacgctgctttaatgcctttgtatcatgctattgcttcccgtatggctttcattttctcctccttgtataaatcctggttgctgtctctttatgaggagttgtggcccgttgtcaggcaacgtggcgtggtgtgcactgtgtttgctgacgcaacccccactggttggggcattgccaccacctgtcagctcctttccgggactttcgctttccccctccctattgccacggcggaactcatcgccgcctgccttgcccgctgctggacaggggctcggctgttgggcactgacaattccgtggtgttgtcggggaaatcatcgtcctttccttggctgctcgcctgtgttgccacctggattctgcgcgggacgtccttctgctacgtcccttcggccctcaatccagcggaccttccttcccgcggcctgctgccggctctgcggcctcttccgcgtcttcgccttcgccctcagacgagtcggatctccctttgggccgcctccccgcgtcgactttaagaccaatgacggccgcaggaacccctagtgatggagttggccactccctctctgcgcgctcgctcgctcactgaggccgggcgaccaaaggtcgcccgacgcccgggctttgcccgggcggcctcagtgagcgagcgagcgcgcagctgcctgcaggggcgcctgatgcggtattttctccttacgcatctgtgcggtatttcacaccgcatacgtcaaagcaaccatagtacgcgccctgtagcggcgcattaagcgcggcgggtgtggtggttacgcgcagcgtgaccgctacacttgccagcgccttagcgcccgctcctttcgctttcttcccttcctttctcgccacgttcgccggctttccccgtcaagctctaaatcgggggctccctttagggttccgatttagtgctttacggcacctcgaccccaaaaaacttgatttgggtgatggttcacgtagtgggccatcgccctgatagacggtttttcgccctttgacgttggagtccacgttctttaatagtggactcttgttccaaactggaacaacactcaactctatctcgggctattcttttgatttataagggattttgccgatttcggtctattggttaaaaaatgagctgatttaacaaaaatttaacgcgaattttaacaaaatattaacgtttacaattttatggtgcactctcagtacaatctgctctgatgccgcatagttaagccagccccgacacccgccaacacccgctgacgcgccctgacgggcttgtctgctcccggcatccgcttacagacaagctgtgaccgtctccgggagctgcatgtgtcagaggttttcaccgtcatcaccgaaacgcgcgagacgaaagggcctcgtgatacgcctatttttataggttaatgtcatgataataatggtttcttagacgtcaggtggcacttttcggggaaatgtgcgcggaacccctatttgtttatttttctaaatacattcaaatatgtatccgctcatgagacaataaccctgataaatgcttcaataatattgaaaaaggaagagtatgagtattcaacatttccgtgtcgcccttattcccttttttgcggcattttgccttcctgtttttgctcacccagaaacgctggtgaaagtaaaagatgctgaagatcagttgggtgcacgagtgggttacatcgaactggatctcaacagcggtaagatccttgagagttttcgccccgaagaacgttttccaatgatgagcacttttaaagttctgctatgtggcgcggtattatcccgtattgacgccgggcaagagcaactcggtcgccgcatacactattctcagaatgacttggttgagtactcaccagtcacagaaaagcatcttacggatggcatgacagtaagagaattatgcagtgctgccataaccatgagtgataacactgcggccaacttacttctgacaacgatcggaggaccgaaggagctaaccgcttttttgcacaacatgggggatcatgtaactcgccttgatcgttgggaaccggagctgaatgaagccataccaaacgacgagcgtgacaccacgatgcctgtagcaatggcaacaacgttgcgcaaactattaactggcgaactacttactctagcttcccggcaacaattaatagactggatggaggcggataaagttgcaggaccacttctgcgctcggcccttccggctggctggtttattgctgataaatctggagccggtgagcgtggaagccgcggtatcattgcagcactggggccagatggtaagccctcccgtatcgtagttatctacacgacggggagtcaggcaactatggatgaacgaaatagacagatcgctgagataggtgcctcactgattaagcattggtaactgtcagaccaagtttactcatatatactttagattgatttaaaacttcatttttaatttaaaaggatctaggtgaagatcctttttgataatctcatgaccaaaatcccttaacgtgagttttcgttccactgagcgtcagaccccgtagaaaagatcaaaggatcttcttgagatcctttttttctgcgcgtaatctgctgcttgcaaacaaaaaaaccaccgctaccagcggtggtttgtttgccggatcaagagctaccaactctttttccgaaggtaactggcttcagcagagcgcagataccaaatactgttcttctagtgtagccgtagttaggccaccacttcaagaactctgtagcaccgcctacatacctcgctctgctaatcctgttaccagtggctgctgccagtggcgataagtcgtgtcttaccgggttggactcaagacgatagttaccggataaggcgcagcggtcgggctgaacggggggttcgtgcacacagcccagcttggagcgaacgacctacaccgaactgagatacctacagcgtgagctatgagaaagcgccacgcttcccgaagggagaaaggcggacaggtatccggtaagcggcagggtcggaacaggagagcgcacgagggagcttccagggggaaacgcctggtatctttatagtcctgtcgggtttcgccacctctgacttgagcgtcgatttttgtgatgctcgtcaggggggcggagcctatggaaaaacgccagcaacgcggcctttttacggttcctggccttttgctggccttttgctcacatgt

SEQ ID NO: 3 - DNA, 7109 bp, Artificial Sequence
  pGW067
cctgcaggcagctgcgcgctcgctcgctcactgaggccgcccgggcgtcgggcgacctttggtcgcccggcctcagtgagcgagcgagcgcgcagagagggagtggccaactccatcactaggggttcctgcggcctctagaaaggatctgcgatcgctccggtgcccgtcagtgggcagagcgcacatcgcccacagtccccgagaagttggggggaggggtcggcaattgaacgggtgcctagagaaggtggcgcggggtaaactgggaaagtgatgtcgtgtactggctccgcctttttcccgagggtgggggagaaccgtatataagtgcagtagtcgccgtgaacgttctttttcgcaacgggtttgccgccagaacacagctgaagcttcgaggggctcgcatctctccttcacgcgcccgccgccctacctgaggccgccatccacgccggttgagtcgcgttctgccgcctcccgcctgtggtgcctcctgaactgcgtccgccgtctaggtaagtttaaagctcaggtcgagaccgggcctttgtccggcgctcccttggagcctacctagactcagccggctctccacgctttgcctgaccctgcttgctcaactctacgtctttgtttcgttttctgttctgcgccgttacagatctggctaactaccggtgccaccatggcttgcaattgtcagttgatgcaggatacaccactcctcaagtttccatgtccaaggctcattcttctctttgtgctgctgattcgtctttcacaagtgtcttcagatgttgatgaacaactgtccaagtcagtgaaagataaggtattgctgccttgccgttacaactctcctcatgaagatgagtctgaagaccgaatctactggcaaaaacatgacaaagtggtgctgtctgtcattgttgggaaactaaaagtgtggcccgagtataagaaccggactttatatgacaacactacctactctcttatcatcctgggcctggtcctttcagaccggggcacatacagctgtgtcgttcaaaagaaggaaagaggaacgtatgaagttaaacacttggctttagtaaagttgtccatcaaagctgacttctctacccccaacataactgagtctggaaacccatctgcagacactaaaaggattacctgctttgcttccgggggtttcccaaagcctcgcttctcttggttggaaaatggaagagaattacctggcatcaatacgacaatttcccaggatcctgaatctgaattgtacaccattagtagccaactagatttcaatacgactcgcaaccacaccattaagtgtctcattaaatatggagatgctcacgtgtcagaggacttcacctgggaaaaacccccagaagaccctcctgatagcaagaacacacttgtgctctttggggcaggattcggcgcagtaataacagtcgtcgtcatcgttgtcatcatcaaatgcttctgtaagcacagaagctgtttcagaagaaatgaggcaagcagagaaacaaacaacagccttaccttcgggcctgaagaagcattagctgaacagaccgtcttccttcgtacgggcagtggagagggcagaggaagtctgctaacatgcggtgacgtcgaggagaatcctggcccaatggagagtgtggtacagccttcagtgtttgtggtggatggacagacggacatcccattcaggcggctggaacagaaccaccggagacggcgctgtggcactgtccaggtcagcctggccctggtgctgctgctaggtgctgggctggccactcagggctggtttctcctgagactgcatcaacgtcttggagacatagtagctcatctgccagatggaggcaaaggctcctgggagaagctgatacaagatcaacgatctcaccaggccaacccagcagcacatcttacaggagccaacgccagcttgataggtattggtggacctctgttatgggagacacgacttggcctggccttcttgaggggcttgacgtatcatgatggggccctggtgaccatggagcccggttactactatgtgtactccaaagtgcagctgagcggcgtgggctgcccccaggggctggccaatggcctccccatcacccatggactatacaagcgcacatcccgctacccgaaggagttagaactgctggtcagtcggcggtcaccctgtggccgggccaacagctcccgagtctggtgggacagcagcttcctgggcggcgtggtacatctggaggctggggaagaggtggtggtccgcgtgcctggaaaccgcctggtcagaccacgtgacggcaccaggtcctatttcggagctttcatggtcactagtggatccggcgcaacaaacttctctctgctgaaacaagccggagatgtcgaagagaatcctggaccgatgaacccaagtgctgccgtcattttctgcctcatcctgctgggtctgagtgggactcaagggatccctctcgcaaggacggtccgctgcaactgcatccatatcgatgacgggccagtgagaatgagggccatagggaagcttgaaatcatccctgcgagcctatcctgcccacgtgttgagatcattgccacgatgaaaaagaatgatgagcagagatgtctgaatccggaatctaagaccatcaagaatttaatgaaagcgtttagccaaaaaaggtctaaaagggctcctgctagcagcggtacccagtgcaccaactacgccctgctgaagctggccggcgatgtggagagcaaccccgggcccatggaccagcacacacttgatgtggaggataccgcggatgccagacatccagcaggtacttcgtgcccctcggatgcggcgctcctcagagataccgggctcctcgcggacgctgcgctcctctcagatactgtgcgccccacaaatgccgcgctccccacggatgctgcctaccctgcggttaatgttcgggatcgcgaggccgcgtggccgcctgcactgaacttctgttcccgccacccaaagctctatggcctagtcgctttggttttgctgcttctgatcgccgcctgtgttcctatcttcacccgcaccgagcctcggccagcgctcacaatcaccacctcgcccaacctgggtacccgagagaataatgcagaccaggtcacccctgtttcccacattggctgccccaacactacacaacagggctctcctgtgttcgccaagctactggctaaaaaccaagcatcgttgtgcaatacaactctgaactggcacagccaagatggagctgggagctcatacctatctcaaggtctgaggtacgaagaagacaaaaaggagttggtggtagacagtcccgggctctactacgtatttttggaactgaagctcagtccaacattcacaaacacaggccacaaggtgcagggctgggtctctcttgttttgcaagcaaagcctcaggtagatgactttgacaacttggccctgacagtggaactgttcccttgctccatggagaacaagttagtggaccgttcctggagtcaactgttgctcctgaaggctggccaccgcctcagtgtgggtctgagggcttatctgcatggagcccaggatgcatacagagactgggagctgtcttatcccaacaccaccagctttggactctttcttgtgaaacccgacaacccatgggaaggcatatgcggtaccgtgaagcagaccctgaacttcgatctgctgaagctggccggcgatgtggagagcaaccccgggcccatgaacgctacacactgcatcttggctttgcagctcttcctcatggctgtttctggctgttactgccacggcacagtcattgaaagcctagaaagtctgaataactattttaactcaagtggcatagatgtggaagaaaagagtctcttcttggatatctggaggaactggcaaaaggatggtgacatgaaaatcctgcagagccagattatctctttctacctcagactctttgaagtcttgaaagacaatcaggccatcagcaacaacataagcgtcattgaatcacacctgattactaccttcttcagcaacagcaaggcgaaaaaggatgcattcatgagtattgccaagtttgaggtcaacaacccacaggtccagcgccaagcattcaatgagctcatccgagtggtccaccagctgttgccggaatccagcctcaggaagcggaaaaggagtcgctgctgagaattcaataaaagatctttattttcattagatctgtgtgttggttttttgtgtgcggccgcaggaacccctagtgatggagttggccactccctctctgcgcgctcgctcgctcactgaggccgggcgaccaaaggtcgcccgacgcccgggctttgcccgggcggcctcagtgagcgagcgagcgcgcagctgcctgcaggggcgcctgatgcggtattttctccttacgcatctgtgcggtatttcacaccgcatacgtcaaagcaaccatagtacgcgccctgtagcggcgcattaagcgcggcgggtgtggtggttacgcgcagcgtgaccgctacacttgccagcgccttagcgcccgctcctttcgctttcttcccttcctttctcgccacgttcgccggctttccccgtcaagctctaaatcgggggctccctttagggttccgatttagtgctttacggcacctcgaccccaaaaaacttgatttgggtgatggttcacgtagtgggccatcgccctgatagacggtttttcgccctttgacgttggagtccacgttctttaatagtggactcttgttccaaactggaacaacactcaactctatctcgggctattcttttgatttataagggattttgccgatttcggtctattggttaaaaaatgagctgatttaacaaaaatttaacgcgaattttaacaaaatattaacgtttacaattttatggtgcactctcagtacaatctgctctgatgccgcatagttaagccagccccgacacccgccaacacccgctgacgcgccctgacgggcttgtctgctcccggcatccgcttacagacaagctgtgaccgtctccgggagctgcatgtgtcagaggttttcaccgtcatcaccgaaacgcgcgagacgaaagggcctcgtgatacgcctatttttataggttaatgtcatgataataatggtttcttagacgtcaggtggcacttttcggggaaatgtgcgcggaacccctatttgtttatttttctaaatacattcaaatatgtatccgctcatgagacaataaccctgataaatgcttcaataatattgaaaaaggaagagtatgagtattcaacatttccgtgtcgcccttattcccttttttgcggcattttgccttcctgtttttgctcacccagaaacgctggtgaaagtaaaagatgctgaagatcagttgggtgcacgagtgggttacatcgaactggatctcaacagcggtaagatccttgagagttttcgccccgaagaacgttttccaatgatgagcacttttaaagttctgctatgtggcgcggtattatcccgtattgacgccgggcaagagcaactcggtcgccgcatacactattctcagaatgacttggttgagtactcaccagtcacagaaaagcatcttacggatggcatgacagtaagagaattatgcagtgctgccataaccatgagtgataacactgcggccaacttacttctgacaacgatcggaggaccgaaggagctaaccgcttttttgcacaacatgggggatcatgtaactcgccttgatcgttgggaaccggagctgaatgaagccataccaaacgacgagcgtgacaccacgatgcctgtagcaatggcaacaacgttgcgcaaactattaactggcgaactacttactctagcttcccggcaacaattaatagactggatggaggcggataaagttgcaggaccacttctgcgctcggcccttccggctggctggtttattgctgataaatctggagccggtgagcgtggaagccgcggtatcattgcagcactggggccagatggtaagccctcccgtatcgtagttatctacacgacggggagtcaggcaactatggatgaacgaaatagacagatcgctgagataggtgcctcactgattaagcattggtaactgtcagaccaagtttactcatatatactttagattgatttaaaacttcatttttaatttaaaaggatctaggtgaagatcctttttgataatctcatgaccaaaatcccttaacgtgagttttcgttccactgagcgtcagaccccgtagaaaagatcaaaggatcttcttgagatcctttttttctgcgcgtaatctgctgcttgcaaacaaaaaaaccaccgctaccagcggtggtttgtttgccggatcaagagctaccaactctttttccgaaggtaactggcttcagcagagcgcagataccaaatactgttcttctagtgtagccgtagttaggccaccacttcaagaactctgtagcaccgcctacatacctcgctctgctaatcctgttaccagtggctgctgccagtggcgataagtcgtgtcttaccgggttggactcaagacgatagttaccggataaggcgcagcggtcgggctgaacggggggttcgtgcacacagcccagcttggagcgaacgacctacaccgaactgagatacctacagcgtgagctatgagaaagcgccacgcttcccgaagggagaaaggcggacaggtatccggtaagcggcagggtcggaacaggagagcgcacgagggagcttccagggggaaacgcctggtatctttatagtcctgtcgggtttcgccacctctgacttgagcgtcgatttttgtgatgctcgtcaggggggcggagcctatggaaaaacgccagcaacgcggcctttttacggttcctggccttttgctggccttttgctcacatgt

SEQ ID NO: 4 - DNA, 13393 bp, Artificial Sequence
  pGW029
  misc_feature (9532)..(9534): n is a, c, g, or t
  misc_feature (9549)..(9551): n is a, c, g, or t
  misc_feature (11851)..(11856): n is a, c, g, or t
ctacagggcgcgtccattcgccattcaggatcgaattaattcttaattaacatcatcaataatataccttattttggattgaagccaatatgataatgagggggtggagtttgtgacgtggcgcggggcgtgggaacggggcgggtgacgtagtagtgtggcggaagtgtgatgttgcaagtgtggcggaacacatgtaagcgacggatgtggcaaaagtgacgtttttggtgtgcgccggtgtacacaggaagtgacaattttcgcgcggttttaggcggatgttgtagtaaatttgggcgtaaccgagtaagatttggccattttcgcgggaaaactgaataagaggaagtgaaatctgaataattttgtgttactcatagcgcgtaatactggtaccgcggccgcctcgagtctagaaagagggcctatttcccatgattccttcatatttgcatatacgatacaaggctgttagagagataattagaattaatttgactgtaaacacaaagatattagtacaaaatacgtgacgtagaaagtaataatttcttgggtagtttgcagttttaaaattatgttttaaaatggactatcatatgcttaccgtaacttgaaagtatttcgatttcttggctttatatatcttgtggaaaggacgaaacaccggaagagcgagctcttctgttttagagctaggccaacatgaggatcacccatgtctgcagggcctagcaagttaaaataaggctagtccgttatcaacttggccaacatgaggatcacccatgtctgcagggccaagtggcaccgagtcggtgcttttttgctagcgtcagtgggcagagcgcacatcgcccacagtccccgagaagttggggggaggggtcggcaattgaacgggtgcctagagaaggtggcgcggggtaaactgggaaagtgatgtcgtgtactggctccgcctttttcccgagggtgggggagaaccgtatataagtgcagtagtcgccgtgaacgttctttttcgcaacgggtttgccgccagaacacagctgaagcttcgaggggctcgcatctctccttcacgcgcccgccgccctacctgaggccgccatccacgccggttgagtcgcgttctgccgcctcccgcctgtggtgcctcctgaactgcgtccgccgtctaggtaagtttaaagctcaggtcgagaccgggcctttgtccggcgctcccttggagcctacctagactcagccggctctccacgctttgcctgaccctgcttgctcaactctacgtctttgtttcgttttctgttctgcgccgttacagatccaagctcgtacggccaccatgaaaaggccggcggccacgaaaaaggccggccaggcaaaaaagaaaaaggacaagaagtacagcatcggcctggccatcggcaccaactctgtgggctgggccgtgatcaccgacgagtacaaggtgcccagcaagaaattcaaggtgctgggcaacaccgaccggcacagcatcaagaagaacctgatcggagccctgctgttcgacagcggcgaaacagccgaggccacccggctgaagagaaccgccagaagaagatacaccagacggaagaaccggatctgctatctgcaagagatcttcagcaacgagatggccaaggtggacgacagcttcttccacagactggaagagtccttcctggtggaagaggataagaagcacgagcggcaccccatcttcggcaacatcgtggacgaggtggcctaccacgagaagtaccccaccatctaccacctgagaaagaaactggtggacagcaccgacaaggccgacctgcggctgatctatctggccctggcccacatgatcaagttccggggccacttcctgatcgagggcgacctgaaccccgacaacagcgacgtggacaagctgttcatccagctggtgcagacctacaaccagctgttcgaggaaaaccccatcaacgccagcggcgtggacgccaaggccatcctgtctgccagactgagcaagagcagacggctggaaaatctgatcgcccagctgcccggcgagaagaagaatggcctgttcggcaacctgattgccctgagcctgggcctgacccccaacttcaagagcaacttcgacctggccgaggatgccaaactgcagctgagcaaggacacctacgacgacgacctggacaacctgctggcccagatcggcgaccagtacgccgacctgtttctggccgccaagaacctgtccgacgccatcctgctgagcgacatcctgagagtgaacaccgagatcaccaaggcccccctgagcgcctctatgatcaagagatacgacgagcaccaccaggacctgaccctgctgaaagctctcgtgcggcagcagctgcctgagaagtacaaagagattttcttcgaccagagcaagaacggctacgccggctacattgacggcggagccagccaggaagagttctacaagttcatcaagcccatcctggaaaagatggacggcaccgaggaactgctcgtgaagctgaacagagaggacctgctgcggaagcagcggaccttcgacaacggcagcatcccccaccagatccacctgggagagctgcacgccattctgcggcggcaggaagatttttacccattcctgaaggacaaccgggaaaagatcgagaagatcctgaccttccgcatcccctactacgtgggccctctggccaggggaaacagcagattcgcctggatgaccagaaagagcgaggaaaccatcaccccctggaacttcgaggaagtggtggacaagggcgcttccgcccagagcttcatcgagcggatgaccaacttcgataagaacctgcccaacgagaaggtgctgcccaagcacagcctgctgtacgagtacttcaccgtgtataacgagctgaccaaagtgaaatacgtgaccgagggaatgagaaagcccgccttcctgagcggcgagcagaaaaaggccatcgtggacctgctgttcaagaccaaccggaaagtgaccgtgaagcagctgaaagaggactacttcaagaaaatcgagtgcttcgactccgtggaaatctccggcgtggaagatcggttcaacgcctccctgggcacataccacgatctgctgaaaattatcaaggacaaggacttcctggacaatgaggaaaacgaggacattctggaagatatcgtgctgaccctgacactgtttgaggacagagagatgatcgaggaacggctgaaaacctatgcccacctgttcgacgacaaagtgatgaagcagctgaagcggcggagatacaccggctggggcaggctgagccggaagctgatcaacggcatccgggacaagcagtccggcaagacaatcctggatttcctgaagtccgacggcttcgccaacagaaacttcatgcagctgatccacgacgacagcctgacctttaaagaggacatccagaaagcccaggtgtccggccagggcgatagcctgcacgagcacattgccaatctggccggcagccccgccattaagaagggcatcctgcagacagtgaaggtggtggacgagctcgtgaaagtgatgggccggcacaagcccgagaacatcgtgatcgaaatggccagagagaaccagaccacccagaagggacagaagaacagccgcgagagaatgaagcggatcgaagagggcatcaaagagctgggcagccagatcctgaaagaacaccccgtggaaaacacccagctgcagaacgagaagctgtacctgtactacctgcagaatgggcgggatatgtacgtggaccaggaactggacatcaaccggctgtccgactacgatgtggaccacatcgtgcctcagagctttctgaaggacgactccatcgacaacaaggtgctgaccagaagcgacaaggcccggggcaagagcgacaacgtgccctccgaagaggtcgtgaagaagatgaagaactactggcggcagctgctgaacgccaagctgattacccagagaaagttcgacaatctgaccaaggccgagagaggcggcctgagcgaactggataaggccggcttcatcaagagacagctggtggaaacccggcagatcacaaagcacgtggcacagatcctggactcccggatgaacactaagtacgacgagaatgacaagctgatccgggaagtgaaagtgatcaccctgaagtccaagctggtgtccgatttccggaaggatttccagttttacaaagtgcgcgagatcaacaactaccaccacgcccacgacgcctacctgaacgccgtcgtgggaaccgccctgatcaaaaagtaccctaagctggaaagcgagttcgtgtacggcgactacaaggtgtacgacgtgcggaagatgatcgccaagagcgagcaggaaatcggcaaggctaccgccaagtacttcttctacagcaacatcatgaactttttcaagaccgagattaccctggccaacggcgagatccggaagcggcctctgatcgagacaaacggcgaaaccggggagatcgtgtgggataagggccgggattttgccaccgtgcggaaagtgctgagcatgccccaagtgaatatcgtgaaaaagaccgaggtgcagacaggcggcttcagcaaagagtctatcctgcccaagaggaacagcgataagctgatcgccagaaagaaggactgggaccctaagaagtacggcggcttcgacagccccaccgtggcctattctgtgctggtggtggccaaagtggaaaagggcaagtccaagaaactgaagagtgtgaaagagctgctggggatcaccatcatggaaagaagcagcttcgagaagaatcccatcgactttctggaagccaagggctacaaagaagtgaaaaaggacctgatcatcaagctgcctaagtactccctgttcgagctggaaaacggccggaagagaatgctggcctctgccggcgaactgcagaagggaaacgaactggccctgccctccaaatatgtgaacttcctgtacctggccagccactatgagaagctgaagggctcccccgaggataatgagcagaaacagctgtttgtggaacagcacaagcactacctggacgagatcatcgagcagatcagcgagttctccaagagagtgatcctggccgacgctaatctggacaaagtgctgtccgcctacaacaagcaccgggataagcccatcagagagcaggccgagaatatcatccacctgtttaccctgaccaatctgggagcccctgccgccttcaagtactttgacaccaccatcgaccggaagaggtacaccagcaccaaagaggtgctggacgccaccctgatccaccagagcatcaccggcctgtacgagacacggatcgacctgtctcagctgggaggcgacagcgctggaggacctaagaaaaagaggaaggtgggatccggacgggctgacgcattggacgattttgatctggatatgctgggaagtgacgccctcgatgattttgaccttgacatgcttggttcggatgcccttgatgactttgacctcgacatgctcggcagtgacgcccttgatgatttcgacctggacatgctgattaactgtacaggaagcggagccactaacttctccctgttgaaacaagcaggggatgtcgaagagaatcccgggccagccaccatggcttcaaactttactcagttcgtgctcgtggacaatggtgggacaggggatgtgacagtggctccttctaatttcgctaatggggtggcagagtggatcagctccaactcacggagccaggcctacaaggtgacatgcagcgtcaggcagtctagtgcccagaagagaaagtataccatcaaggtggaggtccccaaagtggctacccagacagtgggcggagtcgaactgcctgtcgccgcttggaggtcctacctgaacatggagctcactatcccaattttcgctaccaattctgactgtgaactcatcgtgaaggcaatgcaggggctcctcaaagacggtaatcctatcccttccgccatcgccgctaactcaggtatctacagcgctggaggaggtggaagcggaggaggaggaagcggaggaggaggtagcggacctaagaaaaagaggaaggtggcggccgctggatccccttcagggcagatcagcaaccaggccctggctctggcccctagctccgctccagtgctggcccagactatggtgccctctagtgctatggtgcctctggcccagccacctgctccagcccctgtgctgaccccaggaccaccccagtcactgagcgctccagtgcccaagtctacacaggccggcgaggggactctgagtgaagctctgctgcacctgcagttcgacgctgatgaggacctgggagctctgctggggaacagcaccgatcccggagtgttcacagatctggcctccgtggacaactctgagtttcagcagctgctgaatcagggcgtgtccatgtctcatagtacagccgaaccaatgctgatggagtaccccgaagccattacccggctggtgaccggcagccagcggccccccgaccccgctccaactcccctgggaaccagcggcctgcctaatgggctgtccggagatgaagacttctcaagcatcgctgatatggactttagtgccctgctgtcacagatttcctctagtgggcagggaggaggtggaagcggcttcagcgtggacaccagtgccctgctggacctgttcagcccctcggtgaccgtgcccgacatgagcctgcctgaccttgacagcagcctggccagtatccaagagctcctgtctccccaggagccccccaggcctcccgaggcagagaacagcagcccggattcagggaagcagctggtgcactacacagcgcagccgctgttcctgctggaccccggctccgtggacaccgggagcaacgacctgccggtgctgtttgagctgggagagggctcctacttctccgaaggggacggcttcgccgaggaccccaccatctccctgctgacaggctcggagcctcccaaagccaaggaccccactgtctcctaagaattcgatatcaagcttaataaaagatctttattttcattagatctgtgtgttggttttttgtgtagatctgggcgtggttaagggtgggaaagaatatataaggtgggggtcttatgtagttttgtatctgttttgcagcagccgccgccgccatgagcaccaactcgtttgatggaagcattgtgagctcatatttgacaacgcgcatgcccccatgggccggggtgcgtcagaatgtgatgggctccagcattgatggtcgccccgtcctgcccgcaaactctactaccttgacctacgagaccgtgtctggaacgccgttggagactgcagcctccgccgccgcttcagccgctgcagccaccgcccgcgggattgtgactgactttgctttcctgagcccgcttgcaagcagtgcagcttcccgttcatccgcccgcgatgacaagttgacggctcttttggcacaattggattctttgacccgggaacttaatgtcgtttctcagcagctgttggatctgcgccagcaggtttctgccctgaaggcttcctcccctcccaatgcggtttaaaacataaataaaaaaccagactctgtttggatttggatcaagcaagtgtcttgctgtctttatttaggggttttgcgcgcgcggtaggcccgggaccagcggtctcggtcgttgagggtcctgtgtattttttccaggacgtggtaaaggtgactctggatgttcagatacatgggcataagcccgtctctggggtggaggtagcaccactgcagagcttcatgctgcggggtggtgttgtagatgatccagtcgtagcaggagcgctgggcgtggtgcctaaaaatgtctttcagtagcaagctgattgccaggggcaggcccttggtgtaagtgtttacaaagcggttaagctgggatgggtgcatacgtggggatatgagatgcatcttggactgtatttttaggttggctatgttcccagccatatccctccggggattcatgttgtgcagaaccaccagcacagtgtatccggtgcacttgggaaatttgtcatgtagcttagaaggaaatgcgtggaagaacttggagacgcccttgtgacctccaagattttccatgcattcgtccataatgatggcaatgggcccacgggcggcggcctgggcgaagatatttctgggatcactaacgtcatagttgtgttccaggatgagatcgtcataggccatttttacaaagcgcgggcggagggtgccagactgcggtataatggttccatccggcccaggggcgtagttaccctcacagatttgcatttcccacgctttgagttcagatggggggatcatgtctacctgcggggcgatgaagaaaacggtttccggggtaggggagatcagctgggaagaaagcaggttcctgagcagctgcgacttaccgcagccggtgggcccgtaaatcacacctattaccgggtgcaactggtagttaagagagctgcagctgccgtcatccctgagcaggggggccacttcgttaagcatgtccctgactcgcatgttttccctgaccaaatccgccagaaggcgctcgccgcccagcgatagcagttcttgcaaggaagcaaagtttttcaacggtttgagaccgtccgccgtaggcatgcttttgagcgtttgaccaagcagttccaggcggtcccacagctcggtcacctgctctacggcatctcgatccagcatatctcctcgtttcgcgggttggggcggctttcgctgtacggcagtagtcggtgctcgtccagacgggccagggtcatgtctttccacgggcgcagggtcctcgtcagcgtagtctgggtcacggtgaaggggtgcgctccgggctgcgcgctggccagggtgcgcttgaggctggtcctgctggtgctgaagcgctgccggtcttcgccctgcgcgtcggccaggtagcatttgaccatggtgtcatagtccagcccctccgcggcgtggcccttggcgcgcagcttgcccttggaggaggcgccgcacgaggggcagtgcagacttttgagggcgtagagcttgggcgcgagaaataccgattccggggagtaggcatccgcgccgcaggccccgcagacggtctcgcattccacgagccaggtgagctctggccgttcggggtcaaaaaccaggtttcccccatgctttttgatgcgtttcttacctctggtttccatgagccggtgtccacgctcggtgacgaaaaggctgtccgtgtccccgtatacagactnnngtttaaacgaattcnnntataaaatgcaaggtgctgctcaaaaaatcaggcaaagcctcgcgcaaaaaagaaagcacatcgtagtcatgctcatgcagataaaggcaggtaagctccggaaccaccacagaaaaagacaccatttttctctcaaacatgtctgcgggtttctgcataaacacaaaataaaataacaaaaaaacatttaaacattagaagcctgtcttacaacaggaaaaacaacccttataagcataagacggactacggccatgccggcgtgaccgtaaaaaaactggtcaccgtgattaaaaagcaccaccgacagctcctcggtcatgtccggagtcataatgtaagactcggtaaacacatcaggttgattcatcggtcagtgctaaaaagcgaccgaaatagcccgggggaatacatacccgcaggcgtagagacaacattacagcccccataggaggtataacaaaattaataggagagaaaaacacataaacacctgaaaaaccctcctgcctaggcaaaatagcaccctcccgctccagaacaacatacagcgcttcacagcggcagcctaacagtcagccttaccagtaaaaaagaaaacctattaaaaaaacaccactcgacacggcaccagctcaatcagtcacagtgtaaaaaagggccaagtgcagagcgagtatatataggactaaaaaatgacgtaacggttaaagtccacaaaaaacacccagaaaaccgcacgcgaacctacgcccagaaacgaaagccaaaaaacccacaacttcctcaaatcgtcacttccgttttcccacgttacgtaacttcccattttaagaaaactacaattcccaacacatacaagttactccgccctaaaacctacgtcacccgccccgttcccacgccccgcgccacgtcacaaactccaccccctcattatcatattggcttcaatccaaaataaggtatattattgatgattaattaattaaggatcccggtgtgaaataccgcacagatgcgtaaggagaaaataccgcatcaggcgctcttacgcttcctcgctcactgactcgctgcgctcggtcgttcggctgcggcgagcggtatcagctcactcaaaggcggtaatacggttatccacagaatcaggggataacgcaggaaagaacatgtgagcaaaaggccagcaaaaggccaggaaccgtaaaaaggccgcgttgctggcgtttttccataggctccgcccccctgacgagcatcacaaaaatcgacgctcaagtcagaggtggcgaaacccgacaggactataaagataccaggcgtttccccctggaagctccctcgtgcgctctcctgttccgaccctgccgcttaccggatacctgtccgcctttctcccttcgggaagcgtggcgctttctcatagctcacgctgtaggtatctcagttcggtgtaggtcgttcgctccaagctgggctgtgtgcacgaaccccccgttcagcccgaccgctgcgccttatccggtaactatcgtcttgagtccaacccggtaagacacgacttatcgccactggcagcagccactggtaacaggattagcagagcgaggtatgtaggcggtgctacagagttcttgaagtggtggcctaactacggctacactagaaggacagtatttggtatctgcgctctgctgaagccagttaccttcggaaaaagagttggtagctcttgatccggcaaacaaaccaccgctggtagcggtggtttttttgtttgcaagcagcagattacgcgcagaaaaaaaggatctcaagaagatcctttgatcttttctacggggtctgacgctcagtggaacgaaaactcacgttaagggattttggtcatgagattatcaaaaaggatcttcacctagatccttttaaattaaaaatgaagttttaaatcaatctaaagtatatatgagtaaacttggtctgacagttaccaatgcttaatcagtgaggcacctatctcagcgatctgtctatttcgttcatccatagttgcctgactccccgtcgtgtagataactacgatacgggagggcttaccatctggccccagtgctgcaatgataccgcgagacccacgctcaccggctccagatttatcagcaataaaccagccagccggaagggccgagcgcagaagtggtcctgcaactttatccgcctccatccagtctattaattgttgccgggaagctagagtaagtagttcgccagttaatagtttgcgcaacgttgttgnnnnnnaaaaaggatcttcacctagatccttttcacgtagaaagccagtccgcagaaacggtgctgaccccggatgaatgtcagctactgggctatctggacaagggaaaacgcaagcgcaaagagaaagcaggtagcttgcagtgggcttacatggcgatagctagactgggcggttttatggacagcaagcgaaccggaattgccagctggggcgccctctggtaaggttgggaagccctgcaaagtaaactggatggctttctcgccgccaaggatctgatggcgcaggggatcaagctctgatcaagagacaggatgaggatcgtttcgcatgattgaacaagatggattgcacgcaggttctccggccgcttgggtggagaggctattcggctatgactgggcacaacagacaatcggctgctctgatgccgccgtgttccggctgtcagcgcaggggcgcccggttctttttgtcaagaccgacctgtccggtgccctgaatgaactgcaagacgaggcagcgcggctatcgtggctggccacgacgggcgttccttgcgcagctgtgctcgacgttgtcactgaagcgggaagggactggctgctattgggcgaagtgccggggcaggatctcctgtcatctcaccttgctcctgccgagaaagtatccatcatggctgatgcaatgcggcggctgcatacgcttgatccggctacctgcccattcgaccaccaagcgaaacatcgcatcgagcgagcacgtactcggatggaagccggtcttgtcgatcaggatgatctggacgaggagcatcaggggctcgcgccagccgaactgttcgccaggctcaaggcgagcatgcccgacggcgaggatctcgtcgtgacccatggcgatgcctgcttgccgaatatcatggtggaaaatggccgcttttctggattcatcgactgtggccggctgggtgtggcggaccgctatcaggacatagcgttggctacccgtgatattgctgaggagcttggcggcgaatgggctgaccgcttcctcgtgctttacggtatcgccgctcccgattcgcagcgcatcgccttctatcgccttcttgacgagttcttctgaattttgttaaaatttttgttaaatcagctcattttttaaccaataggccgaaatcggcaacatcccttataaatcaaaagaatagaccgcgatagggttgagtgttgttccagtttggaacaagagtccactattaaagaacgtggactccaacgtcaaagggcgaaaaaccgtctatcagggcgatggcccactacgtgaaccatcacccaaatcaagttttttgcggtcgaggtgccgtaaagctctaaatcggaaccctaaagggagcccccgatttagagcttgacggggaaagccggcgaacgtggcgagaaaggaagggaagaaagcgaaaggagcgggcgctagggcgctggcaagtgtagcggtcacgctgcgcgtaaccaccacacccgcgcgcttaatgcgccg

SEQ ID NO: 5 - DNA, 13444 bp, Artificial Sequence
  pGW035
  misc_feature (9583)..(9585): n is a, c, g, or t
  misc_feature (9600)..(9602): n is a, c, g, or t
  misc_feature (11902)..(11907): n is a, c, g, or t
ctacagggcgcgtccattcgccattcaggatcgaattaattcttaattaacatcatcaataatataccttattttggattgaagccaatatgataatgagggggtggagtttgtgacgtggcgcggggcgtgggaacggggcgggtgacgtagtagtgtggcggaagtgtgatgttgcaagtgtggcggaacacatgtaagcgacggatgtggcaaaagtgacgtttttggtgtgcgccggtgtacacaggaagtgacaattttcgcgcggttttaggcggatgttgtagtaaatttgggcgtaaccgagtaagatttggccattttcgcgggaaaactgaataagaggaagtgaaatctgaataattttgtgttactcatagcgcgtaatactggtaccgcggccgcctcgagtctagaaagagggcctatttcccatgattccttcatatttgcatatacgatacaaggctgttagagagataattagaattaatttgactgtaaacacaaagatattagtacaaaatacgtgacgtagaaagtaataatttcttgggtagtttgcagttttaaaattatgttttaaaatggactatcatatgcttaccgtaacttgaaagtatttcgatttcttggctttatatatcttgtggaaaggacgaaacaccggaagagcgagctcttctgttttagagctaggccaacatgaggatcacccatgtctgcagggcctagcaagttaaaataaggctagtccgttatcaacttggccaacatgaggatcacccatgtctgcagggccaagtggcaccgagtcggtgcttttttgctagcgtcagtgggcagagcgcacatcgcccacagtccccgagaagttggggggaggggtcggcaattgaacgggtgcctagagaaggtggcgcggggtaaactgggaaagtgatgtcgtgtactggctccgcctttttcccgagggtgggggagaaccgtatataagtgcagtagtcgccgtgaacgttctttttcgcaacgggtttgccgccagaacacagctgaagcttcgaggggctcgcatctctccttcacgcgcccgccgccctacctgaggccgccatccacgccggttgagtcgcgttctgccgcctcccgcctgtggtgcctcctgaactgcgtccgccgtctaggtaagtttaaagctcaggtcgagaccgggcctttgtccggcgctcccttggagcctacctagactcagccggctctccacgctttgcctgaccctgcttgctcaactctacgtctttgtttcgttttctgttctgcgccgttacagatccaagctcgtacggccaccatgaaaaggccggcggccacgaaaaaggccggccaggcaaaaaagaaaaaggacaagaagtacagcatcggcctggccatcggcaccaactctgtgggctgggccgtgatcaccgacgagtacaaggtgcccagcaagaaattcaaggtgctgggcaacaccgaccggcacagcatcaagaagaacctgatcggagccctgctgttcgacagcggcgaaacagccgaggccacccggctgaagagaaccgccagaagaagatacaccagacggaagaaccggatctgctatctgcaagagatcttcagcaacgagatggccaaggtggacgacagcttcttccacagactggaagagtccttcctggtggaagaggataagaagcacgagcggcaccccatcttcggcaacatcgtggacgaggtggcctaccacgagaagtaccccaccatctaccacctgagaaagaaactggtggacagcaccgacaaggccgacctgcggctgatctatctggccctggcccacatgatcaagttccggggccacttcctgatcgagggcgacctgaaccccgacaacagcgacgtggacaagctgttcatccagctggtgcagacctacaaccagctgttcgaggaaaaccccatcaacgccagcggcgtggacgccaaggccatcctgtctgccagactgagcaagagcagacggctggaaaatctgatcgcccagctgcccggcgagaagaagaatggcctgttcggcaacctgattgccctgagcctgggcctgacccccaacttcaagagcaacttcgacctggccgaggatgccaaactgcagctgagcaaggacacctacgacgacgacctggacaacctgctggcccagatcggcgaccagtacgccgacctgtttctggccgccaagaacctgtccgacgccatcctgctgagcgacatcctgagagtgaacaccgagatcaccaaggcccccctgagcgcctctatgatcaagagatacgacgagcaccaccaggacctgaccctgctgaaagctctcgtgcggcagcagctgcctgagaagtacaaagagattttcttcgaccagagcaagaacggctacgccggctacattgacggcggagccagccaggaagagttctacaagttcatcaagcccatcctggaaaagatggacggcaccgaggaactgctcgtgaagctgaacagagaggacctgctgcggaagcagcggaccttcgacaacggcagcatcccccaccagatccacctgggagagctgcacgccattctgcggcggcaggaagatttttacccattcctgaaggacaaccgggaaaagatcgagaagatcctgaccttccgcatcccctactacgtgggccctctggccaggggaaacagcagattcgcctggatgaccagaaagagcgaggaaaccatcaccccctggaacttcgaggaagtggtggacaagggcgcttccgcccagagcttcatcgagcggatgaccaacttcgataagaacctgcccaacgagaaggtgctgcccaagcacagcctgctgtacgagtacttcaccgtgtataacgagctgaccaaagtgaaatacgtgaccgagggaatgagaaagcccgccttcctgagcggcgagcagaaaaaggccatcgtggacctgctgttcaagaccaaccggaaagtgaccgtgaagcagctgaaagaggactacttcaagaaaatcgagtgcttcgactccgtggaaatctccggcgtggaagatcggttcaacgcctccctgggcacataccacgatctgctgaaaattatcaaggacaaggacttcctggacaatgaggaaaacgaggacattctggaagatatcgtgctgaccctgacactgtttgaggacagagagatgatcgaggaacggctgaaaacctatgcccacctgttcgacgacaaagtgatgaagcagctgaagcggcggagatacaccggctggggcaggctgagccggaagctgatcaacggcatccgggacaagcagtccggcaagacaatcctggatttcctgaagtccgacggcttcgccaacagaaacttcatgcagctgatccacgacgacagcctgacctttaaagaggacatccagaaagcccaggtgtccggccagggcgatagcctgcacgagcacattgccaatctggccggcagccccgccattaagaagggcatcctgcagacagtgaaggtggtggacgagctcgtgaaagtgatgggccggcacaagcccgagaacatcgtgatcgaaatggccagagagaaccagaccacccagaagggacagaagaacagccgcgagagaatgaagcggatcgaagagggcatcaaagagctgggcagccagatcctgaaagaacaccccgtggaaaacacccagctgcagaacgagaagctgtacctgtactacctgcagaatgggcgggatatgtacgtggaccaggaactggacatcaaccggctgtccgactacgatgtggaccacatcgtgcctcagagctttctgaaggacgactccatcgacaacaaggtgctgaccagaagcgacaaggcccggggcaagagcgacaacgtgccctccgaagaggtcgtgaagaagatgaagaactactggcggcagctgctgaacgccaagctgattacccagagaaagttcgacaatctgaccaaggccgagagaggcggcctgagcgaactggataaggccggcttcatcaagagacagctggtggaaacccggcagatcacaaagcacgtggcacagatcctggactcccggatgaacactaagtacgacgagaatgacaagctgatccgggaagtgaaagtgatcaccctgaagtccaagctggtgtccgatttccggaaggatttccagttttacaaagtgcgcgagatcaacaactaccaccacgcccacgacgcctacctgaacgccgtcgtgggaaccgccctgatcaaaaagtaccctaagctggaaagcgagttcgtgtacggcgactacaaggtgtacgacgtgcggaagatgatcgccaagagcgagcaggaaatcggcaaggctaccgccaagtacttcttctacagcaacatcatgaactttttcaagaccgagattaccctggccaacggcgagatccggaagcggcctctgatcgagacaaacggcgaaaccggggagatcgtgtgggataagggccgggattttgccaccgtgcggaaagtgctgagcatgccccaagtgaatatcgtgaaaaagaccgaggtgcagacaggcggcttcagcaaagagtctatcctgcccaagaggaacagcgataagctgatcgccagaaagaaggactgggaccctaagaagtacggcggcttcgacagccccaccgtggcctattctgtgctggtggtggccaaagtggaaaagggcaagtccaagaaactgaagagtgtgaaagagctgctggggatcaccatcatggaaagaagcagcttcgagaagaatcccatcgactttctggaagccaagggctacaaagaagtgaaaaaggacctgatcatcaagctgcctaagtactccctgttcgagctggaaaacggccggaagagaatgctggcctctgccggcgaactgcagaagggaaacgaactggccctgccctccaaatatgtgaacttcctgtacctggccagccactatgagaagctgaagggctcccccgaggataatgagcagaaacagctgtttgtggaacagcacaagcactacctggacgagatcatcgagcagatcagcgagttctccaagagagtgatcctggccgacgctaatctggacaaagtgctgtccgcctacaacaagcaccgggataagcccatcagagagcaggccgagaatatcatccacctgtttaccctgaccaatctgggagcccctgccgccttcaagtactttgacaccaccatcgaccggaagaggtacaccagcaccaaagaggtgctggacgccaccctgatccaccagagcatcaccggcctgtacgagacacggatcgacctgtctcagctgggaggcgacagcgctggaggaggtggaagcggaggaggaggaagcggaggaggaggtagcggacctaagaaaaagaggaaggtggcggccgctggatccggacgggctgacgcattggacgattttgatctggatatgctgggaagtgacgccctcgatgattttgaccttgacatgcttggttcggatgcccttgatgactttgacctcgacatgctcggcagtgacgcccttgatgatttcgacctggacatgctgattaactgtacaggaagcggagccactaacttctccctgttgaaacaagcaggggatgtcgaagagaatcccgggccagccaccatggcttcaaactttactcagttcgtgctcgtggacaatggtgggacaggggatgtgacagtggctccttctaatttcgctaatggggtggcagagtggatcagctccaactcacggagccaggcctacaaggtgacatgcagcgtcaggcagtctagtgcccagaagagaaagtataccatcaaggtggaggtccccaaagtggctacccagacagtgggcggagtcgaactgcctgtcgccgcttggaggtcctacctgaacatggagctcactatcccaattttcgctaccaattctgactgtgaactcatcgtgaaggcaatgcaggggctcctcaaagacggtaatcctatcccttccgccatcgccgctaactcaggtatctacagcgctggaggaggtggaagcggaggaggaggaagcggaggaggaggtagcggacctaagaaaaagaggaaggtggcggccgctggatccccttcagggcagatcagcaaccaggccctggctctggcccctagctccgctccagtgctggcccagactatggtgccctctagtgctatggtgcctctggcccagccacctgctccagcccctgtgctgaccccaggaccaccccagtcactgagcgctccagtgcccaagtctacacaggccggcgaggggactctgagtgaagctctgctgcacctgcagttcgacgctgatgaggacctgggagctctgctggggaacagcaccgatcccggagtgttcacagatctggcctccgtggacaactctgagtttcagcagctgctgaatcagggcgtgtccatgtctcatagtacagccgaaccaatgctgatggagtaccccgaagccattacccggctggtgaccggcagccagcggccccccgaccccgctccaactcccctgggaaccagcggcctgcctaatgggctgtccggagatgaagacttctcaagcatcgctgatatggactttagtgccctgctgtcacagatttcctctagtgggcagggaggaggtggaagcggcttcagcgtggacaccagtgccctgctggacctgttcagcccctcggtgaccgtgcccgacatgagcctgcctgaccttgacagcagcctggccagtatccaagagctcctgtctccccaggagccccccaggcctcccgaggcagagaacagcagcccggattcagggaagcagctggtgcactacacagcgcagccgctgttcctgctggaccccggctccgtggacaccgggagcaacgacctgccggtgctgtttgagctgggagagggctcctacttctccgaaggggacggcttcgccgaggaccccaccatctccctgctgacaggctcggagcctcccaaagccaaggaccccactgtctcctaagaattcgatatcaagcttaataaaagatctttattttcattagatctgtgtgttggttttttgtgtagatctgggcgtggttaagggtgggaaagaatatataaggtgggggtcttatgtagttttgtatctgttttgcagcagccgccgccgccatgagcaccaactcgtttgatggaagcattgtgagctcatatttgacaacgcgcatgcccccatgggccggggtgcgtcagaatgtgatgggctccagcattgatggtcgccccgtcctgcccgcaaactctactaccttgacctacgagaccgtgtctggaacgccgttggagactgcagcctccgccgccgcttcagccgctgcagccaccgcccgcgggattgtgactgactttgctttcctgagcccgcttgcaagcagtgcagcttcccgttcatccgcccgcgatgacaagttgacggctcttttggcacaattggattctttgacccgggaacttaatgtcgtttctcagcagctgttggatctgcgccagcaggtttctgccctgaaggcttcctcccctcccaatgcggtttaaaacataaataaaaaaccagactctgtttggatttggatcaagcaagtgtcttgctgtctttatttaggggttttgcgcgcgcggtaggcccgggaccagcggtctcggtcgttgagggtcctgtgtattttttccaggacgtggtaaaggtgactctggatgttcagatacatgggcataagcccgtctctggggtggaggtagcaccactgcagagcttcatgctgcggggtggtgttgtagatgatccagtcgtagcaggagcgctgggcgtggtgcctaaaaatgtctttcagtagcaagctgattgccaggggcaggcccttggtgtaagtgtttacaaagcggttaagctgggatgggtgcatacgtggggatatgagatgcatcttggactgtatttttaggttggctatgttcccagccatatccctccggggattcatgttgtgcagaaccaccagcacagtgtatccggtgcacttgggaaatttgtcatgtagcttagaaggaaatgcgtggaagaacttggagacgcccttgtgacctccaagattttccatgcattcgtccataatgatggcaatgggcccacgggcggcggcctgggcgaagatatttctgggatcactaacgtcatagttgtgttccaggatgagatcgtcataggccatttttacaaagcgcgggcggagggtgccagactgcggtataatggttccatccggcccaggggcgtagttaccctcacagatttgcatttcccacgctttgagttcagatggggggatcatgtctacctgcggggcgatgaagaaaacggtttccggggtaggggagatcagctgggaagaaagcaggttcctgagcagctgcgacttaccgcagccggtgggcccgtaaatcacacctattaccgggtgcaactggtagttaagagagctgcagctgccgtcatccctgagcaggggggccacttcgttaagcatgtccctgactcgcatgttttccctgaccaaatccgccagaaggcgctcgccgcccagcgatagcagttcttgcaaggaagcaaagtttttcaacggtttgagaccgtccgccgtaggcatgcttttgagcgtttgaccaagcagttccaggcggtcccacagctcggtcacctgctctacggcatctcgatccagcatatctcctcgtttcgcgggttggggcggctttcgctgtacggcagtagtcggtgctcgtccagacgggccagggtcatgtctttccacgggcgcagggtcctcgtcagcgtagtctgggtcacggtgaaggggtgcgctccgggctgcgcgctggccagggtgcgcttgaggctggtcctgctggtgctgaagcgctgccggtcttcgccctgcgcgtcggccaggtagcatttgaccatggtgtcatagtccagcccctccgcggcgtggcccttggcgcgcagcttgcccttggaggaggcgccgcacgaggggcagtgcagacttttgagggcgtagagcttgggcgcgagaaataccgattccggggagtaggcatccgcgccgcaggccccgcagacggtctcgcattccacgagccaggtgagctctggccgttcggggtcaaaaaccaggtttcccccatgctttttgatgcgtttcttacctctggtttccatgagccggtgtccacgctcggtgacgaaaaggctgtccgtgtccccgtatacagactnnngtttaaacgaattcnnntataaaatgcaaggtgctgctcaaaaaatcaggcaaagcctcgcgcaaaaaagaaagcacatcgtagtcatgctcatgcagataaaggcaggtaagctccggaaccaccacagaaaaagacaccatttttctctcaaacatgtctgcgggtttctgcataaacacaaaataaaataacaaaaaaacatttaaacattagaagcctgtcttacaacaggaaaaacaacccttataagcataagacggactacggccatgccggcgtgaccgtaaaaaaactggtcaccgtgattaaaaagcaccaccgacagctcctcggtcatgtccggagtcataatgtaagactcggtaaacacatcaggttgattcatcggtcagtgctaaaaagcgaccgaaatagcccgggggaatacatacccgcaggcgtagagacaacattacagcccccataggaggtataacaaaattaataggagagaaaaacacataaacacctgaaaaaccctcctgcctaggcaaaatagcaccctcccgctccagaacaacatacagcgcttcacagcggcagcctaacagtcagccttaccagtaaaaaagaaaacctattaaaaaaacaccactcgacacggcaccagctcaatcagtcacagtgtaaaaaagggccaagtgcagagcgagtatatataggactaaaaaatgacgtaacggttaaagtccacaaaaaacacccagaaaaccgcacgcgaacctacgcccagaaacgaaagccaaaaaacccacaacttcctcaaatcgtcacttccgttttcccacgttacgtaacttcccattttaagaaaactacaattcccaacacatacaagttactccgccctaaaacctacgtcacccgccccgttcccacgccccgcgccacgtcacaaactccaccccctcattatcatattggcttcaatccaaaataaggtatattattgatgattaattaattaaggatcccggtgtgaaataccgcacagatgcgtaaggagaaaataccgcatcaggcgctcttacgcttcctcgctcactgactcgctgcgctcggtcgttcggctgcggcgagcggtatcagctcactcaaaggcggtaatacggttatccacagaatcaggggataacgcaggaaagaacatgtgagcaaaaggccagcaaaaggccaggaaccgtaaaaaggccgcgttgctggcgtttttccataggctccgcccccctgacgagcatcacaaaaatcgacgctcaagtcagaggtggcgaaacccgacaggactataaagataccaggcgtttccccctggaagctccctcgtgcgctctcctgttccgaccctgccgcttaccggatacctgtccgcctttctcccttcgggaagcgtggcgctttctcatagctcacgctgtaggtatctcagttcggtgtaggtcgttcgctccaagctgggctgtgtgcacgaaccccccgttcagcccgaccgctgcgccttatccggtaactatcgtcttgagtccaacccggtaagacacgacttatcgccactggcagcagccactggtaacaggattagcagagcgaggtatgtaggcggtgctacagagttcttgaagtggtggcctaactacggctacactagaaggacagtatttggtatctgcgctctgctgaagccagttaccttcggaaaaagagttggtagctcttgatccggcaaacaaaccaccgctggtagcggtggtttttttgtttgcaagcagcagattacgcgcagaaaaaaaggatctcaagaagatcctttgatcttttctacggggtctgacgctcagtggaacgaaaactcacgttaagggattttggtcatgagattatcaaaaaggatcttcacctagatccttttaaattaaaaatgaagttttaaatcaatctaaagtatatatgagtaaacttggtctgacagttaccaatgcttaatcagtgaggcacctatctcagcgatctgtctatttcgttcatccatagttgcctgactccccgtcgtgtagataactacgatacgggagggcttaccatctggccccagtgctgcaatgataccgcgagacccacgctcaccggctccagatttatcagcaataaaccagccagccggaagggccgagcgcagaagtggtcctgcaactttatccgcctccatccagtctattaattgttgccgggaagctagagtaagtagttcgccagttaatagtttgcgcaacgttgttgnnnnnnaaaaaggatcttcacctagatccttttcacgtagaaagccagtccgcagaaacggtgctgaccccggatgaatgtcagctactgggctatctggacaagggaaaacgcaagcgcaaagagaaagcaggtagcttgcagtgggcttacatggcgatagctagactgggcggttttatggacagcaagcgaaccggaattgccagctggggcgccctctggtaaggttgggaagccctgcaaagtaaactggatggctttctcgccgccaaggatctgatggcgcaggggatcaagctctgatcaagagacaggatgaggatcgtttcgcatgattgaacaagatggattgcacgcaggttctccggccgcttgggtggagaggctattcggctatgactgggcacaacagacaatcggctgctctgatgccgccgtgttccggctgtcagcgcaggggcgcccggttctttttgtcaagaccgacctgtccggtgccctgaatgaactgcaagacgaggcagcgcggctatcgtggctggccacgacgggcgttccttgcgcagctgtgctcgacgttgtcactgaagcgggaagggactggctgctattgggcgaagtgccggggcaggatctcctgtcatctcaccttgctcctgccgagaaagtatccatcatggctgatgcaatgcggcggctgcatacgcttgatccggctacctgcccattcgaccaccaagcgaaacatcgcatcgagcgagcacgtactcggatggaagccggtcttgtcgatcaggatgatctggacgaggagcatcaggggctcgcgccagccgaactgttcgccaggctcaaggcgagcatgcccgacggcgaggatctcgtcgtgacccatggcgatgcctgcttgccgaatatcatggtggaaaatggccgcttttctggattcatcgactgtggccggctgggtgtggcggaccgctatcaggacatagcgttggctacccgtgatattgctgaggagcttggcggcgaatgggctgaccgcttcctcgtgctttacggtatcgccgctcccgattcgcagcgcatcgccttctatcgccttcttgacgagttcttctgaattttgttaaaatttttgttaaatcagctcattttttaaccaataggccgaaatcggcaacatcccttataaatcaaaagaatagaccgcgatagggttgagtgttgttccagtttggaacaagagtccactattaaagaacgtggactccaacgtcaaagggcgaaaaaccgtctatcagggcgatggcccactacgtgaaccatcacccaaatcaagttttttgcggtcgaggtgccgtaaagctctaaatcggaaccctaaagggagcccccgatttagagcttgacggggaaagccggcgaacgtggcgagaaaggaagggaagaaagcgaaaggagcgggcgctagggcgctggcaagtgtagcggtcacgctgcgcgtaaccaccacacccgcgcgcttaatgcgccg

SEQ ID NO: 6 - DNA, 11777 bp, Artificial Sequence
  pGW063
aattaattaagctagcatcatcaataatataccttattttggattgaagccaatatgataatgagggggtggagtttgtgacgtggcgcggggcgtgggaacggggcgggtgacgtagtagtgtggcggaagtgtgatgttgcaagtgtggcggaacacatgtaagcgacggatgtggcaaaagtgacgtttttggtgtgcgccggtgtacacaggaagtgacaattttcgcgcggttttaggcggatgttgtagtaaatttgggcgtaaccgagtaagatttggccattttcgcgggaaaactgaataagaggaagtgaaatctgaataattttgtgttactcatagcgcgtaatatttgtctagggagatccggtaccgcggccgcctcgagtctagaaagagggcctatttcccatgattccttcatatttgcatatacgatacaaggctgttagagagataattagaattaatttgactgtaaacacaaagatattagtacaaaatacgtgacgtagaaagtaataatttcttgggtagtttgcagttttaaaattatgttttaaaatggactatcatatgcttaccgtaacttgaaagtatttcgatttcttggctttatatatcttgtggaaaggacgaaacaccggaagagcgagctcttctgttttagagctaggccaacatgaggatcacccatgtctgcagggcctagcaagttaaaataaggctagtccgttatcaacttggccaacatgaggatcacccatgtctgcagggccaagtggcaccgagtcggtgcttttttgctagcgtcagtgggcagagcgcacatcgcccacagtccccgagaagttggggggaggggtcggcaattgaacgggtgcctagagaaggtggcgcggggtaaactgggaaagtgatgtcgtgtactggctccgcctttttcccgagggtgggggagaaccgtatataagtgcagtagtcgccgtgaacgttctttttcgcaacgggtttgccgccagaacacagctgaagcttcgaggggctcgcatctctccttcacgcgcccgccgccctacctgaggccgccatccacgccggttgagtcgcgttctgccgcctcccgcctgtggtgcctcctgaactgcgtccgccgtctaggtaagtttaaagctcaggtcgagaccgggcctttgtccggcgctcccttggagcctacctagactcagccggctctccacgctttgcctgaccctgcttgctcaactctacgtctttgtttcgttttctgttctgcgccgttacagatccaagctcgtacggccaccatgaaaaggccggcggccacgaaaaaggccggccaggcaaaaaagaaaaaggacaagaagtacagcatcggcctggccatcggcaccaactctgtgggctgggccgtgatcaccgacgagtacaaggtgcccagcaagaaattcaaggtgctgggcaacaccgaccggcacagcatcaagaagaacctgatcggagccctgctgttcgacagcggcgaaacagccgaggccacccggctgaagagaaccgccagaagaagatacaccagacggaagaaccggatctgctatctgcaagagatcttcagcaacgagatggccaaggtggacgacagcttcttccacagactggaagagtccttcctggtggaagaggataagaagcacgagcggcaccccatcttcggcaacatcgtggacgaggtggcctaccacgagaagtaccccaccatctaccacctgagaaagaaactggtggacagcaccgacaaggccgacctgcggctgatctatctggccctggcccacatgatcaagttccggggccacttcctgatcgagggcgacctgaaccccgacaacagcgacgtggacaagctgttcatccagctggtgcagacctacaaccagctgttcgaggaaaaccccatcaacgccagcggcgtggacgccaaggccatcctgtctgccagactgagcaagagcagacggctggaaaatctgatcgcccagctgcccggcgagaagaagaatggcctgttcggcaacctgattgccctgagcctgggcctgacccccaacttcaagagcaacttcgacctggccgaggatgccaaactgcagctgagcaaggacacctacgacgacgacctggacaacctgctggcccagatcggcgaccagtacgccgacctgtttctggccgccaagaacctgtccgacgccatcctgctgagcgacatcctgagagtgaacaccgagatcaccaaggcccccctgagcgcctctatgatcaagagatacgacgagcaccaccaggacctgaccctgctgaaagctctcgtgcggcagcagctgcctgagaagtacaaagagattttcttcgaccagagcaagaacggctacgccggctacattgacggcggagccagccaggaagagttctacaagttcatcaagcccatcctggaaaagatggacggcaccgaggaactgctcgtgaagctgaacagagaggacctgctgcggaagcagcggaccttcgacaacggcagcatcccccaccagatccacctgggagagctgcacgccattctgcggcggcaggaagatttttacccattcctgaaggacaaccgggaaaagatcgagaagatcctgaccttccgcatcccctactacgtgggccctctggccaggggaaacagcagattcgcctggatgaccagaaagagcgaggaaaccatcaccccctggaacttcgaggaagtggtggacaagggcgcttccgcccagagcttcatcgagcggatgaccaacttcgataagaacctgcccaacgagaaggtgctgcccaagcacagcctgctgtacgagtacttcaccgtgtataacgagctgaccaaagtgaaatacgtgaccgagggaatgagaaagcccgccttcctgagcggcgagcagaaaaaggccatcgtggacctgctgttcaagaccaaccggaaagtgaccgtgaagcagctgaaagaggactacttcaagaaaatcgagtgcttcgactccgtggaaatctccggcgtggaagatcggttcaacgcctccctgggcacataccacgatctgctgaaaattatcaaggacaaggacttcctggacaatgaggaaaacgaggacattctggaagatatcgtgctgaccctgacactgtttgaggacagagagatgatcgaggaacggctgaaaacctatgcccacctgttcgacgacaaagtgatgaagcagctgaagcggcggagatacaccggctggggcaggctgagccggaagctgatcaacggcatccgggacaagcagtccggcaagacaatcctggatttcctgaagtccgacggcttcgccaacagaaacttcatgcagctgatccacgacgacagcctgacctttaaagaggacatccagaaagcccaggtgtccggccagggcgatagcctgcacgagcacattgccaatctggccggcagccccgccattaagaagggcatcctgcagacagtgaaggtggtggacgagctcgtgaaagtgatgggccggcacaagcccgagaacatcgtgatcgaaatggccagagagaaccagaccacccagaagggacagaagaacagccgcgagagaatgaagcggatcgaagagggcatcaaagagctgggcagccagatcctgaaagaacaccccgtggaaaacacccagctgcagaacgagaagctgtacctgtactacctgcagaatgggcgggatatgtacgtggaccaggaactggacatcaaccggctgtccgactacgatgtggaccacatcgtgcctcagagctttctgaaggacgactccatcgacaacaaggtgctgaccagaagcgacaaggcccggggcaagagcgacaacgtgccctccgaagaggtcgtgaagaagatgaagaactactggcggcagctgctgaacgccaagctgattacccagagaaagttcgacaatctgaccaaggccgagagaggcggcctgagcgaactggataaggccggcttcatcaagagacagctggtggaaacccggcagatcacaaagcacgtggcacagatcctggactcccggatgaacactaagtacgacgagaatgacaagctgatccgggaagtgaaagtgatcaccctgaagtccaagctggtgtccgatttccggaaggatttccagttttacaaagtgcgcgagatcaacaactaccaccacgcccacgacgcctacctgaacgccgtcgtgggaaccgccctgatcaaaaagtaccctaagctggaaagcgagttcgtgtacggcgactacaaggtgtacgacgtgcggaagatgatcgccaagagcgagcaggaaatcggcaaggctaccgccaagtacttcttctacagcaacatcatgaactttttcaagaccgagattaccctggccaacggcgagatccggaagcggcctctgatcgagacaaacggcgaaaccggggagatcgtgtgggataagggccgggattttgccaccgtgcggaaagtgctgagcatgccccaagtgaatatcgtgaaaaagaccgaggtgcagacaggcggcttcagcaaagagtctatcctgcccaagaggaacagcgataagctgatcgccagaaagaaggactgggaccctaagaagtacggcggcttcgacagccccaccgtggcctattctgtgctggtggtggccaaagtggaaaagggcaagtccaagaaactgaagagtgtgaaagagctgctggggatcaccatcatggaaagaagcagcttcgagaagaatcccatcgactttctggaagccaagggctacaaagaagtgaaaaaggacctgatcatcaagctgcctaagtactccctgttcgagctggaaaacggccggaagagaatgctggcctctgccggcgaactgcagaagggaaacgaactggccctgccctccaaatatgtgaacttcctgtacctggccagccactatgagaagctgaagggctcccccgaggataatgagcagaaacagctgtttgtggaacagcacaagcactacctggacgagatcatcgagcagatcagcgagttctccaagagagtgatcctggccgacgctaatctggacaaagtgctgtccgcctacaacaagcaccgggataagcccatcagagagcaggccgagaatatcatccacctgtttaccctgaccaatctgggagcccctgccgccttcaagtactttgacaccaccatcgaccggaagaggtacaccagcaccaaagaggtgctggacgccaccctgatccaccagagcatcaccggcctgtacgagacacggatcgacctgtctcagctgggaggcgacagcgctggaggaggtggaagcggaggaggaggaagcggaggaggaggtagcggacctaagaaaaagaggaaggtggcggccgctggatccccttcagggcagatcagcaaccaggccctggctctggcccctagctccgctccagtgctggcccagactatggtgccctctagtgctatggtgcctctggcccagccacctgctccagcccctgtgctgaccccaggaccaccccagtcactgagcgctccagtgcccaagtctacacaggccggcgaggggactctgagtgaagctctgctgcacctgcagttcgacgctgatgaggacctgggagctctgctggggaacagcaccgatcccggagtgttcacagatctggcctccgtggacaactctgagtttcagcagctgctgaatcagggcgtgtccatgtctcatagtacagccgaaccaatgctgatggagtaccccgaagccattacccggctggtgaccggcagccagcggccccccgaccccgctccaactcccctgggaaccagcggcctgcctaatgggctgtccggagatgaagacttctcaagcatcgctgatatggactttagtgccctgctgtcacagatttcctctagtgggcagggaggaggtggaagcggcttcagcgtggacaccagtgccctgctggacctgttcagcccctcggtgaccgtgcccgacatgagcctgcctgaccttgacagcagcctggccagtatccaagagctcctgtctccccaggagccccccaggcctcccgaggcagagaacagcagcccggattcagggaagcagctggtgcactacacagcgcagccgctgttcctgctggaccccggctccgtggacaccgggagcaacgacctgccggtgctgtttgagctgggagagggctcctacttctccgaaggggacggcttcgccgaggaccccaccatctccctgctgacaggctcggagcctcccaaagccaaggaccccactgtctcctaagaattcctgcagcccgggggatccactagttctagagcggccgccaccgcggggagatccagacatgataagatacattgatgagtttggacaaaccacaactagaatgcagtgaaaaaaatgctttatttgtgaaatttgtgatgctattgctttatttgtaaccattataagctgcaataaacaagttaacaacaacaattgcattcattttatgtttcaggttcagggggaggtgtgggaggttttttaaagcaagtaaaacctctacaaatgtggtatggctgattatgatcccggctgcctcgcgcgtttcggtgatgacggtgaaaacctcttgacacatgcagctcccggagacggtcacagcttgtctgtaagcggatgccgggagcagacaagcccgtcagggcgcgtcagcgggtgttggcgggtgtcggggcgcagccatgaggtcgactctagtccccgcggtggcagatctggaaggtgctgaggtacgatgagacccgcaccaggtgcagaccctgcgagtgtggcggtaaacatattaggaaccagcctgtgatgctggatgtgaccgaggagctgaggcccgatcacttggtgctggcctgcacccgcgctgagtttggctctagcgatgaagatacagattgaggtactgaaatgtgtgggcgtggcttaagggtgggaaagaatatataaggtgggggtcttatgtagttttgtatctgttttgcagcagccgccgccgccatgagcaccaactcgtttgatggaagcattgtgagctcatatttgacaacgcgcatgcccccatgggccggggtgcgtcagaatgtgatgggctccagcattgatggtcgccccgtcctgcccgcaaactctactaccttgacctacgagaccgtgtctggaacgccgttggagactgcagcctccgccgccgcttcagccgctgcagccaccgcccgcgggattgtgactgactttgctttcctgagcccgcttgcaagcagtgcagcttcccgttcatccgcccgcgatgacaagttgacggctcttttggcacaattggattctttgacccgggaacttaatgtcgtttctcagcagctgttggatctgcgccagcaggtttctgccctgaaggcttcctcccctcccaatgcggtttaaaacataaataaaaaaccagactctgtttggatttggatcaagcaagtgtcttgctgtctttatttaggggttttgcgcgcgcggtaggcccgggaccagcggtctcggtcgttgagggtcctgtgtattttttccaggacgtggtaaaggtgactctggatgttcagatacatgggcataagcccgtctctggggtggaggtagcaccactgcagagcttcatgctgcggggtggtgttgtagatgatccagtcgtagcaggagcgctgggcgtggtgcctaaaaatgtctttcagtagcaagctgattgccaggggcaggcccttggtgtaagtgtttacaaagcggttaagctgggatgggtgcatacgtggggatatgagatgcatcttggactgtatttttaggttggctatgttcccagccatatccctccggggattcatgttgtgcagaaccaccagcacagtgtatccggtgcacttgggaaatttgtcatgtagcttagaaggaaatgcgtggaagaacttggagacgcccttgtgacctccaagattttccatgcattcgtccataatgatggcaatgggcccacgggcggcggcctgggcgaagatatttctgggatcactaacgtcatagttgtgttccaggatgagatcgtcataggccatttttacaaagcgcgggcggagggtgccagactgcggtataatggttccatccggcccaggggcgtagttaccctcacagatttgcatttcccacgctttgagttcagatggggggatcatgtctacctgcggggcgatgaagaaaacggtttccggggtaggggagatcagctgggaagaaagcaggttcctgagcagctgcgacttaccgcagccggtgggcccgtaaatcacacctattaccgggtgcaactggtagttaagagagctgcagctgccgtcatccctgagcaggggggccacttcgttaagcatgtccctgactcgcatgttttccctgaccaaatccgccagaaggcgctcgccgcccagcgatagcagttcttgcaaggaagcaaagtttttcaacggtttgagaccgtccgccgtaggcatgcttttgagcgtttgaccaagcagttccaggcggtcccacagctcggtcacctgctctacggcatctcgatccagcatatctcctcgtttcgcgggttggggcggctttcgctgtacggcagtagtcggtgctcgtccagacgggccagggtcatgtctttccacgggcgcagggtcctcgtcagcgtagtctgggtcacggtgaaggggtgcgctccgggctgcgcgctggccagggtgcgcttgaggctggtcctgctggtgctgaagcgctgccggtcttcgccctgcgcgtcggccaggtagcatttgaccatggtgtcatagtccagcccctccgcggcgtggcccttggcgcgcagcttgcccttggaggaggcgccgcacgaggggcagtgcagacttttgagggcgtagagcttgggcgcgagaaataccgattccggggagtaggcatccgcgccgcaggccccgcagacggtctcgcattccacgagccaggtgagctctggccgttcggggtcaaaaaccaggtttcccccatgctttttgatgcgtttcttacctctggtttccatgagccggtgtccacgctcggtgacgaaaaggctgtccgtgtccccgtatacagacttgagaggcctgtcctcgaccgatgcccttgagagccttcaacccagtcagctccttccggtgggcgcggggcatgactatcgtcgccgcacttatgactgtcttctttatcatgcaactcgtaggacaggtgccggcagcgctctgggtcattttcggcgaggaccgctttcgctggagcgcgacgatgatcggcctgtcgcttgcggtattcggaatcttgcacgccctcgctcaagccttcgtcactggtcccgccaccaaacgtttcggcgagaagcaggccattatcgccggcatggcggccgacgcgctgggctacgtcttgctggcgttcgcgacgcgaggctggatggccttccccattatgattcttctcgcttccggcggcatcgggatgcccgcgttgcaggccatgctgtccaggcaggtagatgacgaccatcagggacagcttcaaggccagcaaaaggccaggaaccgtaaaaaggccgcgttgctggcgtttttccataggctccgcccccctgacgagcatcacaaaaatcgacgctcaagtcagaggtggcgaaacccgacaggactataaagataccaggcgtttccccctggaagctccctcgtgcgctctcctgttccgaccctgccgcttaccggatacctgtccgcctttctcccttcgggaagcgtggcgctttctcatagctcacgctgtaggtatctcagttcggtgtaggtcgttcgctccaagctgggctgtgtgcacgaaccccccgttcagcccgaccgctgcgccttatccggtaactatcgtcttgagtccaacccggtaagacacgacttatcgccactggcagcagccactggtaacaggattagcagagcgaggtatgtaggcggtgctacagagttcttgaagtggtggcctaactacggctacactagaaggacagtatttggtatctgcgctctgctgaagccagttaccttcggaaaaagagttggtagctcttgatccggcaaacaaaccaccgctggtagcggtggtttttttgtttgcaagcagcagattacgcgcagaaaaaaaggatctcaagaagatcctttgatcttttctacggggtctgacgctcagtggaacgaaaactcacgttaagggattttggtcatgagattatcaaaaaggatcttcacctagatccttttaaattaaaaatgaagttttaaatcaatctaaagtatatatgagtaaacttggtctgacagttaccaatgcttaatcagtgaggcacctatctcagcgatctgtctatttcgttcatccatagttgcctgactccccgtcgtgtagataactacgatacgggagggcttaccatctggccccagtgctgcaatgataccgcgagacccacgctcaccggctccagatttatcagcaataaaccagccagccggaagggccgagcgcagaagtggtcctgcaactttatccgcctccatccagtctattaattgttgccgggaagctagagtaagtagttcgccagttaatagtttgcgcaacgttgttgccattgctgcaggcatcgtggtgtcacgctcgtcgtttggtatggcttcattcagctccggttcccaacgatcaaggcgagttacatgatcccccatgttgtgcaaaaaagcggttagctccttcggtcctccgatcgttgtcagaagtaagttggccgcagtgttatcactcatggttatggcagcactgcataattctcttactgtcatgccatccgtaagatgcttttctgtgactggtgagtactcaaccaagtcattctgagaatagtgtatgcggcgaccgagttgctcttgcccggcgtcaacacgggataataccgcgccacatagcagaactttaaaagtgctcatcattggaaaacgttcttcggggcgaaaactctcaaggatcttaccgctgttgagatccagttcgatgtaacccactcgtgcacccaactgatcttcagcatcttttactttcaccagcgtttctgggtgagcaaaaacaggaaggcaaaatgccgcaaaaaagggaataagggcgacacggaaatgttgaatactcatactcttcctttttcaatattattgaagcatttatcagggttattgtctcatgagcggatacatatttgaatgtatttagaaaaataaacaaataggggttccgcgcacatttccccgaaaagtgccacctgacgtctaagaaaccattattatcatgacattaacctataaaaataggcgtatcacgaggccctttcgtcttcaagaa

SEQ ID NO: 7 - DNA, 33477 bp, Artificial Sequence
  pAdEasy-1
attgtgagctcatatttgacaacgcgcatgcccccatgggccggggtgcgtcagaatgtgatgggctccagcattgatggtcgccccgtcctgcccgcaaactctactaccttgacctacgagaccgtgtctggaacgccgttggagactgcagcctccgccgccgcttcagccgctgcagccaccgcccgcgggattgtgactgactttgctttcctgagcccgcttgcaagcagtgcagcttcccgttcatccgcccgcgatgacaagttgacggctcttttggcacaattggattctttgacccgggaacttaatgtcgtttctcagcagctgttggatctgcgccagcaggtttctgccctgaaggcttcctcccctcccaatgcggtttaaaacataaataaaaaaccagactctgtttggatttggatcaagcaagtgtcttgctgtctttatttaggggttttgcgcgcgcggtaggcccgggaccagcggtctcggtcgttgagggtcctgtgtattttttccaggacgtggtaaaggtgactctggatgttcagatacatgggcataagcccgtctctggggtggaggtagcaccactgcagagcttcatgctgcggggtggtgttgtagatgatccagtcgtagcaggagcgctgggcgtggtgcctaaaaatgtctttcagtagcaagctgattgccaggggcaggcccttggtgtaagtgtttacaaagcggttaagctgggatgggtgcatacgtggggatatgagatgcatcttggactgtatttttaggttggctatgttcccagccatatccctccggggattcatgttgtgcagaaccaccagcacagtgtatccggtgcacttgggaaatttgtcatgtagcttagaaggaaatgcgtggaagaacttggagacgcccttgtgacctccaagattttccatgcattcgtccataatgatggcaatgggcccacgggcggcggcctgggcgaagatatttctgggatcactaacgtcatagttgtgttccaggatgagatcgtcataggccatttttacaaagcgcgggcggagggtgccagactgcggtataatggttccatccggcccaggggcgtagttaccctcacagatttgcatttcccacgctttgagttcagatggggggatcatgtctacctgcggggcgatgaagaaaacggtttccggggtaggggagatcagctgggaagaaagcaggttcctgagcagctgcgacttaccgcagccggtgggcccgtaaatcacacctattaccggctgcaactggtagttaagagagctgcagctgccgtcatccctgagcaggggggccacttcgttaagcatgtccctgactcgcatgttttccctgaccaaatccgccagaaggcgctcgccgcccagcgatagcagttcttgcaaggaagcaaagtttttcaacggtttgagaccgtccgccgtaggcatgcttttgagcgtttgaccaagcagttccaggcggtcccacagctcggtcacctgctctacggcatctcgatccagcatatctcctcgtttcgcgggttggggcggctttcgctgtacggcagtagtcggtgctcgtccagacgggccagggtcatgtctttccacgggcgcagggtcctcgtcagcgtagtctgggtcacggtgaaggggtgcgctccgggctgcgcgctggccagggtgcgcttgaggctggtcctgctggtgctgaagcgctgccggtcttcgccctgcgcgtcggccaggtagcatttgaccatggtgtcatagtccagcccctccgcggcgtggcccttggcgcgcagcttgcccttggaggaggcgccgcacgaggggcagtgcagacttttgagggcgtagagcttgggcgcgagaaataccgattccggggagtaggcatccgcgccgcaggccccgcagacggtctcgcattccacgagccaggtgagctctggccgttcggggtcaaaaaccaggtttcccccatgctttttgatgcgtttcttacctctggtttccatgagccggtgtccacgctcggtgacgaaaaggctgtccgtgtccccgtatacagacttgagaggcctgtcctcgagcggtgttccgcggtcctcctcgtatagaaactcggaccactctgagacaaaggctcgcgtccaggccagcacgaaggaggctaagtgggaggggtagcggtcgttgtccactagggggtccactcgctccagggtgtgaagacacatgtcgccctcttcggcatcaaggaaggtgattggtttgtaggtgtaggccacgtgaccgggtgttcctgaaggggggctataaaagggggtgggggcgcgttcgtcctcactctcttccgcatcgctgtctgcgagggccagctgttggggtgagtactccctctgaaaagcgggcatgacttctgcgctaagattgtcagtttccaaaaacgaggaggatttgatattcacctggcccgcggtgatgcctttgagggtggccgcatccatctggtcagaaaagacaatctttttgttgtcaagcttggtggcaaacgacccgtagagggcgttggacagcaacttggcgatggagcgcagggtttggtttttgtcgcgatcggcgcgctccttggccgcgatgtttagctgcacgtattcgcgcgcaacgcaccgccattcgggaaagacggtggtgcgctcgtcgggcaccaggtgcacgcgccaaccgcggttgtgcagggtgacaaggtcaacgctggtggctacctctccgcgtaggcgctcgttggtccagcagaggcggccgcccttgcgcgagcagaatggcggtagggggtctagctgcgtctcgtccggggggtctgcgtccacggtaaagaccccgggcagcaggcgcgcgtcgaagtagtctatcttgcatccttgcaagtctagcgcctgctgccatgcgcgggcggcaagcgcgcgctcgtatgggttgagtgggggaccccatggcatggggtgggtgagcgcggaggcgtacatgccgcaaatgtcgtaaacgtagaggggctctctgagtattccaagatatgtagggtagcatcttccaccgcggatgctggcgcgcacgtaatcgtatagttcgtgcgagggagcgaggaggtcgggaccgaggttgctacgggcgggctgctctgctcggaagactatctgcctgaagatggcatgtgagttggatgatatggttggacgctggaagacgttgaagctggcgtctgtgagacctaccgcgtcacgcacgaaggaggcgtaggagtcgcgcagcttgttgaccagctcggcggtgacctgcacgtctagggcgcagtagtccagggtttccttgatgatgtcatacttatcctgtcccttttttttccacagctcgcggttgaggacaaactcttcgcggtctttccagtactcttggatcggaaacccgtcggcctccgaacggtaagagcctagcatgtagaactggttgacggcctggtaggcgcagcatcccttttctacgggtagcgcgtatgcctgcgcggccttccggagcgaggtgtgggtgagcgcaaaggtgtccctgaccatgactttgaggtactggtatttgaagtcagtgtcgtcgcatccgccctgctcccagagcaaaaagtccgtgcgctttttggaacgcggatttggcagggcgaaggtgacatcgttgaagagtatctttcccgcgcgaggcataaagttgcgtgtgatgcggaagggtcccggcacctcggaacggttgttaattacctgggcggcgagcacgatctcgtcaaagccgttgatgttgtggcccacaatgtaaagttccaagaagcgcgggatgcccttgatggaaggcaattttttaagttcctcgtaggtgagctcttcaggggagctgagcccgtgctctgaaagggcccagtctgcaagatgagggttggaagcgacgaatgagctccacaggtcacgggccattagcatttgcaggtggtcgcgaaaggtcctaaactggcgacctatggccattttttctggggtgatgcagtagaaggtaagcgggtcttgttcccagcggtcccatccaaggttcgcggctaggtctcgcgcggcagtcactagaggctcatctccgccgaacttcatgaccagcatgaagggcacgagctgcttcccaaaggcccccatccaagtataggtctctacatcgtaggtgacaaagagacgctcggtgcgaggatgcgagccgatcgggaagaactggatctcccgccaccaattggaggagtggctattgatgtggtgaaagtagaagtccctgcgacgggccgaacactcgtgctggcttttgtaaaaacgtgcgcagtactggcagcggtgcacgggctgtacatcctgcacgaggttgacctgacgaccgcgcacaaggaagcagagtgggaatttgagcccctcgcctggcgggtttggctggtggtcttctacttcggctgcttgtccttgaccgtctggctgctcgaggggagttacggtggatcggaccaccacgccgcgcgagcccaaagtccagatgtccgcgcgcggcggtcggagcttgatgacaacatcgcgcagatgggagctgtccatggtctggagctcccgcggcgtcaggtcaggcgggagctcctgcaggtttacctcgcatagacgggtcagggcgcgggctagatccaggtgatacctaatttccaggggctggttggtggcggcgtcgatggcttgcaagaggccgcatccccgcggcgcgactacggtaccgcgcggcgggcggtgggccgcgggggtgtccttggatgatgcatctaaaagcggtgacgcgggcgagcccccggaggtagggggggctccggacccgccgggagagggggcaggggcacgtcggcgccgcgcgcgggcaggagctggtgctgcgcgcgtaggttgctggcgaacgcgacgacgcggcggttgatctcctgaatctggcgcctctgcgtgaagacgacgggcccggtgagcttgaacctgaaagagagttcgacagaatcaatttcggtgtcgttgacggcggcctggcgcaaaatctcctgcacgtctcctgagttgtcttgataggcgatctcggccatgaactgctcgatctcttcctcctggagatctccgcgtccggctcgctccacggtggcggcgaggtcgttggaaatgcgggccatgagctgcgagaaggcgttgaggcctccctcgttccagacgcggctgtagaccacgcccccttcggcatcgcgggcgcgcatgaccacctgcgcgagattgagctccacgtgccgggcgaagacggcgtagtttcgcaggcgctgaaagaggtagttgagggtggtggcggtgtgttctgccacgaagaagtacataacccagcgtcgcaacgtggattcgttgatatcccccaaggcctcaaggcgctccatggcctcgtagaagtccacggcgaagttgaaaaactgggagttgcgcgccgacacggttaactcctcctccagaagacggatgagctcggcgacagtgtcgcgcacctcgcgctcaaaggctacaggggcctcttcttcttcttcaatctcctcttccataagggcctccccttcttcttcttctggcggcggtgggggaggggggacacggcggcgacgacggcgcaccgggaggcggtcgacaaagcgctcgatcatctccccgcggcgacggcgcatggtctcggtgacggcgcggccgttctcgcgggggcgcagttggaagacgccgcccgtcatgtcccggttatgggttggcggggggctgccatgcggcagggatacggcgctaacgatgcatctcaacaattgttgtgtaggtactccgccgccgagggacctgagcgagtccgcatcgaccggatcggaaaacctctcgagaaaggcgtctaaccagtcacagtcgcaaggtaggctgagcaccgtggcgggcggcagcgggcggcggtcggggttgtttctggcggaggtgctgctgatgatgtaattaaagtaggcggtcttgagacggcggatggtcgacagaagcaccatgtccttgggtccggcctgctgaatgcgcaggcggtcggccatgccccaggcttcgttttgacatcggcgcaggtctttgtagtagtcttgcatgagcctttctaccggcacttcttcttctccttcctcttgtcctgcatctcttgcatctatcgctgcggcggcggcggagtttggccgtaggtggcgccctcttcctcccatgcgtgtgaccccgaagcccctcatcggctgaagcagggctaggtcggcgacaacgcgctcggctaatatggcctgctgcacctgcgtgagggtagactggaagtcatccatgtccacaaagcggtggtatgcgcccgtgttgatggtgtaagtgcagttggccataacggaccagttaacggtctggtgacccggctgcgagagctcggtgtacctgagacgcgagtaagccctcgagtcaaatacgtagtcgttgcaagtccgcaccaggtactggtatcccaccaaaaagtgcggcggcggctggcggtagaggggccagcgtagggtggccggggctccgggggcgagatcttccaacataaggcgatgatatccgtagatgtacctggacatccaggtgatgccggcggcggtggtggaggcgcgcggaaagtcgcggacgcggttccagatgttgcgcagcggcaaaaagtgctccatggtcgggacgctctggccggtcaggcgcgcgcaatcgttgacgctctagcgtgcaaaaggagagcctgtaagcgggcactcttccgtggtctggtggataaattcgcaagggtatcatggcggacgaccggggttcgagccccgtatccggccgtccgccgtgatccatgcggttaccgcccgcgtgtcgaacccaggtgtgcgacgtcagacaacgggggagtgctccttttggcttccttccaggcgcggcggctgctgcgctagcttttttggccactggccgcgcgcagcgtaagcggttaggctggaaagcgaaagcattaagtggctcgctccctgtagccggagggttattttccaagggttgagtcgcgggacccccggttcgagtctcggaccggccggactgcggcgaacgggggtttgcctccccgtcatgcaagaccccgcttgcaaattcctccggaaacagggacgagccccttttttgcttttcccagatgcatccggtgctgcggcagatgcgcccccctcctcagcagcggcaagagcaagagcagcggcagacatgcagggcaccctcccctcctcctaccgcgtcaggaggggcgacatccgcggttgacgcggcagcagatggtgattacgaacccccgcggcgccgggcccggcactacctggacttggaggagggcgagggcctggcgcggctaggagcgccctctcctgagcggcacccaagggtgcagctgaagcgtgatacgcgtgaggcgtacgtgccgcggcagaacctgtttcgcgaccgcgagggagaggagcccgaggagatgcgggatcgaaagttccacgcagggcgcgagctgcggcatggcctgaatcgcgagcggttgctgcgcgaggaggactttgagcccgacgcgcgaaccgggattagtcccgcgcgcgcacacgtggcggccgccgacctggtaaccgcatacgagcagacggtgaaccaggagattaactttcaaaaaagctttaacaaccacgtgcgtacgcttgtggcgcgcgaggaggtggctataggactgatgcatctgtgggactttgtaagcgcgctggagcaaaacccaaatagcaagccgctcatggcgcagctgttccttatagtgcagcacagcagggacaacgaggcattcagggatgcgctgctaaacatagtagagcccgagggccgctggctgctcgatttgataaacatcctgcagagcatagtggtgcaggagcgcagcttgagcctggctgacaaggtggccgccatcaactattccatgcttagcctgggcaagttttacgcccgcaagatataccataccccttacgttcccatagacaaggaggtaaagatcgaggggttctacatgcgcatggcgctgaaggtgcttaccttgagcgacgacctgggcgtttatcgcaacgagcgcatccacaaggccgtgagcgtgagccggcggcgcgagctcagcgaccgcgagctgatgcacagcctgcaaagggccctggctggcacgggcagcggcgatagagaggccgagtcctactttgacgcgggcgctgacctgcgctgggccccaagccgacgcgccctggaggcagctggggccggacctgggctggcggtggcacccgcgcgcgctggcaacgtcggcggcgtggaggaatatgacgaggacgatgagtacgagccagaggacggcgagtactaagcggtgatgtttctgatcagatgatgcaagacgcaacggacccggcggtgcgggcggcgctgcagagccagccgtccggccttaactccacggacgactggcgccaggtcatggaccgcatcatgtcgctgactgcgcgcaatcctgacgcgttccggcagcagccgcaggccaaccggctctccgcaattctggaagcggtggtcccggcgcgcgcaaaccccacgcacgagaaggtgctggcgatcgtaaacgcgctggccgaaaacagggccatccggcccgacgaggccggcctggtctacgacgcgctgcttcagcgcgtggctcgttacaacagcggcaacgtgcagaccaacctggaccggctggtgggggatgtgcgcgaggccgtggcgcagcgtgagcgcgcgcagcagcagggcaacctgggctccatggttgcactaaacgccttcctgagtacacagcccgccaacgtgccgcggggacaggaggactacaccaactttgtgagcgcactgcggctaatggtgactgagacaccgcaaagtgaggtgtaccagtctgggccagactattttttccagaccagtagacaaggcctgcagaccgtaaacctgagccaggctttcaaaaacttgcaggggctgtggggggtgcgggctcccacaggcgaccgcgcgaccgtgtctagcttgctgacgcccaactcgcgcctgttgctgctgctaatagcgcccttcacggacagtggcagcgtgtcccgggacacatacctaggtcacttgctgacactgtaccgcgaggccataggtcaggcgcatgtggacgagcatactttccaggagattacaagtgtcagccgcgcgctggggcaggaggacacgggcagcctggaggcaaccctaaactacctgctgaccaaccggcggcagaagatcccctcgttgcacagtttaaacagcgaggaggagcgcattttgcgctacgtgcagcagagcgtgagccttaacctgatgcgcgacggggtaacgcccagcgtggcgctggacatgaccgcgcgcaacatggaaccgggcatgtatgcctcaaaccggccgtttatcaaccgcctaatggactacttgcatcgcgcggccgccgtgaaccccgagtatttcaccaatgccatcttgaacccgcactggctaccgccccctggtttctacaccgggggattcgaggtgcccgagggtaacgatggattcctctgggacgacatagacgacagcgtgttttccccgcaaccgcagaccctgctagagttgcaacagcgcgagcaggcagaggcggcgctgcgaaaggaaagcttccgcaggccaagcagcttgtccgatctaggcgctgcggccccgcggtcagatgctagtagcccatttccaagcttgatagggtctcttaccagcactcgcaccacccgcccgcgcctgctgggcgaggaggagtacctaaacaactcgctgctgcagccgcagcgcgaaaaaaacctgcctccggcatttcccaacaacgggatagagagcctagtggacaagatgagtagatggaagacgtacgcgcaggagcacagggacgtgccaggcccgcgcccgcccacccgtcgtcaaaggcacgaccgtcagcggggtctggtgtgggaggacgatgactcggcagacgacagcagcgtcctggatttgggagggagtggcaacccgtttgcgcaccttcgccccaggctggggagaatgttttaaaaaaaaaaaagcatgatgcaaaataaaaaactcaccaaggccatggcaccgagcgttggttttcttgtattccccttagtatgcggcgcgcggcgatgtatgaggaaggtcctcctccctcctacgagagtgtggtgagcgcggcgccagtggcggcggcgctgggttctcccttcgatgctcccctggacccgccgtttgtgcctccgcggtacctgcggcctaccggggggagaaacagcatccgttactctgagttggcacccctattcgacaccacccgtgtgtacctggtggacaacaagtcaacggatgtggcatccctgaactaccagaacgaccacagcaactttctgaccacggtcattcaaaacaatgactacagcccgggggaggcaagcacacagaccatcaatcttgacgaccggtcgcactggggcggcgacctgaaaaccatcctgcataccaacatgccaaatgtgaacgagttcatgtttaccaataagtttaaggcgcgggtgatggtgtcgcgcttgcctactaaggacaatcaggtggagctgaaatacgagtgggtggagttcacgctgcccgagggcaactactccgagaccatgaccatagaccttatgaacaacgcgatcgtggagcactacttgaaagtgggcagacagaacggggttctggaaagcgacatcggggtaaagtttgacacccgcaacttcagactggggtttgaccccgtcactggtcttgtcatgcctggggtatatacaaacgaagccttccatccagacatcattttgctgccaggatgcggggtggacttcacccacagccgcctgagcaacttgttgggcatccgcaagcggcaacccttccaggagggctttaggatcacctacgatgatctggagggtggtaacattcccgcactgttggatgtggacgcctaccaggcgagcttgaaagatgacaccgaacagggcgggggtggcgcaggcggcagcaacagcagtggcagcggcgcggaagagaactccaacgcggcagccgcggcaatgcagccggtggaggacatgaacgatcatgccattcgcggcgacacctttgccacacgggctgaggagaagcgcgctgaggccgaagcagcggccgaagctgccgcccccgctgcgcaacccgaggtcgagaagcctcagaagaaaccggtgatcaaacccctgacagaggacagcaagaaacgcagttacaacctaataagcaatgacagcaccttcacccagtaccgcagctggtaccttgcatacaactacggcgaccctcagaccggaatccgctcatggaccctgctttgcactcctgacgtaacctgcggctcggagcaggtctactggtcgttgccagacatgatgcaagaccccgtgaccttccgctccacgcgccagatcagcaactttccggtggtgggcgccgagctgttgcccgtgcactccaagagcttctacaacgaccaggccgtctactcccaactcatccgccagtttacctctctgacccacgtgttcaatcgctttcccgagaaccagattttggcgcgcccgccagcccccaccatcaccaccgtcagtgaaaacgttcctgctctcacagatcacgggacgctaccgctgcgcaacagcatcggaggagtccagcgagtgaccattactgacgccagacgccgcacctgcccctacgtttacaaggccctgggcatagtctcgccgcgcgtcctatcgagccgcactttttgagcaagcatgtccatccttatatcgcccagcaataacacaggctggggcctgcgcttcccaagcaagatgtttggcggggccaagaagcgctccgaccaacacccagtgcgcgtgcgcgggcactaccgcgcgccctggggcgcgcacaaacgcggccgcactgggcgcaccaccgtcgatgacgccatcgacgcggtggtggaggaggcgcgcaactacacgcccacgccgccaccagtgtccacagtggacgcggccattcagaccgtggtgcgcggagcccggcgctatgctaaaatgaagagacggcggaggcgcgtagcacgtcgccaccgccgccgacccggcactgccgcccaacgcgcggcggcggccctgcttaaccgcgcacgtcgcaccggccgacgggcggccatgcgggccgctcgaaggctggccgcgggtattgtcactgtgccccccaggtccaggcgacgagcggccgccgcagcagccgcggccattagtgctatgactcagggtcgcaggggcaacgtgtattgggtgcgcgactcggttagcggcctgcgcgtgcccgtgcgcacccgccccccgcgcaactagattgcaagaaaaaactacttagactcgtactgttgtatgtatccagcggcggcggcgcgcaacgaagctatgtccaagcgcaaaatcaaagaagagatgctccaggtcatcgcgccggagatctatggccccccgaagaaggaagagcaggattacaagccccgaaagctaaagcgggtcaaaaagaaaaagaaagatgatgatgatgaacttgacgacgaggtggaactgctgcacgctaccgcgcccaggcgacgggtacagtggaaaggtcgacgcgtaaaacgtgttttgcgacccggcaccaccgtagtctttacgcccggtgagcgctccacccgcacctacaagcgcgtgtatgatgaggtgtacggcgacgaggacctgcttgagcaggccaacgagcgcctcggggagtttgcctacggaaagcggcataaggacatgctggcgttgccgctggacgagggcaacccaacacctagcctaaagcccgtaacactgcagcaggtgctgcccgcgcttgcaccgtccgaagaaaagcgcggcctaaagcgcgagtctggtgacttggcacccaccgtgcagctgatggtacccaagcgccagcgactggaagatgtcttggaaaaaatgaccgtggaacctgggctggagcccgaggtccgcgtgcggccaatcaagcaggtggcgccgggactgggcgtgcagaccgtggacgttcagatacccactaccagtagcaccagtattgccaccgccacagagggcatggagacacaaacgtccccggttgcctcagcggtggcggatgccgcggtgcaggcggtcgctgcggccgcgtccaagacctctacggaggtgcaaacggacccgtggatgtttcgcgtttcagccccccggcgcccgcgccgttcgaggaagtacggcgccgccagcgcgctactgcccgaatatgccctacatccttccattgcgcctacccccggctatcgtggctacacctaccgccccagaagacgagcaactacccgacgccgaaccaccactggaacccgccgccgccgtcgccgtcgccagcccgtgctggccccgatttccgtgcgcagggtggctcgcgaaggaggcaggaccctggtgctgccaacagcgcgctaccaccccagcatcgtttaaaagccggtctttgtggttcttgcagatatggccctcacctgccgcctccgtttcccggtgccgggattccgaggaagaatgcaccgtaggaggggcatggccggccacggcctgacgggcggcatgcgtcgtgcgcaccaccggcggcggcgcgcgtcgcaccgtcgcatgcgcggcggtatcctgcccctccttattccactgatcgccgcggcgattggcgccgtgcccggaattgcatccgtggccttgcaggcgcagagacactgattaaaaacaagttgcatgtggaaaaatcaaaataaaaagtctggactctcacgctcgcttggtcctgtaactattttgtagaatggaagacatcaactttgcgtctctggccccgcgacacggctcgcgcccgttcatgggaaactggcaagatatcggcaccagcaatatgagcggtggcgccttcagctggggctcgctgtggagcggcattaaaaatttcggttccaccgttaagaactatggcagcaaggcctggaacagcagcacaggccagatgctgagggataagttgaaagagcaaaatttccaacaaaaggtggtagatggcctggcctctggcattagcggggtggtggacctggccaaccaggcagtgcaaaataagattaacagtaagcttgatccccgccctcccgtagaggagcctccaccggccgtggagacagtgtctccagaggggcgtggcgaaaagcgtccgcgccccgacagggaagaaactctggtgacgcaaatagacgagcctccctcgtacgaggaggcactaaagcaaggcctgcccaccacccgtcccatcgcgcccatggctaccggagtgctgggccagcacacacccgtaacgctggacctgcctccccccgccgacacccagcagaaacctgtgctgccaggcccgaccgccgttgttgtaacccgtcctagccgcgcgtccctgcgccgcgccgccagcggtccgcgatcgttgcggcccgtagccagtggcaactggcaaagcacactgaacagcatcgtgggtctgggggtgcaatccctgaagcgccgacgatgcttctgatagctaacgtgtcgtatgtgtgtcatgtatgcgtccatgtcgccgccagaggagctgctgagccgccgcgcgcccgctttccaagatggctaccccttcgatgatgccgcagtggtcttacatgcacatctcgggccaggacgcctcggagtacctgagccccgggctggtgcagtttgcccgcgccaccgagacgtacttcagcctgaataacaagtttagaaaccccacggtggcgcctacgcacgacgtgaccacagaccggtcccagcgtttgacgctgcggttcatccctgtggaccgtgaggatactgcgtactcgtacaaggcgcggttcaccctagctgtgggtgataaccgtgtgctggacatggcttccacgtactttgacatccgcggcgtgctggacaggggccctacttttaagccctactctggcactgcctacaacgccctggctcccaagggtgccccaaatccttgcgaatgggatgaagctgctactgctcttgaaataaacctagaagaagaggacgatgacaacgaagacgaagtagacgagcaagctgagcagcaaaaaactcacgtatttgggcaggcgccttattctggtataaatattacaaaggagggtattcaaataggtgtcgaaggtcaaacacctaaatatgccgataaaacatttcaacctgaacctcaaataggagaatctcagtggtacgaaacagaaattaatcatgcagctgggagagtcctaaaaaagactaccccaatgaaaccatgttacggttcatatgcaaaacccacaaatgaaaatggagggcaaggcattcttgtaaagcaacaaaatggaaagctagaaagtcaagtggaaatgcaatttttctcaactactgaggcagccgcaggcaatggtgataacttgactcctaaagtggtattgtacagtgaagatgtagatatagaaaccccagacactcatatttcttacatgcccactattaaggaaggtaactcacgagaactaatgggccaacaatctatgcccaacaggcctaattacattgcttttagggacaattttattggtctaatgtattacaacagcacgggtaatatgggtgttctggcgggccaagcatcgcagttgaatgctgttgtagatttgcaagacagaaacacagagctttcataccagcttttgcttgattccattggtgatagaaccaggtacttttctatgtggaatcaggctgttgacagctatgatccagatgttagaattattgaaaatcatggaactgaagatgaacttccaaattactgctttccactgggaggtgtgattaatacagagactcttaccaaggtaaaacctaaaacaggtcaggaaaatggatgggaaaaagatgctacagaattttcagataaaaatgaaataagagttggaaataattttgccatggaaatcaatctaaatgccaacctgtggagaaatttcctgtactccaacatagcgctgtatttgcccgacaagctaaagtacagtccttccaacgtaaaaatttctgataacccaaacacctacgactacatgaacaagcgagtggtggctcccgggctagtggactgctacattaaccttggagcacgctggtcccttgactatatggacaacgtcaacccatttaaccaccaccgcaatgctggcctgcgctaccgctcaatgttgctgggcaatggtcgctatgtgcccttccacatccaggtgcctcagaagttctttgccattaaaaacctccttctcctgccgggctcatacacctacgagtggaacttcaggaaggatgttaacatggttctgcagagctccctaggaaatgacctaagggttgacggagccagcattaagtttgatagcatttgcctttacgccaccttcttccccatggcccacaacaccgcctccacgcttgaggccatgcttagaaacgacaccaacgaccagtcctttaacgactatctctccgccgccaacatgctctaccctatacccgccaacgctaccaacgtgcccatatccatcccctcccgcaactgggcggctttccgcggctgggccttcacgcgccttaagactaaggaaaccccatcactgggctcgggctacgacccttattacacctactctggctctataccctacctagatggaaccttttacctcaaccacacctttaagaaggtggccattacctttgactcttctgtcagctggcctggcaatgaccgcctgcttacccccaacgagtttgaaattaagcgctcagttgacggggagggttacaacgttgcccagtgtaacatgaccaaagactggttcctggtacaaatgctagctaactataacattggctaccagggcttctatatcccagagagctacaaggaccgcatgtactccttctttagaaacttccagcccatgagccgtcaggtggtggatgatactaaatacaaggactaccaacaggtgggcatcctacaccaacacaacaactctggatttgttggctaccttgcccccaccatgcgcgaaggacaggcctaccctgctaacttcccctatccgcttataggcaagaccgcagttgacagcattacccagaaaaagtttctttgcgatcgcaccctttggcgcatcccattctccagtaactttatgtccatgggcgcactcacagacctgggccaaaaccttctctacgccaactccgcccacgcgctagacatgacttttgaggtggatcccatggacgagcccacccttctttatgttttgtttgaagtctttgacgtggtccgtgtgcaccagccgcaccgcggcgtcatcgaaaccgtgtacctgcgcacgcccttctcggccggcaacgccacaacataaagaagcaagcaacatcaacaacagctgccgccatgggctccagtgagcaggaactgaaagccattgtcaaagatcttggttgtgggccatattttttgggcacctatgacaagcgctttccaggctttgtttctccacacaagctcgcctgcgccatagtcaatacggccggtcgcgagactgggggcgtacactggatggcctttgcctggaacccgcactcaaaaacatgctacctctttgagccctttggcttttctgaccagcgactcaagcaggtttaccagtttgagtacgagtcactcctgcgccgtagcgccattgcttcttcccccgaccgctgtataacgctggaaaagtccacccaaagcgtacaggggcccaactcggccgcctgtggactattctgctgcatgtttctccacgcctttgccaactggccccaaactcccatggatcacaaccccaccatgaaccttattaccggggtacccaactccatgctcaacagtccccaggtacagcccaccctgcgtcgcaaccaggaacagctctacagcttcctggagcgccactcgccctacttccgcagccacagtgcgcagattaggagcgccacttctttttgtcacttgaaaaacatgtaaaaataatgtactagagacactttcaataaaggcaaatgcttttatttgtacactctcgggtgattatttacccccacccttgccgtctgcgccgtttaaaaatcaaaggggttctgccgcgcatcgctatgcgccactggcagggacacgttgcgatactggtgtttagtgctccacttaaactcaggcacaaccatccgcggcagctcggtgaagttttcactccacaggctgcgcaccatcaccaacgcgtttagcaggtcgggcgccgatatcttgaagtcgcagttggggcctccgccctgcgcgcgcgagttgcgatacacagggttgcagcactggaacactatcagcgccgggtggtgcacgctggccagcacgctcttgtcggagatcagatccgcgtccaggtcctccgcgttgctcagggcgaacggagtcaactttggtagctgccttcccaaaaagggcgcgtgcccaggctttgagttgcactcgcaccgtagtggcatcaaaaggtgaccgtgcccggtctgggcgttaggatacagcgcctgcataaaagccttgatctgcttaaaagccacctgagcctttgcgccttcagagaagaacatgccgcaagacttgccggaaaactgattggccggacaggccgcgtcgtgcacgcagcaccttgcgtcggtgttggagatctgcaccacatttcggccccaccggttcttcacgatcttggccttgctagactgctccttcagcgcgcgctgcccgttttcgctcgtcacatccatttcaatcacgtgctccttatttatcataatgcttccgtgtagacacttaagctcgccttcgatctcagcgcagcggtgcagccacaacgcgcagcccgtgggctcgtgatgcttgtaggtcacctctgcaaacgactgcaggtacgcctgcaggaatcgccccatcatcgtcacaaaggtcttgttgctggtgaaggtcagctgcaacccgcggtgctcctcgttcagccaggtcttgcatacggccgccagagcttccacttggtcaggcagtagtttgaagttcgcctttagatcgttatccacgtggtacttgtccatcagcgcgcgcgcagcctccatgcccttctcccacgcagacacgatcggcacactcagcgggttcatcaccgtaatttcactttccgcttcgctgggctcttcctcttcctcttgcgtccgcataccacgcgccactgggtcgtcttcattcagccgccgcactgtgcgcttacctcctttgccatgcttgattagcaccggtgggttgctgaaacccaccatttgtagcgccacatcttctctttcttcctcgctgtccacgattacctctggtgatggcgggcgctcgggcttgggagaagggcgcttctttttcttcttgggcgcaatggccaaatccgccgccgaggtcgatggccgcgggctgggtgtgcgcggcaccagcgcgtcttgtgatgagtcttcctcgtcctcggactcgatacgccgcctcatccgcttttttgggggcgcccggggaggcggcggcgacggggacggggacgacacgtcctccatggttgggggacgtcgcgccgcaccgcgtccgcgctcgggggtggtttcgcgctgctcctcttcccgactggccatttccttctcctataggcagaaaaagatcatggagtcagtcgagaagaaggacagcctaaccgccccctctgagttcgccaccaccgcctccaccgatgccgccaacgcgcctaccaccttccccgtcgaggcacccccgcttgaggaggaggaagtgattatcgagcaggacccaggttttgtaagcgaagacgacgaggaccgctcagtaccaacagaggataaaaagcaagaccaggacaacgcagaggcaaacgaggaacaagtcgggcggggggacgaaaggcatggcgactacctagatgtgggagacgacgtgctgttgaagcatctgcagcgccagtgcgccattatctgcgacgcgttgcaagagcgcagcgatgtgcccctcgccatagcggatgtcagccttgcctacgaacgccacctattctcaccgcgcgtaccccccaaacgccaagaaaacggcacatgcgagcccaacccgcgcctcaacttctaccccgtatttgccgtgccagaggtgcttgccacctatcacatctttttccaaaactgcaagatacccctatcctgccgtgccaaccgcagccgagcggacaagcagctggccttgcggcagggcgctgtcatacctgatatcgcctcgctcaacgaagtgccaaaaatctttgagggtcttggacgcgacgagaagcgcgcggcaaacgctctgcaacaggaaaacagcgaaaatgaaagtcactctggagtgttggtggaactcgagggtgacaacgcgcgcctagccgtactaaaacgcagcatcgaggtcacccactttgcctacccggcacttaacctaccccccaaggtcatgagcacagtcatgagtgagctgatcgtgcgccgtgcgcagcccctggagagggatgcaaatttgcaagaacaaacagaggagggcctacccgcagttggcgacgagcagctagcgcgctggcttcaaacgcgcgagcctgccgacttggaggagcgacgcaaactaatgatggccgcagtgctcgttaccgtggagcttgagtgcatgcagcggttctttgctgacccggagatgcagcgcaagctagaggaaacattgcactacacctttcgacagggctacgtacgccaggcctgcaagatctccaacgtggagctctgcaacctggtctcctaccttggaattttgcacgaaaaccgccttgggcaaaacgtgcttcattccacgctcaagggcgaggcgcgccgcgactacgtccgcgactgcgtttacttatttctatgctacacctggcagacggccatgggcgtttggcagcagtgcttggaggagtgcaacctcaaggagctgcagaaactgctaaagcaaaacttgaaggacctatggacggccttcaacgagcgctccgtggccgcgcacctggcggacatcattttccccgaacgcctgcttaaaaccctgcaacagggtctgccagacttcaccagtcaaagcatgttgcagaactttaggaactttatcctagagcgctcaggaatcttgcccgccacctgctgtgcacttcctagcgactttgtgcccattaagtaccgcgaatgccctccgccgctttggggccactgctaccttctgcagctagccaactaccttgcctaccactctgacataatggaagacgtgagcggtgacggtctactggagtgtcactgtcgctgcaacctatgcaccccgcaccgctccctggtttgcaattcgcagctgcttaacgaaagtcaaattatcggtacctttgagctgcagggtccctcgcctgacgaaaagtccgcggctccggggttgaaactcactccggggctgtggacgtcggcttaccttcgcaaatttgtacctgaggactaccacgcccacgagattaggttctacgaagaccaatcccgcccgcctaatgcggagcttaccgcctgcgtcattacccagggccacattcttggccaattgcaagccatcaacaaagcccgccaagagtttctgctacgaaagggacggggggtttacttggacccccagtccggcgaggagctcaacccaatccccccgccgccgcagccctatcagcagcagccgcgggcccttgcttcccaggatggcacccaaaaagaagctgcagctgccgccgccacccacggacgaggaggaatactgggacagtcaggcagaggaggttttggacgaggaggaggaggacatgatggaagactgggagagcctagacgaggaagcttccgaggtcgaagaggtgtcagacgaaacaccgtcaccctcggtcgcattcccctcgccggcgccccagaaatcggcaaccggttccagcatggctacaacctccgctcctcaggcgccgccggcactgcccgttcgccgacccaaccgtagatgggacaccactggaaccagggccggtaagtccaagcagccgccgccgttagcccaagagcaacaacagcgccaaggctaccgctcatggcgcgggcacaagaacgccatagttgcttgcttgcaagactgtgggggcaacatctccttcgcccgccgctttcttctctaccatcacggcgtggccttcccccgtaacatcctgcattactaccgtcatctctacagcccatactgcaccggcggcagcggcagcaacagcagcggccacacagaagcaaaggcgaccggatagcaagactctgacaaagcccaagaaatccacagcggcggcagcagcaggaggaggagcgctgcgtctggcgcccaacgaacccgtatcgacccgcgagcttagaaacaggatttttcccactctgtatgctatatttcaacagagcaggggccaagaacaagagctgaaaataaaaaacaggtctctgcgatccctcacccgcagctgcctgtatcacaaaagcgaagatcagcttcggcgcacgctggaagacgcggaggctctcttcagtaaatactgcgcgctgactcttaaggactagtttcgcgccctttctcaaatttaagcgcgaaaactacgtcatctccagcggccacacccggcgccagcacctgttgtcagcgccattatgagcaaggaaattcccacgccctacatgtggagttaccagccacaaatgggacttgcggctggagctgcccaagactactcaacccgaataaactacatgagcgcgggaccccacatgatatcccgggtcaacggaatacgcgcccaccgaaaccgaattctcctggaacaggcggctattaccaccacacctcgtaataaccttaatccccgtagttggcccgctgccctggtgtaccaggaaagtcccgctcccaccactgtggtacttcccagagacgcccaggccgaagttcagatgactaactcaggggcgcagcttgcgggcggctttcgtcacagggtgcggtcgcccgggcagggtataactcacctgacaatcagagggcgaggtattcagctcaacgacgagtcggtgagctcctcgcttggtctccgtccggacgggacatttcagatcggcggcgccggccgctcttcattcacgcctcgtcaggcaatcctaactctgcagacctcgtcctctgagccgcgctctggaggcattggaactctgcaatttattgaggagtttgtgccatcggtctactttaaccccttctcgggacctcccggccactatccggatcaatttattcctaactttgacgcggtaaaggactcggcggacggctacgactgaatgttaagtggagaggcagagcaactgcgcctgaaacacctggtccactgtcgccgccacaagtgctttgcccgcgactccggtgagttttgctactttgaattgcccgaggatcatatcgagggcccggcgcacggcgtccggcttaccgcccagggagagcttgcccgtagcctgattcgggagtttacccagcgccccctgctagttgagcgggacaggggaccctgtgttctcactgtgatttgcaactgtcctaaccctggattacatcaagatcctctagttaatgtcaggtcgcctaagtcgattaactagagtacccggggatcttattccctttaactaataaaaaaaaataataaagcatcacttacttaaaatcagttagcaaatttctgtccagtttattcagcagcacctccttgccctcctcccagctctggtattgcagcttcctcctggctgcaaactttctccacaatctaaatggaatgtcagtttcctcctgttcctgtccatccgcacccactatcttcatgttgttgcagatgaagcgcgcaagaccgtctgaagataccttcaaccccgtgtatccatatgacacggaaaccggtcctccaactgtgccttttcttactcctccctttgtatcccccaatgggtttcaagagagtccccctggggtactctctttgcgcctatccgaacctctagttacctccaatggcatgcttgcgctcaaaatgggcaacggcctctctctggacgaggccggcaaccttacctcccaaaatgtaaccactgtgagcccacctctcaaaaaaaccaagtcaaacataaacctggaaatatctgcacccctcacagttacctcagaagccctaactgtggctgccgccgcacctctaatggtcgcgggcaacacactcaccatgcaatcacaggccccgctaaccgtgcacgactccaaacttagcattgccacccaaggacccctcacagtgtcagaaggaaagctagccctgcaaacatcaggccccctcaccaccaccgatagcagtacccttactatcactgcctcaccccctctaactactgccactggtagcttgggcattgacttgaaagagcccatttatacacaaaatggaaaactaggactaaagtacggggctcctttgcatgtaacagacgacctaaacactttgaccgtagcaactggtccaggtgtgactattaataatacttccttgcaaactaaagttactggagccttgggttttgattcacaaggcaatatgcaacttaatgtagcaggaggactaaggattgattctcaaaacagacgccttatacttgatgttagttatccgtttgatgctcaaaaccaactaaatctaagactaggacagggccctctttttataaactcagcccacaacttggatattaactacaacaaaggcctttacttgtttacagcttcaaacaattccaaaaagcttgaggttaacctaagcactgccaaggggttgatgtttgacgctacagccatagccattaatgcaggagatgggcttgaatttggttcacctaatgcaccaaacacaaatcccctcaaaacaaaaattggccatggcctagaatttgattcaaacaaggctatggttcctaaactaggaactggccttagttttgacagcacaggtgccattacagtaggaaacaaaaataatgataagctaactttgtggaccacaccagctccatctcctaactgtagactaaatgcagagaaagatgctaaactcactttggtcttaacaaaatgtggcagtcaaatacttgctacagtttcagttttggctgttaaaggcagtttggctccaatatctggaacagttcaaagtgctcatcttattataagatttgacgaaaatggagtgctactaaacaattccttcctggacccagaatattggaactttagaaatggagatcttactgaaggcacagcctatacaaacgctgttggatttatgcctaacctatcagcttatccaaaatctcacggtaaaactgccaaaagtaacattgtcagtcaagtttacttaaacggagacaaaactaaacctgtaacactaaccattacactaaacggtacacaggaaacaggagacacaactccaagtgcatactctatgtcattttcatgggactggtctggccacaactacattaatgaaatatttgccacatcctcttacactttttcatacattgcccaagaataaagaatcgtttgtgttatgtttcaacgtgtttatttttcaattgcagaaaatttcaagtcatttttcattcagtagtatagccccaccaccacatagcttatacagatcaccgtaccttaatcaaactcacagaaccctagtattcaacctgccacctccctcccaacacacagagtacacagtcctttctccccggctggccttaaaaagcatcatatcatgggtaacagacatattcttaggtgttatattccacacggtttcctgtcgagccaaacgctcatcagtgatattaataaactccccgggcagctcacttaagttcatgtcgctgtccagctgctgagccacaggctgctgtccaacttgcggttgcttaacgggcggcgaaggagaagtccacgcctacatgggggtagagtcataatcgtgcatcaggatagggcggtggtgctgcagcagcgcgcgaataaactgctgccgccgccgctccgtcctgcaggaatacaacatggcagtggtctcctcagcgatgattcgcaccgcccgcagcataaggcgccttgtcctccgggcacagcagcgcaccctgatctcacttaaatcagcacagtaactgcagcacagcaccacaatattgttcaaaatcccacagtgcaaggcgctgtatccaaagctcatggcggggaccacagaacccacgtggccatcataccacaagcgcaggtagattaagtggcgacccctcataaacacgctggacataaacattacctcttttggcatgttgtaattcaccacctcccggtaccatataaacctctgattaaacatggcgccatccaccaccatcctaaaccagctggccaaaacctgcccgccggctatacactgcagggaaccgggactggaacaatgacagtggagagcccaggactcgtaaccatggatcatcatgctcgtcatgatatcaatgttggcacaacacaggcacacgtgcatacacttcctcaggattacaagctcctcccgcgttagaaccatatcccagggaacaacccattcctgaatcagcgtaaatcccacactgcagggaagacctcgcacgtaactcacgttgtgcattgtcaaagtgttacattcgggcagcagcggatgatcctccagtatggtagcgcgggtttctgtctcaaaaggaggtagacgatccctactgtacggagtgcgccgagacaaccgagatcgtgttggtcgtagtgtcatgccaaatggaacgccggacgtagtcatatttcctgaagcaaaaccaggtgcgggcgtgacaaacagatctgcgtctccggtctcgccgcttagatcgctctgtgtagtagttgtagtatatccactctctcaaagcatccaggcgccccctggcttcgggttctatgtaaactccttcatgcgccgctgccctgataacatccaccaccgcagaataagccacacccagccaacctacacattcgttctgcgagtcacacacgggaggagcgggaagagctggaagaaccatgtttttttttttattccaaaagattatccaaaacctcaaaatgaagatctattaagtgaacgcgctcccctccggtggcgtggtcaaactctacagccaaagaacagataatggcatttgtaagatgttgcacaatggcttccaaaaggcaaacggccctcacgtccaagtggacgtaaaggctaaacccttcagggtgaatctcctctataaacattccagcaccttcaaccatgcccaaataattctcatctcgccaccttctcaatatatctctaagcaaatcccgaatattaagtccggccattgtaaaaatctgctccagagcgccctccaccttcagcctcaagcagcgaatcatgattgcaaaaattcaggttcctcacagacctgtataagattcaaaagcggaacattaacaaaaataccgcgatcccgtaggtcccttcgcagggccagctgaacataatcgtgcaggtctgcacggaccagcgcggccacttccccgccaggaaccatgacaaaagaacccacactgattatgacacgcatactcggagctatgctaaccagcgtagccccgatgtaagcttgttgcatgggcggcgatataaaatgcaaggtgctgctcaaaaaatcaggcaaagcctcgcgcaaaaaagaaagcacatcgtagtcatgctcatgcagataaaggcaggtaagctccggaaccaccacagaaaaagacaccatttttctctcaaacatgtctgcgggtttctgcataaacacaaaataaaataacaaaaaaacatttaaacattagaagcctgtcttacaacaggaaaaacaacccttataagcataagacggactacggccatgccggcgtgaccgtaaaaaaactggtcaccgtgattaaaaagcaccaccgacagctcctcggtcatgtccggagtcataatgtaagactcggtaaacacatcaggttgattcacatcggtcagtgctaaaaagcgaccgaaatagcccgggggaatacatacccgcaggcgtagagacaacattacagcccccataggaggtataacaaaattaataggagagaaaaacacataaacacctgaaaaaccctcctgcctaggcaaaatagcaccctcccgctccagaacaacatacagcgcttccacagcggcagccataacagtcagccttaccagtaaaaaagaaaacctattaaaaaaacaccactcgacacggcaccagctcaatcagtcacagtgtaaaaaagggccaagtgcagagcgagtatatataggactaaaaaatgacgtaacggttaaagtccacaaaaaacacccagaaaaccgcacgcgaacctacgcccagaaacgaaagccaaaaaacccacaacttcctcaaatcgtcacttccgttttcccacgttacgtcacttcccattttaagaaaactacaattcccaacacatacaagttactccgccctaaaacctacgtcacccgccccgttcccacgccccgcgccacgtcacaaactccaccccctcattatcatattggcttcaatccaaaataaggtatattattgatgatgttaattaacatgcatggatcctacgtctcgaccgatgcccttgagagccttcaacccagtcagctccttccggtgggcgcggggcatgactatcgtcgccgcacttatgactgtcttctttatcatgcaactcgtaggacaggtgccggcagcgctctgggtcattttcggcgaggaccgctttcgctggagcgcgacgatgatcggcctgtcgcttgcggtattcggaatcttgcacgccctcgctcaagccttcgtcactggtcccgccaccaaacgtttcggcgagaagcaggccattatcgccggcatggcggccgacgcgctgggctacgtcttgctggcgttcgcgacgcgaggctggatggccttccccattatgattcttctcgcttccggcggcatcgggatgcccgcgttgcaggccatgctgtccaggcaggtagatgacgaccatcagggacagcttcaaggatcgctcgcggctcttaccagcctaacttcgatcattggaccgctgatcgtcacggcgatttatgccgcctcggcgagcacatggaacgggttggcatggattgtaggcgccgccctataccttgtctgcctccccgcgttgcgtcgcggtgcatggagccgggccacctcgacctgaatggaagccggcggcacctcgctaacggattcaccactccaagaattggagccaatcaattcttgcggagaactgtgaatgcgcaaaccaacccttggcagaacatatccatcgcgtccgccatctccagcagccgcacgcggcgcatctcgggcagcgttgggtcctggccacgggtgcgcatgatcgtgctcctgtcgttgaggacccggctaggctggcggggttgccttactggttagcagaatgaatcaccgatacgcgagcgaacgtgaagcgactgctgctgcaaaacgtctgcgacctgagcaacaacatgaatggtcttcggtttccgtgtttcgtaaagtctggaaacgcggaagtcagcgccctgcaccattatgttccggatctgcatcgcaggatgctgctggctaccctgtggaacacctacatctgtattaacgaagcgctggcattgaccctgagtgatttttctctggtcccgccgcatccataccgccagttgtttaccctcacaacgttccagtaaccgggcatgttcatcatcagtaacccgtatcgtgagcatcctctctcgtttcatcggtatcattacccccatgaacagaaatcccccttacacggaggcatcagtgaccaaacaggaaaaaaccgcccttaacatggcccgctttatcagaagccagacattaacgcttctggagaaactcaacgagctggacgcggatgaacaggcagacatctgtgaatcgcttcacgaccacgctgatgagctttaccgcagctgcctcgcgcgtttcggtgatgacggtgaaaacctctgacacatgcagctcccggagacggtcacagcttgtctgtaagcggatgccgggagcagacaagcccgtcagggcgcgtcagcgggtgttggcgggtgtcggggcgcagccatgacccagtcacgtagcgatagcggagtgtatactggcttaactatgcggcatcagagcagattgtactgagagtgcaccatatgcggtgtgaaataccgcacagatgcgtaaggagaaaataccgcatcaggcgctcttccgcttcctcgctcactgactcgctgcgctcggtcgttcggctgcggcgagcggtatcagctcactcaaaggcggtaatacggttatccacagaatcaggggataacgcaggaaagaacatgtgagcaaaaggccagcaaaaggccaggaaccgtaaaaaggccgcgttgctggcgtttttccataggctccgcccccctgacgagcatcacaaaaatcgacgctcaagtcagaggtggcgaaacccgacaggactataaagataccaggcgtttccccctggaagctccctcgtgcgctctcctgttccgaccctgccgcttaccggatacctgtccgcctttctcccttcgggaagcgtggcgctttctcatagctcacgctgtaggtatctcagttcggtgtaggtcgttcgctccaagctgggctgtgtgcacgaaccccccgttcagcccgaccgctgcgccttatccggtaactatcgtcttgagtccaacccggtaagacacgacttatcgccactggcagcagccactggtaacaggattagcagagcgaggtatgtaggcggtgctacagagttcttgaagtggtggcctaactacggctacactagaaggacagtatttggtatctgcgctctgctgaagccagttaccttcggaaaaagagttggtagctcttgatccggcaaacaaaccaccgctggtagcggtggtttttttgtttgcaagcagcagattacgcgcagaaaaaaaggatctcaagaagatcctttgatcttttctacggggtctgacgctcagtggaacgaaaactcacgttaagggattttggtcatgagattatcaaaaaggatcttcacctagatccttttaaattaaaaatgaagttttaaatcaatctaaagtatatatgagtaaacttggtctgacagttaccaatgcttaatcagtgaggcacctatctcagcgatctgtctatttcgttcatccatagttgcctgactccccgtcgtgtagataactacgatacgggagggcttaccatctggccccagtgctgcaatgataccgcgagacccacgctcaccggctccagatttatcagcaataaaccagccagccggaagggccgagcgcagaagtggtcctgcaactttatccgcctccatccagtctattaattgttgccgggaagctagagtaagtagttcgccagttaatagtttgcgcaacgttgttgccattgctgcaggcatcgtggtgtcacgctcgtcgtttggtatggcttcattcagctccggttcccaacgatcaaggcgagttacatgatcccccatgttgtgcaaaaaagcggttagctccttcggtcctccgatcgttgtcagaagtaagttggccgcagtgttatcactcatggttatggcagcactgcataattctcttactgtcatgccatccgtaagatgcttttctgtgactggtgagtactcaaccaagtcattctgagaatagtgtatgcggcgaccgagttgctcttgcccggcgtcaacacgggataataccgcgccacatagcagaactttaaaagtgctcatcattggaaaacgttcttcggggcgaaaactctcaaggatcttaccgctgttgagatccagttcgatgtaacccactcgtgcacccaactgatcttcagcatcttttactttcaccagcgtttctgggtgagcaaaaacaggaaggcaaaatgccgcaaaaaagggaataagggcgacacggaaatgttgaatactcatactcttcctttttcaatattattgaagcatttatcagggttattgtctcatgagcggatacatatttgaatgtatttagaaaaataaacaaataggggttccgcgcacatttccccgaaaagtgccacctgtctagctacgaattcttcgacagcttcgaaactagaatcgatttcgaaactagcttaagggtgggaaagaatatataaggtgggggtcttatgtagttttgtatctgttttgcagcagccgccgccgccatgagcaccaactcgtttgatggaagc

SEQ ID NO: 8 - DNA, 8108 bp, Artificial Sequence
  pAD_Track8509
  misc_feature (9)..(11): n is a, c, g, or t
  misc_feature (352)..(354): n is a, c, g, or t
  misc_feature (1942)..(1944): n is a, c, g, or t
  misc_feature (2001)..(2003): n is a, c, g, or t
  misc_feature (4244)..(4246): n is a, c, g, or t
  misc_feature (4261)..(4263): n is a, c, g, or t
  misc_feature (5246)..(5248): n is a, c, g, or t
  misc_feature (5263)..(5265): n is a, c, g, or t
  misc_feature (6566)..(6571): n is a, c, g, or t
ttaattaannntcccttccagctctctgccccttttggattgaagccaatatgataatgagggggtggagtttgtgacgtggcgcggggcgtgggaacggggcgggtgacgtagtagtgtggcggaagtgtgatgttgcaagtgtggcggaacacatgtaagcgacggatgtggcaaaagtgacgtttttggtgtgcgccggtgtacacaggaagtgacaattttcgcgcggttttaggcggatgttgtagtaaatttgggcgtaaccgagtaagatttggccattttcgcgggaaaactgaataagaggaagtgaaatctgaataattttgtgttactcatagcgcgtaannncgcgttaagatacattgatgagtttggacaaaccacaactagaatgcagtgaaaaaaatgctttatttgtgaaatttgtgatgctattgctttatttgtaaccattataagctgcaataaacaagttaacaacaacaattgcattcattttatgtttcaggttcagggggaggtgtgggaggttttttaaagcaagtaaaacctctacaaatgtggtatggctgattatgatcagttatctagatccggtggatctgagtccggacttgtacagctcgtccatgccgagagtgatcccggcggcggtcacgaactccagcaggaccatgtgatcgcgcttctcgttggggtctttgctcagggcggactgggtgctcaggtagtggttgtcgggcagcagcacggggccgtcgccgatgggggtgttctgctggtagtggtcggcgagctgcacgctgccgtcctcgatgttgtggcggatcttgaagttcaccttgatgccgttcttctgcttgtcggccatgatatagacgttgtggctgttgtagttgtactccagcttgtgccccaggatgttgccgtcctccttgaagtcgatgcccttcagctcgatgcggttcaccagggtgtcgccctcgaacttcacctcggcgcgggtcttgtagttgccgtcgtccttgaagaagatggtgcgctcctggacgtagccttcgggcatggcggacttgaagaagtcgtgctgcttcatgtggtcggggtagcggctgaagcactgcacgccgtaggtcagggtggtcacgagggtgggccagggcacgggcagcttgccggtggtgcagatgaacttcagggtcagcttgccgtaggtggcatcgccctcgccctcgccggacacgctgaacttgtggccgtttacgtcgccgtccagctcgaccaggatgggcaccaccccggtgaacagctcctcgcccttgctcaccatggtggcgaccggtagcgctagcggatctgacggttcactaaaccagctctgcttatatagacctcccaccgtacacgcctaccgcccatttgcgtcaatggggcggagttgttacgacattttggaaagtcccgttgattttggtgccaaaacaaactcccattgacgtcaatggggtggagacttggaaatccccgtgagtcaaaccgctatccacgcccattgatgtactgccaaaaccgcatcaccatggtaatagcgatgactaatacgtagatgtactgccaagtaggaaagtcccataaggtcatgtactgggcataatgccaggcgggccatttaccgtcattgacgtcaatagggggcgtacttggcatatgatacacttgatgtactgccaagtgggcagtttaccgtaaatactccacccattgacgtcaatggaaagtccctattggcgttactatgggaacatacgtcattattgacgtcaatgggcgggggtcgttgggcggtcagccaggcgggccatttaccgtaagttatgtaacgcggaactccatatatgggctatgaactaatgaccccgtaattgattactattannnctagcagatctggtaccgtcgacgcggccgcgatatcctcgagaagctttctagagnnntaagggtgggaaagaatatataaggtgggggtcttatgtagttttgtatctgttttgcagcagccgccgccgccatgagcaccaactcgtttgatggaagcattgtgagctcatatttgacaacgcgcatgcccccatgggccggggtgcgtcagaatgtgatgggctccagcattgatggtcgccccgtcctgcccgcaaactctactaccttgacctacgagaccgtgtctggaacgccgttggagactgcagcctccgccgccgcttcagccgctgcagccaccgcccgcgggattgtgactgactttgctttcctgagcccgcttgcaagcagtgcagcttcccgttcatccgcccgcgatgacaagttgacggctcttttggcacaattggattctttgacccgggaacttaatgtcgtttctcagcagctgttggatctgcgccagcaggtttctgccctgaaggcttcctcccctcccaatgcggtttaaaacataaataaaaaaccagactctgtttggatttggatcaagcaagtgtcttgctgtctttatttaggggttttgcgcgcgcggtaggcccgggaccagcggtctcggtcgttgagggtcctgtgtattttttccaggacgtggtaaaggtgactctggatgttcagatacatgggcataagcccgtctctggggtggaggtagcaccactgcagagcttcatgctgcggggtggtgttgtagatgatccagtcgtagcaggagcgctgggcgtggtgcctaaaaatgtctttcagtagcaagctgattgccaggggcaggcccttggtgtaagtgtttacaaagcggttaagctgggatgggtgcatacgtggggatatgagatgcatcttggactgtatttttaggttggctatgttcccagccatatccctccggggattcatgttgtgcagaaccaccagcacagtgtatccggtgcacttgggaaatttgtcatgtagcttagaaggaaatgcgtggaagaacttggagacgcccttgtgacctccaagattttccatgcattcgtccataatgatggcaatgggcccacgggcggcggcctgggcgaagatatttctgggatcactaacgtcatagttgtgttccaggatgagatcgtcataggccatttttacaaagcgcgggcggagggtgccagactgcggtataatggttccatccggcccaggggcgtagttaccctcacagatttgcatttcccacgctttgagttcagatggggggatcatgtctacctgcggggcgatgaagaaaacggtttccggggtaggggagatcagctgggaagaaagcaggttcctgagcagctgcgacttaccgcagccggtgggcccgtaaatcacacctattaccgggtgcaactggtagttaagagagctgcagctgccgtcatccctgagcaggggggccacttcgttaagcatgtccctgactcgcatgttttccctgaccaaatccgccagaaggcgctcgccgcccagcgatagcagttcttgcaaggaagcaaagtttttcaacggtttgagaccgtccgccgtaggcatgcttttgagcgtttgaccaagcagttccaggcggtcccacagctcggtcacctgctctacggcatctcgatccagcatatctcctcgtttcgcgggttggggcggctttcgctgtacggcagtagtcggtgctcgtccagacgggccagggtcatgtctttccacgggcgcagggtcctcgtcagcgtagtctgggtcacggtgaaggggtgcgctccgggctgcgcgctggccagggtgcgcttgaggctggtcctgctggtgctgaagcgctgccggtcttcgccctgcgcgtcggccaggtagcatttgaccatggtgtcatagtccagcccctccgcggcgtggcccttggcgcgcagcttgcccttggaggaggcgccgcacgaggggcagtgcagacttttgagggcgtagagcttgggcgcgagaaataccgattccggggagtaggcatccgcgccgcaggccccgcagacggtctcgcattccacgagccaggtgagctctggccgttcggggtcaaaaaccaggtttcccccatgctttttgatgcgtttcttacctctggtttccatgagccggtgtccacgctcggtgacgaaaaggctgtccgtgtccccgtatacagactnnngtttaaacgaattcnnntataaaatgcaaggtgctgctcaaaaaatcaggcaaagcctcgcgcaaaaaagaaagcacatcgtagtcatgctcatgcagataaaggcaggtaagctccggaaccaccacagaaaaagacaccatttttctctcaaacatgtctgcgggtttctgcataaacacaaaataaaataacaaaaaaacatttaaacattagaagcctgtcttacaacaggaaaaacaacccttataagcataagacggactacggccatgccggcgtgaccgtaaaaaaactggtcaccgtgattaaaaagcaccaccgacagctcctcggtcatgtccggagtcataatgtaagactcggtaaacacatcaggttgattcatcggtcagtgctaaaaagcgaccgaaatagcccgggggaatacatacccgcaggcgtagagacaacattacagcccccataggaggtataacaaaattaataggagagaaaaacacataaacacctgaaaaaccctcctgcctaggcaaaatagcaccctcccgctccagaacaacatacagcgcttcacagcggcagcctaacagtcagccttaccagtaaaaaagaaaacctattaaaaaaacaccactcgacacggcaccagctcaatcagtcacagtgtaaaaaagggccaagtgcagagcgagtatatataggactaaaaaatgacgtaacggttaaagtccacaaaaaacacccagaaaaccgcacgcgaacctacgcccagaaacgaaagccaaaaaacccacaacttcctcaaatcgtcacttccgttttcccacgttacgtaacttcccattttaagaaaactacaattcccaacacatacaagttactccgccctaaaacctacgtcacccgccccgttcccacgccccgcgccacgtcacaaactccaccccctcattatcatattggcttcaatccaaaataaggtatattattgatgatnnnttaattaaggatccnnncggtgtgaaataccgcacagatgcgtaaggagaaaataccgcatcaggcgctcttccgcttcctcgctcactgactcgctgcgctcggtcgttcggctgcggcgagcggtatcagctcactcaaaggcggtaatacggttatccacagaatcaggggataacgcaggaaagaacatgtgagcaaaaggccagcaaaaggccaggaaccgtaaaaaggccgcgttgctggcgtttttccataggctccgcccccctgacgagcatcacaaaaatcgacgctcaagtcagaggtggcgaaacccgacaggactataaagataccaggcgtttccccctggaagctccctcgtgcgctctcctgttccgaccctgccgcttaccggatacctgtccgcctttctcccttcgggaagcgtggcgctttctcatagctcacgctgtaggtatctcagttcggtgtaggtcgttcgctccaagctgggctgtgtgcacgaaccccccgttcagcccgaccgctgcgccttatccggtaactatcgtcttgagtccaacccggtaagacacgacttatcgccactggcagcagccactggtaacaggattagcagagcgaggtatgtaggcggtgctacagagttcttgaagtggtggcctaactacggctacactagaaggacagtatttggtatctgcgctctgctgaagccagttaccttcggaaaaagagttggtagctcttgatccggcaaacaaaccaccgctggtagcggtggtttttttgtttgcaagcagcagattacgcgcagaaaaaaaggatctcaagaagatcctttgatcttttctacggggtctgacgctcagtggaacgaaaactcacgttaagggattttggtcatgagattatcaaaaaggatcttcacctagatccttttaaattaaaaatgaagttttaaatcaatctaaagtatatatgagtaaacttggtctgacagttaccaatgcttaatcagtgaggcacctatctcagcgatctgtctatttcgttcatccatagttgcctgactccccgtcgtgtagataactacgatacgggagggcttaccatctggccccagtgctgcaatgataccgcgagacccacgctcaccggctccagatttatcagcaataaaccagccagccggaagggccgagcgcagaagtggtcctgcaactttatccgcctccatccagtctattaattgttgccgggaagctagagtaagtagttcgccagttaatagtttgcgcaacgttgttgnnnnnnaaaaaggatcttcacctagatccttttcacgtagaaagccagtccgcagaaacggtgctgaccccggatgaatgtcagctactgggctatctggacaagggaaaacgcaagcgcaaagagaaagcaggtagcttgcagtgggcttacatggcgatagctagactgggcggttttatggacagcaagcgaaccggaattgccagctggggcgccctctggtaaggttgggaagccctgcaaagtaaactggatggctttctcgccgccaaggatctgatggcgcaggggatcaagctctgatcaagagacaggatgaggatcgtttcgcatgattgaacaagatggattgcacgcaggttctccggccgcttgggtggagaggctattcggctatgactgggcacaacagacaatcggctgctctgatgccgccgtgttccggctgtcagcgcaggggcgcccggttctttttgtcaagaccgacctgtccggtgccctgaatgaactgcaagacgaggcagcgcggctatcgtggctggccacgacgggcgttccttgcgcagctgtgctcgacgttgtcactgaagcgggaagggactggctgctattgggcgaagtgccggggcaggatctcctgtcatctcaccttgctcctgccgagaaagtatccatcatggctgatgcaatgcggcggctgcatacgcttgatccggctacctgcccattcgaccaccaagcgaaacatcgcatcgagcgagcacgtactcggatggaagccggtcttgtcgatcaggatgatctggacgaagagcatcaggggctcgcgccagccgaactgttcgccaggctcaaggcgagcatgcccgacggcgaggatctcgtcgtgacccatggcgatgcctgcttgccgaatatcatggtggaaaatggccgcttttctggattcatcgactgtggccggctgggtgtggcggaccgctatcaggacatagcgttggctacccgtgatattgctgaagagcttggcggcgaatgggctgaccgcttcctcgtgctttacggtatcgccgctcccgattcgcagcgcatcgccttctatcgccttcttgacgagttcttctgaattttgttaaaatttttgttaaatcagctcattttttaaccaataggccgaaatcggcaacatcccttataaatcaaaagaatagaccgcgatagggttgagtgttgttccagtttggaacaagagtccactattaaagaacgtggactccaacgtcaaagggcgaaaaaccgtctatcagggcgatggcccactacgtgaaccatcacccaaatcaagttttttgcggtcgaggtgccgtaaagctctaaatcggaaccctaaagggagcccccgatttagagcttgacggggaaagccggcgaacgtggcgagaaaggaagggaagaaagcgaaaggagcgggcgctagggcgctggcaagtgtagcggtcacgctgcgcgtaaccaccacacccgcgcgcttaatgcgccg

SEQ ID NO: 9 - DNA, 9237 bp, Artificial Sequence
  pAdTrack-CMV
tgttaacttgtttattgcagcttataatggttacaaataaagcaatagcatcacaaatttcacaaataaagcatttttttcactgcattctagttgtggtttgtccaaactcatcaatgtatcttaacgcggaggtttatcgacgatctgctagtgattaatagtaatcaattacggggtcattagttcatagcccatatatggagttccgcgttacataacttacggtaaatggcccgcctggctgaccgcccaacgacccccgcccattgacgtcaataatgacgtatgttcccatagtaacgccaatagggactttccattgacgtcaatgggtggagtatttacggtaaactgcccacttggcagtacatcaagtgtatcatatgccaagtacgccccctattgacgtcaatgacggtaaatggcccgcctggcattatgcccagtacatgaccttatgggactttcctacttggcagtacatctacgtattagtcatcgctattaccatggtgatgcggttttggcagtacatcaatgggcgtggatagcggtttgactcacggggatttccaagtctccaccccattgacgtcaatgggagtttgttttggcaccaaaatcaacgggactttccaaaatgtcgtaacaactccgccccattgacgcaaatgggcggtaggcgtgtacggtgggaggtctatataagcagagctggtttagtgaaccgtcagatccgctagcgctaccggtcgccaccatggtgagcaagggcgaggagctgttcaccggggtggtgcccatcctggtcgagctggacggcgacgtaaacggccacaagttcagcgtgtccggcgagggcgagggcgatgccacctacggcaagctgaccctgaagttcatctgcaccaccggcaagctgcccgtgccctggcccaccctcgtgaccaccctgacctacggcgtgcagtgcttcagccgctaccccgaccacatgaagcagcacgacttcttcaagtccgccatgcccgaaggctacgtccaggagcgcaccatcttcttcaaggacgacggcaactacaagacccgcgccgaggtgaagttcgagggcgacaccctggtgaaccgcatcgagctgaagggcatcgacttcaaggaggacggcaacatcctggggcacaagctggagtacaactacaacagccacaacgtctatatcatggccgacaagcagaagaacggcatcaaggtgaacttcaagatccgccacaacatcgaggacggcagcgtgcagctcgccgaccactaccagcagaacacccccatcggcgacggccccgtgctgctgcccgacaaccactacctgagcacccagtccgccctgagcaaagaccccaacgagaagcgcgatcacatggtcctgctggagttcgtgaccgccgccgggatcactctcggcatggacgagctgtacaagtccggactcagatccaccggatctagataactgatcataatcagccataccacatttgtagaggttttacttgctttaaaaaacctcccacacctccccctgaacctgaaacataaaatgaatgcaattgttgttgttaacttgtttattgcagcttataatggttacaaataaagcaatagcatcacaaatttcacaaataaagcatttttttcactgcattctagttgtggtttgtccaaactcatcaatgtatcttaacgcgatcaagctagcttgctagactcgactgactataataataaaacgccaactttgacccggaacgcggaaaacacctgagaaaaacacctgggcgagtctccacgtaaacggtcaaagtccccgcggccctagacaaatattacgcgctatgagtaacacaaaattattcagatttcacttcctcttattcagttttcccgcgaaaatggccaaatcttactcggttacgcccaaatttactacaacatccgcctaaaaccgcgcgaaaattgtcacttcctgtgtacaccggcgcacaccaaaaacgtcacttttgccacatccgtcgcttacatgtgttccgccacacttgcaacatcacacttccgccacactactacgtcacccgccccgttcccacgccccgcgccacgtcacaaactccaccccctcattatcatattggcttcaatccaaaataaggtatattattgatgatgttaattaagaattaattcgatcctgaatggcgaatggacgcgccctgtagcggcgcattaagcgcggcgggtgtggtggttacgcgcagcgtgaccgctacacttgccagcgccctagcgcccgctcctttcgctttcttcccttcctttctcgccacgttcgccggctttccccgtcaagctctaaatcgggggctccctttagggttccgatttagtgctttacggcacctcgaccccaaaaaacttgattagggtgatggttcacgtagtgggccatcgccctgatagacggtttttcgccctttgacgttggagtccacgttctttaatagtggactcttgttccaaactggaacaacactcaaccctatctcggtctattcttttgatttataagggattttgccgatttcggcctattggttaaaaaatgagctgatttaacaaaaattttaacaaaattcagaagaactcgtcaagaaggcgatagaaggcgatgcgctgcgaatcgggagcggcgataccgtaaagcacgaggaagcggtcagcccattcgccgccaagctcttcagcaatatcacgggtagccaacgctatgtcctgatagcggtccgccacacccagccggccacagtcgatgaatccagaaaagcggccattttccaccatgatattcggcaagcaggcatcgccatgggtcacgacgagatcctcgccgtcgggcatgctcgccttgagcctggcgaacagttcggctggcgcgagcccctgatgctcttcgtccagatcatcctgatcgacaagaccggcttccatccgagtacgtgctcgctcgatgcgatgtttcgcttggtggtcgaatgggcaggtagccggatcaagcgtatgcagccgccgcattgcatcagccatgatggatactttctcggcaggagcaaggtgagatgacaggagatcctgccccggcacttcgcccaatagcagccagtcccttcccgcttcagtgacaacgtcgagcacagctgcgcaaggaacgcccgtcgtggccagccacgatagccgcgctgcctcgtcttgcagttcattcagggcaccggacaggtcggtcttgacaaaaagaaccgggcgcccctgcgctgacagccggaacacggcggcatcagagcagccgattgtctgttgtgcccagtcatagccgaatagcctctccacccaagcggccggagaacctgcgtgcaatccatcttgttcaatcatgcgaaacgatcctcatcctgtctcttgatcagagcttgatcccctgcgccatcagatccttggcggcaagaaagccatccagtttactttgcagggcttcccaaccttaccagagggcgccccagctggcaattccggttcgcttgctgtccataaaaccgcccagtctagctatcgccatgtaagcccactgcaagctacctgctttctctttgcgcttgcgttttcccttgtccagatagcccagtagctgacattcatccggggtcagcaccgtttctgcggactggctttctacgtgaaaaggatctaggtgaagatcctttttgataatctcatggctgcagcaatggcaacaacgttgcgcaaactattaactggcgaactacttactctagcttcccggcaacaattaatagactggatggaggcggataaagttgcaggaccacttctgcgctcggcccttccggctggctggtttattgctgataaatctggagccggtgagcgtgggtctcgcggtatcattgcagcactggggccagatggtaagccctcccgtatcgtagttatctacacgacggggagtcaggcaactatggatgaacgaaatagacagatcgctgagataggtgcctcactgattaagcattggtaactgtcagaccaagtttactcatatatactttagattgatttaaaacttcatttttaatttaaaaggatctaggtgaagatcctttttgataatctcatgaccaaaatcccttaacgtgagttttcgttccactgagcgtcagaccccgtagaaaagatcaaaggatcttcttgagatcctttttttctgcgcgtaatctgctgcttgcaaacaaaaaaaccaccgctaccagcggtggtttgtttgccggatcaagagctaccaactctttttccgaaggtaactggcttcagcagagcgcagataccaaatactgtccttctagtgtagccgtagttaggccaccacttcaagaactctgtagcaccgcctacatacctcgctctgctaatcctgttaccagtggctgctgccagtggcgataagtcgtgtcttaccgggttggactcaagacgatagttaccggataaggcgcagcggtcgggctgaacggggggttcgtgcacacagcccagcttggagcgaacgacctacaccgaactgagatacctacagcgtgagctatgagaaagcgccacgcttcccgaagggagaaaggcggacaggtatccggtaagcggcagggtcggaacaggagagcgcacgagggagcttccagggggaaacgcctggtatctttatagtcctgtcgggtttcgccacctctgacttgagcgtcgatttttgtgatgctcgtcaggggggcggagcctatggaaaaacgccagcaacgcggcctttttacggttcctggccttttgctggccttttgctcacatgttctttcctgcgttatcccctgattctgtggataaccgtattaccgcctttgagtgagctgataccgctcgccgcagccgaacgaccgagcgcagcgagtcagtgagcgaggaagcggaagagcgcctgatgcggtattttctccttacgcatctgtgcggtatttcacaccgcatatggatccatgcatgttaattaacatcatcaataatataccttattttggattgaagccaatatgataatgagggggtggagtttgtgacgtggcgcggggcgtgggaacggggcgggtgacgtaggttttagggcggagtaacttgtatgtgttgggaattgtagttttcttaaaatgggaagtgacgtaacgtgggaaaacggaagtgacgatttgaggaagttgtgggttttttggctttcgtttctgggcgtaggttcgcgtgcggttttctgggtgttttttgtggactttaaccgttacgtcattttttagtcctatatatactcgctctgcacttggcccttttttacactgtgactgattgagctggtgccgtgtcgagtggtgtttttttaataggttttcttttttactggtaaggctgactgttatggctgccgctgtggaagcgctgtatgttgttctggagcgggagggtgctattttgcctaggcaggagggtttttcaggtgtttatgtgtttttctctcctattaattttgttatacctcctatgggggctgtaatgttgtctctacgcctgcgggtatgtattcccccgggctatttcggtcgctttttagcactgaccgatgtgaatcaacctgatgtgtttaccgagtcttacattatgactccggacatgaccgaggagctgtcggtggtgctttttaatcacggtgaccagtttttttacggtcacgccggcatggccgtagtccgtcttatgcttataagggttgtttttcctgttgtaagacaggcttctaatgtttaaatgtttttttgttattttattttgtgtttatgcagaaacccgcagacatgtttgagagaaaaatggtgtctttttctgtggtggttccggagcttacctgcctttatctgcatgagcatgactacgatgtgctttcttttttgcgcgaggctttgcctgattttttgagcagcaccttgcattttatatcgccgcccatgcaacaagctattgaattcgtttaaactccctctcaagtctgtatacggggacacggacagccttttcgtcaccgagcgtggacaccggctcatggaaaccagaggtaagaaacgcatcaaaaagcatgggggaaacctggtttttgaccccgaacggccagagctcacctggctcgtggaatgcgagaccgtctgcggggcctgcggcgcggatgcctactccccggaatcggtatttctcgcgcccaagctctacgccctcaaaagtctgcactgcccctcgtgcggcgcctcctccaagggcaagctgcgcgccaagggccacgccgcggaggggctggactatgacaccatggtcaaatgctacctggccgacgcgcagggcgaagaccggcagcgcttcagcaccagcaggaccagcctcaagcgcaccctggccagcgcgcagcccggagcgcaccccttcaccgtgacccagactacgctgacgaggaccctgcgcccgtggaaagacatgaccctggcccgtctggacgagcaccgactactgccgtacagcgaaagccgccccaacccgcgaaacgaggagatatgctggatcgagatgccgtagagcaggtgaccgagctgtgggaccgcctggaactgcttggtcaaacgctcaaaagcatgcctacggcggacggtctcaaaccgttgaaaaactttgcttccttgcaagaactgctatcgctgggcggcgagcgccttctggcggatttggtcagggaaaacatgcgagtcagggacatgcttaacgaagtggcccccctgctcagggatgacggcagctgcagctctcttaactaccagttgcagccggtaataggtgtgatttacgggcccaccggctgcggtaagtcgcagctgctcaggaacctgctttcttcccagctgatctcccctaccccggaaaccgttttcttcatcgccccgcaggtagacatgatccccccatctgaactcaaagcgtgggaaatgcaaatctgtgagggtaactacgcccctgggccggatggaaccattataccgcagtctggcaccctccgcccgcgctttgtaaaaatggcctatgacgatctcatcctggaacacaactatgacgttagtgatcccagaaatatcttcgcccaggccgccgcccgtgggcccattgccatcattatggacgaatgcatggaaaatcttggaggtcacaagggcgtctccaagttcttccacgcatttccttctaagctacatgacaaatttcccaagtgcaccggatacactgtgctggtggttctgcacaacatgaatccccggagggatatggctgggaacatagccaacctaaaaatacagtccaagatgcatctcatatccccacgtatgcacccatcccagcttaaccgctttgtaaacacttacaccaagggcctgcccctggcaatcagcttgctactgaaagacatttttaggcaccacgcccagcgctcctgctacgactggatcatctacaacaccaccccgcagcatgaagctctgcagtggtgctacctccaccccagagacgggcttatgcccatgtatctgaacatccagagtcacctttaccacgtcctggaaaaaatacacaggaccctcaacgaccgagaccgctggtcccgggcctaccgcgcgcgcaaaacccctaaataaagacagcaagacacttgcttgatccaaatccaaacagagtctggttttttatttatgttttaaaccgcattgggaggggaggaagccttcagggcagaaacctgctggcgcagatccaacagctgctgagaaacgacattaagttcccgggtcaaagaatccaattgtgccaaaagagccgtcaacttgtcatcgcgggcggatgaacgggaagctgcactgcttgcaagcgggctcaggaaagcaaagtcagtcacaatcccgcgggcggtggctgcagcggctgaagcggcggcggaggctgcagtctccaacggcgttccagacacggtctcgtaggtcaaggtagtagagtttgcgggcaggacggggcgaccatcaatgctggagcccatcacattctgacgcaccccggcccatgggggcatgcgcgttgtcaaatatgagctcacaatgcttccatcaaacgagttggtgctcatggcggcggcggctgctgcaaaacagatacaaaactacataagacccccaccttatatattctttcccacccttaaccacgcccagatcctctagcagtgataaacgtctaatagtaatcaattacggggtcattagttcatagcccatatatggagttccgcgttacataacttacggtaaatggcccgcctggctgaccgcccaacgacccccgcccattgacgtcaataatgacgtatgttcccatagtaacgccaatagggactttccattgacgtcaatgggtggagtatttacggtaaactgcccacttggcagtacatcaagtgtatcatatgccaagtacgccccctattgacgtcaatgacggtaaatggcccgcctggcattatgcccagtacatgaccttatgggactttcctacttggcagtacatctacgtattagtcatcgctattaccatggtgatgcggttttggcagtacatcaatgggcgtggatagcggtttgactcacggggatttccaagtctccaccccattgacgtcaatgggagtttgttttggcaccaaaatcaacgggactttccaaaatgtcgtaacaactccgccccattgacgcaaatgggcggtaggcgtgtacggtgggaggtctatataagcagagctggtttagtgaaccgtcagatccgctagagatctggtaccgtcgacgcggccgctcgagcctaagcttctagataagatatccgatccaccggatctagataactgatcataatcagccataccacatttgtagaggttttacttgctttaaaaaacctcccacacctccccctgaacctgaaacataaaatgaatgcaattgttgt

SEQ ID NO: 10 - DNA, 7658 bp, Artificial Sequence
  pZB3 AAV dSaCas9
aaaacctctgacacatgcagctcccggagacggtcacagcttgtctgtaagcggatgccgggagcagacaagcccgtcagggcgcgtcagcgggtgttggcgggtgtcggggctggcttaactatgcggcatcagagcagattgtactgagagtgcaccataaaattgtaaacgttaatattttgttaaaattcgcgttaaatttttgttaaatcagctcattttttaaccaatagaccgaaatcggcaaaatcccttataaatcaaaagaatagcccgagatagagttgagtgttgttccagtttggaacaagagtccactattaaagaacgtggactccaacgtcaaagggcgaaaaaccgtctatcagggcgatggcccactacgtgaaccatcacccaaatcaagttttttggggtcgaggtgccgtaaagcactaaatcggaaccctaaagggagcccccgatttagagcttgacggggaaagccggcgaacgtggcgagaaaggaagggaagaaagcgaaaggagcgggcgctaaggcgctggcaagtgtagcggtcacgctgcgcgtaaccaccacacccgccgcgcttaatgcgccgctacagggcgcgtactatggttgctttgacgtatgcggtgtgaaataccgcacagatgcgtaaggagaaaataccgcatcaggcgcccctgcaggcagctgcgcgctcgctcgctcactgaggccgcccgggcaaagcccgggcgtcgggcgacctttggtcgcccggcctcagtgagcgagcgagcgcgcagagagggagtggccaactccatcactaggggttcctgcggccgcgagggcctatttcccatgattccttcatatttgcatatacgatacaaggctgttagagagataattggaattaatttgactgtaaacacaaagatattagtacaaaatacgtgacgtagaaagtaataatttcttgggtagtttgcagttttaaaattatgttttaaaatggactatcatatgcttaccgtaacttgaaagtatttcgatttcttggctttatatatcttgtggaaaggacgaaacaccgggagaccacggcaggtctcagttttagtactctggaggccaacatgaggatcacccatgtctgcagggccaacagaatctactaaaacaaggcaaaatgccgtgtttatctcgtcaacttgttggcgagatttttttggccgcctcgaggtacttatataagggggtgggggcgcgttcgtcctcagtcgcgatcgaacactcgagccgagcagacgtgcctacggaccgaccggtgccaccatggccccaaagaagaagcggaaggtcggtatccacggagtcccagcagccaagcggaactacatcctgggcctggccatcggcatcaccagcgtgggctacggcatcatcgactacgagacacgggacgtgatcgatgccggcgtgcggctgttcaaagaggccaacgtggaaaacaacgagggcaggcggagcaagagaggcgccagaaggctgaagcggcggaggcggcatagaatccagagagtgaagaagctgctgttcgactacaacctgctgaccgaccacagcgagctgagcggcatcaacccctacgaggccagagtgaagggcctgagccagaagctgagcgaggaagagttctctgccgccctgctgcacctggccaagagaagaggcgtgcacaacgtgaacgaggtggaagaggacaccggcaacgagctgtccaccaaagagcagatcagccggaacagcaaggccctggaagagaaatacgtggccgaactgcagctggaacggctgaagaaagacggcgaagtgcggggcagcatcaacagattcaagaccagcgactacgtgaaagaagccaaacagctgctgaaggtgcagaaggcctaccaccagctggaccagagcttcatcgacacctacatcgacctgctggaaacccggcggacctactatgagggacctggcgagggcagccccttcggctggaaggacatcaaagaatggtacgagatgctgatgggccactgcacctacttccccgaggaactgcggagcgtgaagtacgcctacaacgccgacctgtacaacgccctgaacgacctgaacaatctcgtgatcaccagggacgagaacgagaagctggaatattacgagaagttccagatcatcgagaacgtgttcaagcagaagaagaagcccaccctgaagcagatcgccaaagaaatcctcgtgaacgaagaggatattaagggctacagagtgaccagcaccggcaagcccgagttcaccaacctgaaggtgtaccacgacatcaaggacattaccgcccggaaagagattattgagaacgccgagctgctggatcagattgccaagatcctgaccatctaccagagcagcgaggacatccaggaagaactgaccaatctgaactccgagctgacccaggaagagatcgagcagatctctaatctgaagggctataccggcacccacaacctgagcctgaaggccatcaacctgatcctggacgagctgtggcacaccaacgacaaccagatcgctatcttcaaccggctgaagctggtgcccaagaaggtggacctgtcccagcagaaagagatccccaccaccctggtggacgacttcatcctgagccccgtcgtgaagagaagcttcatccagagcatcaaagtgatcaacgccatcatcaagaagtacggcctgcccaacgacatcattatcgagctggcccgcgagaagaactccaaggacgcccagaaaatgatcaacgagatgcagaagcggaaccggcagaccaacgagcggatcgaggaaatcatccggaccaccggcaaagagaacgccaagtacctgatcgagaagatcaagctgcacgacatgcaggaaggcaagtgcctgtacagcctggaagccatccctctggaagatctgctgaacaaccccttcaactatgaggtggaccacatcatccccagaagcgtgtccttcgacaacagcttcaacaacaaggtgctcgtgaagcaggaagaagccagcaagaagggcaaccggaccccattccagtacctgagcagcagcgacagcaagatcagctacgaaaccttcaagaagcacatcctgaatctggccaagggcaagggcagaatcagcaagaccaagaaagagtatctgctggaagaacgggacatcaacaggttctccgtgcagaaagacttcatcaaccggaacctggtggataccagatacgccaccagaggcctgatgaacctgctgcggagctacttcagagtgaacaacctggacgtgaaagtgaagtccatcaatggcggcttcaccagctttctgcggcggaagtggaagtttaagaaagagcggaacaaggggtacaagcaccacgccgaggacgccctgatcattgccaacgccgatttcatcttcaaagagtggaagaaactggacaaggccaaaaaagtgatggaaaaccagatgttcgaggaaaagcaggccgagagcatgcccgagatcgaaaccgagcaggagtacaaagagatcttcatcaccccccaccagatcaagcacattaaggacttcaaggactacaagtacagccaccgggtggacaagaagcctaatagagagctgattaacgacaccctgtactccacccggaaggacgacaagggcaacaccctgatcgtgaacaatctgaacggcctgtacgacaaggacaatgacaagctgaaaaagctgatcaacaagagccccgaaaagctgctgatgtaccaccacgacccccagacctaccagaaactgaagctgattatggaacagtacggcgacgagaagaatcccctgtacaagtactacgaggaaaccgggaactacctgaccaagtactccaaaaaggacaacggccccgtgatcaagaagattaagtattacggcaacaaactgaacgcccatctggacatcaccgacgactaccccaacagcagaaacaaggtcgtgaagctgtccctgaagccctacagattcgacgtgtacctggacaatggcgtgtacaagttcgtgaccgtgaagaatctggatgtgatcaaaaaagaaaactactacgaagtgaatagcaagtgctatgaggaagctaagaagctgaagaagatcagcaaccaggccgagtttatcgcctccttctacaacaacgatctgatcaagatcaacggcgagctgtatagagtgatcggcgtgaacaacgacctgctgaaccggatcgaagtgaacatgatcgacatcacctaccgcgagtacctggaaaacatgaacgacaagaggccccccaggatcattaagacaatcgcctccaagacccagagcattaagaagtacagcacagacattctgggcaacctgtatgaagtgaaatctaagaagcaccctcagatcatcaaaaagggcaaaaggccggcggccacgaaaaaggccggccaggcaaaaaagaaaaagggatccgaggccagcggttccggacgggctgacgcattggacgattttgatctggatatgctgggaagtgacgccctcgatgattttgaccttgacatgcttggttcggatgcccttgatgactttgacctcgacatgctcggcagtgacgcccttgatgatttcgacctggacatgctgattaactctagaagttccggatctccgaaaaagaaacgcaaagttggttcgggaggtggttcgggtggctctggatcagtgctgcctcaggctcctgctcctgcaccagctccagccatggtgtctgcactggctcaggcaccagcacccgtgcctgtgctggctcctggacctccacaggctgtggctccaccagcccctaaacctacacaggccggcgagggcacactgtctgaagctctgctgcagctgcagttcgacgacgaggatctgggagccctgctgggaaacagcaccgatcctgccgtgttcaccgacctggccagcgtggacaacagcgagttccagcagctgctgaaccagggcatccctgtggcccctcacaccaccgagcccatgctgatggaataccccgaggccatcacccggctcgtgacaggcgctcagaggcctcctgatccagctcctgcccctctgggagcaccaggcctgcctaatggactgctgtctggcgacgaggacttcagctctatcgccgatatggatttctcagccttgctgtcaggcggtggtagtggtgggagcggtagtgacctttcccatccgcccccaaggggccatctggatgagctgacaaccacacttgagtccatgaccgaggatctgaacctggactcacccctgaccccggaattgaacgagattctggataccttcctgaacgacgagtgcctcttgcatgccatgcatatcagcacaggactgtccatcttcgacacatctctgttttaggaattcaaataaaatacgaaatgaaataaaatacgaaatgcaattgggccgcaggaacccctagtgatggagttggccactccctctctgcgcgctcgctcgctcactgaggccgggcgaccaaaggtcgcccgacgcccgggctttgcccgagcggcctcagtgagcgagcgagcgcgcagctgcctgcaggacatgtgagcaaaaggccagcaaaaggccaggaaccgtaaaaaggccgcgttgctggcgtttttccataggctccgcccccctgacgagcatcacaaaaatcgacgctcaagtcagaggtggcgaaacccgacaggactataaagataccaggcgtttccccctggaagctccctcgtgcgctctcctgttccgaccctgccgcttaccggatacctgtccgcctttctcccttcgggaagcgtggcgctttctcatagctcacgctgtaggtatctcagttcggtgtaggtcgttcgctccaagctgggctgtgtgcacgaaccccccgttcagcccgaccgctgcgccttatccggtaactatcgtcttgagtccaacccggtaagacacgacttatcgccactggcagcagccactggtaacaggattagcagagcgaggtatgtaggcggtgctacagagttcttgaagtggtggcctaactacggctacactagaagaacagtatttggtatctgcgctctgctgaagccagttaccttcggaaaaagagttggtagctcttgatccggcaaacaaaccaccgctggtagcggtggtttttttgtttgcaagcagcagattacgcgcagaaaaaaaggatctcaagaagatcctttgatcttttctacggggtctgacgctcagtggaacgaaaactcacgttaagggattttggtcatgagattatcaaaaaggatcttcacctagatccttttaaattaaaaatgaagttttaaatcaatctaaagtatatatgagtaaacttggtctgacagttaccaatgcttaatcagtgaggcacctatctcagcgatctgtctatttcgttcatccatagttgcctgactccccgtcgtgtagataactacgatacgggagggcttaccatctggccccagtgctgcaatgataccgcggcttccacgctcaccggctccagatttatcagcaataaaccagccagccggaagggccgagcgcagaagtggtcctgcaactttatccgcctccatccagtctattaattgttgccgggaagctagagtaagtagttcgccagttaatagtttgcgcaacgttgttgccattgctacaggcatcgtggtgtcacgctcgtcgtttggtatggcttcattcagctccggttcccaacgatcaaggcgagttacatgatcccccatgttgtgcaaaaaagcggttagctccttcggtcctccgatcgttgtcagaagtaagttggccgcagtgttatcactcatggttatggcagcactgcataattctcttactgtcatgccatccgtaagatgcttttctgtgactggtgagtactcaaccaagtcattctgagaatagtgtatgcggcgaccgagttgctcttgcccggcgtcaatacgggataataccgcgccacatagcagaactttaaaagtgctcatcattggaaaacgttcttcggggcgaaaactctcaaggatcttaccgctgttgagatccagttcgatgtaacccactcgtgcacccaactgatcttcagcatcttttactttcaccagcgtttctgggtgagcaaaaacaggaaggcaaaatgccgcaaaaaagggaataagggcgacacggaaatgttgaatactcatactcttcctttttcaatattattgaagcatttatcagggttattgtctcatgagcggatacatatttgaatgtatttagaaaaataaacaaataggggttccgcgcacatttccccgaaaagtgccacctgacgtctaagaaaccattattatcatgacattaacctataaaaataggcgtatcacgaggccctttcgtctcgcgcgtttcggtgatgacggtg

SEQ ID NO: 11 - DNA, 6668 bp, Artificial Sequence
  pGW047
cctgcaggcagctgcgcgctcgctcgctcactgaggccgcccgggcaaagcccgggcgtcgggcgacctttggtcgcccggcctcagtgagcgagcgagcgcgcagagagggagtggccaactccatcactaggggttcctgcggccgcacgcgttctagaaagagggcctatttcccatgattccttcatatttgcatatacgatacaaggctgttagagagataattggaattaatttgactgtaaacacaaagatattagtacaaaatacgtgacgtagaaagtaataatttcttgggtagtttgcagttttaaaattatgttttaaaatggactatcatatgcttaccgtaacttgaaagtatttcgatttcttggctttatatatcttgtggaaaggacgaaacaccggaagagcgagctcttctgttttagtactctggaggccaacatgaggatcacccatgtctgcagggccaacagaatctactaaaacaaggcaaaatgccgtgtttatctcgtcaactggccaacatgaggatcacccatgtctgcagggcctgttggcgagatttttttgctagctgcaaagatggataaagttttaaacagagaggaatctttgcagctaatggaccttctaggtcttgaaaggagtgggaattggctccggtgcccgtcagtgggcagagcgcacatcgcccacagtccccgagaagttggggggaggggtcggcaattgaaccggtgcctagagaaggtggcgcggggtaaactgggaaagtgatgtcgtgtactggctccgcctttttcccgagggtgggggagaaccgtatataagtgcagtagtcgccgtgaacgttctttttcgcaacgggtttgccgccagaacacaggtaagtgccgtgtgtggttcccgcgggcctggcctctttacgggttatggcccttgcgtgccttgaattacttccacctggctgcagtacgtgattcttgatcccgagcttcgggttggaagtgggtgggagagttcgaggccttgcgcttaaggagccccttcgcctcgtgcttgagttgaggcctggcctgggcgctggggccgccgcgtgcgaatctggtggcaccttcgcgcctgtctcgctgctttcgataagtctctagccatttaaaatttttgatgacctgctgcgacgctttttttctggcaagatagtcttgtaaatgcgggccaagatctgcacactggtatttcggtttttggggccgcgggcggcgacggggcccgtgcgtcccagcgcacatgttcggcgaggcggggcctgcgagcgcggccaccgagaatcggacgggggtagtctcaagctggccggcctgctctggtgcctggcctcgcgccgccgtgtatcgccccgccctgggcggcaaggctggcccggtcggcaccagttgcgtgagcggaaagatggccgcttcccggccctgctgcagggagctcaaaatgaaggacgcggcgctcgggagagcgggcgggtgagtcacccacacaaaggaaaagggcctttccgtcctcagccgtcgcttcatgtgactccacggagtaccgggcgccgtccaggcacctcgattagttctcgagcttttggagtacgtcgtctttaggttggggggaggggttttatgcgatggagtttccccacactgagtgggtggagactgaagttaggccagcttggcacttgatgtaattctccttggaatttgccctttttgagtttggatcttggttcattctcaagcctcagacagtggttcaaagtttttttcttccatttcaggtgtcgtgacgtacggccaccatggcttcaaactttactcagttcgtgctcgtggacaatggtgggacaggggatgtgacagtggctccttctaatttcgctaatggggtggcagagtggatcagctccaactcacggagccaggcctacaaggtgacatgcagcgtcaggcagtctagtgcccagaagagaaagtataccatcaaggtggaggtccccaaagtggctacccagacagtgggcggagtcgaactgcctgtcgccgcttggaggtcctacctgaacatggagctcactatcccaattttcgctaccaattctgactgtgaactcatcgtgaaggcaatgcaggggctcctcaaagacggtaatcctatcccttccgccatcgccgctaactcaggtatctacagcgctggaggaggtggaagcggaggaggaggaagcggaggaggaggtagcggacctaagaaaaagaggaaggtggcggccgctggatccccttcagggcagatcagcaaccaggccctggctctggcccctagctccgctccagtgctggcccagactatggtgccctctagtgctatggtgcctctggcccagccacctgctccagcccctgtgctgaccccaggaccaccccagtcactgagcgctccagtgcccaagtctacacaggccggcgaggggactctgagtgaagctctgctgcacctgcagttcgacgctgatgaggacctgggagctctgctggggaacagcaccgatcccggagtgttcacagatctggcctccgtggacaactctgagtttcagcagctgctgaatcagggcgtgtccatgtctcatagtacagccgaaccaatgctgatggagtaccccgaagccattacccggctggtgaccggcagccagcggccccccgaccccgctccaactcccctgggaaccagcggcctgcctaatgggctgtccggagatgaagacttctcaagcatcgctgatatggactttagtgccctgctgtcacagatttcctctagtgggcagggaggaggtggaagcggcttcagcgtggacaccagtgccctgctggacctgttcagcccctcggtgaccgtgcccgacatgagcctgcctgaccttgacagcagcctggccagtatccaagagctcctgtctccccaggagccccccaggcctcccgaggcagagaacagcagcccggattcagggaagcagctggtgcactacacagcgcagccgctgttcctgctggaccccggctccgtggacaccgggagcaacgacctgccggtgctgtttgagctgggagagggctcctacttctccgaaggggacggcttcgccgaggaccccaccatctccctgctgacaggctcggagcctcccaaagccaaggaccccactgtctcctaagaattcacgcgttaagtcgacaatcaacctctggattacaaaatttgtgaaagattgactggtattcttaactatgttgctccttttacgctatgtggatacgctgctttaatgcctttgtatcatgctattgcttcccgtatggctttcattttctcctccttgtataaatcctggttgctgtctctttatgaggagttgtggcccgttgtcaggcaacgtggcgtggtgtgcactgtgtttgctgacgcaacccccactggttggggcattgccaccacctgtcagctcctttccgggactttcgctttccccctccctattgccacggcggaactcatcgccgcctgccttgcccgctgctggacaggggctcggctgttgggcactgacaattccgtggtgttgtcggggaaatcatcgtcctttccttggctgctcgcctgtgttgccacctggattctgcgcgggacgtccttctgctacgtcccttcggccctcaatccagcggaccttccttcccgcggcctgctgccggctctgcggcctcttccgcgtcttcgccttcgccctcagacgagtcggatctccctttgggccgcctccccgcgtcgactttaagaccaatgacgtgcggaccgagcggccgcaggaacccctagtgatggagttggccactccctctctgcgcgctcgctcgctcactgaggccgggcgaccaaaggtcgcccgacgcccgggctttgcccgggcggcctcagtgagcgagcgagcgcgcagctgcctgcaggggcgcctgatgcggtattttctccttacgcatctgtgcggtatttcacaccgcatacgtcaaagcaaccatagtacgcgccctgtagcggcgcattaagcgcggcgggtgtggtggttacgcgcagcgtgaccgctacacttgccagcgccctagcgcccgctcctttcgctttcttcccttcctttctcgccacgttcgccggctttccccgtcaagctctaaatcgggggctccctttagggttccgatttagtgctttacggcacctcgaccccaaaaaacttgatttgggtgatggttcacgtagtgggccatcgccctgatagacggtttttcgccctttgacgttggagtccacgttctttaatagtggactcttgttccaaactggaacaacactcaaccctatctcgggctattcttttgatttataagggattttgccgatttcggcctattggttaaaaaatgagctgatttaacaaaaatttaacgcgaattttaacaaaatattaacgtttacaattttatggtgcactctcagtacaatctgctctgatgccgcatagttaagccagccccgacacccgccaacacccgctgacgcgccctgacgggcttgtctgctcccggcatccgcttacagacaagctgtgaccgtctccgggagctgcatgtgtcagaggttttcaccgtcatcaccgaaacgcgcgagacgaaagggcctcgtgatacgcctatttttataggttaatgtcatgataataatggtttcttagacgtcaggtggcacttttcggggaaatgtgcgcggaacccctatttgtttatttttctaaatacattcaaatatgtatccgctcatgagacaataaccctgataaatgcttcaataatattgaaaaaggaagagtatgagtattcaacatttccgtgtcgcccttattcccttttttgcggcattttgccttcctgtttttgctcacccagaaacgctggtgaaagtaaaagatgctgaagatcagttgggtgcacgagtgggttacatcgaactggatctcaacagcggtaagatccttgagagttttcgccccgaagaacgttttccaatgatgagcacttttaaagttctgctatgtggcgcggtattatcccgtattgacgccgggcaagagcaactcggtcgccgcatacactattctcagaatgacttggttgagtactcaccagtcacagaaaagcatcttacggatggcatgacagtaagagaattatgcagtgctgccataaccatgagtgataacactgcggccaacttacttctgacaacgatcggaggaccgaaggagctaaccgcttttttgcacaacatgggggatcatgtaactcgccttgatcgttgggaaccggagctgaatgaagccataccaaacgacgagcgtgacaccacgatgcctgtagcaatggcaacaacgttgcgcaaactattaactggcgaactacttactctagcttcccggcaacaattaatagactggatggaggcggataaagttgcaggaccacttctgcgctcggcccttccggctggctggtttattgctgataaatctggagccggtgagcgtgggtctcgcggtatcattgcagcactggggccagatggtaagccctcccgtatcgtagttatctacacgacggggagtcaggcaactatggatgaacgaaatagacagatcgctgagataggtgcctcactgattaagcattggtaactgtcagaccaagtttactcatatatactttagattgatttaaaacttcatttttaatttaaaaggatctaggtgaagatcctttttgataatctcatgaccaaaatcccttaacgtgagttttcgttccactgagcgtcagaccccgtagaaaagatcaaaggatcttcttgagatcctttttttctgcgcgtaatctgctgcttgcaaacaaaaaaaccaccgctaccagcggtggtttgtttgccggatcaagagctaccaactctttttccgaaggtaactggcttcagcagagcgcagataccaaatactgtccttctagtgtagccgtagttaggccaccacttcaagaactctgtagcaccgcctacatacctcgctctgctaatcctgttaccagtggctgctgccagtggcgataagtcgtgtcttaccgggttggactcaagacgatagttaccggataaggcgcagcggtcgggctgaacggggggttcgtgcacacagcccagcttggagcgaacgacctacaccgaactgagatacctacagcgtgagctatgagaaagcgccacgcttcccgaagggagaaaggcggacaggtatccggtaagcggcagggtcggaacaggagagcgcacgagggagcttccagggggaaacgcctggtatctttatagtcctgtcgggtttcgccacctctgacttgagcgtcgatttttgtgatgctcgtcaggggggcggagcctatggaaaaacgccagcaacgcggcctttttacggttcctggccttttgctggccttttgctcacatgt

SEQ ID NO: 12 - DNA, 7489 bp, Artificial Sequence
  pGW060
cctgcaggcagctgcgcgctcgctcgctcactgaggccgcccgggcgtcgggcgacctttggtcgcccggcctcagtgagcgagcgagcgcgcagagagggagtggccaactccatcactaggggttcctgcggcctctagaaaggatctgcgatcgctccggtgcccgtcagtgggcagagcgcacatcgcccacagtccccgagaagttggggggaggggtcggcaattgaacgggtgcctagagaaggtggcgcggggtaaactgggaaagtgatgtcgtgtactggctccgcctttttcccgagggtgggggagaaccgtatataagtgcagtagtcgccgtgaacgttctttttcgcaacgggtttgccgccagaacacagctgaagcttcgaggggctcgcatctctccttcacgcgcccgccgccctacctgaggccgccatccacgccggttgagtcgcgttctgccgcctcccgcctgtggtgcctcctgaactgcgtccgccgtctaggtaagtttaaagctcaggtcgagaccgggcctttgtccggcgctcccttggagcctacctagactcagccggctctccacgctttgcctgaccctgcttgctcaactctacgtctttgtttcgttttctgttctgcgccgttacagatctggctaactaccggtgccaccatggccccaaagaagaagcggaaggtcggtatccacggagtcccagcagccaagcggaactacatcctgggcctggccatcggcatcaccagcgtgggctacggcatcatcgactacgagacacgggacgtgatcgatgccggcgtgcggctgttcaaagaggccaacgtggaaaacaacgagggcaggcggagcaagagaggcgccagaaggctgaagcggcggaggcggcatagaatccagagagtgaagaagctgctgttcgactacaacctgctgaccgaccacagcgagctgagcggcatcaacccctacgaggccagagtgaagggcctgagccagaagctgagcgaggaagagttctctgccgccctgctgcacctggccaagagaagaggcgtgcacaacgtgaacgaggtggaagaggacaccggcaacgagctgtccaccaaagagcagatcagccggaacagcaaggccctggaagagaaatacgtggccgaactgcagctggaacggctgaagaaagacggcgaagtgcggggcagcatcaacagattcaagaccagcgactacgtgaaagaagccaaacagctgctgaaggtgcagaaggcctaccaccagctggaccagagcttcatcgacacctacatcgacctgctggaaacccggcggacctactatgagggacctggcgagggcagccccttcggctggaaggacatcaaagaatggtacgagatgctgatgggccactgcacctacttccccgaggaactgcggagcgtgaagtacgcctacaacgccgacctgtacaacgccctgaacgacctgaacaatctcgtgatcaccagggacgagaacgagaagctggaatattacgagaagttccagatcatcgagaacgtgttcaagcagaagaagaagcccaccctgaagcagatcgccaaagaaatcctcgtgaacgaagaggatattaagggctacagagtgaccagcaccggcaagcccgagttcaccaacctgaaggtgtaccacgacatcaaggacattaccgcccggaaagagattattgagaacgccgagctgctggatcagattgccaagatcctgaccatctaccagagcagcgaggacatccaggaagaactgaccaatctgaactccgagctgacccaggaagagatcgagcagatctctaatctgaagggctataccggcacccacaacctgagcctgaaggccatcaacctgatcctggacgagctgtggcacaccaacgacaaccagatcgctatcttcaaccggctgaagctggtgcccaagaaggtggacctgtcccagcagaaagagatccccaccaccctggtggacgacttcatcctgagccccgtcgtgaagagaagcttcatccagagcatcaaagtgatcaacgccatcatcaagaagtacggcctgcccaacgacatcattatcgagctggcccgcgagaagaactccaaggacgcccagaaaatgatcaacgagatgcagaagcggaaccggcagaccaacgagcggatcgaggaaatcatccggaccaccggcaaagagaacgccaagtacctgatcgagaagatcaagctgcacgacatgcaggaaggcaagtgcctgtacagcctggaagccatccctctggaagatctgctgaacaaccccttcaactatgaggtggaccacatcatccccagaagcgtgtccttcgacaacagcttcaacaacaaggtgctcgtgaagcaggaagaagccagcaagaagggcaaccggaccccattccagtacctgagcagcagcgacagcaagatcagctacgaaaccttcaagaagcacatcctgaatctggccaagggcaagggcagaatcagcaagaccaagaaagagtatctgctggaagaacgggacatcaacaggttctccgtgcagaaagacttcatcaaccggaacctggtggataccagatacgccaccagaggcctgatgaacctgctgcggagctacttcagagtgaacaacctggacgtgaaagtgaagtccatcaatggcggcttcaccagctttctgcggcggaagtggaagtttaagaaagagcggaacaaggggtacaagcaccacgccgaggacgccctgatcattgccaacgccgatttcatcttcaaagagtggaagaaactggacaaggccaaaaaagtgatggaaaaccagatgttcgaggaaaagcaggccgagagcatgcccgagatcgaaaccgagcaggagtacaaagagatcttcatcaccccccaccagatcaagcacattaaggacttcaaggactacaagtacagccaccgggtggacaagaagcctaatagagagctgattaacgacaccctgtactccacccggaaggacgacaagggcaacaccctgatcgtgaacaatctgaacggcctgtacgacaaggacaatgacaagctgaaaaagctgatcaacaagagccccgaaaagctgctgatgtaccaccacgacccccagacctaccagaaactgaagctgattatggaacagtacggcgacgagaagaatcccctgtacaagtactacgaggaaaccgggaactacctgaccaagtactccaaaaaggacaacggccccgtgatcaagaagattaagtattacggcaacaaactgaacgcccatctggacatcaccgacgactaccccaacagcagaaacaaggtcgtgaagctgtccctgaagccctacagattcgacgtgtacctggacaatggcgtgtacaagttcgtgaccgtgaagaatctggatgtgatcaaaaaagaaaactactacgaagtgaatagcaagtgctatgaggaagctaagaagctgaagaagatcagcaaccaggccgagtttatcgcctccttctacaacaacgatctgatcaagatcaacggcgagctgtatagagtgatcggcgtgaacaacgacctgctgaaccggatcgaagtgaacatgatcgacatcacctaccgcgagtacctggaaaacatgaacgacaagaggccccccaggatcattaagacaatcgcctccaagacccagagcattaagaagtacagcacagacattctgggcaacctgtatgaagtgaaatctaagaagcaccctcagatcatcaaaaagggcaaaaggccggcggccacgaaaaaggccggccaggcaaaaaagaaaaagggatccggacgggctgacgcattggacgattttgatctggatatgctgggaagtgacgccctcgatgattttgaccttgacatgcttggttcggatgcccttgatgactttgacctcgacatgctcggcagtgacgcccttgatgatttcgacctggacatgctgatttaagaattcacgcgttaagtcgacaatcaacctctggattacaaaatttgtgaaagattgactggtattcttaactatgttgctccttttacgctatgtggatacgctgctttaatgcctttgtatcatgctattgcttcccgtatggctttcattttctcctccttgtataaatcctggttgctgtctctttatgaggagttgtggcccgttgtcaggcaacgtggcgtggtgtgcactgtgtttgctgacgcaacccccactggttggggcattgccaccacctgtcagctcctttccgggactttcgctttccccctccctattgccacggcggaactcatcgccgcctgccttgcccgctgctggacaggggctcggctgttgggcactgacaattccgtggtgttgtcggggaaatcatcgtcctttccttggctgctcgcctgtgttgccacctggattctgcgcgggacgtccttctgctacgtcccttcggccctcaatccagcggaccttccttcccgcggcctgctgccggctctgcggcctcttccgcgtcttcgccttcgccctcagacgagtcggatctccctttgggccgcctccccgcgtcgactttaagaccaatgacggccgcaggaacccctagtgatggagttggccactccctctctgcgcgctcgctcgctcactgaggccgggcgaccaaaggtcgcccgacgcccgggctttgcccgggcggcctcagtgagcgagcgagcgcgcagctgcctgcaggggcgcctgatgcggtattttctccttacgcatctgtgcggtatttcacaccgcatacgtcaaagcaaccatagtacgcgccctgtagcggcgcattaagcgcggcgggtgtggtggttacgcgcagcgtgaccgctacacttgccagcgccttagcgcccgctcctttcgctttcttcccttcctttctcgccacgttcgccggctttccccgtcaagctctaaatcgggggctccctttagggttccgatttagtgctttacggcacctcgaccccaaaaaacttgatttgggtgatggttcacgtagtgggccatcgccctgatagacggtttttcgccctttgacgttggagtccacgttctttaatagtggactcttgttccaaactggaacaacactcaactctatctcgggctattcttttgatttataagggattttgccgatttcggtctattggttaaaaaatgagctgatttaacaaaaatttaacgcgaattttaacaaaatattaacgtttacaattttatggtgcactctcagtacaatctgctctgatgccgcatagttaagccagccccgacacccgccaacacccgctgacgcgccctgacgggcttgtctgctcccggcatccgcttacagacaagctgtgaccgtctccgggagctgcatgtgtcagaggttttcaccgtcatcaccgaaacgcgcgagacgaaagggcctcgtgatacgcctatttttataggttaatgtcatgataataatggtttcttagacgtcaggtggcacttttcggggaaatgtgcgcggaacccctatttgtttatttttctaaatacattcaaatatgtatccgctcatgagacaataaccctgataaatgcttcaataatattgaaaaaggaagagtatgagtattcaacatttccgtgtcgcccttattcccttttttgcggcattttgccttcctgtttttgctcacccagaaacgctggtgaaagtaaaagatgctgaagatcagttgggtgcacgagtgggttacatcgaactggatctcaacagcggtaagatccttgagagttttcgccccgaagaacgttttccaatgatgagcacttttaaagttctgctatgtggcgcggtattatcccgtattgacgccgggcaagagcaactcggtcgccgcatacactattctcagaatgacttggttgagtactcaccagtcacagaaaagcatcttacggatggcatgacagtaagagaattatgcagtgctgccataaccatgagtgataacactgcggccaacttacttctgacaacgatcggaggaccgaaggagctaaccgcttttttgcacaacatgggggatcatgtaactcgccttgatcgttgggaaccggagctgaatgaagccataccaaacgacgagcgtgacaccacgatgcctgtagcaatggcaacaacgttgcgcaaactattaactggcgaactacttactctagcttcccggcaacaattaatagactggatggaggcggataaagttgcaggaccacttctgcgctcggcccttccggctggctggtttattgctgataaatctggagccggtgagcgtggaagccgcggtatcattgcagcactggggccagatggtaagccctcccgtatcgtagttatctacacgacggggagtcaggcaactatggatgaacgaaatagacagatcgctgagataggtgcctcactgattaagcattggtaactgtcagaccaagtttactcatatatactttagattgatttaaaacttcatttttaatttaaaaggatctaggtgaagatcctttttgataatctcatgaccaaaatcccttaacgtgagttttcgttccactgagcgtcagaccccgtagaaaagatcaaaggatcttcttgagatcctttttttctgcgcgtaatctgctgcttgcaaacaaaaaaaccaccgctaccagcggtggtttgtttgccggatcaagagctaccaactctttttccgaaggtaactggcttcagcagagcgcagataccaaatactgttcttctagtgtagccgtagttaggccaccacttcaagaactctgtagcaccgcctacatacctcgctctgctaatcctgttaccagtggctgctgccagtggcgataagtcgtgtcttaccgggttggactcaagacgatagttaccggataaggcgcagcggtcgggctgaacggggggttcgtgcacacagcccagcttggagcgaacgacctacaccgaactgagatacctacagcgtgagctatgagaaagcgccacgcttcccgaagggagaaaggcggacaggtatccggtaagcggcagggtcggaacaggagagcgcacgagggagcttccagggggaaacgcctggtatctttatagtcctgtcgggtttcgccacctctgacttgagcgtcgatttttgtgatgctcgtcaggggggcggagcctatggaaaaacgccagcaacgcggcctttttacggttcctggccttttgctggccttttgctcacatgt

SEQ ID NO: 13 - DNA, 6726 bp, Artificial Sequence
  pGW045
cctgcaggcagctgcgcgctcgctcgctcactgaggccgcccgggcaaagcccgggcgtcgggcgacctttggtcgcccggcctcagtgagcgagcgagcgcgcagagagggagtggccaactccatcactaggggttcctgcggccgcacgcgttctagaaagagggcctatttcccatgattccttcatatttgcatatacgatacaaggctgttagagagataattggaattaatttgactgtaaacacaaagatattagtacaaaatacgtgacgtagaaagtaataatttcttgggtagtttgcagttttaaaattatgttttaaaatggactatcatatgcttaccgtaacttgaaagtatttcgatttcttggctttatatatcttgtggaaaggacgaaacaccggaagagcgagctcttctgttttagagctaggccaacatgaggatcacccatgtctgcagggcctagcaagttaaaataaggctagtccgttatcaacttggccaacatgaggatcacccatgtctgcagggccaagtggcaccgagtcggtgcttttttggatccaagcttggcgtaactagatcttgagacaaatgggacagcagagatccagtttggttaattagctagctgcaaagatggataaagttttaaacagagaggaatctttgcagctaatggaccttctaggtcttgaaaggagtgggaattggctccggtgcccgtcagtgggcagagcgcacatcgcccacagtccccgagaagttggggggaggggtcggcaattgaaccggtgcctagagaaggtggcgcggggtaaactgggaaagtgatgtcgtgtactggctccgcctttttcccgagggtgggggagaaccgtatataagtgcagtagtcgccgtgaacgttctttttcgcaacgggtttgccgccagaacacaggtaagtgccgtgtgtggttcccgcgggcctggcctctttacgggttatggcccttgcgtgccttgaattacttccacctggctgcagtacgtgattcttgatcccgagcttcgggttggaagtgggtgggagagttcgaggccttgcgcttaaggagccccttcgcctcgtgcttgagttgaggcctggcctgggcgctggggccgccgcgtgcgaatctggtggcaccttcgcgcctgtctcgctgctttcgataagtctctagccatttaaaatttttgatgacctgctgcgacgctttttttctggcaagatagtcttgtaaatgcgggccaagatctgcacactggtatttcggtttttggggccgcgggcggcgacggggcccgtgcgtcccagcgcacatgttcggcgaggcggggcctgcgagcgcggccaccgagaatcggacgggggtagtctcaagctggccggcctgctctggtgcctggcctcgcgccgccgtgtatcgccccgccctgggcggcaaggctggcccggtcggcaccagttgcgtgagcggaaagatggccgcttcccggccctgctgcagggagctcaaaatgaaggacgcggcgctcgggagagcgggcgggtgagtcacccacacaaaggaaaagggcctttccgtcctcagccgtcgcttcatgtgactccacggagtaccgggcgccgtccaggcacctcgattagttctcgagcttttggagtacgtcgtctttaggttggggggaggggttttatgcgatggagtttccccacactgagtgggtggagactgaagttaggccagcttggcacttgatgtaattctccttggaatttgccctttttgagtttggatcttggttcattctcaagcctcagacagtggttcaaagtttttttcttccatttcaggtgtcgtgacgtacggccaccatggcttcaaactttactcagttcgtgctcgtggacaatggtgggacaggggatgtgacagtggctccttctaatttcgctaatggggtggcagagtggatcagctccaactcacggagccaggcctacaaggtgacatgcagcgtcaggcagtctagtgcccagaagagaaagtataccatcaaggtggaggtccccaaagtggctacccagacagtgggcggagtcgaactgcctgtcgccgcttggaggtcctacctgaacatggagctcactatcccaattttcgctaccaattctgactgtgaactcatcgtgaaggcaatgcaggggctcctcaaagacggtaatcctatcccttccgccatcgccgctaactcaggtatctacagcgctggaggaggtggaagcggaggaggaggaagcggaggaggaggtagcggacctaagaaaaagaggaaggtggcggccgctggatccccttcagggcagatcagcaaccaggccctggctctggcccctagctccgctccagtgctggcccagactatggtgccctctagtgctatggtgcctctggcccagccacctgctccagcccctgtgctgaccccaggaccaccccagtcactgagcgctccagtgcccaagtctacacaggccggcgaggggactctgagtgaagctctgctgcacctgcagttcgacgctgatgaggacctgggagctctgctggggaacagcaccgatcccggagtgttcacagatctggcctccgtggacaactctgagtttcagcagctgctgaatcagggcgtgtccatgtctcatagtacagccgaaccaatgctgatggagtaccccgaagccattacccggctggtgaccggcagccagcggccccccgaccccgctccaactcccctgggaaccagcggcctgcctaatgggctgtccggagatgaagacttctcaagcatcgctgatatggactttagtgccctgctgtcacagatttcctctagtgggcagggaggaggtggaagcggcttcagcgtggacaccagtgccctgctggacctgttcagcccctcggtgaccgtgcccgacatgagcctgcctgaccttgacagcagcctggccagtatccaagagctcctgtctccccaggagccccccaggcctcccgaggcagagaacagcagcccggattcagggaagcagctggtgcactacacagcgcagccgctgttcctgctggaccccggctccgtggacaccgggagcaacgacctgccggtgctgtttgagctgggagagggctcctacttctccgaaggggacggcttcgccgaggaccccaccatctccctgctgacaggctcggagcctcccaaagccaaggaccccactgtctcctaagaattcacgcgttaagtcgacaatcaacctctggattacaaaatttgtgaaagattgactggtattcttaactatgttgctccttttacgctatgtggatacgctgctttaatgcctttgtatcatgctattgcttcccgtatggctttcattttctcctccttgtataaatcctggttgctgtctctttatgaggagttgtggcccgttgtcaggcaacgtggcgtggtgtgcactgtgtttgctgacgcaacccccactggttggggcattgccaccacctgtcagctcctttccgggactttcgctttccccctccctattgccacggcggaactcatcgccgcctgccttgcccgctgctggacaggggctcggctgttgggcactgacaattccgtggtgttgtcggggaaatcatcgtcctttccttggctgctcgcctgtgttgccacctggattctgcgcgggacgtccttctgctacgtcccttcggccctcaatccagcggaccttccttcccgcggcctgctgccggctctgcggcctcttccgcgtcttcgccttcgccctcagacgagtcggatctccctttgggccgcctccccgcgtcgactttaagaccaatgacgtgcggaccgagcggccgcaggaacccctagtgatggagttggccactccctctctgcgcgctcgctcgctcactgaggccgggcgaccaaaggtcgcccgacgcccgggctttgcccgggcggcctcagtgagcgagcgagcgcgcagctgcctgcaggggcgcctgatgcggtattttctccttacgcatctgtgcggtatttcacaccgcatacgtcaaagcaaccatagtacgcgccctgtagcggcgcattaagcgcggcgggtgtggtggttacgcgcagcgtgaccgctacacttgccagcgccctagcgcccgctcctttcgctttcttcccttcctttctcgccacgttcgccggctttccccgtcaagctctaaatcgggggctccctttagggttccgatttagtgctttacggcacctcgaccccaaaaaacttgatttgggtgatggttcacgtagtgggccatcgccctgatagacggtttttcgccctttgacgttggagtccacgttctttaatagtggactcttgttccaaactggaacaacactcaaccctatctcgggctattcttttgatttataagggattttgccgatttcggcctattggttaaaaaatgagctgatttaacaaaaatttaacgcgaattttaacaaaatattaacgtttacaattttatggtgcactctcagtacaatctgctctgatgccgcatagttaagccagccccgacacccgccaacacccgctgacgcgccctgacgggcttgtctgctcccggcatccgcttacagacaagctgtgaccgtctccgggagctgcatgtgtcagaggttttcaccgtcatcaccgaaacgcgcgagacgaaagggcctcgtgatacgcctatttttataggttaatgtcatgataataatggtttcttagacgtcaggtggcacttttcggggaaatgtgcgcggaacccctatttgtttatttttctaaatacattcaaatatgtatccgctcatgagacaataaccctgataaatgcttcaataatattgaaaaaggaagagtatgagtattcaacatttccgtgtcgcccttattcccttttttgcggcattttgccttcctgtttttgctcacccagaaacgctggtgaaagtaaaagatgctgaagatcagttgggtgcacgagtgggttacatcgaactggatctcaacagcggtaagatccttgagagttttcgccccgaagaacgttttccaatgatgagcacttttaaagttctgctatgtggcgcggtattatcccgtattgacgccgggcaagagcaactcggtcgccgcatacactattctcagaatgacttggttgagtactcaccagtcacagaaaagcatcttacggatggcatgacagtaagagaattatgcagtgctgccataaccatgagtgataacactgcggccaacttacttctgacaacgatcggaggaccgaaggagctaaccgcttttttgcacaacatgggggatcatgtaactcgccttgatcgttgggaaccggagctgaatgaagccataccaaacgacgagcgtgacaccacgatgcctgtagcaatggcaacaacgttgcgcaaactattaactggcgaactacttactctagcttcccggcaacaattaatagactggatggaggcggataaagttgcaggaccacttctgcgctcggcccttccggctggctggtttattgctgataaatctggagccggtgagcgtgggtctcgcggtatcattgcagcactggggccagatggtaagccctcccgtatcgtagttatctacacgacggggagtcaggcaactatggatgaacgaaatagacagatcgctgagataggtgcctcactgattaagcattggtaactgtcagaccaagtttactcatatatactttagattgatttaaaacttcatttttaatttaaaaggatctaggtgaagatcctttttgataatctcatgaccaaaatcccttaacgtgagttttcgttccactgagcgtcagaccccgtagaaaagatcaaaggatcttcttgagatcctttttttctgcgcgtaatctgctgcttgcaaacaaaaaaaccaccgctaccagcggtggtttgtttgccggatcaagagctaccaactctttttccgaaggtaactggcttcagcagagcgcagataccaaatactgtccttctagtgtagccgtagttaggccaccacttcaagaactctgtagcaccgcctacatacctcgctctgctaatcctgttaccagtggctgctgccagtggcgataagtcgtgtcttaccgggttggactcaagacgatagttaccggataaggcgcagcggtcgggctgaacggggggttcgtgcacacagcccagcttggagcgaacgacctacaccgaactgagatacctacagcgtgagctatgagaaagcgccacgcttcccgaagggagaaaggcggacaggtatccggtaagcggcagggtcggaacaggagagcgcacgagggagcttccagggggaaacgcctggtatctttatagtcctgtcgggtttcgccacctctgacttgagcgtcgatttttgtgatgctcgtcaggggggcggagcctatggaaaaacgccagcaacgcggcctttttacggttcctggccttttgctggccttttgctcacatgt

SEQ ID NO: 14 - DNA, 7428 bp, Artificial Sequence
  pRC119
cctgcaggcagctgcgcgctcgctcgctcactgaggccgcccgggcaaagcccgggcgtcgggcgacctttggtcgcccggcctcagtgagcgagcgagcgcgcagagagggagtggccaactccatcactaggggttcctgcggccgcacgcgttctaggtcttgaaaggagtgggaattggctccggtgcccgtcagtgggcagagcgcacatcgcccacagtccccgagaagttggggggaggggtcggcaattgatccggtgcctagagaaggtggcgcggggtaaactgggaaagtgatgtcgtgtactggctccgcctttttcccgagggtgggggagaaccgtatataagtgcagtagtcgccgtgaacgttctttttcgcaacgggtttgccgccagaacacaggtgtcgtgacgcgcgtacggccaccatgacacagttcgagggctttaccaacctgtatcaggtgagcaagacactgcggtttgagctgatcccacagggcaagaccctgaagcacatccaggagcagggcttcatcgaggaggacaaggcccgcaatgatcactacaaggagctgaagcccatcatcgatcggatctacaagacctatgccgaccagtgcctgcagctggtgcagctggattgggagaacctgagcgccgccatcgactcctatagaaaggagaaaaccgaggagacaaggaacgccctgatcgaggagcaggccacatatcgcaatgccatccacgactacttcatcggccggacagacaacctgaccgatgccatcaataagagacacgccgagatctacaagggcctgttcaaggccgagctgtttaatggcaaggtgctgaagcagctgggcaccgtgaccacaaccgagcacgagaacgccctgctgcggagcttcgacaagtttacaacctacttctccggcttttatagaaacaggaagaacgtgttcagcgccgaggatatcagcacagccatcccacaccgcatcgtgcaggacaacttccccaagtttaaggagaattgtcacatcttcacacgcctgatcaccgccgtgcccagcctgcgggagcactttgagaacgtgaagaaggccatcggcatcttcgtgagcacctccatcgaggaggtgttttccttccctttttataaccagctgctgacacagacccagatcgacctgtataaccagctgctgggaggaatctctcgggaggcaggcaccgagaagatcaagggcctgaacgaggtgctgaatctggccatccagaagaatgatgagacagcccacatcatcgcctccctgccacacagattcatccccctgtttaagcagatcctgtccgataggaacaccctgtctttcatcctggaggagtttaagagcgacgaggaagtgatccagtccttctgcaagtacaagacactgctgagaaacgagaacgtgctggagacagccgaggccctgtttaacgagctgaacagcatcgacctgacacacatcttcatcagccacaagaagctggagacaatcagcagcgccctgtgcgaccactgggatacactgaggaatgccctgtatgagcggagaatctccgagctgacaggcaagatcaccaagtctgccaaggagaaggtgcagcgcagcctgaagcacgaggatatcaacctgcaggagatcatctctgccgcaggcaaggagctgagcgaggccttcaagcagaaaaccagcgagatcctgtcccacgcacacgccgccctggatcagccactgcctacaaccctgaagaagcaggaggagaaggagatcctgaagtctcagctggacagcctgctgggcctgtaccacctgctggactggtttgccgtggatgagtccaacgaggtggaccccgagttctctgcccggctgaccggcatcaagctggagatggagccttctctgagcttctacaacaaggccagaaattatgccaccaagaagccctactccgtggagaagttcaagctgaactttcagatgcctacactggccagaggctgggacgtgaatagagagaagaacaatggcgccatcctgtttgtgaagaacggcctgtactatctgggcatcatgccaaagcagaagggcaggtataaggccctgagcttcgagcccacagagaaaaccagcgagggctttgataagatgtactatgactacttccctgatgccgccaagatgatcccaaagtgcagcacccagctgaaggccgtgacagcccactttcagacccacacaacccccatcctgctgtccaacaatttcatcgagcctctggagatcacaaaggagatctacgacctgaacaatcctgagaaggagccaaagaagtttcagacagcctacgccaagaaaaccggcgaccagaagggctacagagaggccctgtgcaagtggatcgacttcacaagggattttctgtccaagtataccaagacaacctctatcgatctgtctagcctgcggccatcctctcagtataaggacctgggcgagtactatgccgagctgaatcccctgctgtaccacatcagcttccagagaatcgccgagaaggagatcatggatgccgtggagacaggcaagctgtacctgttccagatctataacaaggactttgccaagggccaccacggcaagcctaatctgcacacactgtattggaccggcctgttttctccagagaacctggccaagacaagcatcaagctgaatggccaggccgagctgttctaccgccctaagtccaggatgaagaggatggcacaccggctgggagagaagatgctgaacaagaagctgaaggatcagaaaaccccaatccccgacaccctgtaccaggagctgtacgactatgtgaatcacagactgtcccacgacctgtctgatgaggccagggccctgctgcccaacgtgatcaccaaggaggtgtctcacgagatcatcaaggataggcgctttaccagcgacaagttctttttccacgtgcctatcacactgaactatcaggccgccaattccccatctaagttcaaccagagggtgaatgcctacctgaaggagcaccccgagacacctatcatcggcatcgcccggggcgagagaaacctgatctatatcacagtgatcgactccaccggcaagatcctggagcagcggagcctgaacaccatccagcagtttgattaccagaagaagctggacaacagggagaaggagagggtggcagcaaggcaggcctggtctgtggtgggcacaatcaaggatctgaagcagggctatctgagccaggtcatccacgagatcgtggacctgatgatccactaccaggccgtggtggtgctggagaacctgaatttcggctttaagagcaagaggaccggcatcgccgagaaggccgtgtaccagcagttcgagaagatgctgatcgataagctgaattgcctggtgctgaaggactatccagcagagaaagtgggaggcgtgctgaacccataccagctgacagaccagttcacctcctttgccaagatgggcacccagtctggcttcctgttttacgtgcctgccccatatacatctaagatcgatcccctgaccggcttcgtggaccccttcgtgtggaaaaccatcaagaatcacgagagccgcaagcacttcctggagggcttcgactttctgcactacgacgtgaaaaccggcgacttcatcctgcactttaagatgaacagaaatctgtccttccagaggggcctgcccggctttatgcctgcatgggatatcgtgttcgagaagaacgagacacagtttgacgccaagggcacccctttcatcgccggcaagagaatcgtgccagtgatcgagaatcacagattcaccggcagataccgggacctgtatcctgccaacgagctgatcgccctgctggaggagaagggcatcgtgttcagggatggctccaacatcctgccaaagctgctggagaatgacgattctcacgccatcgacacgatggtggccctgatccgcagcgtgctgcagatgcggaactccaatgccgccacaggcgaggactatatcaacagccccgtgcgcgatctgaatggcgtgtgcttcgactcccggtttcagaacccagagtggccaatggacgccgatgccaatggcgcctaccacatcgccctgaagggccagctgctgctgaatcacctgaaggagagcaaggatctgaagctgcagaacggcatctccaatcaggactggctggcctacatccaggagctgcgcaacaaaaggccggcggccacgaaaaaggccggccaggcaaaaaagaaaaagggcagtggtagtggagaagagctgttgtcaaaaaattatcacttggagaatgaggtagcccgccttaagaaaggcagcggatcaggcgaggaacttctgagcaagaattaccatctcgaaaacgaagtggcacgcttgaagaagggttcaggttccggggaggagctcctctccaagaactaccacctggagaacgaagtcgctcgcctgaagaaatgaaataaaagatctttattttcattagatctgtgtgttggttttttgtgtgcggaccgagcggccgcaggaacccctagtgatggagttggccactccctctctgcgcgctcgctcgctcactgaggccgggcgaccaaaggtcgcccgacgcccgggctttgcccgggcggcctcagtgagcgagcgagcgcgcagctgcctgcaggggcgcctgatgcggtattttctccttacgcatctgtgcggtatttcacaccgcatacgtcaaagcaaccatagtacgcgccctgtagcggcgcattaagcgcggcgggtgtggtggttacgcgcagcgtgaccgctacacttgccagcgccctagcgcccgctcctttcgctttcttcccttcctttctcgccacgttcgccggctttccccgtcaagctctaaatcgggggctccctttagggttccgatttagtgctttacggcacctcgaccccaaaaaacttgatttgggtgatggttcacgtagtgggccatcgccctgatagacggtttttcgccctttgacgttggagtccacgttctttaatagtggactcttgttccaaactggaacaacactcaaccctatctcgggctattcttttgatttataagggattttgccgatttcggcctattggttaaaaaatgagctgatttaacaaaaatttaacgcgaattttaacaaaatattaacgtttacaattttatggtgcactctcagtacaatctgctctgatgccgcatagttaagccagccccgacacccgccaacacccgctgacgcgccctgacgggcttgtctgctcccggcatccgcttacagacaagctgtgaccgtctccgggagctgcatgtgtcagaggttttcaccgtcatcaccgaaacgcgcgagacgaaagggcctcgtgatacgcctatttttataggttaatgtcatgataataatggtttcttagacgtcaggtggcacttttcggggaaatgtgcgcggaacccctatttgtttatttttctaaatacattcaaatatgtatccgctcatgagacaataaccctgataaatgcttcaataatattgaaaaaggaagagtatgagtattcaacatttccgtgtcgcccttattcccttttttgcggcattttgccttcctgtttttgctcacccagaaacgctggtgaaagtaaaagatgctgaagatcagttgggtgcacgagtgggttacatcgaactggatctcaacagcggtaagatccttgagagttttcgccccgaagaacgttttccaatgatgagcacttttaaagttctgctatgtggcgcggtattatcccgtattgacgccgggcaagagcaactcggtcgccgcatacactattctcagaatgacttggttgagtactcaccagtcacagaaaagcatcttacggatggcatgacagtaagagaattatgcagtgctgccataaccatgagtgataacactgcggccaacttacttctgacaacgatcggaggaccgaaggagctaaccgcttttttgcacaacatgggggatcatgtaactcgccttgatcgttgggaaccggagctgaatgaagccataccaaacgacgagcgtgacaccacgatgcctgtagcaatggcaacaacgttgcgcaaactattaactggcgaactacttactctagcttcccggcaacaattaatagactggatggaggcggataaagttgcaggaccacttctgcgctcggcccttccggctggctggtttattgctgataaatctggagccggtgagcgtgggtctcgcggtatcattgcagcactggggccagatggtaagccctcccgtatcgtagttatctacacgacggggagtcaggcaactatggatgaacgaaatagacagatcgctgagataggtgcctcactgattaagcattggtaactgtcagaccaagtttactcatatatactttagattgatttaaaacttcatttttaatttaaaaggatctaggtgaagatcctttttgataatctcatgaccaaaatcccttaacgtgagttttcgttccactgagcgtcagaccccgtagaaaagatcaaaggatcttcttgagatcctttttttctgcgcgtaatctgctgcttgcaaacaaaaaaaccaccgctaccagcggtggtttgtttgccggatcaagagctaccaactctttttccgaaggtaactggcttcagcagagcgcagataccaaatactgtccttctagtgtagccgtagttaggccaccacttcaagaactctgtagcaccgcctacatacctcgctctgctaatcctgttaccagtggctgctgccagtggcgataagtcgtgtcttaccgggttggactcaagacgatagttaccggataaggcgcagcggtcgggctgaacggggggttcgtgcacacagcccagcttggagcgaacgacctacaccgaactgagatacctacagcgtgagctatgagaaagcgccacgcttcccgaagggagaaaggcggacaggtatccggtaagcggcagggtcggaacaggagagcgcacgagggagcttccagggggaaacgcctggtatctttatagtcctgtcgggtttcgccacctctgacttgagcgtcgatttttgtgatgctcgtcaggggggcggagcctatggaaaaacgccagcaacgcggcctttttacggttcctggccttttgctggccttttgctcacatgt

SEQ ID NO: 15 - DNA, 7335 bp, Artificial Sequence
  pRC120
cctgcaggcagctgcgcgctcgctcgctcactgaggccgcccgggcaaagcccgggcgtcgggcgacctttggtcgcccggcctcagtgagcgagcgagcgcgcagagagggagtggccaactccatcactaggggttcctgcggccgcacgcgttctaggtcttgaaaggagtgggaattggctccggtgcccgtcagtgggcagagcgcacatcgcccacagtccccgagaagttggggggaggggtcggcaattgatccggtgcctagagaaggtggcgcggggtaaactgggaaagtgatgtcgtgtactggctccgcctttttcccgagggtgggggagaaccgtatataagtgcagtagtcgccgtgaacgttctttttcgcaacgggtttgccgccagaacacaggtgtcgtgacgcgcgtacggccaccatgtcaaagctggagaaattcaccaactgttatagcctgtctaagaccctgcgcttcaaggcaatcccagtgggcaagacacaagagaacattgacaacaaacggctcctggtggaggatgagaagagggctgaagattacaagggcgttaagaagctgctggataggtactatctgtcattcatcaacgatgtcctccacagtatcaagctgaagaatctgaacaattacatttctctgttccggaagaagacacggaccgagaaggagaacaaagagctggagaatctggagatcaacctgaggaaagaaatagctaaggctttcaaagggaacgagggttacaagtccctgttcaagaaagacattatcgagactattctgcctgagttcctggacgataaagatgagatcgccctcgtcaattccttcaatgggtttaccacagcctttaccggcttcttcgacaatagagagaatatgttctctgaagaggccaaatccactagcatcgcctttcgctgcataaacgagaacctgactaggtacatcagcaatatggacatctttgagaaagtcgatgccatattcgacaaacatgaggtgcaggagattaaggagaagatcctgaactcagattacgatgtcgaagatttcttcgagggagagttcttcaacttcgtgctcacacaagagggcattgatgtgtacaatgcaatcattggagggttcgtgacagagagtggcgagaagataaagggcctgaacgagtatatcaacctctacaaccagaaaaccaagcagaaactgcctaagttcaagccactgtacaaacaagtgctctcagatagggaaagcctgagcttctacggtgaagggtatacatcagatgaagaagtgctcgaagtgttccgcaacaccctcaataagaacagtgaaatcttctcttcaatcaagaagctggagaaactgttcaagaatttcgatgagtactcctctgccggaatctttgtgaagaatggccctgcaatatccactattagcaaagacatctttggcgagtggaacgttatcagggataagtggaatgccgagtacgatgatattcatctcaagaagaaagccgtggttacagagaaatacgaggatgatagacgcaagagctttaagaagattggtagcttctctctcgaacagctgcaggagtacgccgacgctgacctgtcagtcgtggagaaactcaaggagatcataatccagaaggtggatgaaatctacaaagtgtatggaagctctgagaaactcttcgatgcagactttgttctggagaagagtctgaagaagaacgacgcagtggttgctatcatgaaggacctgctggattctgttaagtctttcgagaattacattaaggcattctttggtgaagggaaggagacaaatagggacgagagcttctatggcgactttgttctggcctacgacatcctcctcaaggttgaccacatctatgacgctatacggaattacgttacccagaagccctatagcaaagacaagttcaagctgtatttccagaatccacagtttatgggtgggtgggataaagacaaagaaacagattacagggccactatcctgcggtacggcagcaaatactatctggctatcatggataagaagtacgccaaatgcctccagaagatcgacaaggacgacgtgaacggtaactacgagaagatcaattacaagctcctgccaggacctaacaagatgctgcccaaggtgttcttctccaagaaatggatggcctactataacccaagcgaggacattcagaagatatacaagaatgggacattcaagaagggcgatatgttcaacctcaacgactgccacaagctgattgatttcttcaaggatagcatttctcgctatcccaagtggtctaatgcatacgatttcaacttcagcgagactgagaagtacaaagacatcgctggcttctaccgggaggtggaagagcaaggctataaggtgtcattcgaatccgcttctaagaaggaagtggataagctcgtggaagagggtaagctgtacatgttccagatatacaacaaagacttcagcgataagagccacggcactccaaacctccatactatgtatttcaagctgctgtttgacgagaacaaccacggacagattaggctgtcaggaggcgcagaactcttcatgcgcagagcttcactgaagaaggaggaactcgttgtccacccagccaatagccctatagccaataagaatccagacaatcctaagaaaaccactactctgtcttacgatgtgtataaggataagagattctctgaagatcagtacgaactgcacatacccattgccattaacaagtgccctaagaacatcttcaagattaacacagaggttagagtgctcctgaaacacgacgataacccttatgttataggcattgctcgcggagagagaaacctgctgtacatcgtcgtggtggacggcaaaggcaacatcgtggaacagtacagtctcaatgaaatcattaacaatttcaacggaatccgcattaagaccgactaccattctctcctcgacaagaaggagaaagaaaggttcgaagcaagacagaattggacaagtatagagaatatcaaagaactgaaggctgggtacatctctcaggttgtgcacaagatatgtgagctggtggagaagtacgacgctgttatcgccctcgcggacctgaatagcggcttcaagaactccagggtgaaggtggagaagcaggtgtatcagaagttcgagaagatgctgatcgacaagctcaactatatggtggacaagaaatccaatccttgcgctactggtggagccctgaagggctatcaaatcaccaataagttcgaatctttcaagtctatgagcacccagaatggcttcatcttctacatacccgcatggctgacatccaagattgatccctctaccggatttgttaatctgctcaagactaagtacacctctattgctgactcaaagaagttcatatcatcatttgaccgcatcatgtacgtgccagaagaggacctgttcgagtttgccctggattacaagaatttctctcggactgacgccgactacatcaagaagtggaagctctactcttatggtaatcggattcgcatattccgcaatcccaagaagaataacgtgttcgattgggaggaagtttgcctcaccagcgcttacaaggagctgttcaataagtatgggattaactaccagcagggcgacataagagccctgctgtgcgaacaatctgataaggcattctattcctctttcatggcactgatgtcactgatgctgcaaatgcgcaattccatcaccggaagaacagacgtggcctttctgatctctcctgtcaagaactcagatggcatcttctacgattcccgcaactatgaagcacaggagaatgctatcctgcctaagaatgccgatgcaaatggagcctataacatcgccagaaaggtcctctgggccataggacaattcaagaaagctgaagatgagaagctggacaaggtgaagatcgccatttcaaacaaagagtggctcgaatatgctcagacctcagtgaagcataaaaggccggcggccacgaaaaaggccggccaggcaaaaaagaaaaagggcagcggtagtggggaggagcttctttctaaaaattatcatcttgaaaatgaagtggcacgactcaagaaaggctctgggtccggtgaggaactcctgtccaagaactatcatcttgaaaacgaagtcgcccgccttaaaaaaggctcaggctcaggtgaagaattgttgagcaaaaactatcaccttgagaatgaggttgcccggctcaaaaaagggtctggcagcggcgaggaactcctttcaaagaactaccatctcgaaaatgaagttgctcggttgaagaagggttcaggatctggcgaggagcttctgtccaagaactaccatttggagaacgaggtcgcaagacttaaaaaatgaaataaaagatctttattttcattagatctgtgtgttggttttttgtgtgcggaccgagcggccgcaggaacccctagtgatggagttggccactccctctctgcgcgctcgctcgctcactgaggccgggcgaccaaaggtcgcccgacgcccgggctttgcccgggcggcctcagtgagcgagcgagcgcgcagctgcctgcaggggcgcctgatgcggtattttctccttacgcatctgtgcggtatttcacaccgcatacgtcaaagcaaccatagtacgcgccctgtagcggcgcattaagcgcggcgggtgtggtggttacgcgcagcgtgaccgctacacttgccagcgccctagcgcccgctcctttcgctttcttcccttcctttctcgccacgttcgccggctttccccgtcaagctctaaatcgggggctccctttagggttccgatttagtgctttacggcacctcgaccccaaaaaacttgatttgggtgatggttcacgtagtgggccatcgccctgatagacggtttttcgccctttgacgttggagtccacgttctttaatagtggactcttgttccaaactggaacaacactcaaccctatctcgggctattcttttgatttataagggattttgccgatttcggcctattggttaaaaaatgagctgatttaacaaaaatttaacgcgaattttaacaaaatattaacgtttacaattttatggtgcactctcagtacaatctgctctgatgccgcatagttaagccagccccgacacccgccaacacccgctgacgcgccctgacgggcttgtctgctcccggcatccgcttacagacaagctgtgaccgtctccgggagctgcatgtgtcagaggttttcaccgtcatcaccgaaacgcgcgagacgaaagggcctcgtgatacgcctatttttataggttaatgtcatgataataatggtttcttagacgtcaggtggcacttttcggggaaatgtgcgcggaacccctatttgtttatttttctaaatacattcaaatatgtatccgctcatgagacaataaccctgataaatgcttcaataatattgaaaaaggaagagtatgagtattcaacatttccgtgtcgcccttattcccttttttgcggcattttgccttcctgtttttgctcacccagaaacgctggtgaaagtaaaagatgctgaagatcagttgggtgcacgagtgggttacatcgaactggatctcaacagcggtaagatccttgagagttttcgccccgaagaacgttttccaatgatgagcacttttaaagttctgctatgtggcgcggtattatcccgtattgacgccgggcaagagcaactcggtcgccgcatacactattctcagaatgacttggttgagtactcaccagtcacagaaaagcatcttacggatggcatgacagtaagagaattatgcagtgctgccataaccatgagtgataacactgcggccaacttacttctgacaacgatcggaggaccgaaggagctaaccgcttttttgcacaacatgggggatcatgtaactcgccttgatcgttgggaaccggagctgaatgaagccataccaaacgacgagcgtgacaccacgatgcctgtagcaatggcaacaacgttgcgcaaactattaactggcgaactacttactctagcttcccggcaacaattaatagactggatggaggcggataaagttgcaggaccacttctgcgctcggcccttccggctggctggtttattgctgataaatctggagccggtgagcgtgggtctcgcggtatcattgcagcactggggccagatggtaagccctcccgtatcgtagttatctacacgacggggagtcaggcaactatggatgaacgaaatagacagatcgctgagataggtgcctcactgattaagcattggtaactgtcagaccaagtttactcatatatactttagattgatttaaaacttcatttttaatttaaaaggatctaggtgaagatcctttttgataatctcatgaccaaaatcccttaacgtgagttttcgttccactgagcgtcagaccccgtagaaaagatcaaaggatcttcttgagatcctttttttctgcgcgtaatctgctgcttgcaaacaaaaaaaccaccgctaccagcggtggtttgtttgccggatcaagagctaccaactctttttccgaaggtaactggcttcagcagagcgcagataccaaatactgtccttctagtgtagccgtagttaggccaccacttcaagaactctgtagcaccgcctacatacctcgctctgctaatcctgttaccagtggctgctgccagtggcgataagtcgtgtcttaccgggttggactcaagacgatagttaccggataaggcgcagcggtcgggctgaacggggggttcgtgcacacagcccagcttggagcgaacgacctacaccgaactgagatacctacagcgtgagctatgagaaagcgccacgcttcccgaagggagaaaggcggacaggtatccggtaagcggcagggtcggaacaggagagcgcacgagggagcttccagggggaaacgcctggtatctttatagtcctgtcgggtttcgccacctctgacttgagcgtcgatttttgtgatgctcgtcaggggggcggagcctatggaaaaacgccagcaacgcggcctttttacggttcctggccttttgctggccttttgctcacatgt

SEQ ID NO: 16 - DNA, 5810 bp, Artificial Sequence
  pRC121b
cctgcaggcagctgcgcgctcgctcgctcactgaggccgcccgggcgtcgggcgacctttggtcgcccggcctcagtgagcgagcgagcgcgcagagagggagtggccaactccatcactaggggttcctgcggcctctagaaaggatctgcgatcgctccggtgcccgtcagtgggcagagcgcacatcgcccacagtccccgagaagttggggggaggggtcggcaattgaacgggtgcctagagaaggtggcgcggggtaaactgggaaagtgatgtcgtgtactggctccgcctttttcccgagggtgggggagaaccgtatataagtgcagtagtcgccgtgaacgttctttttcgcaacgggtttgccgccagaacacagctgaagcttcgaggggctcgcatctctccttcacgcgcccgccgccctacctgaggccgccatccacgccggttgagtcgcgttctgccgcctcccgcctgtggtgcctcctgaactgcgtccgccgtctaggtaagtttaaagctcaggtcgagaccgggcctttgtccggcgctcccttggagcctacctagactcagccggctctccacgctttgcctgaccctgcttgctcaactctacgtctttgtttcgttttctgttctgcgccgttacagatctggctaactaccggtgccaccatgggcccagccgccaaacgagtcaagctggatggccccgatatcgtcatgactcaatcaccctcatcactgtcagccagcgtcggtgaccgggtaacaattacttgtagatcatcaactggggccgtcactacctccaactatgccagttgggttcaagagaaacccggcaagctctttaagggactgatcggtgggaccaataatcgggcccccggtgtgccttctcgctttagcgggagtttgataggcgataaagccacattgacaatatcatctcttcaacccgaggacttcgctacctatttttgtgctttgtggtatagtaaccattgggtatttggccaaggaactaaggtagagttgaagcgggggggcggcggctctggtggaggaggtagtgggggcggtggctcttccggagggggttccgaagtaaagcttttggagagcggcggcggcctggtccagcctggaggatctctcaagcttagctgcgccgtcagcggcttttccctcactgattatggtgtaaattgggtgaggcaggctccaggcagggggttggagtggataggggtgatatggggggatggcatcacagattataattctgcacttaaggataggtttattatcagtaaggacaacggtaagaacaccgtttatcttcagatgtctaaggtgcggtccgatgatactgccctctattattgtgtaaccggccttttcgattactggggccaagggactttggtaaccgtgtcatcatatccctatgacgtccctgactacgcagggggaggagggggatccggtggcggtggtagtggaggaggtggatctggaggagggggaagcggtaccccagctgcgaaacgagttaaattggatggtggtggcgggtcctcaggtttgcccaatggattggatggtgatgaagacttctcagacatcgcagatatggactttagtgccttgctgagccaaatctcatctggctcatcaggtcttcccaacggattggatggcgatgaggacttttccgacatcgcagacatggacttttccgctctgttgagccagataagttctggctcctccggactccctaatggcttggatggagatgaggattttagcgatatagcagacatggattttagcgcattgctctcacaaatctccagtggcgggggtggtagtggattttcagtggatacttccgcacttctcgatttgttttctcccagtgtcaccgtcccagacatgagtcttcctgacctcgactcttctctcgccagtattcaggaactgctcagtccacaggagcctcctcgccctcctgaagcagagaatagttccccagattcaggaaagcagctggtgcactacacagcacagccactgttcctcttggaccctgggagtgtagacacaggctcaaacgatctccccgttctttttgaacttggcgaaggttcctattttagcgagggggacggattcgccgaggaccctactatcagtctccttacaggtagcgagccacccaaagctaaagaccccaccgtgagctagtgactcgaggattcgtcagtagggttgtaaaggtttttcttttcctgagaaaacaaccttttgttttctcaggttttgctttttggcctttccctagctttaaaaaaaaaaaagcaaaactcaccgaggcagttccataggatggctagcaagatcctggtattggtctgcgagaagagcgagctcttcaatcaacctctggattacaaaatttgtgaaagattgactggtattcttaactatgttgctccttttacgctatgtggatacgctgctttaatgcctttgtatcatgctattgcttcccgtatggctttcattttctcctccttgtataaatcctggttgctgtctctttatgaggagttgtggcccgttgtcaggcaacgtggcgtggtgtgcactgtgtttgctgacgcaacccccactggttggggcattgccaccacctgtcagctcctttccgggactttcgctttccccctccctattgccacggcggaactcatcgccgcctgccttgcccgctgctggacaggggctcggctgttgggcactgacaattccgtggtgttgtcggggaaatcatcgtcctttccttggctgctcgcctgtgttgccacctggattctgcgcgggacgtccttctgctacgtcccttcggccctcaatccagcggaccttccttcccgcggcctgctgccggctctgcggcctcttccgcgtcttcgccttcgccctcagacgagtcggatctccctttgggccgcctccccgcgtcgactttaagaccaatcggccgcaggaacccctagtgatggagttggccactccctctctgcgcgctcgctcgctcactgaggccgggcgaccaaaggtcgcccgacgcccgggctttgcccgggcggcctcagtgagcgagcgagcgcgcagctgcctgcaggggcgcctgatgcggtattttctccttacgcatctgtgcggtatttcacaccgcatacgtcaaagcaaccatagtacgcgccctgtagcggcgcattaagcgcggcgggtgtggtggttacgcgcagcgtgaccgctacacttgccagcgccttagcgcccgctcctttcgctttcttcccttcctttctcgccacgttcgccggctttccccgtcaagctctaaatcgggggctccctttagggttccgatttagtgctttacggcacctcgaccccaaaaaacttgatttgggtgatggttcacgtagtgggccatcgccctgatagacggtttttcgccctttgacgttggagtccacgttctttaatagtggactcttgttccaaactggaacaacactcaactctatctcgggctattcttttgatttataagggattttgccgatttcggtctattggttaaaaaatgagctgatttaacaaaaatttaacgcgaattttaacaaaatattaacgtttacaattttatggtgcactctcagtacaatctgctctgatgccgcatagttaagccagccccgacacccgccaacacccgctgacgcgccctgacgggcttgtctgctcccggcatccgcttacagacaagctgtgaccgtctccgggagctgcatgtgtcagaggttttcaccgtcatcaccgaaacgcgcgagacgaaagggcctcgtgatacgcctatttttataggttaatgtcatgataataatggtttcttagacgtcaggtggcacttttcggggaaatgtgcgcggaacccctatttgtttatttttctaaatacattcaaatatgtatccgctcatgagacaataaccctgataaatgcttcaataatattgaaaaaggaagagtatgagtattcaacatttccgtgtcgcccttattcccttttttgcggcattttgccttcctgtttttgctcacccagaaacgctggtgaaagtaaaagatgctgaagatcagttgggtgcacgagtgggttacatcgaactggatctcaacagcggtaagatccttgagagttttcgccccgaagaacgttttccaatgatgagcacttttaaagttctgctatgtggcgcggtattatcccgtattgacgccgggcaagagcaactcggtcgccgcatacactattctcagaatgacttggttgagtactcaccagtcacagaaaagcatcttacggatggcatgacagtaagagaattatgcagtgctgccataaccatgagtgataacactgcggccaacttacttctgacaacgatcggaggaccgaaggagctaaccgcttttttgcacaacatgggggatcatgtaactcgccttgatcgttgggaaccggagctgaatgaagccataccaaacgacgagcgtgacaccacgatgcctgtagcaatggcaacaacgttgcgcaaactattaactggcgaactacttactctagcttcccggcaacaattaatagactggatggaggcggataaagttgcaggaccacttctgcgctcggcccttccggctggctggtttattgctgataaatctggagccggtgagcgtggaagccgcggtatcattgcagcactggggccagatggtaagccctcccgtatcgtagttatctacacgacggggagtcaggcaactatggatgaacgaaatagacagatcgctgagataggtgcctcactgattaagcattggtaactgtcagaccaagtttactcatatatactttagattgatttaaaacttcatttttaatttaaaaggatctaggtgaagatcctttttgataatctcatgaccaaaatcccttaacgtgagttttcgttccactgagcgtcagaccccgtagaaaagatcaaaggatcttcttgagatcctttttttctgcgcgtaatctgctgcttgcaaacaaaaaaaccaccgctaccagcggtggtttgtttgccggatcaagagctaccaactctttttccgaaggtaactggcttcagcagagcgcagataccaaatactgttcttctagtgtagccgtagttaggccaccacttcaagaactctgtagcaccgcctacatacctcgctctgctaatcctgttaccagtggctgctgccagtggcgataagtcgtgtcttaccgggttggactcaagacgatagttaccggataaggcgcagcggtcgggctgaacggggggttcgtgcacacagcccagcttggagcgaacgacctacaccgaactgagatacctacagcgtgagctatgagaaagcgccacgcttcccgaagggagaaaggcggacaggtatccggtaagcggcagggtcggaacaggagagcgcacgagggagcttccagggggaaacgcctggtatctttatagtcctgtcgggtttcgccacctctgacttgagcgtcgatttttgtgatgctcgtcaggggggcggagcctatggaaaaacgccagcaacgcggcctttttacggttcctggccttttgctggccttttgctcacatgt

SEQ ID NO: 17 - DNA, 6689 bp, Artificial Sequence
  pRC124
cctgcaggcagctgcgcgctcgctcgctcactgaggccgcccgggcgtcgggcgacctttggtcgcccggcctcagtgagcgagcgagcgcgcagagagggagtggccaactccatcactaggggttcctgcggcctctagaaaggatctgcgatcgctccggtgcccgtcagtgggcagagcgcacatcgcccacagtccccgagaagttggggggaggggtcggcaattgaacgggtgcctagagaaggtggcgcggggtaaactgggaaagtgatgtcgtgtactggctccgcctttttcccgagggtgggggagaaccgtatataagtgcagtagtcgccgtgaacgttctttttcgcaacgggtttgccgccagaacacagctgaagcttcgaggggctcgcatctctccttcacgcgcccgccgccctacctgaggccgccatccacgccggttgagtcgcgttctgccgcctcccgcctgtggtgcctcctgaactgcgtccgccgtctaggtaagtttaaagctcaggtcgagaccgggcctttgtccggcgctcccttggagcctacctagactcagccggctctccacgctttgcctgaccctgcttgctcaactctacgtctttgtttcgttttctgttctgcgccgttacagatctggctaactaccggtgccaccatgcccgctgcgaaacgagttaaattggatggatcctcaaagctggagaaattcaccaactgttatagcctgtctaagaccctgcgcttcaaggcaatcccagtgggcaagacacaagagaacattgacaacaaacggctcctggtggaggatgagaagagggctgaagattacaagggcgttaagaagctgctggataggtactatctgtcattcatcaacgatgtcctccacagtatcaagctgaagaatctgaacaattacatttctctgttccggaagaagacacggaccgagaaggagaacaaagagctggagaatctggagatcaacctgaggaaagaaatagctaaggctttcaaagggaacgagggttacaagtccctgttcaagaaagacattatcgagactattctgcctgagttcctggacgataaagatgagatcgccctcgtcaattccttcaatgggtttaccacagcctttaccggcttcttcgacaatagagagaatatgttctctgaagaggccaaatccactagcatcgcctttcgctgcataaacgagaacctgactaggtacatcagcaatatggacatctttgagaaagtcgatgccatattcgacaaacatgaggtgcaggagattaaggagaagatcctgaactcagattacgatgtcgaagatttcttcgagggagagttcttcaacttcgtgctcacacaagagggcattgatgtgtacaatgcaatcattggagggttcgtgacagagagtggcgagaagataaagggcctgaacgagtatatcaacctctacaaccagaaaaccaagcagaaactgcctaagttcaagccactgtacaaacaagtgctctcagatagggaaagcctgagcttctacggtgaagggtatacatcagatgaagaagtgctcgaagtgttccgcaacaccctcaataagaacagtgaaatcttctcttcaatcaagaagctggagaaactgttcaagaatttcgatgagtactcctctgccggaatctttgtgaagaatggccctgcaatatccactattagcaaagacatctttggcgagtggaacgttatcagggataagtggaatgccgagtacgatgatattcatctcaagaagaaagccgtggttacagagaaatacgaggatgatagacgcaagagctttaagaagattggtagcttctctctcgaacagctgcaggagtacgccgacgctgacctgtcagtcgtggagaaactcaaggagatcataatccagaaggtggatgaaatctacaaagtgtatggaagctctgagaaactcttcgatgcagactttgttctggagaagagtctgaagaagaacgacgcagtggttgctatcatgaaggacctgctggattctgttaagtctttcgagaattacattaaggcattctttggtgaagggaaggagacaaatagggacgagagcttctatggcgactttgttctggcctacgacatcctcctcaaggttgaccacatctatgacgctatacggaattacgttacccagaagccctatagcaaagacaagttcaagctgtatttccagaatccacagtttatgggtgggtgggataaagacaaagaaacagattacagggccactatcctgcggtacggcagcaaatactatctggctatcatggataagaagtacgccaaatgcctccagaagatcgacaaggacgacgtgggtaccagtccagctgcgaaacgagttaaattggatggtggtggcgggtcctcaggtttgcccaatggattggatggtgatgaagacttctcagacatcgcagatatggactttagtgccttgctgagccaaatctcatctggctcatcaggtcttcccaacggattggatggcgatgaggacttttccgacatcgcagacatggacttttccgctctgttgagccagataagttctggctcctccggactccctaatggcttggatggagatgaggattttagcgatatagcagacatggattttagcgcattgctctcacaaatctccagtggcgggggtggtagtggattttcagtggatacttccgcacttctcgatttgttttctcccagtgtcaccgtcccagacatgagtcttcctgacctcgactcttctctcgccagtattcaggaactgctcagtccacaggagcctcctcgccctcctgaagcagagaatagttccccagattcaggaaagcagctggtgcactacacagcacagccactgttcctcttggaccctgggagtgtagacacaggctcaaacgatctccccgttctttttgaacttggcgaaggttcctattttagcgagggggacggattcgccgaggaccctactatcagtctccttacaggtagcgagccacccaaagctaaagaccccaccgtgagctagtgactcgaggattcgtcagtagggttgtaaaggtttttcttttcctgagaaaacaaccttttgttttctcaggttttgctttttggcctttccctagctttaaaaaaaaaaaagcaaaactcaccgaggcagttccataggatggctagcaagatcctggtattggtctgcgagaagagcgagctcttcaatcaacctctggattacaaaatttgtgaaagattgactggtattcttaactatgttgctccttttacgctatgtggatacgctgctttaatgcctttgtatcatgctattgcttcccgtatggctttcattttctcctccttgtataaatcctggttgctgtctctttatgaggagttgtggcccgttgtcaggcaacgtggcgtggtgtgcactgtgtttgctgacgcaacccccactggttggggcattgccaccacctgtcagctcctttccgggactttcgctttccccctccctattgccacggcggaactcatcgccgcctgccttgcccgctgctggacaggggctcggctgttgggcactgacaattccgtggtgttgtcggggaaatcatcgtcctttccttggctgctcgcctgtgttgccacctggattctgcgcgggacgtccttctgctacgtcccttcggccctcaatccagcggaccttccttcccgcggcctgctgccggctctgcggcctcttccgcgtcttcgccttcgccctcagacgagtcggatctccctttgggccgcctccccgccggccgcaggaacccctagtgatggagttggccactccctctctgcgcgctcgctcgctcactgaggccgggcgaccaaaggtcgcccgacgcccgggctttgcccgggcggcctcagtgagcgagcgagcgcgcagctgcctgcaggggcgcctgatgcggtattttctccttacgcatctgtgcggtatttcacaccgcatacgtcaaagcaaccatagtacgcgccctgtagcggcgcattaagcgcggcgggtgtggtggttacgcgcagcgtgaccgctacacttgccagcgccttagcgcccgctcctttcgctttcttcccttcctttctcgccacgttcgccggctttccccgtcaagctctaaatcgggggctccctttagggttccgatttagtgctttacggcacctcgaccccaaaaaacttgatttgggtgatggttcacgtagtgggccatcgccctgatagacggtttttcgccctttgacgttggagtccacgttctttaatagtggactcttgttccaaactggaacaacactcaactctatctcgggctattcttttgatttataagggattttgccgatttcggtctattggttaaaaaatgagctgatttaacaaaaatttaacgcgaattttaacaaaatattaacgtttacaattttatggtgcactctcagtacaatctgctctgatgccgcatagttaagccagccccgacacccgccaacacccgctgacgcgccctgacgggcttgtctgctcccggcatccgcttacagacaagctgtgaccgtctccgggagctgcatgtgtcagaggttttcaccgtcatcaccgaaacgcgcgagacgaaagggcctcgtgatacgcctatttttataggttaatgtcatgataataatggtttcttagacgtcaggtggcacttttcggggaaatgtgcgcggaacccctatttgtttatttttctaaatacattcaaatatgtatccgctcatgagacaataaccctgataaatgcttcaataatattgaaaaaggaagagtatgagtattcaacatttccgtgtcgcccttattcccttttttgcggcattttgccttcctgtttttgctcacccagaaacgctggtgaaagtaaaagatgctgaagatcagttgggtgcacgagtgggttacatcgaactggatctcaacagcggtaagatccttgagagttttcgccccgaagaacgttttccaatgatgagcacttttaaagttctgctatgtggcgcggtattatcccgtattgacgccgggcaagagcaactcggtcgccgcatacactattctcagaatgacttggttgagtactcaccagtcacagaaaagcatcttacggatggcatgacagtaagagaattatgcagtgctgccataaccatgagtgataacactgcggccaacttacttctgacaacgatcggaggaccgaaggagctaaccgcttttttgcacaacatgggggatcatgtaactcgccttgatcgttgggaaccggagctgaatgaagccataccaaacgacgagcgtgacaccacgatgcctgtagcaatggcaacaacgttgcgcaaactattaactggcgaactacttactctagcttcccggcaacaattaatagactggatggaggcggataaagttgcaggaccacttctgcgctcggcccttccggctggctggtttattgctgataaatctggagccggtgagcgtggaagccgcggtatcattgcagcactggggccagatggtaagccctcccgtatcgtagttatctacacgacggggagtcaggcaactatggatgaacgaaatagacagatcgctgagataggtgcctcactgattaagcattggtaactgtcagaccaagtttactcatatatactttagattgatttaaaacttcatttttaatttaaaaggatctaggtgaagatcctttttgataatctcatgaccaaaatcccttaacgtgagttttcgttccactgagcgtcagaccccgtagaaaagatcaaaggatcttcttgagatcctttttttctgcgcgtaatctgctgcttgcaaacaaaaaaaccaccgctaccagcggtggtttgtttgccggatcaagagctaccaactctttttccgaaggtaactggcttcagcagagcgcagataccaaatactgttcttctagtgtagccgtagttaggccaccacttcaagaactctgtagcaccgcctacatacctcgctctgctaatcctgttaccagtggctgctgccagtggcgataagtcgtgtcttaccgggttggactcaagacgatagttaccggataaggcgcagcggtcgggctgaacggggggttcgtgcacacagcccagcttggagcgaacgacctacaccgaactgagatacctacagcgtgagctatgagaaagcgccacgcttcccgaagggagaaaggcggacaggtatccggtaagcggcagggtcggaacaggagagcgcacgagggagcttccagggggaaacgcctggtatctttatagtcctgtcgggtttcgccacctctgacttgagcgtcgatttttgtgatgctcgtcaggggggcggagcctatggaaaaacgccagcaacgcggcctttttacggttcctggccttttgctggccttttgctcacatgt

SEQ ID NO: 18 - DNA, 6904 bp, Artificial Sequence
  pRC126
cctgcaggcagctgcgcgctcgctcgctcactgaggccgcccgggcgtcgggcgacctttggtcgcccggcctcagtgagcgagcgagcgcgcagagagggagtggccaactccatcactaggggttcctgcggcctctagaaaggatctgcgatcgctccggtgcccgtcagtgggcagagcgcacatcgcccacagtccccgagaagttggggggaggggtcggcaattgaacgggtgcctagagaaggtggcgcggggtaaactgggaaagtgatgtcgtgtactggctccgcctttttcccgagggtgggggagaaccgtatataagtgcagtagtcgccgtgaacgttctttttcgcaacgggtttgccgccagaacacagctgaagcttcgaggggctcgcatctctccttcacgcgcccgccgccctacctgaggccgccatccacgccggttgagtcgcgttctgccgcctcccgcctgtggtgcctcctgaactgcgtccgccgtctaggtaagtttaaagctcaggtcgagaccgggcctttgtccggcgctcccttggagcctacctagactcagccggctctccacgctttgcctgaccctgcttgctcaactctacgtctttgtttcgttttctgttctgcgccgttacagatctggctaactaccggtgccaccatgcccgctgcgaaacgagttaaattggatggtggtggcgggtcctcaggtttgcccaatggattggatggtgatgaagacttctcagacatcgcagatatggactttagtgccttgctgagccaaatctcatctggctcatcaggtcttcccaacggattggatggcgatgaggacttttccgacatcgcagacatggacttttccgctctgttgagccagataagttctggctcctccggactccctaatggcttggatggagatgaggattttagcgatatagcagacatggattttagcgcattgctctcacaaatctccagtggcgggggtggtagtggattttcagtggatacttccgcacttctcgatttgttttctcccagtgtcaccgtcccagacatgagtcttcctgacctcgactcttctctcgccagtattcaggaactgctcagtccacaggagcctcctcgccctcctgaagcagagaatagttccccagattcaggaaagcagctggtgcactacacagcacagccactgttcctcttggaccctgggagtgtagacacaggctcaaacgatctccccgttctttttgaacttggcgaaggttcctattttagcgagggggacggattcgccgaggaccctactatcagtctccttacaggtagcgagccacccaaagctaaagaccccaccgtgagcggtggtggcgggtccggtaacggtaactacgagaagatcaattacaagctcctgccaggacctaacaagatgctgcccaaggtgttcttctccaagaaatggatggcctactataacccaagcgaggacattcagaagatatacaagaatgggacattcaagaagggcgatatgttcaacctcaacgactgccacaagctgattgatttcttcaaggatagcatttctcgctatcccaagtggtctaatgcatacgatttcaacttcagcgagactgagaagtacaaagacatcgctggcttctaccgggaggtggaagagcaaggctataaggtgtcattcgaatccgcttctaagaaggaagtggataagctcgtggaagagggtaagctgtacatgttccagatatacaacaaagacttcagcgataagagccacggcactccaaacctccatactatgtatttcaagctgctgtttgacgagaacaaccacggacagattaggctgtcaggaggcgcagaactcttcatgcgcagagcttcactgaagaaggaggaactcgttgtccacccagccaatagccctatagccaataagaatccagacaatcctaagaaaaccactactctgtcttacgatgtgtataaggataagagattctctgaagatcagtacgaactgcacatacccattgccattaacaagtgccctaagaacatcttcaagattaacacagaggttagagtgctcctgaaacacgacgataacccttatgttataggcattgctcgcggagagagaaacctgctgtacatcgtcgtggtggacggcaaaggcaacatcgtggaacagtacagtctcaatgaaatcattaacaatttcaacggaatccgcattaagaccgactaccattctctcctcgacaagaaggagaaagaaaggttcgaagcaagacagaattggacaagtatagagaatatcaaagaactgaaggctgggtacatctctcaggttgtgcacaagatatgtgagctggtggagaagtacgacgctgttatcgccctcgcggacctgaatagcggcttcaagaactccagggtgaaggtggagaagcaggtgtatcagaagttcgagaagatgctgatcgacaagctcaactatatggtggacaagaaatccaatccttgcgctactggtggagccctgaagggctatcaaatcaccaataagttcgaatctttcaagtctatgagcacccagaatggcttcatcttctacatacccgcatggctgacatccaagattgatccctctaccggatttgttaatctgctcaagactaagtacacctctattgctgactcaaagaagttcatatcatcatttgaccgcatcatgtacgtgccagaagaggacctgttcgagtttgccctggattacaagaatttctctcggactgacgccgactacatcaagaagtggaagctctactcttatggtaatcggattcgcatattccgcaatcccaagaagaataacgtgttcgattgggaggaagtttgcctcaccagcgcttacaaggagctgttcaataagtatgggattaactaccagcagggcgacataagagccctgctgtgcgaacaatctgataaggcattctattcctctttcatggcactgatgtcactgatgctgcaaatgcgcaattccatcaccggaagaacagacgtggcctttctgatctctcctgtcaagaactcagatggcatcttctacgattcccgcaactatgaagcacaggagaatgctatcctgcctaagaatgccgatgcaaatggagcctataacatcgccagaaaggtcctctgggccataggacaattcaagaaagctgaagatgagaagctggacaaggtgaagatcgccatttcaaacaaagagtggctcgaatatgctcagacctcagtgaagcatggtacccccgctgcgaaacgagttaaattggatggtggtggcgggtcctcaggtttgcccaatggattggatggtgatgaagacttctcagacatcgcagatatggactttagtgccttgctgagccaaatctcatctggctcatcaggtcttcccaacggattggatggcgatgaggacttttccgacatcgcagacatggacttttccgctctgttgagccagataagttctggctcctccggactccctaatggcttggatggagatgaggattttagcgatatagcagacatggattttagcgcattgctctcacaaatctccagtggcgggggtggtagtggattttcagtggatacttccgcacttctcgatttgttttctcccagtgtcaccgtcccagacatgagtcttcctgacctcgactcttctctcgccagtattcaggaactgctcagtccacaggagcctcctcgccctcctgaagcagagaatagttccccagattcaggaaagcagctggtgcactacacagcacagccactgttcctcttggaccctgggagtgtagacacaggctcaaacgatctccccgttctttttgaacttggcgaaggttcctattttagcgagggggacggattcgccgaggaccctactatcagtctccttacaggtagcgagccacccaaagctaaagaccccaccgtgagctagtgactcgagaataaaagatctttattttcattagatctgtgtgttggttttttgtgtcggccgcaggaacccctagtgatggagttggccactccctctctgcgcgctcgctcgctcactgaggccgggcgaccaaaggtcgcccgacgcccgggctttgcccgggcggcctcagtgagcgagcgagcgcgcagctgcctgcaggggcgcctgatgcggtattttctccttacgcatctgtgcggtatttcacaccgcatacgtcaaagcaaccatagtacgcgccctgtagcggcgcattaagcgcggcgggtgtggtggttacgcgcagcgtgaccgctacacttgccagcgccttagcgcccgctcctttcgctttcttcccttcctttctcgccacgttcgccggctttccccgtcaagctctaaatcgggggctccctttagggttccgatttagtgctttacggcacctcgaccccaaaaaacttgatttgggtgatggttcacgtagtgggccatcgccctgatagacggtttttcgccctttgacgttggagtccacgttctttaatagtggactcttgttccaaactggaacaacactcaactctatctcgggctattcttttgatttataagggattttgccgatttcggtctattggttaaaaaatgagctgatttaacaaaaatttaacgcgaattttaacaaaatattaacgtttacaattttatggtgcactctcagtacaatctgctctgatgccgcatagttaagccagccccgacacccgccaacacccgctgacgcgccctgacgggcttgtctgctcccggcatccgcttacagacaagctgtgaccgtctccgggagctgcatgtgtcagaggttttcaccgtcatcaccgaaacgcgcgagacgaaagggcctcgtgatacgcctatttttataggttaatgtcatgataataatggtttcttagacgtcaggtggcacttttcggggaaatgtgcgcggaacccctatttgtttatttttctaaatacattcaaatatgtatccgctcatgagacaataaccctgataaatgcttcaataatattgaaaaaggaagagtatgagtattcaacatttccgtgtcgcccttattcccttttttgcggcattttgccttcctgtttttgctcacccagaaacgctggtgaaagtaaaagatgctgaagatcagttgggtgcacgagtgggttacatcgaactggatctcaacagcggtaagatccttgagagttttcgccccgaagaacgttttccaatgatgagcacttttaaagttctgctatgtggcgcggtattatcccgtattgacgccgggcaagagcaactcggtcgccgcatacactattctcagaatgacttggttgagtactcaccagtcacagaaaagcatcttacggatggcatgacagtaagagaattatgcagtgctgccataaccatgagtgataacactgcggccaacttacttctgacaacgatcggaggaccgaaggagctaaccgcttttttgcacaacatgggggatcatgtaactcgccttgatcgttgggaaccggagctgaatgaagccataccaaacgacgagcgtgacaccacgatgcctgtagcaatggcaacaacgttgcgcaaactattaactggcgaactacttactctagcttcccggcaacaattaatagactggatggaggcggataaagttgcaggaccacttctgcgctcggcccttccggctggctggtttattgctgataaatctggagccggtgagcgtggaagccgcggtatcattgcagcactggggccagatggtaagccctcccgtatcgtagttatctacacgacggggagtcaggcaactatggatgaacgaaatagacagatcgctgagataggtgcctcactgattaagcattggtaactgtcagaccaagtttactcatatatactttagattgatttaaaacttcatttttaatttaaaaggatctaggtgaagatcctttttgataatctcatgaccaaaatcccttaacgtgagttttcgttccactgagcgtcagaccccgtagaaaagatcaaaggatcttcttgagatcctttttttctgcgcgtaatctgctgcttgcaaacaaaaaaaccaccgctaccagcggtggtttgtttgccggatcaagagctaccaactctttttccgaaggtaactggcttcagcagagcgcagataccaaatactgttcttctagtgtagccgtagttaggccaccacttcaagaactctgtagcaccgcctacatacctcgctctgctaatcctgttaccagtggctgctgccagtggcgataagtcgtgtcttaccgggttggactcaagacgatagttaccggataaggcgcagcggtcgggctgaacggggggttcgtgcacacagcccagcttggagcgaacgacctacaccgaactgagatacctacagcgtgagctatgagaaagcgccacgcttcccgaagggagaaaggcggacaggtatccggtaagcggcagggtcggaacaggagagcgcacgagggagcttccagggggaaacgcctggtatctttatagtcctgtcgggtttcgccacctctgacttgagcgtcgatttttgtgatgctcgtcaggggggcggagcctatggaaaaacgccagcaacgcggcctttttacggttcctggccttttgctggccttttgctcacatgt

SEQ ID NO: 19 - DNA, 20 bp, Artificial Sequence
  CD80 sg2
tccaggcctgttctgagcac

SEQ ID NO: 20 - DNA, 20 bp, Artificial Sequence
  LIGHT sg2
gaggaggtacgtgaggaaag

SEQ ID NO: 21 - DNA, 20 bp, Artificial Sequence
  CXCL10 sg3
gcaatgccctcggtttacag

SEQ ID NO: 22 - DNA, 20 bp, Artificial Sequence
  4-1BBL sg2
acagggcctggacagggaag

SEQ ID NO: 23 - DNA, 20 bp, Artificial Sequence
  GITRL sg1
agtgcttagcagtgttccaa

SEQ ID NO: 24 - DNA, 7151 bp, Artificial Sequence
  pGW071
cctgcaggcagctgcgcgctcgctcgctcactgaggccgcccgggcgtcgggcgacctttggtcgcccggcctcagtgagcgagcgagcgcgcagagagggagtggccaactccatcactaggggttcctgcggcctctagaaaggatctgcgatcgctccggtgcccgtcagtgggcagagcgcacatcgcccacagtccccgagaagttggggggaggggtcggcaattgaacgggtgcctagagaaggtggcgcggggtaaactgggaaagtgatgtcgtgtactggctccgcctttttcccgagggtgggggagaaccgtatataagtgcagtagtcgccgtgaacgttctttttcgcaacgggtttgccgccagaacacagctgaagcttcgaggggctcgcatctctccttcacgcgcccgccgccctacctgaggccgccatccacgccggttgagtcgcgttctgccgcctcccgcctgtggtgcctcctgaactgcgtccgccgtctaggtaagtttaaagctcaggtcgagaccgggcctttgtccggcgctcccttggagcctacctagactcagccggctctccacgctttgcctgaccctgcttgctcaactctacgtctttgtttcgttttctgttctgcgccgttacagatctggctaactaccggtgccaccatggcttgcaattgtcagttgatgcaggatacaccactcctcaagtttccatgtccaaggctcattcttctctttgtgctgctgattcgtctttcacaagtgtcttcagatgttgatgaacaactgtccaagtcagtgaaagataaggtattgctgccttgccgttacaactctcctcatgaagatgagtctgaagaccgaatctactggcaaaaacatgacaaagtggtgctgtctgtcattgttgggaaactaaaagtgtggcccgagtataagaaccggactttatatgacaacactacctactctcttatcatcctgggcctggtcctttcagaccggggcacatacagctgtgtcgttcaaaagaaggaaagaggaacgtatgaagttaaacacttggctttagtaaagttgtccatcaaagctgacttctctacccccaacataactgagtctggaaacccatctgcagacactaaaaggattacctgctttgcttccgggggtttcccaaagcctcgcttctcttggttggaaaatggaagagaattacctggcatcaatacgacaatttcccaggatcctgaatctgaattgtacaccattagtagccaactagatttcaatacgactcgcaaccacaccattaagtgtctcattaaatatggagatgctcacgtgtcagaggacttcacctgggaaaaacccccagaagaccctcctgatagcaagaacacacttgtgctctttggggcaggattcggcgcagtaataacagtcgtcgtcatcgttgtcatcatcaaatgcttctgtaagcacagaagctgtttcagaagaaatgaggcaagcagagaaacaaacaacagccttaccttcgggcctgaagaagcattagctgaacagaccgtcttccttcgtacgggcagtggagagggcagaggaagtctgctaacatgcggtgacgtcgaggagaatcctggcccaatggagagtgtggtacagccttcagtgtttgtggtggatggacagacggacatcccattcaggcggctggaacagaaccaccggagacggcgctgtggcactgtccaggtcagcctggccctggtgctgctgctaggtgctgggctggccactcagggctggtttctcctgagactgcatcaacgtcttggagacatagtagctcatctgccagatggaggcaaaggctcctgggagaagctgatacaagatcaacgatctcaccaggccaacccagcagcacatcttacaggagccaacgccagcttgataggtattggtggacctctgttatgggagacacgacttggcctggccttcttgaggggcttgacgtatcatgatggggccctggtgaccatggagcccggttactactatgtgtactccaaagtgcagctgagcggcgtgggctgcccccaggggctggccaatggcctccccatcacccatggactatacaagcgcacatcccgctacccgaaggagttagaactgctggtcagtcggcggtcaccctgtggccgggccaacagctcccgagtctggtgggacagcagcttcctgggcggcgtggtacatctggaggctggggaagaggtggtggtccgcgtgcctggaaaccgcctggtcagaccacgtgacggcaccaggtcctatttcggagctttcatggtcactagtggatccggcgcaacaaacttctctctgctgaaacaagccggagatgtcgaagagaatcctggaccgatgaacccaagtgctgccgtcattttctgcctcatcctgctgggtctgagtgggactcaagggatccctctcgcaaggacggtccgctgcaactgcatccatatcgatgacgggccagtgagaatgagggccatagggaagcttgaaatcatccctgcgagcctatcctgcccacgtgttgagatcattgccacgatgaaaaagaatgatgagcagagatgtctgaatccggaatctaagaccatcaagaatttaatgaaagcgtttagccaaaaaaggtctaaaagggctcctgctagcagcggtacccagtgcaccaactacgccctgctgaagctggccggcgatgtggagagcaaccccgggcccatggaccagcacacacttgatgtggaggataccgcggatgccagacatccagcaggtacttcgtgcccctcggatgcggcgctcctcagagataccgggctcctcgcggacgctgcgctcctctcagatactgtgcgccccacaaatgccgcgctccccacggatgctgcctaccctgcggttaatgttcgggatcgcgaggccgcgtggccgcctgcactgaacttctgttcccgccacccaaagctctatggcctagtcgctttggttttgctgcttctgatcgccgcctgtgttcctatcttcacccgcaccgagcctcggccagcgctcacaatcaccacctcgcccaacctgggtacccgagagaataatgcagaccaggtcacccctgtttcccacattggctgccccaacactacacaacagggctctcctgtgttcgccaagctactggctaaaaaccaagcatcgttgtgcaatacaactctgaactggcacagccaagatggagctgggagctcatacctatctcaaggtctgaggtacgaagaagacaaaaaggagttggtggtagacagtcccgggctctactacgtatttttggaactgaagctcagtccaacattcacaaacacaggccacaaggtgcagggctgggtctctcttgttttgcaagcaaagcctcaggtagatgactttgacaacttggccctgacagtggaactgttcccttgctccatggagaacaagttagtggaccgttcctggagtcaactgttgctcctgaaggctggccaccgcctcagtgtgggtctgagggcttatctgcatggagcccaggatgcatacagagactgggagctgtcttatcccaacaccaccagctttggactctttcttgtgaaacccgacaacccatgggaaggcatatgcggtaccgtgaagcagaccctgaacttcgatctgctgaagctggccggcgatgtggagagcaaccccgggcccatgtacagcatgcagctcgcatcctgtgtcacattgacacttgtgctccttgtcaacagcgcacccacttcaagctccacttcaagctctacagcggaagcacagcagcagcagcagcagcagcagcagcagcagcagcacctggagcagctgttgatggacctacaggagctcctgagcaggatggagaattacaggaacctgaaactccccaggatgctcaccttcaaattttacttgcccaagcaggccacagaattgaaagatcttcagtgcctagaagatgaacttggacctctgcggcatgttctggatttgactcaaagcaaaagctttcaattggaagatgctgagaatttcatcagcaatatcagagtaactgttgtaaaactaaagggctctgacaacacatttgagtgccaattcgatgatgagtcagcaactgtggtggactttctgaggagatggatagccttctgtcaaagcatcatctcaacaagccctcaataagaattcaataaaagatctttattttcattagatctgtgtgttggttttttgtgtgcggccgcaggaacccctagtgatggagttggccactccctctctgcgcgctcgctcgctcactgaggccgggcgaccaaaggtcgcccgacgcccgggctttgcccgggcggcctcagtgagcgagcgagcgcgcagctgcctgcaggggcgcctgatgcggtattttctccttacgcatctgtgcggtatttcacaccgcatacgtcaaagcaaccatagtacgcgccctgtagcggcgcattaagcgcggcgggtgtggtggttacgcgcagcgtgaccgctacacttgccagcgccttagcgcccgctcctttcgctttcttcccttcctttctcgccacgttcgccggctttccccgtcaagctctaaatcgggggctccctttagggttccgatttagtgctttacggcacctcgaccccaaaaaacttgatttgggtgatggttcacgtagtgggccatcgccctgatagacggtttttcgccctttgacgttggagtccacgttctttaatagtggactcttgttccaaactggaacaacactcaactctatctcgggctattcttttgatttataagggattttgccgatttcggtctattggttaaaaaatgagctgatttaacaaaaatttaacgcgaattttaacaaaatattaacgtttacaattttatggtgcactctcagtacaatctgctctgatgccgcatagttaagccagccccgacacccgccaacacccgctgacgcgccctgacgggcttgtctgctcccggcatccgcttacagacaagctgtgaccgtctccgggagctgcatgtgtcagaggttttcaccgtcatcaccgaaacgcgcgagacgaaagggcctcgtgatacgcctatttttataggttaatgtcatgataataatggtttcttagacgtcaggtggcacttttcggggaaatgtgcgcggaacccctatttgtttatttttctaaatacattcaaatatgtatccgctcatgagacaataaccctgataaatgcttcaataatattgaaaaaggaagagtatgagtattcaacatttccgtgtcgcccttattcccttttttgcggcattttgccttcctgtttttgctcacccagaaacgctggtgaaagtaaaagatgctgaagatcagttgggtgcacgagtgggttacatcgaactggatctcaacagcggtaagatccttgagagttttcgccccgaagaacgttttccaatgatgagcacttttaaagttctgctatgtggcgcggtattatcccgtattgacgccgggcaagagcaactcggtcgccgcatacactattctcagaatgacttggttgagtactcaccagtcacagaaaagcatcttacggatggcatgacagtaagagaattatgcagtgctgccataaccatgagtgataacactgcggccaacttacttctgacaacgatcggaggaccgaaggagctaaccgcttttttgcacaacatgggggatcatgtaactcgccttgatcgttgggaaccggagctgaatgaagccataccaaacgacgagcgtgacaccacgatgcctgtagcaatggcaacaacgttgcgcaaactattaactggcgaactacttactctagcttcccggcaacaattaatagactggatggaggcggataaagttgcaggaccacttctgcgctcggcccttccggctggctggtttattgctgataaatctggagccggtgagcgtggaagccgcggtatcattgcagcactggggccagatggtaagccctcccgtatcgtagttatctacacgacggggagtcaggcaactatggatgaacgaaatagacagatcgctgagataggtgcctcactgattaagcattggtaactgtcagaccaagtttactcatatatactttagattgatttaaaacttcatttttaatttaaaaggatctaggtgaagatcctttttgataatctcatgaccaaaatcccttaacgtgagttttcgttccactgagcgtcagaccccgtagaaaagatcaaaggatcttcttgagatcctttttttctgcgcgtaatctgctgcttgcaaacaaaaaaaccaccgctaccagcggtggtttgtttgccggatcaagagctaccaactctttttccgaaggtaactggcttcagcagagcgcagataccaaatactgttcttctagtgtagccgtagttaggccaccacttcaagaactctgtagcaccgcctacatacctcgctctgctaatcctgttaccagtggctgctgccagtggcgataagtcgtgtcttaccgggttggactcaagacgatagttaccggataaggcgcagcggtcgggctgaacggggggttcgtgcacacagcccagcttggagcgaacgacctacaccgaactgagatacctacagcgtgagctatgagaaagcgccacgcttcccgaagggagaaaggcggacaggtatccggtaagcggcagggtcggaacaggagagcgcacgagggagcttccagggggaaacgcctggtatctttatagtcctgtcgggtttcgccacctctgacttgagcgtcgatttttgtgatgctcgtcaggggggcggagcctatggaaaaacgccagcaacgcggcctttttacggttcctggccttttgctggccttttgctcacatgt

SEQ ID NO: 25 - DNA, 3956 bp, Artificial Sequence
  pGW072
cctgcaggcagctgcgcgctcgctcgctcactgaggccgcccgggcgtcgggcgacctttggtcgcccggcctcagtgagcgagcgagcgcgcagagagggagtggccaactccatcactaggggttcctgcggcctctagaaaggatctgcgatcgctccggtgcccgtcagtgggcagagcgcacatcgcccacagtccccgagaagttggggggaggggtcggcaattgaacgggtgcctagagaaggtggcgcggggtaaactgggaaagtgatgtcgtgtactggctccgcctttttcccgagggtgggggagaaccgtatataagtgcagtagtcgccgtgaacgttctttttcgcaacgggtttgccgccagaacacagctgaagcttcgaggggctcgcatctctccttcacgcgcccgccgccctacctgaggccgccatccacgccggttgagtcgcgttctgccgcctcccgcctgtggtgcctcctgaactgcgtccgccgtctaggtaagtttaaagctcaggtcgagaccgggcctttgtccggcgctcccttggagcctacctagactcagccggctctccacgctttgcctgaccctgcttgctcaactctacgtctttgtttcgttttctgttctgcgccgttacagatctggctaactaccggtgccaccatgaacgctacacactgcatcttggctttgcagctcttcctcatggctgtttctggctgttactgccacggcacagtcattgaaagcctagaaagtctgaataactattttaactcaagtggcatagatgtggaagaaaagagtctcttcttggatatctggaggaactggcaaaaggatggtgacatgaaaatcctgcagagccagattatctctttctacctcagactctttgaagtcttgaaagacaatcaggccatcagcaacaacataagcgtcattgaatcacacctgattactaccttcttcagcaacagcaaggcgaaaaaggatgcattcatgagtattgccaagtttgaggtcaacaacccacaggtccagcgccaagcattcaatgagctcatccgagtggtccaccagctgttgccggaatccagcctcaggaagcggaaaaggagtcgctgctgagaattcaataaaagatctttattttcattagatctgtgtgttggttttttgtgtgcggccgcaggaacccctagtgatggagttggccactccctctctgcgcgctcgctcgctcactgaggccgggcgaccaaaggtcgcccgacgcccgggctttgcccgggcggcctcagtgagcgagcgagcgcgcagctgcctgcaggggcgcctgatgcggtattttctccttacgcatctgtgcggtatttcacaccgcatacgtcaaagcaaccatagtacgcgccctgtagcggcgcattaagcgcggcgggtgtggtggttacgcgcagcgtgaccgctacacttgccagcgccttagcgcccgctcctttcgctttcttcccttcctttctcgccacgttcgccggctttccccgtcaagctctaaatcgggggctccctttagggttccgatttagtgctttacggcacctcgaccccaaaaaacttgatttgggtgatggttcacgtagtgggccatcgccctgatagacggtttttcgccctttgacgttggagtccacgttctttaatagtggactcttgttccaaactggaacaacactcaactctatctcgggctattcttttgatttataagggattttgccgatttcggtctattggttaaaaaatgagctgatttaacaaaaatttaacgcgaattttaacaaaatattaacgtttacaattttatggtgcactctcagtacaatctgctctgatgccgcatagttaagccagccccgacacccgccaacacccgctgacgcgccctgacgggcttgtctgctcccggcatccgcttacagacaagctgtgaccgtctccgggagctgcatgtgtcagaggttttcaccgtcatcaccgaaacgcgcgagacgaaagggcctcgtgatacgcctatttttataggttaatgtcatgataataatggtttcttagacgtcaggtggcacttttcggggaaatgtgcgcggaacccctatttgtttatttttctaaatacattcaaatatgtatccgctcatgagacaataaccctgataaatgcttcaataatattgaaaaaggaagagtatgagtattcaacatttccgtgtcgcccttattcccttttttgcggcattttgccttcctgtttttgctcacccagaaacgctggtgaaagtaaaagatgctgaagatcagttgggtgcacgagtgggttacatcgaactggatctcaacagcggtaagatccttgagagttttcgccccgaagaacgttttccaatgatgagcacttttaaagttctgctatgtggcgcggtattatcccgtattgacgccgggcaagagcaactcggtcgccgcatacactattctcagaatgacttggttgagtactcaccagtcacagaaaagcatcttacggatggcatgacagtaagagaattatgcagtgctgccataaccatgagtgataacactgcggccaacttacttctgacaacgatcggaggaccgaaggagctaaccgcttttttgcacaacatgggggatcatgtaactcgccttgatcgttgggaaccggagctgaatgaagccataccaaacgacgagcgtgacaccacgatgcctgtagcaatggcaacaacgttgcgcaaactattaactggcgaactacttactctagcttcccggcaacaattaatagactggatggaggcggataaagttgcaggaccacttctgcgctcggcccttccggctggctggtttattgctgataaatctggagccggtgagcgtggaagccgcggtatcattgcagcactggggccagatggtaagccctcccgtatcgtagttatctacacgacggggagtcaggcaactatggatgaacgaaatagacagatcgctgagataggtgcctcactgattaagcattggtaactgtcagaccaagtttactcatatatactttagattgatttaaaacttcatttttaatttaaaaggatctaggtgaagatcctttttgataatctcatgaccaaaatcccttaacgtgagttttcgttccactgagcgtcagaccccgtagaaaagatcaaaggatcttcttgagatcctttttttctgcgcgtaatctgctgcttgcaaacaaaaaaaccaccgctaccagcggtggtttgtttgccggatcaagagctaccaactctttttccgaaggtaactggcttcagcagagcgcagataccaaatactgttcttctagtgtagccgtagttaggccaccacttcaagaactctgtagcaccgcctacatacctcgctctgctaatcctgttaccagtggctgctgccagtggcgataagtcgtgtcttaccgggttggactcaagacgatagttaccggataaggcgcagcggtcgggctgaacggggggttcgtgcacacagcccagcttggagcgaacgacctacaccgaactgagatacctacagcgtgagctatgagaaagcgccacgcttcccgaagggagaaaggcggacaggtatccggtaagcggcagggtcggaacaggagagcgcacgagggagcttccagggggaaacgcctggtatctttatagtcctgtcgggtttcgccacctctgacttgagcgtcgatttttgtgatgctcgtcaggggggcggagcctatggaaaaacgccagcaacgcggcctttttacggttcctggccttttgctggccttttgctcacatgt

SEQ ID NO: 26 - DNA, 7163 bp, Artificial Sequence
  pGW073
cctgcaggcagctgcgcgctcgctcgctcactgaggccgcccgggcgtcgggcgacctttggtcgcccggcctcagtgagcgagcgagcgcgcagagagggagtggccaactccatcactaggggttcctgcggcctctagaaaggatctgcgatcgctccggtgcccgtcagtgggcagagcgcacatcgcccacagtccccgagaagttggggggaggggtcggcaattgaacgggtgcctagagaaggtggcgcggggtaaactgggaaagtgatgtcgtgtactggctccgcctttttcccgagggtgggggagaaccgtatataagtgcagtagtcgccgtgaacgttctttttcgcaacgggtttgccgccagaacacagctgaagcttcgaggggctcgcatctctccttcacgcgcccgccgccctacctgaggccgccatccacgccggttgagtcgcgttctgccgcctcccgcctgtggtgcctcctgaactgcgtccgccgtctaggtaagtttaaagctcaggtcgagaccgggcctttgtccggcgctcccttggagcctacctagactcagccggctctccacgctttgcctgaccctgcttgctcaactctacgtctttgtttcgttttctgttctgcgccgttacagatctggctaactaccggtgccaccatggcttgcaattgtcagttgatgcaggatacaccactcctcaagtttccatgtccaaggctcattcttctctttgtgctgctgattcgtctttcacaagtgtcttcagatgttgatgaacaactgtccaagtcagtgaaagataaggtattgctgccttgccgttacaactctcctcatgaagatgagtctgaagaccgaatctactggcaaaaacatgacaaagtggtgctgtctgtcattgttgggaaactaaaagtgtggcccgagtataagaaccggactttatatgacaacactacctactctcttatcatcctgggcctggtcctttcagaccggggcacatacagctgtgtcgttcaaaagaaggaaagaggaacgtatgaagttaaacacttggctttagtaaagttgtccatcaaagctgacttctctacccccaacataactgagtctggaaacccatctgcagacactaaaaggattacctgctttgcttccgggggtttcccaaagcctcgcttctcttggttggaaaatggaagagaattacctggcatcaatacgacaatttcccaggatcctgaatctgaattgtacaccattagtagccaactagatttcaatacgactcgcaaccacaccattaagtgtctcattaaatatggagatgctcacgtgtcagaggacttcacctgggaaaaacccccagaagaccctcctgatagcaagaacacacttgtgctctttggggcaggattcggcgcagtaataacagtcgtcgtcatcgttgtcatcatcaaatgcttctgtaagcacagaagctgtttcagaagaaatgaggcaagcagagaaacaaacaacagccttaccttcgggcctgaagaagcattagctgaacagaccgtcttccttcgtacgggcagtggagagggcagaggaagtctgctaacatgcggtgacgtcgaggagaatcctggcccaatggagagtgtggtacagccttcagtgtttgtggtggatggacagacggacatcccattcaggcggctggaacagaaccaccggagacggcgctgtggcactgtccaggtcagcctggccctggtgctgctgctaggtgctgggctggccactcagggctggtttctcctgagactgcatcaacgtcttggagacatagtagctcatctgccagatggaggcaaaggctcctgggagaagctgatacaagatcaacgatctcaccaggccaacccagcagcacatcttacaggagccaacgccagcttgataggtattggtggacctctgttatgggagacacgacttggcctggccttcttgaggggcttgacgtatcatgatggggccctggtgaccatggagcccggttactactatgtgtactccaaagtgcagctgagcggcgtgggctgcccccaggggctggccaatggcctccccatcacccatggactatacaagcgcacatcccgctacccgaaggagttagaactgctggtcagtcggcggtcaccctgtggccgggccaacagctcccgagtctggtgggacagcagcttcctgggcggcgtggtacatctggaggctggggaagaggtggtggtccgcgtgcctggaaaccgcctggtcagaccacgtgacggcaccaggtcctatttcggagctttcatggtcactagtggatccggcgcaacaaacttctctctgctgaaacaagccggagatgtcgaagagaatcctggaccgatgaacccaagtgctgccgtcattttctgcctcatcctgctgggtctgagtgggactcaagggatccctctcgcaaggacggtccgctgcaactgcatccatatcgatgacgggccagtgagaatgagggccatagggaagcttgaaatcatccctgcgagcctatcctgcccacgtgttgagatcattgccacgatgaaaaagaatgatgagcagagatgtctgaatccggaatctaagaccatcaagaatttaatgaaagcgtttagccaaaaaaggtctaaaagggctcctgctagcagcggtacccagtgcaccaactacgccctgctgaagctggccggcgatgtggagagcaaccccgggcccatggaccagcacacacttgatgtggaggataccgcggatgccagacatccagcaggtacttcgtgcccctcggatgcggcgctcctcagagataccgggctcctcgcggacgctgcgctcctctcagatactgtgcgccccacaaatgccgcgctccccacggatgctgcctaccctgcggttaatgttcgggatcgcgaggccgcgtggccgcctgcactgaacttctgttcccgccacccaaagctctatggcctagtcgctttggttttgctgcttctgatcgccgcctgtgttcctatcttcacccgcaccgagcctcggccagcgctcacaatcaccacctcgcccaacctgggtacccgagagaataatgcagaccaggtcacccctgtttcccacattggctgccccaacactacacaacagggctctcctgtgttcgccaagctactggctaaaaaccaagcatcgttgtgcaatacaactctgaactggcacagccaagatggagctgggagctcatacctatctcaaggtctgaggtacgaagaagacaaaaaggagttggtggtagacagtcccgggctctactacgtatttttggaactgaagctcagtccaacattcacaaacacaggccacaaggtgcagggctgggtctctcttgttttgcaagcaaagcctcaggtagatgactttgacaacttggccctgacagtggaactgttcccttgctccatggagaacaagttagtggaccgttcctggagtcaactgttgctcctgaaggctggccaccgcctcagtgtgggtctgagggcttatctgcatggagcccaggatgcatacagagactgggagctgtcttatcccaacaccaccagctttggactctttcttgtgaaacccgacaacccatgggaaggcatatgcggtaccgtgaagcagaccctgaacttcgatctgctgaagctggccggcgatgtggagagcaaccccgggcccatggaggaaatgcctttgagagagtcaagtcctcaaagggcagagaggtgcaagaagtcatggctcttgtgcatagtggctctgttactgatgctgctctgttctttgggtacactgatctatacttcactcaagccaactgccatcgagtcctgcatggttaagtttgaactatcatcctcaaaatggcacatgacatctcccaaacctcactgtgtgaatacgacatctgatgggaagctgaagatactgcagagtggcacatatttaatctacggccaagtgattcctgtggataagaaatacataaaagacaatgcccccttcgtagtacagatatataaaaagaatgatgtcctacaaactctaatgaatgattttcaaatcttgcctataggaggggtttatgaactgcatgctggagataacatatatctgaagttcaactctaaagaccatattcagaaaaataacacatactgggggatcatcttaatgcctgatctaccattcatctcttaggaattcaataaaagatctttattttcattagatctgtgtgttggttttttgtgtgcggccgcaggaacccctagtgatggagttggccactccctctctgcgcgctcgctcgctcactgaggccgggcgaccaaaggtcgcccgacgcccgggctttgcccgggcggcctcagtgagcgagcgagcgcgcagctgcctgcaggggcgcctgatgcggtattttctccttacgcatctgtgcggtatttcacaccgcatacgtcaaagcaaccatagtacgcgccctgtagcggcgcattaagcgcggcgggtgtggtggttacgcgcagcgtgaccgctacacttgccagcgccttagcgcccgctcctttcgctttcttcccttcctttctcgccacgttcgccggctttccccgtcaagctctaaatcgggggctccctttagggttccgatttagtgctttacggcacctcgaccccaaaaaacttgatttgggtgatggttcacgtagtgggccatcgccctgatagacggtttttcgccctttgacgttggagtccacgttctttaatagtggactcttgttccaaactggaacaacactcaactctatctcgggctattcttttgatttataagggattttgccgatttcggtctattggttaaaaaatgagctgatttaacaaaaatttaacgcgaattttaacaaaatattaacgtttacaattttatggtgcactctcagtacaatctgctctgatgccgcatagttaagccagccccgacacccgccaacacccgctgacgcgccctgacgggcttgtctgctcccggcatccgcttacagacaagctgtgaccgtctccgggagctgcatgtgtcagaggttttcaccgtcatcaccgaaacgcgcgagacgaaagggcctcgtgatacgcctatttttataggttaatgtcatgataataatggtttcttagacgtcaggtggcacttttcggggaaatgtgcgcggaacccctatttgtttatttttctaaatacattcaaatatgtatccgctcatgagacaataaccctgataaatgcttcaataatattgaaaaaggaagagtatgagtattcaacatttccgtgtcgcccttattcccttttttgcggcattttgccttcctgtttttgctcacccagaaacgctggtgaaagtaaaagatgctgaagatcagttgggtgcacgagtgggttacatcgaactggatctcaacagcggtaagatccttgagagttttcgccccgaagaacgttttccaatgatgagcacttttaaagttctgctatgtggcgcggtattatcccgtattgacgccgggcaagagcaactcggtcgccgcatacactattctcagaatgacttggttgagtactcaccagtcacagaaaagcatcttacggatggcatgacagtaagagaattatgcagtgctgccataaccatgagtgataacactgcggccaacttacttctgacaacgatcggaggaccgaaggagctaaccgcttttttgcacaacatgggggatcatgtaactcgccttgatcgttgggaaccggagctgaatgaagccataccaaacgacgagcgtgacaccacgatgcctgtagcaatggcaacaacgttgcgcaaactattaactggcgaactacttactctagcttcccggcaacaattaatagactggatggaggcggataaagttgcaggaccacttctgcgctcggcccttccggctggctggtttattgctgataaatctggagccggtgagcgtggaagccgcggtatcattgcagcactggggccagatggtaagccctcccgtatcgtagttatctacacgacggggagtcaggcaactatggatgaacgaaatagacagatcgctgagataggtgcctcactgattaagcattggtaactgtcagaccaagtttactcatatatactttagattgatttaaaacttcatttttaatttaaaaggatctaggtgaagatcctttttgataatctcatgaccaaaatcccttaacgtgagttttcgttccactgagcgtcagaccccgtagaaaagatcaaaggatcttcttgagatcctttttttctgcgcgtaatctgctgcttgcaaacaaaaaaaccaccgctaccagcggtggtttgtttgccggatcaagagctaccaactctttttccgaaggtaactggcttcagcagagcgcagataccaaatactgttcttctagtgtagccgtagttaggccaccacttcaagaactctgtagcaccgcctacatacctcgctctgctaatcctgttaccagtggctgctgccagtggcgataagtcgtgtcttaccgggttggactcaagacgatagttaccggataaggcgcagcggtcgggctgaacggggggttcgtgcacacagcccagcttggagcgaacgacctacaccgaactgagatacctacagcgtgagctatgagaaagcgccacgcttcccgaagggagaaaggcggacaggtatccggtaagcggcagggtcggaacaggagagcgcacgagggagcttccagggggaaacgcctggtatctttatagtcctgtcgggtttcgccacctctgacttgagcgtcgatttttgtgatgctcgtcaggggggcggagcctatggaaaaacgccagcaacgcggcctttttacggttcctggccttttgctggccttttgctcacatgt

SEQ ID NO: 27 - DNA, 3491 bp, Artificial Sequence
  pGW078
cctgcaggcagctgcgcgctcgctcgctcactgaggccgcccgggcgtcgggcgacctttggtcgcccggcctcagtgagcgagcgagcgcgcagagagggagtggccaactccatcactaggggttcctgcggcctctagaaaggatctgcgatcgctccggtgcccgtcagtgggcagagcgcacatcgcccacagtccccgagaagttggggggaggggtcggcaattgaacgggtgcctagagaaggtggcgcggggtaaactgggaaagtgatgtcgtgtactggctccgcctttttcccgagggtgggggagaaccgtatataagtgcagtagtcgccgtgaacgttctttttcgcaacgggtttgccgccagaacacagctgaagcttcgaggggctcgcatctctccttcacgcgcccgccgccctacctgaggccgccatccacgccggttgagtcgcgttctgccgcctcccgcctgtggtgcctcctgaactgcgtccgccgtctaggtaagtttaaagctcaggtcgagaccgggcctttgtccggcgctcccttggagcctacctagactcagccggctctccacgctttgcctgaccctgcttgctcaactctacgtctttgtttcgttttctgttctgcgccgttacagatctggctaactaccggtgccacctgagaattcaataaaagatctttattttcattagatctgtgtgttggttttttgtgtgcggccgcaggaacccctagtgatggagttggccactccctctctgcgcgctcgctcgctcactgaggccgggcgaccaaaggtcgcccgacgcccgggctttgcccgggcggcctcagtgagcgagcgagcgcgcagctgcctgcaggggcgcctgatgcggtattttctccttacgcatctgtgcggtatttcacaccgcatacgtcaaagcaaccatagtacgcgccctgtagcggcgcattaagcgcggcgggtgtggtggttacgcgcagcgtgaccgctacacttgccagcgccttagcgcccgctcctttcgctttcttcccttcctttctcgccacgttcgccggctttccccgtcaagctctaaatcgggggctccctttagggttccgatttagtgctttacggcacctcgaccccaaaaaacttgatttgggtgatggttcacgtagtgggccatcgccctgatagacggtttttcgccctttgacgttggagtccacgttctttaatagtggactcttgttccaaactggaacaacactcaactctatctcgggctattcttttgatttataagggattttgccgatttcggtctattggttaaaaaatgagctgatttaacaaaaatttaacgcgaattttaacaaaatattaacgtttacaattttatggtgcactctcagtacaatctgctctgatgccgcatagttaagccagccccgacacccgccaacacccgctgacgcgccctgacgggcttgtctgctcccggcatccgcttacagacaagctgtgaccgtctccgggagctgcatgtgtcagaggttttcaccgtcatcaccgaaacgcgcgagacgaaagggcctcgtgatacgcctatttttataggttaatgtcatgataataatggtttcttagacgtcaggtggcacttttcggggaaatgtgcgcggaacccctatttgtttatttttctaaatacattcaaatatgtatccgctcatgagacaataaccctgataaatgcttcaataatattgaaaaaggaagagtatgagtattcaacatttccgtgtcgcccttattcccttttttgcggcattttgccttcctgtttttgctcacccagaaacgctggtgaaagtaaaagatgctgaagatcagttgggtgcacgagtgggttacatcgaactggatctcaacagcggtaagatccttgagagttttcgccccgaagaacgttttccaatgatgagcacttttaaagttctgctatgtggcgcggtattatcccgtattgacgccgggcaagagcaactcggtcgccgcatacactattctcagaatgacttggttgagtactcaccagtcacagaaaagcatcttacggatggcatgacagtaagagaattatgcagtgctgccataaccatgagtgataacactgcggccaacttacttctgacaacgatcggaggaccgaaggagctaaccgcttttttgcacaacatgggggatcatgtaactcgccttgatcgttgggaaccggagctgaatgaagccataccaaacgacgagcgtgacaccacgatgcctgtagcaatggcaacaacgttgcgcaaactattaactggcgaactacttactctagcttcccggcaacaattaatagactggatggaggcggataaagttgcaggaccacttctgcgctcggcccttccggctggctggtttattgctgataaatctggagccggtgagcgtggaagccgcggtatcattgcagcactggggccagatggtaagccctcccgtatcgtagttatctacacgacggggagtcaggcaactatggatgaacgaaatagacagatcgctgagataggtgcctcactgattaagcattggtaactgtcagaccaagtttactcatatatactttagattgatttaaaacttcatttttaatttaaaaggatctaggtgaagatcctttttgataatctcatgaccaaaatcccttaacgtgagttttcgttccactgagcgtcagaccccgtagaaaagatcaaaggatcttcttgagatcctttttttctgcgcgtaatctgctgcttgcaaacaaaaaaaccaccgctaccagcggtggtttgtttgccggatcaagagctaccaactctttttccgaaggtaactggcttcagcagagcgcagataccaaatactgttcttctagtgtagccgtagttaggccaccacttcaagaactctgtagcaccgcctacatacctcgctctgctaatcctgttaccagtggctgctgccagtggcgataagtcgtgtcttaccgggttggactcaagacgatagttaccggataaggcgcagcggtcgggctgaacggggggttcgtgcacacagcccagcttggagcgaacgacctacaccgaactgagatacctacagcgtgagctatgagaaagcgccacgcttcccgaagggagaaaggcggacaggtatccggtaagcggcagggtcggaacaggagagcgcacgagggagcttccagggggaaacgcctggtatctttatagtcctgtcgggtttcgccacctctgacttgagcgtcgatttttgtgatgctcgtcaggggggcggagcctatggaaaaacgccagcaacgcggcctttttacggttcctggccttttgctggccttttgctcacatgt

SEQ ID NO: 28 - DNA, 7322 bp, Artificial Sequence
  pGW090
cctgcaggcagctgcgcgctcgctcgctcactgaggccgcccgggcgtcgggcgacctttggtcgcccggcctcagtgagcgagcgagcgcgcagagagggagtggccaactccatcactaggggttcctgcggcctctagaaaggatctgcgatcgctccggtgcccgtcagtgggcagagcgcacatcgcccacagtccccgagaagttggggggaggggtcggcaattgaacgggtgcctagagaaggtggcgcggggtaaactgggaaagtgatgtcgtgtactggctccgcctttttcccgagggtgggggagaaccgtatataagtgcagtagtcgccgtgaacgttctttttcgcaacgggtttgccgccagaacacagctgaagcttcgaggggctcgcatctctccttcacgcgcccgccgccctacctgaggccgccatccacgccggttgagtcgcgttctgccgcctcccgcctgtggtgcctcctgaactgcgtccgccgtctaggtaagtttaaagctcaggtcgagaccgggcctttgtccggcgctcccttggagcctacctagactcagccggctctccacgctttgcctgaccctgcttgctcaactctacgtctttgtttcgttttctgttctgcgccgttacagatctggctaactaccggtgccaccatggcttgcaattgtcagttgatgcaggatacaccactcctcaagtttccatgtccaaggctcattcttctctttgtgctgctgattcgtctttcacaagtgtcttcagatgttgatgaacaactgtccaagtcagtgaaagataaggtattgctgccttgccgttacaactctcctcatgaagatgagtctgaagaccgaatctactggcaaaaacatgacaaagtggtgctgtctgtcattgttgggaaactaaaagtgtggcccgagtataagaaccggactttatatgacaacactacctactctcttatcatcctgggcctggtcctttcagaccggggcacatacagctgtgtcgttcaaaagaaggaaagaggaacgtatgaagttaaacacttggctttagtaaagttgtccatcaaagctgacttctctacccccaacataactgagtctggaaacccatctgcagacactaaaaggattacctgctttgcttccgggggtttcccaaagcctcgcttctcttggttggaaaatggaagagaattacctggcatcaatacgacaatttcccaggatcctgaatctgaattgtacaccattagtagccaactagatttcaatacgactcgcaaccacaccattaagtgtctcattaaatatggagatgctcacgtgtcagaggacttcacctgggaaaaacccccagaagaccctcctgatagcaagaacacacttgtgctctttggggcaggattcggcgcagtaataacagtcgtcgtcatcgttgtcatcatcaaatgcttctgtaagcacagaagctgtttcagaagaaatgaggcaagcagagaaacaaacaacagccttaccttcgggcctgaagaagcattagctgaacagaccgtcttccttcgtacgggcagtggagagggcagaggaagtctgctaacatgcggtgacgtcgaggagaatcctggcccaatggagagtgtggtacagccttcagtgtttgtggtggatggacagacggacatcccattcaggcggctggaacagaaccaccggagacggcgctgtggcactgtccaggtcagcctggccctggtgctgctgctaggtgctgggctggccactcagggctggtttctcctgagactgcatcaacgtcttggagacatagtagctcatctgccagatggaggcaaaggctcctgggagaagctgatacaagatcaacgatctcaccaggccaacccagcagcacatcttacaggagccaacgccagcttgataggtattggtggacctctgttatgggagacacgacttggcctggccttcttgaggggcttgacgtatcatgatggggccctggtgaccatggagcccggttactactatgtgtactccaaagtgcagctgagcggcgtgggctgcccccaggggctggccaatggcctccccatcacccatggactatacaagcgcacatcccgctacccgaaggagttagaactgctggtcagtcggcggtcaccctgtggccgggccaacagctcccgagtctggtgggacagcagcttcctgggcggcgtggtacatctggaggctggggaagaggtggtggtccgcgtgcctggaaaccgcctggtcagaccacgtgacggcaccaggtcctatttcggagctttcatggtcactagtggatccggcgcaacaaacttctctctgctgaaacaagccggagatgtcgaagagaatcctggaccgatgtacagcatgcagctcgcatcctgtgtcacattgacacttgtgctccttgtcaacagcgcacccacttcaagctccacttcaagctctacagcggaagcacagcagcagcagcagcagcagcagcagcagcagcagcacctggagcagctgttgatggacctacaggagctcctgagcaggatggagaattacaggaacctgaaactccccaggatgctcaccttcaaattttacttgcccaagcaggccacagaattgaaagatcttcagtgcctagaagatgaacttggacctctgcggcatgttctggatttgactcaaagcaaaagctttcaattggaagatgctgagaatttcatcagcaatatcagagtaactgttgtaaaactaaagggctctgacaacacatttgagtgccaattcgatgatgagtcagcaactgtggtggactttctgaggagatggatagccttctgtcaaagcatcatctcaacaagccctcaagctagcagcggtacccagtgcaccaactacgccctgctgaagctggccggcgatgtggagagcaaccccgggcccatggaccagcacacacttgatgtggaggataccgcggatgccagacatccagcaggtacttcgtgcccctcggatgcggcgctcctcagagataccgggctcctcgcggacgctgcgctcctctcagatactgtgcgccccacaaatgccgcgctccccacggatgctgcctaccctgcggttaatgttcgggatcgcgaggccgcgtggccgcctgcactgaacttctgttcccgccacccaaagctctatggcctagtcgctttggttttgctgcttctgatcgccgcctgtgttcctatcttcacccgcaccgagcctcggccagcgctcacaatcaccacctcgcccaacctgggtacccgagagaataatgcagaccaggtcacccctgtttcccacattggctgccccaacactacacaacagggctctcctgtgttcgccaagctactggctaaaaaccaagcatcgttgtgcaatacaactctgaactggcacagccaagatggagctgggagctcatacctatctcaaggtctgaggtacgaagaagacaaaaaggagttggtggtagacagtcccgggctctactacgtatttttggaactgaagctcagtccaacattcacaaacacaggccacaaggtgcagggctgggtctctcttgttttgcaagcaaagcctcaggtagatgactttgacaacttggccctgacagtggaactgttcccttgctccatggagaacaagttagtggaccgttcctggagtcaactgttgctcctgaaggctggccaccgcctcagtgtgggtctgagggcttatctgcatggagcccaggatgcatacagagactgggagctgtcttatcccaacaccaccagctttggactctttcttgtgaaacccgacaacccatgggaaggcatatgcggtaccgtgaagcagaccctgaacttcgatctgctgaagctggccggcgatgtggagagcaaccccgggcccatgaacgctacacactgcatcttggctttgcagctcttcctcatggctgtttctggctgttactgccacggcacagtcattgaaagcctagaaagtctgaataactattttaactcaagtggcatagatgtggaagaaaagagtctcttcttggatatctggaggaactggcaaaaggatggtgacatgaaaatcctgcagagccagattatctctttctacctcagactctttgaagtcttgaaagacaatcaggccatcagcaacaacataagcgtcattgaatcacacctgattactaccttcttcagcaacagcaaggcgaaaaaggatgcattcatgagtattgccaagtttgaggtcaacaacccacaggtccagcgccaagcattcaatgagctcatccgagtggtccaccagctgttgccggaatccagcctcaggaagcggaaaaggagtcgctgctgagaattcaataaaagatctttattttcattagatctgtgtgttggttttttgtgtgcggccgcaggaacccctagtgatggagttggccactccctctctgcgcgctcgctcgctcactgaggccgggcgaccaaaggtcgcccgacgcccgggctttgcccgggcggcctcagtgagcgagcgagcgcgcagctgcctgcaggggcgcctgatgcggtattttctccttacgcatctgtgcggtatttcacaccgcatacgtcaaagcaaccatagtacgcgccctgtagcggcgcattaagcgcggcgggtgtggtggttacgcgcagcgtgaccgctacacttgccagcgccttagcgcccgctcctttcgctttcttcccttcctttctcgccacgttcgccggctttccccgtcaagctctaaatcgggggctccctttagggttccgatttagtgctttacggcacctcgaccccaaaaaacttgatttgggtgatggttcacgtagtgggccatcgccctgatagacggtttttcgccctttgacgttggagtccacgttctttaatagtggactcttgttccaaactggaacaacactcaactctatctcgggctattcttttgatttataagggattttgccgatttcggtctattggttaaaaaatgagctgatttaacaaaaatttaacgcgaattttaacaaaatattaacgtttacaattttatggtgcactctcagtacaatctgctctgatgccgcatagttaagccagccccgacacccgccaacacccgctgacgcgccctgacgggcttgtctgctcccggcatccgcttacagacaagctgtgaccgtctccgggagctgcatgtgtcagaggttttcaccgtcatcaccgaaacgcgcgagacgaaagggcctcgtgatacgcctatttttataggttaatgtcatgataataatggtttcttagacgtcaggtggcacttttcggggaaatgtgcgcggaacccctatttgtttatttttctaaatacattcaaatatgtatccgctcatgagacaataaccctgataaatgcttcaataatattgaaaaaggaagagtatgagtattcaacatttccgtgtcgcccttattcccttttttgcggcattttgccttcctgtttttgctcacccagaaacgctggtgaaagtaaaagatgctgaagatcagttgggtgcacgagtgggttacatcgaactggatctcaacagcggtaagatccttgagagttttcgccccgaagaacgttttccaatgatgagcacttttaaagttctgctatgtggcgcggtattatcccgtattgacgccgggcaagagcaactcggtcgccgcatacactattctcagaatgacttggttgagtactcaccagtcacagaaaagcatcttacggatggcatgacagtaagagaattatgcagtgctgccataaccatgagtgataacactgcggccaacttacttctgacaacgatcggaggaccgaaggagctaaccgcttttttgcacaacatgggggatcatgtaactcgccttgatcgttgggaaccggagctgaatgaagccataccaaacgacgagcgtgacaccacgatgcctgtagcaatggcaacaacgttgcgcaaactattaactggcgaactacttactctagcttcccggcaacaattaatagactggatggaggcggataaagttgcaggaccacttctgcgctcggcccttccggctggctggtttattgctgataaatctggagccggtgagcgtggaagccgcggtatcattgcagcactggggccagatggtaagccctcccgtatcgtagttatctacacgacggggagtcaggcaactatggatgaacgaaatagacagatcgctgagataggtgcctcactgattaagcattggtaactgtcagaccaagtttactcatatatactttagattgatttaaaacttcatttttaatttaaaaggatctaggtgaagatcctttttgataatctcatgaccaaaatcccttaacgtgagttttcgttccactgagcgtcagaccccgtagaaaagatcaaaggatcttcttgagatcctttttttctgcgcgtaatctgctgcttgcaaacaaaaaaaccaccgctaccagcggtggtttgtttgccggatcaagagctaccaactctttttccgaaggtaactggcttcagcagagcgcagataccaaatactgttcttctagtgtagccgtagttaggccaccacttcaagaactctgtagcaccgcctacatacctcgctctgctaatcctgttaccagtggctgctgccagtggcgataagtcgtgtcttaccgggttggactcaagacgatagttaccggataaggcgcagcggtcgggctgaacggggggttcgtgcacacagcccagcttggagcgaacgacctacaccgaactgagatacctacagcgtgagctatgagaaagcgccacgcttcccgaagggagaaaggcggacaggtatccggtaagcggcagggtcggaacaggagagcgcacgagggagcttccagggggaaacgcctggtatctttatagtcctgtcgggtttcgccacctctgacttgagcgtcgatttttgtgatgctcgtcaggggggcggagcctatggaaaaacgccagcaacgcggcctttttacggttcctggccttttgctggccttttgctcacatgt

SEQ ID NO: 29 - DNA, 7334 bp, Artificial Sequence
  pGW091
cctgcaggcagctgcgcgctcgctcgctcactgaggccgcccgggcgtcgggcgacctttggtcgcccggcctcagtgagcgagcgagcgcgcagagagggagtggccaactccatcactaggggttcctgcggcctctagaaaggatctgcgatcgctccggtgcccgtcagtgggcagagcgcacatcgcccacagtccccgagaagttggggggaggggtcggcaattgaacgggtgcctagagaaggtggcgcggggtaaactgggaaagtgatgtcgtgtactggctccgcctttttcccgagggtgggggagaaccgtatataagtgcagtagtcgccgtgaacgttctttttcgcaacgggtttgccgccagaacacagctgaagcttcgaggggctcgcatctctccttcacgcgcccgccgccctacctgaggccgccatccacgccggttgagtcgcgttctgccgcctcccgcctgtggtgcctcctgaactgcgtccgccgtctaggtaagtttaaagctcaggtcgagaccgggcctttgtccggcgctcccttggagcctacctagactcagccggctctccacgctttgcctgaccctgcttgctcaactctacgtctttgtttcgttttctgttctgcgccgttacagatctggctaactaccggtgccaccatggcttgcaattgtcagttgatgcaggatacaccactcctcaagtttccatgtccaaggctcattcttctctttgtgctgctgattcgtctttcacaagtgtcttcagatgttgatgaacaactgtccaagtcagtgaaagataaggtattgctgccttgccgttacaactctcctcatgaagatgagtctgaagaccgaatctactggcaaaaacatgacaaagtggtgctgtctgtcattgttgggaaactaaaagtgtggcccgagtataagaaccggactttatatgacaacactacctactctcttatcatcctgggcctggtcctttcagaccggggcacatacagctgtgtcgttcaaaagaaggaaagaggaacgtatgaagttaaacacttggctttagtaaagttgtccatcaaagctgacttctctacccccaacataactgagtctggaaacccatctgcagacactaaaaggattacctgctttgcttccgggggtttcccaaagcctcgcttctcttggttggaaaatggaagagaattacctggcatcaatacgacaatttcccaggatcctgaatctgaattgtacaccattagtagccaactagatttcaatacgactcgcaaccacaccattaagtgtctcattaaatatggagatgctcacgtgtcagaggacttcacctgggaaaaacccccagaagaccctcctgatagcaagaacacacttgtgctctttggggcaggattcggcgcagtaataacagtcgtcgtcatcgttgtcatcatcaaatgcttctgtaagcacagaagctgtttcagaagaaatgaggcaagcagagaaacaaacaacagccttaccttcgggcctgaagaagcattagctgaacagaccgtcttccttcgtacgggcagtggagagggcagaggaagtctgctaacatgcggtgacgtcgaggagaatcctggcccaatggagagtgtggtacagccttcagtgtttgtggtggatggacagacggacatcccattcaggcggctggaacagaaccaccggagacggcgctgtggcactgtccaggtcagcctggccctggtgctgctgctaggtgctgggctggccactcagggctggtttctcctgagactgcatcaacgtcttggagacatagtagctcatctgccagatggaggcaaaggctcctgggagaagctgatacaagatcaacgatctcaccaggccaacccagcagcacatcttacaggagccaacgccagcttgataggtattggtggacctctgttatgggagacacgacttggcctggccttcttgaggggcttgacgtatcatgatggggccctggtgaccatggagcccggttactactatgtgtactccaaagtgcagctgagcggcgtgggctgcccccaggggctggccaatggcctccccatcacccatggactatacaagcgcacatcccgctacccgaaggagttagaactgctggtcagtcggcggtcaccctgtggccgggccaacagctcccgagtctggtgggacagcagcttcctgggcggcgtggtacatctggaggctggggaagaggtggtggtccgcgtgcctggaaaccgcctggtcagaccacgtgacggcaccaggtcctatttcggagctttcatggtcactagtggatccggcgcaacaaacttctctctgctgaaacaagccggagatgtcgaagagaatcctggaccgatggaggaaatgcctttgagagagtcaagtcctcaaagggcagagaggtgcaagaagtcatggctcttgtgcatagtggctctgttactgatgctgctctgttctttgggtacactgatctatacttcactcaagccaactgccatcgagtcctgcatggttaagtttgaactatcatcctcaaaatggcacatgacatctcccaaacctcactgtgtgaatacgacatctgatgggaagctgaagatactgcagagtggcacatatttaatctacggccaagtgattcctgtggataagaaatacataaaagacaatgcccccttcgtagtacagatatataaaaagaatgatgtcctacaaactctaatgaatgattttcaaatcttgcctataggaggggtttatgaactgcatgctggagataacatatatctgaagttcaactctaaagaccatattcagaaaaataacacatactgggggatcatcttaatgcctgatctaccattcatctctgctagcagcggtacccagtgcaccaactacgccctgctgaagctggccggcgatgtggagagcaaccccgggcccatggaccagcacacacttgatgtggaggataccgcggatgccagacatccagcaggtacttcgtgcccctcggatgcggcgctcctcagagataccgggctcctcgcggacgctgcgctcctctcagatactgtgcgccccacaaatgccgcgctccccacggatgctgcctaccctgcggttaatgttcgggatcgcgaggccgcgtggccgcctgcactgaacttctgttcccgccacccaaagctctatggcctagtcgctttggttttgctgcttctgatcgccgcctgtgttcctatcttcacccgcaccgagcctcggccagcgctcacaatcaccacctcgcccaacctgggtacccgagagaataatgcagaccaggtcacccctgtttcccacattggctgccccaacactacacaacagggctctcctgtgttcgccaagctactggctaaaaaccaagcatcgttgtgcaatacaactctgaactggcacagccaagatggagctgggagctcatacctatctcaaggtctgaggtacgaagaagacaaaaaggagttggtggtagacagtcccgggctctactacgtatttttggaactgaagctcagtccaacattcacaaacacaggccacaaggtgcagggctgggtctctcttgttttgcaagcaaagcctcaggtagatgactttgacaacttggccctgacagtggaactgttcccttgctccatggagaacaagttagtggaccgttcctggagtcaactgttgctcctgaaggctggccaccgcctcagtgtgggtctgagggcttatctgcatggagcccaggatgcatacagagactgggagctgtcttatcccaacaccaccagctttggactctttcttgtgaaacccgacaacccatgggaaggcatatgcggtaccgtgaagcagaccctgaacttcgatctgctgaagctggccggcgatgtggagagcaaccccgggcccatgaacgctacacactgcatcttggctttgcagctcttcctcatggctgtttctggctgttactgccacggcacagtcattgaaagcctagaaagtctgaataactattttaactcaagtggcatagatgtggaagaaaagagtctcttcttggatatctggaggaactggcaaaaggatggtgacatgaaaatcctgcagagccagattatctctttctacctcagactctttgaagtcttgaaagacaatcaggccatcagcaacaacataagcgtcattgaatcacacctgattactaccttcttcagcaacagcaaggcgaaaaaggatgcattcatgagtattgccaagtttgaggtcaacaacccacaggtccagcgccaagcattcaatgagctcatccgagtggtccaccagctgttgccggaatccagcctcaggaagcggaaaaggagtcgctgctgagaattcaataaaagatctttattttcattagatctgtgtgttggttttttgtgtgcggccgcaggaacccctagtgatggagttggccactccctctctgcgcgctcgctcgctcactgaggccgggcgaccaaaggtcgcccgacgcccgggctttgcccgggcggcctcagtgagcgagcgagcgcgcagctgcctgcaggggcgcctgatgcggtattttctccttacgcatctgtgcggtatttcacaccgcatacgtcaaagcaaccatagtacgcgccctgtagcggcgcattaagcgcggcgggtgtggtggttacgcgcagcgtgaccgctacacttgccagcgccttagcgcccgctcctttcgctttcttcccttcctttctcgccacgttcgccggctttccccgtcaagctctaaatcgggggctccctttagggttccgatttagtgctttacggcacctcgaccccaaaaaacttgatttgggtgatggttcacgtagtgggccatcgccctgatagacggtttttcgccctttgacgttggagtccacgttctttaatagtggactcttgttccaaactggaacaacactcaactctatctcgggctattcttttgatttataagggattttgccgatttcggtctattggttaaaaaatgagctgatttaacaaaaatttaacgcgaattttaacaaaatattaacgtttacaattttatggtgcactctcagtacaatctgctctgatgccgcatagttaagccagccccgacacccgccaacacccgctgacgcgccctgacgggcttgtctgctcccggcatccgcttacagacaagctgtgaccgtctccgggagctgcatgtgtcagaggttttcaccgtcatcaccgaaacgcgcgagacgaaagggcctcgtgatacgcctatttttataggttaatgtcatgataataatggtttcttagacgtcaggtggcacttttcggggaaatgtgcgcggaacccctatttgtttatttttctaaatacattcaaatatgtatccgctcatgagacaataaccctgataaatgcttcaataatattgaaaaaggaagagtatgagtattcaacatttccgtgtcgcccttattcccttttttgcggcattttgccttcctgtttttgctcacccagaaacgctggtgaaagtaaaagatgctgaagatcagttgggtgcacgagtgggttacatcgaactggatctcaacagcggtaagatccttgagagttttcgccccgaagaacgttttccaatgatgagcacttttaaagttctgctatgtggcgcggtattatcccgtattgacgccgggcaagagcaactcggtcgccgcatacactattctcagaatgacttggttgagtactcaccagtcacagaaaagcatcttacggatggcatgacagtaagagaattatgcagtgctgccataaccatgagtgataacactgcggccaacttacttctgacaacgatcggaggaccgaaggagctaaccgcttttttgcacaacatgggggatcatgtaactcgccttgatcgttgggaaccggagctgaatgaagccataccaaacgacgagcgtgacaccacgatgcctgtagcaatggcaacaacgttgcgcaaactattaactggcgaactacttactctagcttcccggcaacaattaatagactggatggaggcggataaagttgcaggaccacttctgcgctcggcccttccggctggctggtttattgctgataaatctggagccggtgagcgtggaagccgcggtatcattgcagcactggggccagatggtaagccctcccgtatcgtagttatctacacgacggggagtcaggcaactatggatgaacgaaatagacagatcgctgagataggtgcctcactgattaagcattggtaactgtcagaccaagtttactcatatatactttagattgatttaaaacttcatttttaatttaaaaggatctaggtgaagatcctttttgataatctcatgaccaaaatcccttaacgtgagttttcgttccactgagcgtcagaccccgtagaaaagatcaaaggatcttcttgagatcctttttttctgcgcgtaatctgctgcttgcaaacaaaaaaaccaccgctaccagcggtggtttgtttgccggatcaagagctaccaactctttttccgaaggtaactggcttcagcagagcgcagataccaaatactgttcttctagtgtagccgtagttaggccaccacttcaagaactctgtagcaccgcctacatacctcgctctgctaatcctgttaccagtggctgctgccagtggcgataagtcgtgtcttaccgggttggactcaagacgatagttaccggataaggcgcagcggtcgggctgaacggggggttcgtgcacacagcccagcttggagcgaacgacctacaccgaactgagatacctacagcgtgagctatgagaaagcgccacgcttcccgaagggagaaaggcggacaggtatccggtaagcggcagggtcggaacaggagagcgcacgagggagcttccagggggaaacgcctggtatctttatagtcctgtcgggtttcgccacctctgacttgagcgtcgatttttgtgatgctcgtcaggggggcggagcctatggaaaaacgccagcaacgcggcctttttacggttcctggccttttgctggccttttgctcacatgt

SEQ ID NO: 30 - DNA, 7805 bp, Artificial Sequence
  pGW096
cctgcaggcagctgcgcgctcgctcgctcactgaggccgcccgggcgtcgggcgacctttggtcgcccggcctcagtgagcgagcgagcgcgcagagagggagtggccaactccatcactaggggttcctgcggcctctagaaaggatctgcgatcgctccggtgcccgtcagtgggcagagcgcacatcgcccacagtccccgagaagttggggggaggggtcggcaattgaacgggtgcctagagaaggtggcgcggggtaaactgggaaagtgatgtcgtgtactggctccgcctttttcccgagggtgggggagaaccgtatataagtgcagtagtcgccgtgaacgttctttttcgcaacgggtttgccgccagaacacagctgaagcttcgaggggctcgcatctctccttcacgcgcccgccgccctacctgaggccgccatccacgccggttgagtcgcgttctgccgcctcccgcctgtggtgcctcctgaactgcgtccgccgtctaggtaagtttaaagctcaggtcgagaccgggcctttgtccggcgctcccttggagcctacctagactcagccggctctccacgctttgcctgaccctgcttgctcaactctacgtctttgtttcgttttctgttctgcgccgttacagatctggctaactaccggtgccaccatgaacgctacacactgcatcttggctttgcagctcttcctcatggctgtttctggctgttactgccacggcacagtcattgaaagcctagaaagtctgaataactattttaactcaagtggcatagatgtggaagaaaagagtctcttcttggatatctggaggaactggcaaaaggatggtgacatgaaaatcctgcagagccagattatctctttctacctcagactctttgaagtcttgaaagacaatcaggccatcagcaacaacataagcgtcattgaatcacacctgattactaccttcttcagcaacagcaaggcgaaaaaggatgcattcatgagtattgccaagtttgaggtcaacaacccacaggtccagcgccaagcattcaatgagctcatccgagtggtccaccagctgttgccggaatccagcctcaggaagcggaaaaggagtcgctgcggatccggcgcaacaaacttctctctgctgaaacaagccggagatgtcgaagagaatcctggaccgatggcttgcaattgtcagttgatgcaggatacaccactcctcaagtttccatgtccaaggctcattcttctctttgtgctgctgattcgtctttcacaagtgtcttcagatgttgatgaacaactgtccaagtcagtgaaagataaggtattgctgccttgccgttacaactctcctcatgaagatgagtctgaagaccgaatctactggcaaaaacatgacaaagtggtgctgtctgtcattgttgggaaactaaaagtgtggcccgagtataagaaccggactttatatgacaacactacctactctcttatcatcctgggcctggtcctttcagaccggggcacatacagctgtgtcgttcaaaagaaggaaagaggaacgtatgaagttaaacacttggctttagtaaagttgtccatcaaagctgacttctctacccccaacataactgagtctggaaacccatctgcagacactaaaaggattacctgctttgcttccgggggtttcccaaagcctcgcttctcttggttggaaaatggaagagaattacctggcatcaatacgacaatttcccaggatcctgaatctgaattgtacaccattagtagccaactagatttcaatacgactcgcaaccacaccattaagtgtctcattaaatatggagatgctcacgtgtcagaggacttcacctgggaaaaacccccagaagaccctcctgatagcaagaacacacttgtgctctttggggcaggattcggcgcagtaataacagtcgtcgtcatcgttgtcatcatcaaatgcttctgtaagcacagaagctgtttcagaagaaatgaggcaagcagagaaacaaacaacagccttaccttcgggcctgaagaagcattagctgaacagaccgtcttccttcgtacgggcagtggagagggcagaggaagtctgctaacatgcggtgacgtcgaggagaatcctggcccaatggagagtgtggtacagccttcagtgtttgtggtggatggacagacggacatcccattcaggcggctggaacagaaccaccggagacggcgctgtggcactgtccaggtcagcctggccctggtgctgctgctaggtgctgggctggccactcagggctggtttctcctgagactgcatcaacgtcttggagacatagtagctcatctgccagatggaggcaaaggctcctgggagaagctgatacaagatcaacgatctcaccaggccaacccagcagcacatcttacaggagccaacgccagcttgataggtattggtggacctctgttatgggagacacgacttggcctggccttcttgaggggcttgacgtatcatgatggggccctggtgaccatggagcccggttactactatgtgtactccaaagtgcagctgagcggcgtgggctgcccccaggggctggccaatggcctccccatcacccatggactatacaagcgcacatcccgctacccgaaggagttagaactgctggtcagtcggcggtcaccctgtggccgggccaacagctcccgagtctggtgggacagcagcttcctgggcggcgtggtacatctggaggctggggaagaggtggtggtccgcgtgcctggaaaccgcctggtcagaccacgtgacggcaccaggtcctatttcggagctttcatggtcactagtggatccggcgcaacaaacttctctctgctgaaacaagccggagatgtcgaagagaatcctggaccgatgtgtcctcagaagctaaccatctcctggtttgccatcgttttgctggtgtctccactcatggccatgtgggagctggagaaagacgtttatgttgtagaggtggactggactcccgatgcccctggagaaacagtgaacctcacctgtgacacgcctgaagaagatgacatcacctggacctcagaccagagacatggagtcataggctctggaaagaccctgaccatcactgtcaaagagtttctagatgctggccagtacacctgccacaaaggaggcgagactctgagccactcacatctgctgctccacaagaaggaaaatggaatttggtccactgaaattttaaaaaatttcaaaaacaagactttcctgaagtgtgaagcaccaaattactccggacggttcacgtgctcatggctggtgcaaagaaacatggacttgaagttcaacatcaagagcagtagcagttcccctgactctcgggcagtgacatgtggaatggcgtctctgtctgcagagaaggtcacactggaccaaagggactatgagaagtattcagtgtcctgccaggaggatgtcacctgcccaactgccgaggagaccctgcccattgaactggcgttggaagcacggcagcagaataaatatgagaactacagcaccagcttcttcatcagggacatcatcaaaccagacccgcccaagaacttgcagatgaagcctttgaagaactcacaggtggaggtcagctgggagtaccctgactcctggagcactccccattcctacttctccctcaagttctttgttcgaatccagcgcaagaaagaaaagatgaaggagacagaggaggggtgtaaccagaaaggtgcgttcctcgtagagaagacatctaccgaagtccaatgcaaaggcgggaatgtctgcgtgcaagctcaggatcgctattacaattcctcatgcagcaagtgggcatgtgttccctgcagggtccgatccgctagcagcggtacccagtgcaccaactacgccctgctgaagctggccggcgatgtggagagcaaccccgggcccatggaccagcacacacttgatgtggaggataccgcggatgccagacatccagcaggtacttcgtgcccctcggatgcggcgctcctcagagataccgggctcctcgcggacgctgcgctcctctcagatactgtgcgccccacaaatgccgcgctccccacggatgctgcctaccctgcggttaatgttcgggatcgcgaggccgcgtggccgcctgcactgaacttctgttcccgccacccaaagctctatggcctagtcgctttggttttgctgcttctgatcgccgcctgtgttcctatcttcacccgcaccgagcctcggccagcgctcacaatcaccacctcgcccaacctgggtacccgagagaataatgcagaccaggtcacccctgtttcccacattggctgccccaacactacacaacagggctctcctgtgttcgccaagctactggctaaaaaccaagcatcgttgtgcaatacaactctgaactggcacagccaagatggagctgggagctcatacctatctcaaggtctgaggtacgaagaagacaaaaaggagttggtggtagacagtcccgggctctactacgtatttttggaactgaagctcagtccaacattcacaaacacaggccacaaggtgcagggctgggtctctcttgttttgcaagcaaagcctcaggtagatgactttgacaacttggccctgacagtggaactgttcccttgctccatggagaacaagttagtggaccgttcctggagtcaactgttgctcctgaaggctggccaccgcctcagtgtgggtctgagggcttatctgcatggagcccaggatgcatacagagactgggagctgtcttatcccaacaccaccagctttggactctttcttgtgaaacccgacaacccatgggaatgagaattcaataaaagatctttattttcattagatctgtgtgttggttttttgtgtgcggccgcaggaacccctagtgatggagttggccactccctctctgcgcgctcgctcgctcactgaggccgggcgaccaaaggtcgcccgacgcccgggctttgcccgggcggcctcagtgagcgagcgagcgcgcagctgcctgcaggggcgcctgatgcggtattttctccttacgcatctgtgcggtatttcacaccgcatacgtcaaagcaaccatagtacgcgccctgtagcggcgcattaagcgcggcgggtgtggtggttacgcgcagcgtgaccgctacacttgccagcgccttagcgcccgctcctttcgctttcttcccttcctttctcgccacgttcgccggctttccccgtcaagctctaaatcgggggctccctttagggttccgatttagtgctttacggcacctcgaccccaaaaaacttgatttgggtgatggttcacgtagtgggccatcgccctgatagacggtttttcgccctttgacgttggagtccacgttctttaatagtggactcttgttccaaactggaacaacactcaactctatctcgggctattcttttgatttataagggattttgccgatttcggtctattggttaaaaaatgagctgatttaacaaaaatttaacgcgaattttaacaaaatattaacgtttacaattttatggtgcactctcagtacaatctgctctgatgccgcatagttaagccagccccgacacccgccaacacccgctgacgcgccctgacgggcttgtctgctcccggcatccgcttacagacaagctgtgaccgtctccgggagctgcatgtgtcagaggttttcaccgtcatcaccgaaacgcgcgagacgaaagggcctcgtgatacgcctatttttataggttaatgtcatgataataatggtttcttagacgtcaggtggcacttttcggggaaatgtgcgcggaacccctatttgtttatttttctaaatacattcaaatatgtatccgctcatgagacaataaccctgataaatgcttcaataatattgaaaaaggaagagtatgagtattcaacatttccgtgtcgcccttattcccttttttgcggcattttgccttcctgtttttgctcacccagaaacgctggtgaaagtaaaagatgctgaagatcagttgggtgcacgagtgggttacatcgaactggatctcaacagcggtaagatccttgagagttttcgccccgaagaacgttttccaatgatgagcacttttaaagttctgctatgtggcgcggtattatcccgtattgacgccgggcaagagcaactcggtcgccgcatacactattctcagaatgacttggttgagtactcaccagtcacagaaaagcatcttacggatggcatgacagtaagagaattatgcagtgctgccataaccatgagtgataacactgcggccaacttacttctgacaacgatcggaggaccgaaggagctaaccgcttttttgcacaacatgggggatcatgtaactcgccttgatcgttgggaaccggagctgaatgaagccataccaaacgacgagcgtgacaccacgatgcctgtagcaatggcaacaacgttgcgcaaactattaactggcgaactacttactctagcttcccggcaacaattaatagactggatggaggcggataaagttgcaggaccacttctgcgctcggcccttccggctggctggtttattgctgataaatctggagccggtgagcgtggaagccgcggtatcattgcagcactggggccagatggtaagccctcccgtatcgtagttatctacacgacggggagtcaggcaactatggatgaacgaaatagacagatcgctgagataggtgcctcactgattaagcattggtaactgtcagaccaagtttactcatatatactttagattgatttaaaacttcatttttaatttaaaaggatctaggtgaagatcctttttgataatctcatgaccaaaatcccttaacgtgagttttcgttccactgagcgtcagaccccgtagaaaagatcaaaggatcttcttgagatcctttttttctgcgcgtaatctgctgcttgcaaacaaaaaaaccaccgctaccagcggtggtttgtttgccggatcaagagctaccaactctttttccgaaggtaactggcttcagcagagcgcagataccaaatactgttcttctagtgtagccgtagttaggccaccacttcaagaactctgtagcaccgcctacatacctcgctctgctaatcctgttaccagtggctgctgccagtggcgataagtcgtgtcttaccgggttggactcaagacgatagttaccggataaggcgcagcggtcgggctgaacggggggttcgtgcacacagcccagcttggagcgaacgacctacaccgaactgagatacctacagcgtgagctatgagaaagcgccacgcttcccgaagggagaaaggcggacaggtatccggtaagcggcagggtcggaacaggagagcgcacgagggagcttccagggggaaacgcctggtatctttatagtcctgtcgggtttcgccacctctgacttgagcgtcgatttttgtgatgctcgtcaggggggcggagcctatggaaaaacgccagcaacgcggcctttttacggttcctggccttttgctggccttttgctcacatgt

SEQ ID NO: 31 - DNA, 4495 bp, Artificial Sequence
  pGW097
cctgcaggcagctgcgcgctcgctcgctcactgaggccgcccgggcgtcgggcgacctttggtcgcccggcctcagtgagcgagcgagcgcgcagagagggagtggccaactccatcactaggggttcctgcggcctctagaaaggatctgcgatcgctccggtgcccgtcagtgggcagagcgcacatcgcccacagtccccgagaagttggggggaggggtcggcaattgaacgggtgcctagagaaggtggcgcggggtaaactgggaaagtgatgtcgtgtactggctccgcctttttcccgagggtgggggagaaccgtatataagtgcagtagtcgccgtgaacgttctttttcgcaacgggtttgccgccagaacacagctgaagcttcgaggggctcgcatctctccttcacgcgcccgccgccctacctgaggccgccatccacgccggttgagtcgcgttctgccgcctcccgcctgtggtgcctcctgaactgcgtccgccgtctaggtaagtttaaagctcaggtcgagaccgggcctttgtccggcgctcccttggagcctacctagactcagccggctctccacgctttgcctgaccctgcttgctcaactctacgtctttgtttcgttttctgttctgcgccgttacagatctggctaactaccggtgccacatgtgtcctcagaagctaaccatctcctggtttgccatcgttttgctggtgtctccactcatggccatgtgggagctggagaaagacgtttatgttgtagaggtggactggactcccgatgcccctggagaaacagtgaacctcacctgtgacacgcctgaagaagatgacatcacctggacctcagaccagagacatggagtcataggctctggaaagaccctgaccatcactgtcaaagagtttctagatgctggccagtacacctgccacaaaggaggcgagactctgagccactcacatctgctgctccacaagaaggaaaatggaatttggtccactgaaattttaaaaaatttcaaaaacaagactttcctgaagtgtgaagcaccaaattactccggacggttcacgtgctcatggctggtgcaaagaaacatggacttgaagttcaacatcaagagcagtagcagttcccctgactctcgggcagtgacatgtggaatggcgtctctgtctgcagagaaggtcacactggaccaaagggactatgagaagtattcagtgtcctgccaggaggatgtcacctgcccaactgccgaggagaccctgcccattgaactggcgttggaagcacggcagcagaataaatatgagaactacagcaccagcttcttcatcagggacatcatcaaaccagacccgcccaagaacttgcagatgaagcctttgaagaactcacaggtggaggtcagctgggagtaccctgactcctggagcactccccattcctacttctccctcaagttctttgttcgaatccagcgcaagaaagaaaagatgaaggagacagaggaggggtgtaaccagaaaggtgcgttcctcgtagagaagacatctaccgaagtccaatgcaaaggcgggaatgtctgcgtgcaagctcaggatcgctattacaattcctcatgcagcaagtgggcatgtgttccctgcagggtccgatcctaggaattcaataaaagatctttattttcattagatctgtgtgttggttttttgtgtgcggccgcaggaacccctagtgatggagttggccactccctctctgcgcgctcgctcgctcactgaggccgggcgaccaaaggtcgcccgacgcccgggctttgcccgggcggcctcagtgagcgagcgagcgcgcagctgcctgcaggggcgcctgatgcggtattttctccttacgcatctgtgcggtatttcacaccgcatacgtcaaagcaaccatagtacgcgccctgtagcggcgcattaagcgcggcgggtgtggtggttacgcgcagcgtgaccgctacacttgccagcgccttagcgcccgctcctttcgctttcttcccttcctttctcgccacgttcgccggctttccccgtcaagctctaaatcgggggctccctttagggttccgatttagtgctttacggcacctcgaccccaaaaaacttgatttgggtgatggttcacgtagtgggccatcgccctgatagacggtttttcgccctttgacgttggagtccacgttctttaatagtggactcttgttccaaactggaacaacactcaactctatctcgggctattcttttgatttataagggattttgccgatttcggtctattggttaaaaaatgagctgatttaacaaaaatttaacgcgaattttaacaaaatattaacgtttacaattttatggtgcactctcagtacaatctgctctgatgccgcatagttaagccagccccgacacccgccaacacccgctgacgcgccctgacgggcttgtctgctcccggcatccgcttacagacaagctgtgaccgtctccgggagctgcatgtgtcagaggttttcaccgtcatcaccgaaacgcgcgagacgaaagggcctcgtgatacgcctatttttataggttaatgtcatgataataatggtttcttagacgtcaggtggcacttttcggggaaatgtgcgcggaacccctatttgtttatttttctaaatacattcaaatatgtatccgctcatgagacaataaccctgataaatgcttcaataatattgaaaaaggaagagtatgagtattcaacatttccgtgtcgcccttattcccttttttgcggcattttgccttcctgtttttgctcacccagaaacgctggtgaaagtaaaagatgctgaagatcagttgggtgcacgagtgggttacatcgaactggatctcaacagcggtaagatccttgagagttttcgccccgaagaacgttttccaatgatgagcacttttaaagttctgctatgtggcgcggtattatcccgtattgacgccgggcaagagcaactcggtcgccgcatacactattctcagaatgacttggttgagtactcaccagtcacagaaaagcatcttacggatggcatgacagtaagagaattatgcagtgctgccataaccatgagtgataacactgcggccaacttacttctgacaacgatcggaggaccgaaggagctaaccgcttttttgcacaacatgggggatcatgtaactcgccttgatcgttgggaaccggagctgaatgaagccataccaaacgacgagcgtgacaccacgatgcctgtagcaatggcaacaacgttgcgcaaactattaactggcgaactacttactctagcttcccggcaacaattaatagactggatggaggcggataaagttgcaggaccacttctgcgctcggcccttccggctggctggtttattgctgataaatctggagccggtgagcgtggaagccgcggtatcattgcagcactggggccagatggtaagccctcccgtatcgtagttatctacacgacggggagtcaggcaactatggatgaacgaaatagacagatcgctgagataggtgcctcactgattaagcattggtaactgtcagaccaagtttactcatatatactttagattgatttaaaacttcatttttaatttaaaaggatctaggtgaagatcctttttgataatctcatgaccaaaatcccttaacgtgagttttcgttccactgagcgtcagaccccgtagaaaagatcaaaggatcttcttgagatcctttttttctgcgcgtaatctgctgcttgcaaacaaaaaaaccaccgctaccagcggtggtttgtttgccggatcaagagctaccaactctttttccgaaggtaactggcttcagcagagcgcagataccaaatactgttcttctagtgtagccgtagttaggccaccacttcaagaactctgtagcaccgcctacatacctcgctctgctaatcctgttaccagtggctgctgccagtggcgataagtcgtgtcttaccgggttggactcaagacgatagttaccggataaggcgcagcggtcgggctgaacggggggttcgtgcacacagcccagcttggagcgaacgacctacaccgaactgagatacctacagcgtgagctatgagaaagcgccacgcttcccgaagggagaaaggcggacaggtatccggtaagcggcagggtcggaacaggagagcgcacgagggagcttccagggggaaacgcctggtatctttatagtcctgtcgggtttcgccacctctgacttgagcgtcgatttttgtgatgctcgtcaggggggcggagcctatggaaaaacgccagcaacgcggcctttttacggttcctggccttttgctggccttttgctcacatgt

SEQ ID NO: 32 - DNA, 6803 bp, Artificial Sequence
  pGW098
cctgcaggcagctgcgcgctcgctcgctcactgaggccgcccgggcgtcgggcgacctttggtcgcccggcctcagtgagcgagcgagcgcgcagagagggagtggccaactccatcactaggggttcctgcggcctctagaaaggatctgcgatcgctccggtgcccgtcagtgggcagagcgcacatcgcccacagtccccgagaagttggggggaggggtcggcaattgaacgggtgcctagagaaggtggcgcggggtaaactgggaaagtgatgtcgtgtactggctccgcctttttcccgagggtgggggagaaccgtatataagtgcagtagtcgccgtgaacgttctttttcgcaacgggtttgccgccagaacacagctgaagcttcgaggggctcgcatctctccttcacgcgcccgccgccctacctgaggccgccatccacgccggttgagtcgcgttctgccgcctcccgcctgtggtgcctcctgaactgcgtccgccgtctaggtaagtttaaagctcaggtcgagaccgggcctttgtccggcgctcccttggagcctacctagactcagccggctctccacgctttgcctgaccctgcttgctcaactctacgtctttgtttcgttttctgttctgcgccgttacagatctggctaactaccggtgccaccatgaacgctacacactgcatcttggctttgcagctcttcctcatggctgtttctggctgttactgccacggcacagtcattgaaagcctagaaagtctgaataactattttaactcaagtggcatagatgtggaagaaaagagtctcttcttggatatctggaggaactggcaaaaggatggtgacatgaaaatcctgcagagccagattatctctttctacctcagactctttgaagtcttgaaagacaatcaggccatcagcaacaacataagcgtcattgaatcacacctgattactaccttcttcagcaacagcaaggcgaaaaaggatgcattcatgagtattgccaagtttgaggtcaacaacccacaggtccagcgccaagcattcaatgagctcatccgagtggtccaccagctgttgccggaatccagcctcaggaagcggaaaaggagtcgctgcggatccggcgcaacaaacttctctctgctgaaacaagccggagatgtcgaagagaatcctggaccgatggcttgcaattgtcagttgatgcaggatacaccactcctcaagtttccatgtccaaggctcattcttctctttgtgctgctgattcgtctttcacaagtgtcttcagatgttgatgaacaactgtccaagtcagtgaaagataaggtattgctgccttgccgttacaactctcctcatgaagatgagtctgaagaccgaatctactggcaaaaacatgacaaagtggtgctgtctgtcattgttgggaaactaaaagtgtggcccgagtataagaaccggactttatatgacaacactacctactctcttatcatcctgggcctggtcctttcagaccggggcacatacagctgtgtcgttcaaaagaaggaaagaggaacgtatgaagttaaacacttggctttagtaaagttgtccatcaaagctgacttctctacccccaacataactgagtctggaaacccatctgcagacactaaaaggattacctgctttgcttccgggggtttcccaaagcctcgcttctcttggttggaaaatggaagagaattacctggcatcaatacgacaatttcccaggatcctgaatctgaattgtacaccattagtagccaactagatttcaatacgactcgcaaccacaccattaagtgtctcattaaatatggagatgctcacgtgtcagaggacttcacctgggaaaaacccccagaagaccctcctgatagcaagaacacacttgtgctctttggggcaggattcggcgcagtaataacagtcgtcgtcatcgttgtcatcatcaaatgcttctgtaagcacagaagctgtttcagaagaaatgaggcaagcagagaaacaaacaacagccttaccttcgggcctgaagaagcattagctgaacagaccgtcttccttcgtacgggcagtggagagggcagaggaagtctgctaacatgcggtgacgtcgaggagaatcctggcccaatggagagtgtggtacagccttcagtgtttgtggtggatggacagacggacatcccattcaggcggctggaacagaaccaccggagacggcgctgtggcactgtccaggtcagcctggccctggtgctgctgctaggtgctgggctggccactcagggctggtttctcctgagactgcatcaacgtcttggagacatagtagctcatctgccagatggaggcaaaggctcctgggagaagctgatacaagatcaacgatctcaccaggccaacccagcagcacatcttacaggagccaacgccagcttgataggtattggtggacctctgttatgggagacacgacttggcctggccttcttgaggggcttgacgtatcatgatggggccctggtgaccatggagcccggttactactatgtgtactccaaagtgcagctgagcggcgtgggctgcccccaggggctggccaatggcctccccatcacccatggactatacaagcgcacatcccgctacccgaaggagttagaactgctggtcagtcggcggtcaccctgtggccgggccaacagctcccgagtctggtgggacagcagcttcctgggcggcgtggtacatctggaggctggggaagaggtggtggtccgcgtgcctggaaaccgcctggtcagaccacgtgacggcaccaggtcctatttcggagctttcatggtcactagtggatccggcgcaacaaacttctctctgctgaaacaagccggagatgtcgaagagaatcctggaccgatgtgtcctcagaagctaaccatctcctggtttgccatcgttttgctggtgtctccactcatggccatgtgggagctggagaaagacgtttatgttgtagaggtggactggactcccgatgcccctggagaaacagtgaacctcacctgtgacacgcctgaagaagatgacatcacctggacctcagaccagagacatggagtcataggctctggaaagaccctgaccatcactgtcaaagagtttctagatgctggccagtacacctgccacaaaggaggcgagactctgagccactcacatctgctgctccacaagaaggaaaatggaatttggtccactgaaattttaaaaaatttcaaaaacaagactttcctgaagtgtgaagcaccaaattactccggacggttcacgtgctcatggctggtgcaaagaaacatggacttgaagttcaacatcaagagcagtagcagttcccctgactctcgggcagtgacatgtggaatggcgtctctgtctgcagagaaggtcacactggaccaaagggactatgagaagtattcagtgtcctgccaggaggatgtcacctgcccaactgccgaggagaccctgcccattgaactggcgttggaagcacggcagcagaataaatatgagaactacagcaccagcttcttcatcagggacatcatcaaaccagacccgcccaagaacttgcagatgaagcctttgaagaactcacaggtggaggtcagctgggagtaccctgactcctggagcactccccattcctacttctccctcaagttctttgttcgaatccagcgcaagaaagaaaagatgaaggagacagaggaggggtgtaaccagaaaggtgcgttcctcgtagagaagacatctaccgaagtccaatgcaaaggcgggaatgtctgcgtgcaagctcaggatcgctattacaattcctcatgcagcaagtgggcatgtgttccctgcagggtccgatcctgagaattcaataaaagatctttattttcattagatctgtgtgttggttttttgtgtgcggccgcaggaacccctagtgatggagttggccactccctctctgcgcgctcgctcgctcactgaggccgggcgaccaaaggtcgcccgacgcccgggctttgcccgggcggcctcagtgagcgagcgagcgcgcagctgcctgcaggggcgcctgatgcggtattttctccttacgcatctgtgcggtatttcacaccgcatacgtcaaagcaaccatagtacgcgccctgtagcggcgcattaagcgcggcgggtgtggtggttacgcgcagcgtgaccgctacacttgccagcgccttagcgcccgctcctttcgctttcttcccttcctttctcgccacgttcgccggctttccccgtcaagctctaaatcgggggctccctttagggttccgatttagtgctttacggcacctcgaccccaaaaaacttgatttgggtgatggttcacgtagtgggccatcgccctgatagacggtttttcgccctttgacgttggagtccacgttctttaatagtggactcttgttccaaactggaacaacactcaactctatctcgggctattcttttgatttataagggattttgccgatttcggtctattggttaaaaaatgagctgatttaacaaaaatttaacgcgaattttaacaaaatattaacgtttacaattttatggtgcactctcagtacaatctgctctgatgccgcatagttaagccagccccgacacccgccaacacccgctgacgcgccctgacgggcttgtctgctcccggcatccgcttacagacaagctgtgaccgtctccgggagctgcatgtgtcagaggttttcaccgtcatcaccgaaacgcgcgagacgaaagggcctcgtgatacgcctatttttataggttaatgtcatgataataatggtttcttagacgtcaggtggcacttttcggggaaatgtgcgcggaacccctatttgtttatttttctaaatacattcaaatatgtatccgctcatgagacaataaccctgataaatgcttcaataatattgaaaaaggaagagtatgagtattcaacatttccgtgtcgcccttattcccttttttgcggcattttgccttcctgtttttgctcacccagaaacgctggtgaaagtaaaagatgctgaagatcagttgggtgcacgagtgggttacatcgaactggatctcaacagcggtaagatccttgagagttttcgccccgaagaacgttttccaatgatgagcacttttaaagttctgctatgtggcgcggtattatcccgtattgacgccgggcaagagcaactcggtcgccgcatacactattctcagaatgacttggttgagtactcaccagtcacagaaaagcatcttacggatggcatgacagtaagagaattatgcagtgctgccataaccatgagtgataacactgcggccaacttacttctgacaacgatcggaggaccgaaggagctaaccgcttttttgcacaacatgggggatcatgtaactcgccttgatcgttgggaaccggagctgaatgaagccataccaaacgacgagcgtgacaccacgatgcctgtagcaatggcaacaacgttgcgcaaactattaactggcgaactacttactctagcttcccggcaacaattaatagactggatggaggcggataaagttgcaggaccacttctgcgctcggcccttccggctggctggtttattgctgataaatctggagccggtgagcgtggaagccgcggtatcattgcagcactggggccagatggtaagccctcccgtatcgtagttatctacacgacggggagtcaggcaactatggatgaacgaaatagacagatcgctgagataggtgcctcactgattaagcattggtaactgtcagaccaagtttactcatatatactttagattgatttaaaacttcatttttaatttaaaaggatctaggtgaagatcctttttgataatctcatgaccaaaatcccttaacgtgagttttcgttccactgagcgtcagaccccgtagaaaagatcaaaggatcttcttgagatcctttttttctgcgcgtaatctgctgcttgcaaacaaaaaaaccaccgctaccagcggtggtttgtttgccggatcaagagctaccaactctttttccgaaggtaactggcttcagcagagcgcagataccaaatactgttcttctagtgtagccgtagttaggccaccacttcaagaactctgtagcaccgcctacatacctcgctctgctaatcctgttaccagtggctgctgccagtggcgataagtcgtgtcttaccgggttggactcaagacgatagttaccggataaggcgcagcggtcgggctgaacggggggttcgtgcacacagcccagcttggagcgaacgacctacaccgaactgagatacctacagcgtgagctatgagaaagcgccacgcttcccgaagggagaaaggcggacaggtatccggtaagcggcagggtcggaacaggagagcgcacgagggagcttccagggggaaacgcctggtatctttatagtcctgtcgggtttcgccacctctgacttgagcgtcgatttttgtgatgctcgtcaggggggcggagcctatggaaaaacgccagcaacgcggcctttttacggttcctggccttttgctggccttttgctcacatgt

SEQ ID NO: 33 - DNA, 6092 bp, Artificial Sequence
  pGW099
cctgcaggcagctgcgcgctcgctcgctcactgaggccgcccgggcgtcgggcgacctttggtcgcccggcctcagtgagcgagcgagcgcgcagagagggagtggccaactccatcactaggggttcctgcggcctctagaaaggatctgcgatcgctccggtgcccgtcagtgggcagagcgcacatcgcccacagtccccgagaagttggggggaggggtcggcaattgaacgggtgcctagagaaggtggcgcggggtaaactgggaaagtgatgtcgtgtactggctccgcctttttcccgagggtgggggagaaccgtatataagtgcagtagtcgccgtgaacgttctttttcgcaacgggtttgccgccagaacacagctgaagcttcgaggggctcgcatctctccttcacgcgcccgccgccctacctgaggccgccatccacgccggttgagtcgcgttctgccgcctcccgcctgtggtgcctcctgaactgcgtccgccgtctaggtaagtttaaagctcaggtcgagaccgggcctttgtccggcgctcccttggagcctacctagactcagccggctctccacgctttgcctgaccctgcttgctcaactctacgtctttgtttcgttttctgttctgcgccgttacagatctggctaactaccggtgccaccatgaacgctacacactgcatcttggctttgcagctcttcctcatggctgtttctggctgttactgccacggcacagtcattgaaagcctagaaagtctgaataactattttaactcaagtggcatagatgtggaagaaaagagtctcttcttggatatctggaggaactggcaaaaggatggtgacatgaaaatcctgcagagccagattatctctttctacctcagactctttgaagtcttgaaagacaatcaggccatcagcaacaacataagcgtcattgaatcacacctgattactaccttcttcagcaacagcaaggcgaaaaaggatgcattcatgagtattgccaagtttgaggtcaacaacccacaggtccagcgccaagcattcaatgagctcatccgagtggtccaccagctgttgccggaatccagcctcaggaagcggaaaaggagtcgctgcggatccggcgcaacaaacttctctctgctgaaacaagccggagatgtcgaagagaatcctggaccgatggcttgcaattgtcagttgatgcaggatacaccactcctcaagtttccatgtccaaggctcattcttctctttgtgctgctgattcgtctttcacaagtgtcttcagatgttgatgaacaactgtccaagtcagtgaaagataaggtattgctgccttgccgttacaactctcctcatgaagatgagtctgaagaccgaatctactggcaaaaacatgacaaagtggtgctgtctgtcattgttgggaaactaaaagtgtggcccgagtataagaaccggactttatatgacaacactacctactctcttatcatcctgggcctggtcctttcagaccggggcacatacagctgtgtcgttcaaaagaaggaaagaggaacgtatgaagttaaacacttggctttagtaaagttgtccatcaaagctgacttctctacccccaacataactgagtctggaaacccatctgcagacactaaaaggattacctgctttgcttccgggggtttcccaaagcctcgcttctcttggttggaaaatggaagagaattacctggcatcaatacgacaatttcccaggatcctgaatctgaattgtacaccattagtagccaactagatttcaatacgactcgcaaccacaccattaagtgtctcattaaatatggagatgctcacgtgtcagaggacttcacctgggaaaaacccccagaagaccctcctgatagcaagaacacacttgtgctctttggggcaggattcggcgcagtaataacagtcgtcgtcatcgttgtcatcatcaaatgcttctgtaagcacagaagctgtttcagaagaaatgaggcaagcagagaaacaaacaacagccttaccttcgggcctgaagaagcattagctgaacagaccgtcttccttcgtacgggcagtggagagggcagaggaagtctgctaacatgcggtgacgtcgaggagaatcctggcccaatggagagtgtggtacagccttcagtgtttgtggtggatggacagacggacatcccattcaggcggctggaacagaaccaccggagacggcgctgtggcactgtccaggtcagcctggccctggtgctgctgctaggtgctgggctggccactcagggctggtttctcctgagactgcatcaacgtcttggagacatagtagctcatctgccagatggaggcaaaggctcctgggagaagctgatacaagatcaacgatctcaccaggccaacccagcagcacatcttacaggagccaacgccagcttgataggtattggtggacctctgttatgggagacacgacttggcctggccttcttgaggggcttgacgtatcatgatggggccctggtgaccatggagcccggttactactatgtgtactccaaagtgcagctgagcggcgtgggctgcccccaggggctggccaatggcctccccatcacccatggactatacaagcgcacatcccgctacccgaaggagttagaactgctggtcagtcggcggtcaccctgtggccgggccaacagctcccgagtctggtgggacagcagcttcctgggcggcgtggtacatctggaggctggggaagaggtggtggtccgcgtgcctggaaaccgcctggtcagaccacgtgacggcaccaggtcctatttcggagctttcatggtcactagtggatccggcgcaacaaacttctctctgctgaaacaagccggagatgtcgaagagaatcctggaccgatgaacccaagtgctgccgtcattttctgcctcatcctgctgggtctgagtgggactcaagggatccctctcgcaaggacggtccgctgcaactgcatccatatcgatgacgggccagtgagaatgagggccatagggaagcttgaaatcatccctgcgagcctatcctgcccacgtgttgagatcattgccacgatgaaaaagaatgatgagcagagatgtctgaatccggaatctaagaccatcaagaatttaatgaaagcgtttagccaaaaaaggtctaaaagggctccttgagaattcaataaaagatctttattttcattagatctgtgtgttggttttttgtgtgcggccgcaggaacccctagtgatggagttggccactccctctctgcgcgctcgctcgctcactgaggccgggcgaccaaaggtcgcccgacgcccgggctttgcccgggcggcctcagtgagcgagcgagcgcgcagctgcctgcaggggcgcctgatgcggtattttctccttacgcatctgtgcggtatttcacaccgcatacgtcaaagcaaccatagtacgcgccctgtagcggcgcattaagcgcggcgggtgtggtggttacgcgcagcgtgaccgctacacttgccagcgccttagcgcccgctcctttcgctttcttcccttcctttctcgccacgttcgccggctttccccgtcaagctctaaatcgggggctccctttagggttccgatttagtgctttacggcacctcgaccccaaaaaacttgatttgggtgatggttcacgtagtgggccatcgccctgatagacggtttttcgccctttgacgttggagtccacgttctttaatagtggactcttgttccaaactggaacaacactcaactctatctcgggctattcttttgatttataagggattttgccgatttcggtctattggttaaaaaatgagctgatttaacaaaaatttaacgcgaattttaacaaaatattaacgtttacaattttatggtgcactctcagtacaatctgctctgatgccgcatagttaagccagccccgacacccgccaacacccgctgacgcgccctgacgggcttgtctgctcccggcatccgcttacagacaagctgtgaccgtctccgggagctgcatgtgtcagaggttttcaccgtcatcaccgaaacgcgcgagacgaaagggcctcgtgatacgcctatttttataggttaatgtcatgataataatggtttcttagacgtcaggtggcacttttcggggaaatgtgcgcggaacccctatttgtttatttttctaaatacattcaaatatgtatccgctcatgagacaataaccctgataaatgcttcaataatattgaaaaaggaagagtatgagtattcaacatttccgtgtcgcccttattcccttttttgcggcattttgccttcctgtttttgctcacccagaaacgctggtgaaagtaaaagatgctgaagatcagttgggtgcacgagtgggttacatcgaactggatctcaacagcggtaagatccttgagagttttcgccccgaagaacgttttccaatgatgagcacttttaaagttctgctatgtggcgcggtattatcccgtattgacgccgggcaagagcaactcggtcgccgcatacactattctcagaatgacttggttgagtactcaccagtcacagaaaagcatcttacggatggcatgacagtaagagaattatgcagtgctgccataaccatgagtgataacactgcggccaacttacttctgacaacgatcggaggaccgaaggagctaaccgcttttttgcacaacatgggggatcatgtaactcgccttgatcgttgggaaccggagctgaatgaagccataccaaacgacgagcgtgacaccacgatgcctgtagcaatggcaacaacgttgcgcaaactattaactggcgaactacttactctagcttcccggcaacaattaatagactggatggaggcggataaagttgcaggaccacttctgcgctcggcccttccggctggctggtttattgctgataaatctggagccggtgagcgtggaagccgcggtatcattgcagcactggggccagatggtaagccctcccgtatcgtagttatctacacgacggggagtcaggcaactatggatgaacgaaatagacagatcgctgagataggtgcctcactgattaagcattggtaactgtcagaccaagtttactcatatatactttagattgatttaaaacttcatttttaatttaaaaggatctaggtgaagatcctttttgataatctcatgaccaaaatcccttaacgtgagttttcgttccactgagcgtcagaccccgtagaaaagatcaaaggatcttcttgagatcctttttttctgcgcgtaatctgctgcttgcaaacaaaaaaaccaccgctaccagcggtggtttgtttgccggatcaagagctaccaactctttttccgaaggtaactggcttcagcagagcgcagataccaaatactgttcttctagtgtagccgtagttaggccaccacttcaagaactctgtagcaccgcctacatacctcgctctgctaatcctgttaccagtggctgctgccagtggcgataagtcgtgtcttaccgggttggactcaagacgatagttaccggataaggcgcagcggtcgggctgaacggggggttcgtgcacacagcccagcttggagcgaacgacctacaccgaactgagatacctacagcgtgagctatgagaaagcgccacgcttcccgaagggagaaaggcggacaggtatccggtaagcggcagggtcggaacaggagagcgcacgagggagcttccagggggaaacgcctggtatctttatagtcctgtcgggtttcgccacctctgacttgagcgtcgatttttgtgatgctcgtcaggggggcggagcctatggaaaaacgccagcaacgcggcctttttacggttcctggccttttgctggccttttgctcacatgt

SEQ ID NO: 34 - DNA, 7094 bp, Artificial Sequence
  pGW100
cctgcaggcagctgcgcgctcgctcgctcactgaggccgcccgggcgtcgggcgacctttggtcgcccggcctcagtgagcgagcgagcgcgcagagagggagtggccaactccatcactaggggttcctgcggcctctagaaaggatctgcgatcgctccggtgcccgtcagtgggcagagcgcacatcgcccacagtccccgagaagttggggggaggggtcggcaattgaacgggtgcctagagaaggtggcgcggggtaaactgggaaagtgatgtcgtgtactggctccgcctttttcccgagggtgggggagaaccgtatataagtgcagtagtcgccgtgaacgttctttttcgcaacgggtttgccgccagaacacagctgaagcttcgaggggctcgcatctctccttcacgcgcccgccgccctacctgaggccgccatccacgccggttgagtcgcgttctgccgcctcccgcctgtggtgcctcctgaactgcgtccgccgtctaggtaagtttaaagctcaggtcgagaccgggcctttgtccggcgctcccttggagcctacctagactcagccggctctccacgctttgcctgaccctgcttgctcaactctacgtctttgtttcgttttctgttctgcgccgttacagatctggctaactaccggtgccaccatgaacgctacacactgcatcttggctttgcagctcttcctcatggctgtttctggctgttactgccacggcacagtcattgaaagcctagaaagtctgaataactattttaactcaagtggcatagatgtggaagaaaagagtctcttcttggatatctggaggaactggcaaaaggatggtgacatgaaaatcctgcagagccagattatctctttctacctcagactctttgaagtcttgaaagacaatcaggccatcagcaacaacataagcgtcattgaatcacacctgattactaccttcttcagcaacagcaaggcgaaaaaggatgcattcatgagtattgccaagtttgaggtcaacaacccacaggtccagcgccaagcattcaatgagctcatccgagtggtccaccagctgttgccggaatccagcctcaggaagcggaaaaggagtcgctgcggatccggcgcaacaaacttctctctgctgaaacaagccggagatgtcgaagagaatcctggaccgatggcttgcaattgtcagttgatgcaggatacaccactcctcaagtttccatgtccaaggctcattcttctctttgtgctgctgattcgtctttcacaagtgtcttcagatgttgatgaacaactgtccaagtcagtgaaagataaggtattgctgccttgccgttacaactctcctcatgaagatgagtctgaagaccgaatctactggcaaaaacatgacaaagtggtgctgtctgtcattgttgggaaactaaaagtgtggcccgagtataagaaccggactttatatgacaacactacctactctcttatcatcctgggcctggtcctttcagaccggggcacatacagctgtgtcgttcaaaagaaggaaagaggaacgtatgaagttaaacacttggctttagtaaagttgtccatcaaagctgacttctctacccccaacataactgagtctggaaacccatctgcagacactaaaaggattacctgctttgcttccgggggtttcccaaagcctcgcttctcttggttggaaaatggaagagaattacctggcatcaatacgacaatttcccaggatcctgaatctgaattgtacaccattagtagccaactagatttcaatacgactcgcaaccacaccattaagtgtctcattaaatatggagatgctcacgtgtcagaggacttcacctgggaaaaacccccagaagaccctcctgatagcaagaacacacttgtgctctttggggcaggattcggcgcagtaataacagtcgtcgtcatcgttgtcatcatcaaatgcttctgtaagcacagaagctgtttcagaagaaatgaggcaagcagagaaacaaacaacagccttaccttcgggcctgaagaagcattagctgaacagaccgtcttccttcgtacgggcagtggagagggcagaggaagtctgctaacatgcggtgacgtcgaggagaatcctggcccaatggagagtgtggtacagccttcagtgtttgtggtggatggacagacggacatcccattcaggcggctggaacagaaccaccggagacggcgctgtggcactgtccaggtcagcctggccctggtgctgctgctaagtgctgggctggccactcagggctggtttctcctgagactgcatcaacgtcttggagacatagtagctcatctgccagatggaggcaaaggctcctgggagaagctgatacaagatcaacgatctcaccaggccaacccagcagcacatcttacaggagccaacgccagcttgataggtattggtggacctctgttatgggagacacgacttggcctggccttcttgaggggcttgacgtatcatgatggggccctggtgaccatggagcccggttactactatgtgtactccaaagtgcagctgagcggcgtgggctgcccccaggggctggccaatggcctccccatcacccatggactatacaagcgcacatcccgctacccgaaggagttagaactgctggtcagtcggcggtcaccctgtggccgggccaacagctcccgagtctggtgggacagcagcttcctgggcggcgtggtacatctggaggctggggaagaggtggtggtccgcgtgcctggaaaccgcctggtcagaccacgtgacggcaccaggtcctatttcggagctttcatggtcactagtggatccggcgcaacaaacttctctctgctgaaacaagccggagatgtcgaagagaatcctggaccgatgaacccaagtgctgccgtcattttctgcctcatcctgctgggtctgagtgggactcaagggatccctctcgcaaggacggtccgctgcaactgcatccatatcgatgacgggccagtgagaatgagggccatagggaagcttgaaatcatccctgcgagcctatcctgcccacgtgttgagatcattgccacgatgaaaaagaatgatgagcagagatgtctgaatccggaatctaagaccatcaagaatttaatgaaagcgtttagccaaaaaaggtctaaaagggctcctgctagcagcggtacccagtgcaccaactacgccctgctgaagctggccggcgatgtggagagcaaccccgggcccatggaccagcacacacttgatgtggaggataccgcggatgccagacatccagcaggtacttcgtgcccctcggatgcggcgctcctcagagataccgggctcctcgcggacgctgcgctcctctcagatactgtgcgccccacaaatgccgcgctccccacggatgctgcctaccctgcggttaatgttcgggatcgcgaggccgcgtggccgcctgcactgaacttctgttcccgccacccaaagctctatggcctagtcgctttggttttgctgcttctgatcgccgcctgtgttcctatcttcacccgcaccgagcctcggccagcgctcacaatcaccacctcgcccaacctgggtacccgagagaataatgcagaccaggtcacccctgtttcccacattggctgccccaacactacacaacagggctctcctgtgttcgccaagctactggctaaaaaccaagcatcgttgtgcaatacaactctgaactggcacagccaagatggagctgggagctcatacctatctcaaggtctgaggtacgaagaagacaaaaaggagttggtggtagacagtcccgggctctactacgtatttttggaactgaagctcagtccaacattcacaaacacaggccacaaggtgcagggctgggtctctcttgttttgcaagcaaagcctcaggtagatgactttgacaacttggccctgacagtggaactgttcccttgctccatggagaacaagttagtggaccgttcctggagtcaactgttgctcctgaaggctggccaccgcctcagtgtgggtctgagggcttatctgcatggagcccaggatgcatacagagactgggagctgtcttatcccaacaccaccagctttggactctttcttgtgaaacccgacaacccatgggaatgagaattcaataaaagatctttattttcattagatctgtgtgttggttttttgtgtgcggccgcaggaacccctagtgatggagttggccactccctctctgcgcgctcgctcgctcactgaggccgggcgaccaaaggtcgcccgacgcccgggctttgcccgggcggcctcagtgagcgagcgagcgcgcagctgcctgcaggggcgcctgatgcggtattttctccttacgcatctgtgcggtatttcacaccgcatacgtcaaagcaaccatagtacgcgccctgtagcggcgcattaagcgcggcgggtgtggtggttacgcgcagcgtgaccgctacacttgccagcgccttagcgcccgctcctttcgctttcttcccttcctttctcgccacgttcgccggctttccccgtcaagctctaaatcgggggctccctttagggttccgatttagtgctttacggcacctcgaccccaaaaaacttgatttgggtgatggttcacgtagtgggccatcgccctgatagacggtttttcgccctttgacgttggagtccacgttctttaatagtggactcttgttccaaactggaacaacactcaactctatctcgggctattcttttgatttataagggattttgccgatttcggtctattggttaaaaaatgagctgatttaacaaaaatttaacgcgaattttaacaaaatattaacgtttacaattttatggtgcactctcagtacaatctgctctgatgccgcatagttaagccagccccgacacccgccaacacccgctgacgcgccctgacgggcttgtctgctcccggcatccgcttacagacaagctgtgaccgtctccgggagctgcatgtgtcagaggttttcaccgtcatcaccgaaacgcgcgagacgaaagggcctcgtgatacgcctatttttataggttaatgtcatgataataatggtttcttagacgtcaggtggcacttttcggggaaatgtgcgcggaacccctatttgtttatttttctaaatacattcaaatatgtatccgctcatgagacaataaccctgataaatgcttcaataatattgaaaaaggaagagtatgagtattcaacatttccgtgtcgcccttattcccttttttgcggcattttgccttcctgtttttgctcacccagaaacgctggtgaaagtaaaagatgctgaagatcagttgggtgcacgagtgggttacatcgaactggatctcaacagcggtaagatccttgagagttttcgccccgaagaacgttttccaatgatgagcacttttaaagttctgctatgtggcgcggtattatcccgtattgacgccgggcaagagcaactcggtcgccgcatacactattctcagaatgacttggttgagtactcaccagtcacagaaaagcatcttacggatggcatgacagtaagagaattatgcagtgctgccataaccatgagtgataacactgcggccaacttacttctgacaacgatcggaggaccgaaggagctaaccgcttttttgcacaacatgggggatcatgtaactcgccttgatcgttgggaaccggagctgaatgaagccataccaaacgacgagcgtgacaccacgatgcctgtagcaatggcaacaacgttgcgcaaactattaactggcgaactacttactctagcttcccggcaacaattaatagactggatggaggcggataaagttgcaggaccacttctgcgctcggcccttccggctggctggtttattgctgataaatctggagccggtgagcgtggaagccgcggtatcattgcagcactggggccagatggtaagccctcccgtatcgtagttatctacacgacggggagtcaggcaactatggatgaacgaaatagacagatcgctgagataggtgcctcactgattaagcattggtaactgtcagaccaagtttactcatatatactttagattgatttaaaacttcatttttaatttaaaaggatctaggtgaagatcctttttgataatctcatgaccaaaatcccttaacgtgagttttcgttccactgagcgtcagaccccgtagaaaagatcaaaggatcttcttgagatcctttttttctgcgcgtaatctgctgcttgcaaacaaaaaaaccaccgctaccagcggtggtttgtttgccggatcaagagctaccaactctttttccgaaggtaactggcttcagcagagcgcagataccaaatactgttcttctagtgtagccgtagttaggccaccacttcaagaactctgtagcaccgcctacatacctcgctctgctaatcctgttaccagtggctgctgccagtggcgataagtcgtgtcttaccgggttggactcaagacgatagttaccggataaggcgcagcggtcgggctgaacggggggttcgtgcacacagcccagcttggagcgaacgacctacaccgaactgagatacctacagcgtgagctatgagaaagcgccacgcttcccgaagggagaaaggcggacaggtatccggtaagcggcagggtcggaacaggagagcgcacgagggagcttccagggggaaacgcctggtatctttatagtcctgtcgggtttcgccacctctgacttgagcgtcgatttttgtgatgctcgtcaggggggcggagcctatggaaaaacgccagcaacgcggcctttttacggttcctggccttttgctggccttttgctcacatgt

SEQ ID NO: 35 - DNA, 6728 bp, Artificial Sequence
  pGW101
cctgcaggcagctgcgcgctcgctcgctcactgaggccgcccgggcgtcgggcgacctttggtcgcccggcctcagtgagcgagcgagcgcgcagagagggagtggccaactccatcactaggggttcctgcggcctctagaaaggatctgcgatcgctccggtgcccgtcagtgggcagagcgcacatcgcccacagtccccgagaagttggggggaggggtcggcaattgaacgggtgcctagagaaggtggcgcggggtaaactgggaaagtgatgtcgtgtactggctccgcctttttcccgagggtgggggagaaccgtatataagtgcagtagtcgccgtgaacgttctttttcgcaacgggtttgccgccagaacacagctgaagcttcgaggggctcgcatctctccttcacgcgcccgccgccctacctgaggccgccatccacgccggttgagtcgcgttctgccgcctcccgcctgtggtgcctcctgaactgcgtccgccgtctaggtaagtttaaagctcaggtcgagaccgggcctttgtccggcgctcccttggagcctacctagactcagccggctctccacgctttgcctgaccctgcttgctcaactctacgtctttgtttcgttttctgttctgcgccgttacagatctggctaactaccggtgccaccatgaacgctacacactgcatcttggctttgcagctcttcctcatggctgtttctggctgttactgccacggcacagtcattgaaagcctagaaagtctgaataactattttaactcaagtggcatagatgtggaagaaaagagtctcttcttggatatctggaggaactggcaaaaggatggtgacatgaaaatcctgcagagccagattatctctttctacctcagactctttgaagtcttgaaagacaatcaggccatcagcaacaacataagcgtcattgaatcacacctgattactaccttcttcagcaacagcaaggcgaaaaaggatgcattcatgagtattgccaagtttgaggtcaacaacccacaggtccagcgccaagcattcaatgagctcatccgagtggtccaccagctgttgccggaatccagcctcaggaagcggaaaaggagtcgctgcggatccggcgcaacaaacttctctctgctgaaacaagccggagatgtcgaagagaatcctggaccgatggcttgcaattgtcagttgatgcaggatacaccactcctcaagtttccatgtccaaggctcattcttctctttgtgctgctgattcgtctttcacaagtgtcttcagatgttgatgaacaactgtccaagtcagtgaaagataaggtattgctgccttgccgttacaactctcctcatgaagatgagtctgaagaccgaatctactggcaaaaacatgacaaagtggtgctgtctgtcattgttgggaaactaaaagtgtggcccgagtataagaaccggactttatatgacaacactacctactctcttatcatcctgggcctggtcctttcagaccggggcacatacagctgtgtcgttcaaaagaaggaaagaggaacgtatgaagttaaacacttggctttagtaaagttgtccatcaaagctgacttctctacccccaacataactgagtctggaaacccatctgcagacactaaaaggattacctgctttgcttccgggggtttcccaaagcctcgcttctcttggttggaaaatggaagagaattacctggcatcaatacgacaatttcccaggatcctgaatctgaattgtacaccattagtagccaactagatttcaatacgactcgcaaccacaccattaagtgtctcattaaatatggagatgctcacgtgtcagaggacttcacctgggaaaaacccccagaagaccctcctgatagcaagaacacacttgtgctctttggggcaggattcggcgcagtaataacagtcgtcgtcatcgttgtcatcatcaaatgcttctgtaagcacagaagctgtttcagaagaaatgaggcaagcagagaaacaaacaacagccttaccttcgggcctgaagaagcattagctgaacagaccgtcttccttcgtacgggcagtggagagggcagaggaagtctgctaacatgcggtgacgtcgaggagaatcctggcccaatggagagtgtggtacagccttcagtgtttgtggtggatggacagacggacatcccattcaggcggctggaacagaaccaccggagacggcgctgtggcactgtccaggtcagcctggccctggtgctgctgctaggtgctgggctggccactcagggctggtttctcctgagactgcatcaacgtcttggagacatagtagctcatctgccagatggaggcaaaggctcctgggagaagctgatacaagatcaacgatctcaccaggccaacccagcagcacatcttacaggagccaacgccagcttgataggtattggtggacctctgttatgggagacacgacttggcctggccttcttgaggggcttgacgtatcatgatggggccctggtgaccatggagcccggttactactatgtgtactccaaagtgcagctgagcggcgtgggctgcccccaggggctggccaatggcctccccatcacccatggactatacaagcgcacatcccgctacccgaaggagttagaactgctggtcagtcggcggtcaccctgtggccgggccaacagctcccgagtctggtgggacagcagcttcctgggcggcgtggtacatctggaggctggggaagaggtggtggtccgcgtgcctggaaaccgcctggtcagaccacgtgacggcaccaggtcctatttcggagctttcatggtcactagcagcggtacccagtgcaccaactacgccctgctgaagctggccggcgatgtggagagcaaccccgggcccatggaccagcacacacttgatgtggaggataccgcggatgccagacatccagcaggtacttcgtgcccctcggatgcggcgctcctcagagataccgggctcctcgcggacgctgcgctcctctcagatactgtgcgccccacaaatgccgcgctccccacggatgctgcctaccctgcggttaatgttcgggatcgcgaggccgcgtggccgcctgcactgaacttctgttcccgccacccaaagctctatggcctagtcgctttggttttgctgcttctgatcgccgcctgtgttcctatcttcacccgcaccgagcctcggccagcgctcacaatcaccacctcgcccaacctgggtacccgagagaataatgcagaccaggtcacccctgtttcccacattggctgccccaacactacacaacagggctctcctgtgttcgccaagctactggctaaaaaccaagcatcgttgtgcaatacaactctgaactggcacagccaagatggagctgggagctcatacctatctcaaggtctgaggtacgaagaagacaaaaaggagttggtggtagacagtcccgggctctactacgtatttttggaactgaagctcagtccaacattcacaaacacaggccacaaggtgcagggctgggtctctcttgttttgcaagcaaagcctcaggtagatgactttgacaacttggccctgacagtggaactgttcccttgctccatggagaacaagttagtggaccgttcctggagtcaactgttgctcctgaaggctggccaccgcctcagtgtgggtctgagggcttatctgcatggagcccaggatgcatacagagactgggagctgtcttatcccaacaccaccagctttggactctttcttgtgaaacccgacaacccatgggaatgagaattcaataaaagatctttattttcattagatctgtgtgttggttttttgtgtgcggccgcaggaacccctagtgatggagttggccactccctctctgcgcgctcgctcgctcactgaggccgggcgaccaaaggtcgcccgacgcccgggctttgcccgggcggcctcagtgagcgagcgagcgcgcagctgcctgcaggggcgcctgatgcggtattttctccttacgcatctgtgcggtatttcacaccgcatacgtcaaagcaaccatagtacgcgccctgtagcggcgcattaagcgcggcgggtgtggtggttacgcgcagcgtgaccgctacacttgccagcgccttagcgcccgctcctttcgctttcttcccttcctttctcgccacgttcgccggctttccccgtcaagctctaaatcgggggctccctttagggttccgatttagtgctttacggcacctcgaccccaaaaaacttgatttgggtgatggttcacgtagtgggccatcgccctgatagacggtttttcgccctttgacgttggagtccacgttctttaatagtggactcttgttccaaactggaacaacactcaactctatctcgggctattcttttgatttataagggattttgccgatttcggtctattggttaaaaaatgagctgatttaacaaaaatttaacgcgaattttaacaaaatattaacgtttacaattttatggtgcactctcagtacaatctgctctgatgccgcatagttaagccagccccgacacccgccaacacccgctgacgcgccctgacgggcttgtctgctcccggcatccgcttacagacaagctgtgaccgtctccgggagctgcatgtgtcagaggttttcaccgtcatcaccgaaacgcgcgagacgaaagggcctcgtgatacgcctatttttataggttaatgtcatgataataatggtttcttagacgtcaggtggcacttttcggggaaatgtgcgcggaacccctatttgtttatttttctaaatacattcaaatatgtatccgctcatgagacaataaccctgataaatgcttcaataatattgaaaaaggaagagtatgagtattcaacatttccgtgtcgcccttattcccttttttgcggcattttgccttcctgtttttgctcacccagaaacgctggtgaaagtaaaagatgctgaagatcagttgggtgcacgagtgggttacatcgaactggatctcaacagcggtaagatccttgagagttttcgccccgaagaacgttttccaatgatgagcacttttaaagttctgctatgtggcgcggtattatcccgtattgacgccgggcaagagcaactcggtcgccgcatacactattctcagaatgacttggttgagtactcaccagtcacagaaaagcatcttacggatggcatgacagtaagagaattatgcagtgctgccataaccatgagtgataacactgcggccaacttacttctgacaacgatcggaggaccgaaggagctaaccgcttttttgcacaacatgggggatcatgtaactcgccttgatcgttgggaaccggagctgaatgaagccataccaaacgacgagcgtgacaccacgatgcctgtagcaatggcaacaacgttgcgcaaactattaactggcgaactacttactctagcttcccggcaacaattaatagactggatggaggcggataaagttgcaggaccacttctgcgctcggcccttccggctggctggtttattgctgataaatctggagccggtgagcgtggaagccgcggtatcattgcagcactggggccagatggtaagccctcccgtatcgtagttatctacacgacggggagtcaggcaactatggatgaacgaaatagacagatcgctgagataggtgcctcactgattaagcattggtaactgtcagaccaagtttactcatatatactttagattgatttaaaacttcatttttaatttaaaaggatctaggtgaagatcctttttgataatctcatgaccaaaatcccttaacgtgagttttcgttccactgagcgtcagaccccgtagaaaagatcaaaggatcttcttgagatcctttttttctgcgcgtaatctgctgcttgcaaacaaaaaaaccaccgctaccagcggtggtttgtttgccggatcaagagctaccaactctttttccgaaggtaactggcttcagcagagcgcagataccaaatactgttcttctagtgtagccgtagttaggccaccacttcaagaactctgtagcaccgcctacatacctcgctctgctaatcctgttaccagtggctgctgccagtggcgataagtcgtgtcttaccgggttggactcaagacgatagttaccggataaggcgcagcggtcgggctgaacggggggttcgtgcacacagcccagcttggagcgaacgacctacaccgaactgagatacctacagcgtgagctatgagaaagcgccacgcttcccgaagggagaaaggcggacaggtatccggtaagcggcagggtcggaacaggagagcgcacgagggagcttccagggggaaacgcctggtatctttatagtcctgtcgggtttcgccacctctgacttgagcgtcgatttttgtgatgctcgtcaggggggcggagcctatggaaaaacgccagcaacgcggcctttttacggttcctggccttttgctggccttttgctcacatgt

SEQ ID NO: 36 - DNA, 4412 bp, Artificial Sequence
  pGW102
cctgcaggcagctgcgcgctcgctcgctcactgaggccgcccgggcgtcgggcgacctttggtcgcccggcctcagtgagcgagcgagcgcgcagagagggagtggccaactccatcactaggggttcctgcggcctctagaaaggatctgcgatcgctccggtgcccgtcagtgggcagagcgcacatcgcccacagtccccgagaagttggggggaggggtcggcaattgaacgggtgcctagagaaggtggcgcggggtaaactgggaaagtgatgtcgtgtactggctccgcctttttcccgagggtgggggagaaccgtatataagtgcagtagtcgccgtgaacgttctttttcgcaacgggtttgccgccagaacacagctgaagcttcgaggggctcgcatctctccttcacgcgcccgccgccctacctgaggccgccatccacgccggttgagtcgcgttctgccgcctcccgcctgtggtgcctcctgaactgcgtccgccgtctaggtaagtttaaagctcaggtcgagaccgggcctttgtccggcgctcccttggagcctacctagactcagccggctctccacgctttgcctgaccctgcttgctcaactctacgtctttgtttcgttttctgttctgcgccgttacagatctggctaactaccggtgccaccatggcttgcaattgtcagttgatgcaggatacaccactcctcaagtttccatgtccaaggctcattcttctctttgtgctgctgattcgtctttcacaagtgtcttcagatgttgatgaacaactgtccaagtcagtgaaagataaggtattgctgccttgccgttacaactctcctcatgaagatgagtctgaagaccgaatctactggcaaaaacatgacaaagtggtgctgtctgtcattgttgggaaactaaaagtgtggcccgagtataagaaccggactttatatgacaacactacctactctcttatcatcctgggcctggtcctttcagaccggggcacatacagctgtgtcgttcaaaagaaggaaagaggaacgtatgaagttaaacacttggctttagtaaagttgtccatcaaagctgacttctctacccccaacataactgagtctggaaacccatctgcagacactaaaaggattacctgctttgcttccgggggtttcccaaagcctcgcttctcttggttggaaaatggaagagaattacctggcatcaatacgacaatttcccaggatcctgaatctgaattgtacaccattagtagccaactagatttcaatacgactcgcaaccacaccattaagtgtctcattaaatatggagatgctcacgtgtcagaggacttcacctgggaaaaacccccagaagaccctcctgatagcaagaacacacttgtgctctttggggcaggattcggcgcagtaataacagtcgtcgtcatcgttgtcatcatcaaatgcttctgtaagcacagaagctgtttcagaagaaatgaggcaagcagagaaacaaacaacagccttaccttcgggcctgaagaagcattagctgaacagaccgtcttccttcgttaggaattcaataaaagatctttattttcattagatctgtgtgttggttttttgtgtgcggccgcaggaacccctagtgatggagttggccactccctctctgcgcgctcgctcgctcactgaggccgggcgaccaaaggtcgcccgacgcccgggctttgcccgggcggcctcagtgagcgagcgagcgcgcagctgcctgcaggggcgcctgatgcggtattttctccttacgcatctgtgcggtatttcacaccgcatacgtcaaagcaaccatagtacgcgccctgtagcggcgcattaagcgcggcgggtgtggtggttacgcgcagcgtgaccgctacacttgccagcgccttagcgcccgctcctttcgctttcttcccttcctttctcgccacgttcgccggctttccccgtcaagctctaaatcgggggctccctttagggttccgatttagtgctttacggcacctcgaccccaaaaaacttgatttgggtgatggttcacgtagtgggccatcgccctgatagacggtttttcgccctttgacgttggagtccacgttctttaatagtggactcttgttccaaactggaacaacactcaactctatctcgggctattcttttgatttataagggattttgccgatttcggtctattggttaaaaaatgagctgatttaacaaaaatttaacgcgaattttaacaaaatattaacgtttacaattttatggtgcactctcagtacaatctgctctgatgccgcatagttaagccagccccgacacccgccaacacccgctgacgcgccctgacgggcttgtctgctcccggcatccgcttacagacaagctgtgaccgtctccgggagctgcatgtgtcagaggttttcaccgtcatcaccgaaacgcgcgagacgaaagggcctcgtgatacgcctatttttataggttaatgtcatgataataatggtttcttagacgtcaggtggcacttttcggggaaatgtgcgcggaacccctatttgtttatttttctaaatacattcaaatatgtatccgctcatgagacaataaccctgataaatgcttcaataatattgaaaaaggaagagtatgagtattcaacatttccgtgtcgcccttattcccttttttgcggcattttgccttcctgtttttgctcacccagaaacgctggtgaaagtaaaagatgctgaagatcagttgggtgcacgagtgggttacatcgaactggatctcaacagcggtaagatccttgagagttttcgccccgaagaacgttttccaatgatgagcacttttaaagttctgctatgtggcgcggtattatcccgtattgacgccgggcaagagcaactcggtcgccgcatacactattctcagaatgacttggttgagtactcaccagtcacagaaaagcatcttacggatggcatgacagtaagagaattatgcagtgctgccataaccatgagtgataacactgcggccaacttacttctgacaacgatcggaggaccgaaggagctaaccgcttttttgcacaacatgggggatcatgtaactcgccttgatcgttgggaaccggagctgaatgaagccataccaaacgacgagcgtgacaccacgatgcctgtagcaatggcaacaacgttgcgcaaactattaactggcgaactacttactctagcttcccggcaacaattaatagactggatggaggcggataaagttgcaggaccacttctgcgctcggcccttccggctggctggtttattgctgataaatctggagccggtgagcgtggaagccgcggtatcattgcagcactggggccagatggtaagccctcccgtatcgtagttatctacacgacggggagtcaggcaactatggatgaacgaaatagacagatcgctgagataggtgcctcactgattaagcattggtaactgtcagaccaagtttactcatatatactttagattgatttaaaacttcatttttaatttaaaaggatctaggtgaagatcctttttgataatctcatgaccaaaatcccttaacgtgagttttcgttccactgagcgtcagaccccgtagaaaagatcaaaggatcttcttgagatcctttttttctgcgcgtaatctgctgcttgcaaacaaaaaaaccaccgctaccagcggtggtttgtttgccggatcaagagctaccaactctttttccgaaggtaactggcttcagcagagcgcagataccaaatactgttcttctagtgtagccgtagttaggccaccacttcaagaactctgtagcaccgcctacatacctcgctctgctaatcctgttaccagtggctgctgccagtggcgataagtcgtgtcttaccgggttggactcaagacgatagttaccggataaggcgcagcggtcgggctgaacggggggttcgtgcacacagcccagcttggagcgaacgacctacaccgaactgagatacctacagcgtgagctatgagaaagcgccacgcttcccgaagggagaaaggcggacaggtatccggtaagcggcagggtcggaacaggagagcgcacgagggagcttccagggggaaacgcctggtatctttatagtcctgtcgggtttcgccacctctgacttgagcgtcgatttttgtgatgctcgtcaggggggcggagcctatggaaaaacgccagcaacgcggcctttttacggttcctggccttttgctggccttttgctcacatgt

SEQ ID NO: 37 - DNA, 4208 bp, Artificial Sequence
  pGW103
cctgcaggcagctgcgcgctcgctcgctcactgaggccgcccgggcgtcgggcgacctttggtcgcccggcctcagtgagcgagcgagcgcgcagagagggagtggccaactccatcactaggggttcctgcggcctctagaaaggatctgcgatcgctccggtgcccgtcagtgggcagagcgcacatcgcccacagtccccgagaagttggggggaggggtcggcaattgaacgggtgcctagagaaggtggcgcggggtaaactgggaaagtgatgtcgtgtactggctccgcctttttcccgagggtgggggagaaccgtatataagtgcagtagtcgccgtgaacgttctttttcgcaacgggtttgccgccagaacacagctgaagcttcgaggggctcgcatctctccttcacgcgcccgccgccctacctgaggccgccatccacgccggttgagtcgcgttctgccgcctcccgcctgtggtgcctcctgaactgcgtccgccgtctaggtaagtttaaagctcaggtcgagaccgggcctttgtccggcgctcccttggagcctacctagactcagccggctctccacgctttgcctgaccctgcttgctcaactctacgtctttgtttcgttttctgttctgcgccgttacagatctggctaactaccggtgccaccatggagagtgtggtacagccttcagtgtttgtggtggatggacagacggacatcccattcaggcggctggaacagaaccaccggagacggcgctgtggcactgtccaggtcagcctggccctggtgctgctgctaggtgctgggctggccactcagggctggtttctcctgagactgcatcaacgtcttggagacatagtagctcatctgccagatggaggcaaaggctcctgggagaagctgatacaagatcaacgatctcaccaggccaacccagcagcacatcttacaggagccaacgccagcttgataggtattggtggacctctgttatgggagacacgacttggcctggccttcttgaggggcttgacgtatcatgatggggccctggtgaccatggagcccggttactactatgtgtactccaaagtgcagctgagcggcgtgggctgcccccaggggctggccaatggcctccccatcacccatggactatacaagcgcacatcccgctacccgaaggagttagaactgctggtcagtcggcggtcaccctgtggccgggccaacagctcccgagtctggtgggacagcagcttcctgggcggcgtggtacatctggaggctggggaagaggtggtggtccgcgtgcctggaaaccgcctggtcagaccacgtgacggcaccaggtcctatttcggagctttcatggtctgagaattcaataaaagatctttattttcattagatctgtgtgttggttttttgtgtgcggccgcaggaacccctagtgatggagttggccactccctctctgcgcgctcgctcgctcactgaggccgggcgaccaaaggtcgcccgacgcccgggctttgcccgggcggcctcagtgagcgagcgagcgcgcagctgcctgcaggggcgcctgatgcggtattttctccttacgcatctgtgcggtatttcacaccgcatacgtcaaagcaaccatagtacgcgccctgtagcggcgcattaagcgcggcgggtgtggtggttacgcgcagcgtgaccgctacacttgccagcgccttagcgcccgctcctttcgctttcttcccttcctttctcgccacgttcgccggctttccccgtcaagctctaaatcgggggctccctttagggttccgatttagtgctttacggcacctcgaccccaaaaaacttgatttgggtgatggttcacgtagtgggccatcgccctgatagacggtttttcgccctttgacgttggagtccacgttctttaatagtggactcttgttccaaactggaacaacactcaactctatctcgggctattcttttgatttataagggattttgccgatttcggtctattggttaaaaaatgagctgatttaacaaaaatttaacgcgaattttaacaaaatattaacgtttacaattttatggtgcactctcagtacaatctgctctgatgccgcatagttaagccagccccgacacccgccaacacccgctgacgcgccctgacgggcttgtctgctcccggcatccgcttacagacaagctgtgaccgtctccgggagctgcatgtgtcagaggttttcaccgtcatcaccgaaacgcgcgagacgaaagggcctcgtgatacgcctatttttataggttaatgtcatgataataatggtttcttagacgtcaggtggcacttttcggggaaatgtgcgcggaacccctatttgtttatttttctaaatacattcaaatatgtatccgctcatgagacaataaccctgataaatgcttcaataatattgaaaaaggaagagtatgagtattcaacatttccgtgtcgcccttattcccttttttgcggcattttgccttcctgtttttgctcacccagaaacgctggtgaaagtaaaagatgctgaagatcagttgggtgcacgagtgggttacatcgaactggatctcaacagcggtaagatccttgagagttttcgccccgaagaacgttttccaatgatgagcacttttaaagttctgctatgtggcgcggtattatcccgtattgacgccgggcaagagcaactcggtcgccgcatacactattctcagaatgacttggttgagtactcaccagtcacagaaaagcatcttacggatggcatgacagtaagagaattatgcagtgctgccataaccatgagtgataacactgcggccaacttacttctgacaacgatcggaggaccgaaggagctaaccgcttttttgcacaacatgggggatcatgtaactcgccttgatcgttgggaaccggagctgaatgaagccataccaaacgacgagcgtgacaccacgatgcctgtagcaatggcaacaacgttgcgcaaactattaactggcgaactacttactctagcttcccggcaacaattaatagactggatggaggcggataaagttgcaggaccacttctgcgctcggcccttccggctggctggtttattgctgataaatctggagccggtgagcgtggaagccgcggtatcattgcagcactggggccagatggtaagccctcccgtatcgtagttatctacacgacggggagtcaggcaactatggatgaacgaaatagacagatcgctgagataggtgcctcactgattaagcattggtaactgtcagaccaagtttactcatatatactttagattgatttaaaacttcatttttaatttaaaaggatctaggtgaagatcctttttgataatctcatgaccaaaatcccttaacgtgagttttcgttccactgagcgtcagaccccgtagaaaagatcaaaggatcttcttgagatcctttttttctgcgcgtaatctgctgcttgcaaacaaaaaaaccaccgctaccagcggtggtttgtttgccggatcaagagctaccaactctttttccgaaggtaactggcttcagcagagcgcagataccaaatactgttcttctagtgtagccgtagttaggccaccacttcaagaactctgtagcaccgcctacatacctcgctctgctaatcctgttaccagtggctgctgccagtggcgataagtcgtgtcttaccgggttggactcaagacgatagttaccggataaggcgcagcggtcgggctgaacggggggttcgtgcacacagcccagcttggagcgaacgacctacaccgaactgagatacctacagcgtgagctatgagaaagcgccacgcttcccgaagggagaaaggcggacaggtatccggtaagcggcagggtcggaacaggagagcgcacgagggagcttccagggggaaacgcctggtatctttatagtcctgtcgggtttcgccacctctgacttgagcgtcgatttttgtgatgctcgtcaggggggcggagcctatggaaaaacgccagcaacgcggcctttttacggttcctggccttttgctggccttttgctcacatgt

SEQ ID NO: 38 - DNA, 3785 bp, Artificial Sequence
  pGW104
cctgcaggcagctgcgcgctcgctcgctcactgaggccgcccgggcgtcgggcgacctttggtcgcccggcctcagtgagcgagcgagcgcgcagagagggagtggccaactccatcactaggggttcctgcggcctctagaaaggatctgcgatcgctccggtgcccgtcagtgggcagagcgcacatcgcccacagtccccgagaagttggggggaggggtcggcaattgaacgggtgcctagagaaggtggcgcggggtaaactgggaaagtgatgtcgtgtactggctccgcctttttcccgagggtgggggagaaccgtatataagtgcagtagtcgccgtgaacgttctttttcgcaacgggtttgccgccagaacacagctgaagcttcgaggggctcgcatctctccttcacgcgcccgccgccctacctgaggccgccatccacgccggttgagtcgcgttctgccgcctcccgcctgtggtgcctcctgaactgcgtccgccgtctaggtaagtttaaagctcaggtcgagaccgggcctttgtccggcgctcccttggagcctacctagactcagccggctctccacgctttgcctgaccctgcttgctcaactctacgtctttgtttcgttttctgttctgcgccgttacagatctggctaactaccggtgccaccatgaacccaagtgctgccgtcattttctgcctcatcctgctgggtctgagtgggactcaagggatccctctcgcaaggacggtccgctgcaactgcatccatatcgatgacgggccagtgagaatgagggccatagggaagcttgaaatcatccctgcgagcctatcctgcccacgtgttgagatcattgccacgatgaaaaagaatgatgagcagagatgtctgaatccggaatctaagaccatcaagaatttaatgaaagcgtttagccaaaaaaggtctaaaagggctccttgagaattcaataaaagatctttattttcattagatctgtgtgttggttttttgtgtgcggccgcaggaacccctagtgatggagttggccactccctctctgcgcgctcgctcgctcactgaggccgggcgaccaaaggtcgcccgacgcccgggctttgcccgggcggcctcagtgagcgagcgagcgcgcagctgcctgcaggggcgcctgatgcggtattttctccttacgcatctgtgcggtatttcacaccgcatacgtcaaagcaaccatagtacgcgccctgtagcggcgcattaagcgcggcgggtgtggtggttacgcgcagcgtgaccgctacacttgccagcgccttagcgcccgctcctttcgctttcttcccttcctttctcgccacgttcgccggctttccccgtcaagctctaaatcgggggctccctttagggttccgatttagtgctttacggcacctcgaccccaaaaaacttgatttgggtgatggttcacgtagtgggccatcgccctgatagacggtttttcgccctttgacgttggagtccacgttctttaatagtggactcttgttccaaactggaacaacactcaactctatctcgggctattcttttgatttataagggattttgccgatttcggtctattggttaaaaaatgagctgatttaacaaaaatttaacgcgaattttaacaaaatattaacgtttacaattttatggtgcactctcagtacaatctgctctgatgccgcatagttaagccagccccgacacccgccaacacccgctgacgcgccctgacgggcttgtctgctcccggcatccgcttacagacaagctgtgaccgtctccgggagctgcatgtgtcagaggttttcaccgtcatcaccgaaacgcgcgagacgaaagggcctcgtgatacgcctatttttataggttaatgtcatgataataatggtttcttagacgtcaggtggcacttttcggggaaatgtgcgcggaacccctatttgtttatttttctaaatacattcaaatatgtatccgctcatgagacaataaccctgataaatgcttcaataatattgaaaaaggaagagtatgagtattcaacatttccgtgtcgcccttattcccttttttgcggcattttgccttcctgtttttgctcacccagaaacgctggtgaaagtaaaagatgctgaagatcagttgggtgcacgagtgggttacatcgaactggatctcaacagcggtaagatccttgagagttttcgccccgaagaacgttttccaatgatgagcacttttaaagttctgctatgtggcgcggtattatcccgtattgacgccgggcaagagcaactcggtcgccgcatacactattctcagaatgacttggttgagtactcaccagtcacagaaaagcatcttacggatggcatgacagtaagagaattatgcagtgctgccataaccatgagtgataacactgcggccaacttacttctgacaacgatcggaggaccgaaggagctaaccgcttttttgcacaacatgggggatcatgtaactcgccttgatcgttgggaaccggagctgaatgaagccataccaaacgacgagcgtgacaccacgatgcctgtagcaatggcaacaacgttgcgcaaactattaactggcgaactacttactctagcttcccggcaacaattaatagactggatggaggcggataaagttgcaggaccacttctgcgctcggcccttccggctggctggtttattgctgataaatctggagccggtgagcgtggaagccgcggtatcattgcagcactggggccagatggtaagccctcccgtatcgtagttatctacacgacggggagtcaggcaactatggatgaacgaaatagacagatcgctgagataggtgcctcactgattaagcattggtaactgtcagaccaagtttactcatatatactttagattgatttaaaacttcatttttaatttaaaaggatctaggtgaagatcctttttgataatctcatgaccaaaatcccttaacgtgagttttcgttccactgagcgtcagaccccgtagaaaagatcaaaggatcttcttgagatcctttttttctgcgcgtaatctgctgcttgcaaacaaaaaaaccaccgctaccagcggtggtttgtttgccggatcaagagctaccaactctttttccgaaggtaactggcttcagcagagcgcagataccaaatactgttcttctagtgtagccgtagttaggccaccacttcaagaactctgtagcaccgcctacatacctcgctctgctaatcctgttaccagtggctgctgccagtggcgataagtcgtgtcttaccgggttggactcaagacgatagttaccggataaggcgcagcggtcgggctgaacggggggttcgtgcacacagcccagcttggagcgaacgacctacaccgaactgagatacctacagcgtgagctatgagaaagcgccacgcttcccgaagggagaaaggcggacaggtatccggtaagcggcagggtcggaacaggagagcgcacgagggagcttccagggggaaacgcctggtatctttatagtcctgtcgggtttcgccacctctgacttgagcgtcgatttttgtgatgctcgtcaggggggcggagcctatggaaaaacgccagcaacgcggcctttttacggttcctggccttttgctggccttttgctcacatgt

SEQ ID NO: 39 - DNA, 4418 bp, Artificial Sequence
  pGW105
cctgcaggcagctgcgcgctcgctcgctcactgaggccgcccgggcgtcgggcgacctttggtcgcccggcctcagtgagcgagcgagcgcgcagagagggagtggccaactccatcactaggggttcctgcggcctctagaaaggatctgcgatcgctccggtgcccgtcagtgggcagagcgcacatcgcccacagtccccgagaagttggggggaggggtcggcaattgaacgggtgcctagagaaggtggcgcggggtaaactgggaaagtgatgtcgtgtactggctccgcctttttcccgagggtgggggagaaccgtatataagtgcagtagtcgccgtgaacgttctttttcgcaacgggtttgccgccagaacacagctgaagcttcgaggggctcgcatctctccttcacgcgcccgccgccctacctgaggccgccatccacgccggttgagtcgcgttctgccgcctcccgcctgtggtgcctcctgaactgcgtccgccgtctaggtaagtttaaagctcaggtcgagaccgggcctttgtccggcgctcccttggagcctacctagactcagccggctctccacgctttgcctgaccctgcttgctcaactctacgtctttgtttcgttttctgttctgcgccgttacagatctggctaactaccggtgccaccatggaccagcacacacttgatgtggaggataccgcggatgccagacatccagcaggtacttcgtgcccctcggatgcggcgctcctcagagataccgggctcctcgcggacgctgcgctcctctcagatactgtgcgccccacaaatgccgcgctccccacggatgctgcctaccctgcggttaatgttcgggatcgcgaggccgcgtggccgcctgcactgaacttctgttcccgccacccaaagctctatggcctagtcgctttggttttgctgcttctgatcgccgcctgtgttcctatcttcacccgcaccgagcctcggccagcgctcacaatcaccacctcgcccaacctgggtacccgagagaataatgcagaccaggtcacccctgtttcccacattggctgccccaacactacacaacagggctctcctgtgttcgccaagctactggctaaaaaccaagcatcgttgtgcaatacaactctgaactggcacagccaagatggagctgggagctcatacctatctcaaggtctgaggtacgaagaagacaaaaaggagttggtggtagacagtcccgggctctactacgtatttttggaactgaagctcagtccaacattcacaaacacaggccacaaggtgcagggctgggtctctcttgttttgcaagcaaagcctcaggtagatgactttgacaacttggccctgacagtggaactgttcccttgctccatggagaacaagttagtggaccgttcctggagtcaactgttgctcctgaaggctggccaccgcctcagtgtgggtctgagggcttatctgcatggagcccaggatgcatacagagactgggagctgtcttatcccaacaccaccagctttggactctttcttgtgaaacccgacaacccatgggaatgagaattcaataaaagatctttattttcattagatctgtgtgttggttttttgtgtgcggccgcaggaacccctagtgatggagttggccactccctctctgcgcgctcgctcgctcactgaggccgggcgaccaaaggtcgcccgacgcccgggctttgcccgggcggcctcagtgagcgagcgagcgcgcagctgcctgcaggggcgcctgatgcggtattttctccttacgcatctgtgcggtatttcacaccgcatacgtcaaagcaaccatagtacgcgccctgtagcggcgcattaagcgcggcgggtgtggtggttacgcgcagcgtgaccgctacacttgccagcgccttagcgcccgctcctttcgctttcttcccttcctttctcgccacgttcgccggctttccccgtcaagctctaaatcgggggctccctttagggttccgatttagtgctttacggcacctcgaccccaaaaaacttgatttgggtgatggttcacgtagtgggccatcgccctgatagacggtttttcgccctttgacgttggagtccacgttctttaatagtggactcttgttccaaactggaacaacactcaactctatctcgggctattcttttgatttataagggattttgccgatttcggtctattggttaaaaaatgagctgatttaacaaaaatttaacgcgaattttaacaaaatattaacgtttacaattttatggtgcactctcagtacaatctgctctgatgccgcatagttaagccagccccgacacccgccaacacccgctgacgcgccctgacgggcttgtctgctcccggcatccgcttacagacaagctgtgaccgtctccgggagctgcatgtgtcagaggttttcaccgtcatcaccgaaacgcgcgagacgaaagggcctcgtgatacgcctatttttataggttaatgtcatgataataatggtttcttagacgtcaggtggcacttttcggggaaatgtgcgcggaacccctatttgtttatttttctaaatacattcaaatatgtatccgctcatgagacaataaccctgataaatgcttcaataatattgaaaaaggaagagtatgagtattcaacatttccgtgtcgcccttattcccttttttgcggcattttgccttcctgtttttgctcacccagaaacgctggtgaaagtaaaagatgctgaagatcagttgggtgcacgagtgggttacatcgaactggatctcaacagcggtaagatccttgagagttttcgccccgaagaacgttttccaatgatgagcacttttaaagttctgctatgtggcgcggtattatcccgtattgacgccgggcaagagcaactcggtcgccgcatacactattctcagaatgacttggttgagtactcaccagtcacagaaaagcatcttacggatggcatgacagtaagagaattatgcagtgctgccataaccatgagtgataacactgcggccaacttacttctgacaacgatcggaggaccgaaggagctaaccgcttttttgcacaacatgggggatcatgtaactcgccttgatcgttgggaaccggagctgaatgaagccataccaaacgacgagcgtgacaccacgatgcctgtagcaatggcaacaacgttgcgcaaactattaactggcgaactacttactctagcttcccggcaacaattaatagactggatggaggcggataaagttgcaggaccacttctgcgctcggcccttccggctggctggtttattgctgataaatctggagccggtgagcgtggaagccgcggtatcattgcagcactggggccagatggtaagccctcccgtatcgtagttatctacacgacggggagtcaggcaactatggatgaacgaaatagacagatcgctgagataggtgcctcactgattaagcattggtaactgtcagaccaagtttactcatatatactttagattgatttaaaacttcatttttaatttaaaaggatctaggtgaagatcctttttgataatctcatgaccaaaatcccttaacgtgagttttcgttccactgagcgtcagaccccgtagaaaagatcaaaggatcttcttgagatcctttttttctgcgcgtaatctgctgcttgcaaacaaaaaaaccaccgctaccagcggtggtttgtttgccggatcaagagctaccaactctttttccgaaggtaactggcttcagcagagcgcagataccaaatactgttcttctagtgtagccgtagttaggccaccacttcaagaactctgtagcaccgcctacatacctcgctctgctaatcctgttaccagtggctgctgccagtggcgataagtcgtgtcttaccgggttggactcaagacgatagttaccggataaggcgcagcggtcgggctgaacggggggttcgtgcacacagcccagcttggagcgaacgacctacaccgaactgagatacctacagcgtgagctatgagaaagcgccacgcttcccgaagggagaaaggcggacaggtatccggtaagcggcagggtcggaacaggagagcgcacgagggagcttccagggggaaacgcctggtatctttatagtcctgtcgggtttcgccacctctgacttgagcgtcgatttttgtgatgctcgtcaggggggcggagcctatggaaaaacgccagcaacgcggcctttttacggttcctggccttttgctggccttttgctcacatgt

SEQ ID NO: 40 - DNA, 6676 bp, Artificial Sequence
  pGW110
cctgcaggcagctgcgcgctcgctcgctcactgaggccgcccgggcgtcgggcgacctttggtcgcccggcctcagtgagcgagcgagcgcgcagagagggagtggccaactccatcactaggggttcctgcggcctctagaaaggatctgcgatcgctccggtgcccgtcagtgggcagagcgcacatcgcccacagtccccgagaagttggggggaggggtcggcaattgaacgggtgcctagagaaggtggcgcggggtaaactgggaaagtgatgtcgtgtactggctccgcctttttcccgagggtgggggagaaccgtatataagtgcagtagtcgccgtgaacgttctttttcgcaacgggtttgccgccagaacacagctgaagcttcgaggggctcgcatctctccttcacgcgcccgccgccctacctgaggccgccatccacgccggttgagtcgcgttctgccgcctcccgcctgtggtgcctcctgaactgcgtccgccgtctaggtaagtttaaagctcaggtcgagaccgggcctttgtccggcgctcccttggagcctacctagactcagccggctctccacgctttgcctgaccctgcttgctcaactctacgtctttgtttcgttttctgttctgcgccgttacagatctggctaactaccggtgccaccatggcttgcaattgtcagttgatgcaggatacaccactcctcaagtttccatgtccaaggctcattcttctctttgtgctgctgattcgtctttcacaagtgtcttcagatgttgatgaacaactgtccaagtcagtgaaagataaggtattgctgccttgccgttacaactctcctcatgaagatgagtctgaagaccgaatctactggcaaaaacatgacaaagtggtgctgtctgtcattgctgggaaactaaaagtgtggcccgagtataagaaccggactttatatgacaacactacctactctcttatcatcctgggcctggtcctttcagaccggggcacatacagctgtgtcgttcaaaagaaggaaagaggaacgtatgaagttaaacacttggctttagtaaagttgtccatcaaagctgacttctctacccccaacataactgagtctggaaacccatctgcagacactaaaaggattacctgctttgcttccgggggtttcccaaagcctcgcttctcttggttggaaaatggaagagaattacctggcatcaatacgacaatttcccaggatcctgaatctgaattgtacaccattagtagccaactagatttcaatacgactcgcaaccacaccattaagtgtctcattaaatatggagatgctcacgtgtcagaggacttcacctgggaaaaacccccagaagaccctcctgatagcaagaacacacttgtgctctttggggcaggattcggcgcagtaataacagtcgtcgtcatcgttgtcatcatcaaatgcttctgtaagcacagaagctgtttcagaagaaatgaggcaagcagagaaacaaacaacagccttaccttcgggcctgaagaagcattagctgaacagaccgtcttccttcgtacgggcagtggagagggcagaggaagtctgctaacatgcggtgacgtcgaggagaatcctggcccaatggagagtgtggtacagccttcagtgtttgtggtggatggacagacggacatcccattcaggcggctggaacagaaccaccggagacggcgctgtggcactgtccaggtcagcctggccctggtgctgctgctaagtgctgggctggccactcagggctggtttctcctgagactgcatcaacgtcttggagacatagtagctcatctgccagatggaggcaaaggctcctgggagaagctgatacaagatcaacgatctcaccaggccaacccagcagcacatcttacaggagccaacgccagcttgataggtattggtggacctctgttatgggagacacgacttggcctggccttcttgaggggcttgacgtatcatgatggggccctggtgaccatggagcccggttactactatgtgtactccaaagtgcagctgagcggcgtgggctgcccccaggggctggccaatggcctccccatcacccatggactatacaagcgcacatcccgctacccgaaggagttagaactgctggtcagtcggcggtcaccctgtggccgggccaacagctcccgagtctggtgggacagcagcttcctgggcggcgtggtacatctggaggctggggaagaggtggtggtccgcgtgcctggaaaccgcctggtcagaccacgtgacggcaccaggtcctatttcggagctttcatggtcactagtggatccggcgcaacaaacttctctctgctgaaacaagccggagatgtcgaagagaatcctggaccgatgaacccaagtgctgccgtcattttctgcctcatcctgctgggtctgagtgggactcaagggatccctctcgcaaggacggtccgctgcaactgcatccatatcgatgacgggccagtgagaatgagggccatagggaagcttgaaatcatccctgcgagcctatcctgcccacgtgttgagatcattgccacgatgaaaaagaatgatgagcagagatgtctgaatccggaatctaagaccatcaagaatttaatgaaagcgtttagccaaaaaaggtctaaaagggctcctagcggtacccagtgcaccaactacgccctgctgaagctggccggcgatgtggagagcaaccccgggcccgctagcatgaacgctacacactgcatcttggctttgcagctcttcctcatggctgtttctggctgttactgccacggcacagtcattgaaagcctagaaagtctgaataactattttaactcaagtggcatagatgtggaagaaaagagtctcttcttggatatctggaggaactggcaaaaggatggtgacatgaaaatcctgcagagccagattatctctttctacctcagactctttgaagtcttgaaagacaatcaggccatcagcaacaacataagcgtcattgaatcacacctgattactaccttcttcagcaacagcaaggcgaaaaaggatgcattcatgagtattgccaagtttgaggtcaacaacccacaggtgcagcgccaagcattcaatgagctcatccgagtggtccaccagctgttgccggaatccagcctcaggaagcggaaaaggagtcgctgctgagaattcacgcgttaagtcgacaatcaacctctggattacaaaatttgtgaaagattgactggtattcttaactatgttgctccttttacgctatgtggatacgctgctttaatgcctttgtatcatgctattgcttcccgtatggctttcattttctcctccttgtataaatcctggttgctgtctctttatgaggagttgtggcccgttgtcaggcaacgtggcgtggtgtgcactgtgtttgctgacgcaacccccactggttggggcattgccaccacctgtcagctcctttccgggactttcgctttccccctccctattgccacggcggaactcatcgccgcctgccttgcccgctgctggacaggggctcggctgttgggcactgacaattccgtggtgttgtcggggaaatcatcgtcctttccttggctgctcgcctgtgttgccacctggattctgcgcgggacgtccttctgctacgtcccttcggccctcaatccagcggaccttccttcccgcggcctgctgccggctctgcggcctcttccgcgtcttcgccttcgccctcagacgagtcggatctccctttgggccgcctccccgcgtcgactttaagaccaatgacggccgcaggaacccctagtgatggagttggccactccctctctgcgcgctcgctcgctcactgaggccgggcgaccaaaggtcgcccgacgcccgggctttgcccgggcggcctcagtgagcgagcgagcgcgcagctgcctgcaggggcgcctgatgcggtattttctccttacgcatctgtgcggtatttcacaccgcatacgtcaaagcaaccatagtacgcgccctgtagcggcgcattaagcgcggcgggtgtggtggttacgcgcagcgtgaccgctacacttgccagcgccttagcgcccgctcctttcgctttcttcccttcctttctcgccacgttcgccggctttccccgtcaagctctaaatcgggggctccctttagggttccgatttagtgctttacggcacctcgaccccaaaaaacttgatttgggtgatggttcacgtagtgggccatcgccctgatagacggtttttcgccctttgacgttggagtccacgttctttaatagtggactcttgttccaaactggaacaacactcaactctatctcgggctattcttttgatttataagggattttgccgatttcggtctattggttaaaaaatgagctgatttaacaaaaatttaacgcgaattttaacaaaatattaacgtttacaattttatggtgcactctcagtacaatctgctctgatgccgcatagttaagccagccccgacacccgccaacacccgctgacgcgccctgacgggcttgtctgctcccggcatccgcttacagacaagctgtgaccgtctccgggagctgcatgtgtcagaggttttcaccgtcatcaccgaaacgcgcgagacgaaagggcctcgtgatacgcctatttttataggttaatgtcatgataataatggtttcttagacgtcaggtggcacttttcggggaaatgtgcgcggaacccctatttgtttatttttctaaatacattcaaatatgtatccgctcatgagacaataaccctgataaatgcttcaataatattgaaaaaggaagagtatgagtattcaacatttccgtgtcgcccttattcccttttttgcggcattttgccttcctgtttttgctcacccagaaacgctggtgaaagtaaaagatgctgaagatcagttgggtgcacgagtgggttacatcgaactggatctcaacagcggtaagatccttgagagttttcgccccgaagaacgttttccaatgatgagcacttttaaagttctgctatgtggcgcggtattatcccgtattgacgccgggcaagagcaactcggtcgccgcatacactattctcagaatgacttggttgagtactcaccagtcacagaaaagcatcttacggatggcatgacagtaagagaattatgcagtgctgccataaccatgagtgataacactgcggccaacttacttctgacaacgatcggaggaccgaaggagctaaccgcttttttgcacaacatgggggatcatgtaactcgccttgatcgttgggaaccggagctgaatgaagccataccaaacgacgagcgtgacaccacgatgcctgtagcaatggcaacaacgttgcgcaaactattaactggcgaactacttactctagcttcccggcaacaattaatagactggatggaggcggataaagttgcaggaccacttctgcgctcggcccttccggctggctggtttattgctgataaatctggagccggtgagcgtggaagccgcggtatcattgcagcactggggccagatggtaagccctcccgtatcgtagttatctacacgacggggagtcaggcaactatggatgaacgaaatagacagatcgctgagataggtgcctcactgattaagcattggtaactgtcagaccaagtttactcatatatactttagattgatttaaaacttcatttttaatttaaaaggatctaggtgaagatcctttttgataatctcatgaccaaaatcccttaacgtgagttttcgttccactgagcgtcagaccccgtagaaaagatcaaaggatcttcttgagatcctttttttctgcgcgtaatctgctgcttgcaaacaaaaaaaccaccgctaccagcggtggtttgtttgccggatcaagagctaccaactctttttccgaaggtaactggcttcagcagagcgcagataccaaatactgttcttctagtgtagccgtagttaggccaccacttcaagaactctgtagcaccgcctacatacctcgctctgctaatcctgttaccagtggctgctgccagtggcgataagtcgtgtcttaccgggttggactcaagacgatagttaccggataaggcgcagcggtcgggctgaacggggggttcgtgcacacagcccagcttggagcgaacgacctacaccgaactgagatacctacagcgtgagctatgagaaagcgccacgcttcccgaagggagaaaggcggacaggtatccggtaagcggcagggtcggaacaggagagcgcacgagggagcttccagggggaaacgcctggtatctttatagtcctgtcgggtttcgccacctctgacttgagcgtcgatttttgtgatgctcgtcaggggggcggagcctatggaaaaacgccagcaacgcggcctttttacggttcctggccttttgctggccttttgctcacatgt

SEQ ID NO: 41 - DNA, 5689 bp, Artificial Sequence
  pGW111
cctgcaggcagctgcgcgctcgctcgctcactgaggccgcccgggcgtcgggcgacctttggtcgcccggcctcagtgagcgagcgagcgcgcagagagggagtggccaactccatcactaggggttcctgcggcctctagaaaggatctgcgatcgctccggtgcccgtcagtgggcagagcgcacatcgcccacagtccccgagaagttggggggaggggtcggcaattgaacgggtgcctagagaaggtggcgcggggtaaactgggaaagtgatgtcgtgtactggctccgcctttttcccgagggtgggggagaaccgtatataagtgcagtagtcgccgtgaacgttctttttcgcaacgggtttgccgccagaacacagctgaagcttcgaggggctcgcatctctccttcacgcgcccgccgccctacctgaggccgccatccacgccggttgagtcgcgttctgccgcctcccgcctgtggtgcctcctgaactgcgtccgccgtctaggtaagtttaaagctcaggtcgagaccgggcctttgtccggcgctcccttggagcctacctagactcagccggctctccacgctttgcctgaccctgcttgctcaactctacgtctttgtttcgttttctgttctgcgccgttacagatctggctaactaccggtgccaccatggagagtgtggtacagccttcagtgtttgtggtggatggacagacggacatcccattcaggcggctggaacagaaccaccggagacggcgctgtggcactgtccaggtcagcctggccctggtgctgctgctaagtgctgggctggccactcagggctggtttctcctgagactgcatcaacgtcttggagacatagtagctcatctgccagatggaggcaaaggctcctgggagaagctgatacaagatcaacgatctcaccaggccaacccagcagcacatcttacaggagccaacgccagcttgataggtattggtggacctctgttatgggagacacgacttggcctggccttcttgaggggcttgacgtatcatgatggggccctggtgaccatggagcccggttactactatgtgtactccaaagtgcagctgagcggcgtgggctgcccccaggggctggccaatggcctccccatcacccatggactatacaagcgcacatcccgctacccgaaggagttagaactgctggtcagtcggcggtcaccctgtggccgggccaacagctcccgagtctggtgggacagcagcttcctgggcggcgtggtacatctggaggctggggaagaggtggtggtccgcgtgcctggaaaccgcctggtcagaccacgtgacggcaccaggtcctatttcggagctttcatggtcactagtggatccggcgcaacaaacttctctctgctgaaacaagccggagatgtcgaagagaatcctggaccgatgaacccaagtgctgccgtcattttctgcctcatcctgctgggtctgagtgggactcaagggatccctctcgcaaggacggtccgctgcaactgcatccatatcgatgacgggccagtgagaatgagggccatagggaagcttgaaatcatccctgcgagcctatcctgcccacgtgttgagatcattgccacgatgaaaaagaatgatgagcagagatgtctgaatccggaatctaagaccatcaagaatttaatgaaagcgtttagccaaaaaaggtctaaaagggctcctagcggtacccagtgcaccaactacgccctgctgaagctggccggcgatgtggagagcaaccccgggcccgctagcatgaacgctacacactgcatcttggctttgcagctcttcctcatggctgtttctggctgttactgccacggcacagtcattgaaagcctagaaagtctgaataactattttaactcaagtggcatagatgtggaagaaaagagtctcttcttggatatctggaggaactggcaaaaggatggtgacatgaaaatcctgcagagccagattatctctttctacctcagactctttgaagtcttgaaagacaatcaggccatcagcaacaacataagcgtcattgaatcacacctgattactaccttcttcagcaacagcaaggcgaaaaaggatgcattcatgagtattgccaagtttgaggtcaacaacccacaggtccagcgccaagcattcaatgagctcatccgagtggtccaccagctgttgccggaatccagcctcaggaagcggaaaaggagtcgctgctgagaattcacgcgttaagtcgacaatcaacctctggattacaaaatttgtgaaagattgactggtattcttaactatgttgctccttttacgctatgtggatacgctgctttaatgcctttgtatcatgctattgcttcccgtatggctttcattttctcctccttgtataaatcctggttgctgtctctttatgaggagttgtggcccgttgtcaggcaacgtggcgtggtgtgcactgtgtttgctgacgcaacccccactggttggggcattgccaccacctgtcagctcctttccgggactttcgctttccccctccctattgccacggcggaactcatcgccgcctgccttgcccgctgctggacaggggctcggctgttgggcactgacaattccgtggtgttgtcggggaaatcatcgtcctttccttggctgctcgcctgtgttgccacctggattctgcgcgggacgtccttctgctacgtcccttcggccctcaatccagcggaccttccttcccgcggcctgctgccggctctgcggcctcttccgcgtcttcgccttcgccctcagacgagtcggatctccctttgggccgcctccccgcgtcgactttaagaccaatgacggccgcaggaacccctagtgatggagttggccactccctctctgcgcgctcgctcgctcactgaggccgggcgaccaaaggtcgcccgacgcccgggctttgcccgggcggcctcagtgagcgagcgagcgcgcagctgcctgcaggggcgcctgatgcggtattttctccttacgcatctgtgcggtatttcacaccgcatacgtcaaagcaaccatagtacgcgccctgtagcggcgcattaagcgcggcgggtgtggtggttacgcgcagcgtgaccgctacacttgccagcgccttagcgcccgctcctttcgctttcttcccttcctttctcgccacgttcgccggctttccccgtcaagctctaaatcgggggctccctttagggttccgatttagtgctttacggcacctcgaccccaaaaaacttgatttgggtgatggttcacgtagtgggccatcgccctgatagacggtttttcgccctttgacgttggagtccacgttctttaatagtggactcttgttccaaactggaacaacactcaactctatctcgggctattcttttgatttataagggattttgccgatttcggtctattggttaaaaaatgagctgatttaacaaaaatttaacgcgaattttaacaaaatattaacgtttacaattttatggtgcactctcagtacaatctgctctgatgccgcatagttaagccagccccgacacccgccaacacccgctgacgcgccctgacgggcttgtctgctcccggcatccgcttacagacaagctgtgaccgtctccgggagctgcatgtgtcagaggttttcaccgtcatcaccgaaacgcgcgagacgaaagggcctcgtgatacgcctatttttataggttaatgtcatgataataatggtttcttagacgtcaggtggcacttttcggggaaatgtgcgcggaacccctatttgtttatttttctaaatacattcaaatatgtatccgctcatgagacaataaccctgataaatgcttcaataatattgaaaaaggaagagtatgagtattcaacatttccgtgtcgcccttattcccttttttgcggcattttgccttcctgtttttgctcacccagaaacgctggtgaaagtaaaagatgctgaagatcagttgggtgcacgagtgggttacatcgaactggatctcaacagcggtaagatccttgagagttttcgccccgaagaacgttttccaatgatgagcacttttaaagttctgctatgtggcgcggtattatcccgtattgacgccgggcaagagcaactcggtcgccgcatacactattctcagaatgacttggttgagtactcaccagtcacagaaaagcatcttacggatggcatgacagtaagagaattatgcagtgctgccataaccatgagtgataacactgcggccaacttacttctgacaacgatcggaggaccgaaggagctaaccgcttttttgcacaacatgggggatcatgtaactcgccttgatcgttgggaaccggagctgaatgaagccataccaaacgacgagcgtgacaccacgatgcctgtagcaatggcaacaacgttgcgcaaactattaactggcgaactacttactctagcttcccggcaacaattaatagactggatggaggcggataaagttgcaggaccacttctgcgctcggcccttccggctggctggtttattgctgataaatctggagccggtgagcgtggaagccgcggtatcattgcagcactggggccagatggtaagccctcccgtatcgtagttatctacacgacggggagtcaggcaactatggatgaacgaaatagacagatcgctgagataggtgcctcactgattaagcattggtaactgtcagaccaagtttactcatatatactttagattgatttaaaacttcatttttaatttaaaaggatctaggtgaagatcctttttgataatctcatgaccaaaatcccttaacgtgagttttcgttccactgagcgtcagaccccgtagaaaagatcaaaggatcttcttgagatcctttttttctgcgcgtaatctgctgcttgcaaacaaaaaaaccaccgctaccagcggtggtttgtttgccggatcaagagctaccaactctttttccgaaggtaactggcttcagcagagcgcagataccaaatactgttcttctagtgtagccgtagttaggccaccacttcaagaactctgtagcaccgcctacatacctcgctctgctaatcctgttaccagtggctgctgccagtggcgataagtcgtgtcttaccgggttggactcaagacgatagttaccggataaggcgcagcggtcgggctgaacggggggttcgtgcacacagcccagcttggagcgaacgacctacaccgaactgagatacctacagcgtgagctatgagaaagcgccacgcttcccgaagggagaaaggcggacaggtatccggtaagcggcagggtcggaacaggagagcgcacgagggagcttccagggggaaacgcctggtatctttatagtcctgtcgggtttcgccacctctgacttgagcgtcgatttttgtgatgctcgtcaggggggcggagcctatggaaaaacgccagcaacgcggcctttttacggttcctggccttttgctggccttttgctcacatgt

SEQ ID NO: 42 - DNA, 6679 bp, Artificial Sequence
  pGW112
cctgcaggcagctgcgcgctcgctcgctcactgaggccgcccgggcgtcgggcgacctttggtcgcccggcctcagtgagcgagcgagcgcgcagagagggagtggccaactccatcactaggggttcctgcggcctctagaaaggatctgcgatcgctccggtgcccgtcagtgggcagagcgcacatcgcccacagtccccgagaagttggggggaggggtcggcaattgaacgggtgcctagagaaggtggcgcggggtaaactgggaaagtgatgtcgtgtactggctccgcctttttcccgagggtgggggagaaccgtatataagtgcagtagtcgccgtgaacgttctttttcgcaacgggtttgccgccagaacacagctgaagcttcgaggggctcgcatctctccttcacgcgcccgccgccctacctgaggccgccatccacgccggttgagtcgcgttctgccgcctcccgcctgtggtgcctcctgaactgcgtccgccgtctaggtaagtttaaagctcaggtcgagaccgggcctttgtccggcgctcccttggagcctacctagactcagccggctctccacgctttgcctgaccctgcttgctcaactctacgtctttgtttcgttttctgttctgcgccgttacagatctggctaactaccggtgccaccatggaccagcacacacttgatgtggaggataccgcggatgccagacatccagcaggtacttcgtgcccctcggatgcggcgctcctcagagataccgggctcctcgcggacgctgcgctcctctcagatactgtgcgccccacaaatgccgcgctccccacggatgctgcctaccctgcggttaatgttcgggatcgcgaggccgcgtggccgcctgcactgaacttctgttcccgccacccaaagctctatggcctagtcgctttggttttgctgcttctgatcgccgcctgtgttcctatcttcacccgcaccgagcctcggccagcgctcacaatcaccacctcgcccaacctgggtacccgagagaataatgcagaccaggtcacccctgtttcccacattggctgccccaacactacacaacagggctctcctgtgttcgccaagctactggctaaaaaccaagcatcgttgtgcaatacaactctgaactggcacagccaagatggagctgggagctcatacctatctcaaggtctgaggtacgaagaagacaaaaaggagttggtggtagacagtcccgggctctactacgtatttttggaactgaagctcagtccaacattcacaaacacaggccacaaggtgcagggctgggtctctcttgttttgcaagcaaagcctcaggtagatgactttgacaacttggccctgacagtggaactgttcccttgctccatggagaacaagttagtggaccgttcctggagtcaactgttgctcctgaaggctggccaccgcctcagtgtgggtctgagggcttatctgcatggagcccaggatgcatacagagactgggagctgtcttatcccaacaccaccagctttggactctttcttgtgaaacccgacaacccatgggaaggcagtggagagggcagaggaagtctgctaacatgcggtgacgtcgaggagaatcctggcccaatggagagtgtggtacagccttcagtgtttgtggtggatggacagacggacatcccattcaggcggctggaacagaaccaccggagacggcgctgtggcactgtccaggtcagcctggccctggtgctgctgctaagtgctgggctggccactcagggctggtttctcctgagactgcatcaacgtcttggagacatagtagctcatctgccagatggaggcaaaggctcctgggagaagctgatacaagatcaacgatctcaccaggccaacccagcagcacatcttacaggagccaacgccagcttgataggtattggtggacctctgttatgggagacacgacttggcctggccttcttgaggggcttgacgtatcatgatggggccctggtgaccatggagcccggttactactatgtgtactccaaagtgcagctgagcggcgtgggctgcccccaggggctggccaatggcctccccatcacccatggactatacaagcgcacatcccgctacccgaaggagttagaactgctggtcagtcggcggtcaccctgtggccgggccaacagctcccgagtctggtgggacagcagcttcctgggcggcgtggtacatctggaggctggggaagaggtggtggtccgcgtgcctggaaaccgcctggtcagaccacgtgacggcaccaggtcctatttcggagctttcatggtcactagtggatccggcgcaacaaacttctctctgctgaaacaagccggagatgtcgaagagaatcctggaccgatgaacccaagtgctgccgtcattttctgcctcatcctgctgggtctgagtgggactcaagggatccctctcgcaaggacggtccgctgcaactgcatccatatcgatgacgggccagtgagaatgagggccatagggaagcttgaaatcatccctgcgagcctatcctgcccacgtgttgagatcattgccacgatgaaaaagaatgatgagcagagatgtctgaatccggaatctaagaccatcaagaatttaatgaaagcgtttagccaaaaaaggtctaaaagggctcctagcggtacccagtgcaccaactacgccctgctgaagctggccggcgatgtggagagcaaccccgggcccgctagcatgaacgctacacactgcatcttggctttgcagctcttcctcatggctgtttctggctgttactgccacggcacagtcattgaaagcctagaaagtctgaataactattttaactcaagtggcatagatgtggaagaaaagagtctcttcttggatatctggaggaactggcaaaaggatggtgacatgaaaatcctgcagagccagattatctctttctacctcagactctttgaagtcttgaaagacaatcaggccatcagcaacaacataagcgtcattgaatcacacctgattactaccttcttcagcaacagcaaggcgaaaaaggatgcattcatgagtattgccaagtttgaggtcaacaacccacaggtccagcgccaagcattcaatgagctcatccgagtggtccaccagctgttgccggaatccagcctcaggaagcggaaaaggagtcgctgctgagaattcacgcgttaagtcgacaatcaacctctggattacaaaatttgtgaaagattgactggtattcttaactatgttgctccttttacgctatgtggatacgctgctttaatgcctttgtatcatgctattgcttcccgtatggctttcattttctcctccttgtataaatcctggttgctgtctctttatgaggagttgtggcccgttgtcaggcaacgtggcgtggtgtgcactgtgtttgctgacgcaacccccactggttggggcattgccaccacctgtcagctcctttccgggactttcgctttccccctccctattgccacggcggaactcatcgccgcctgccttgcccgctgctggacaggggctcggctgttgggcactgacaattccgtggtgttgtcggggaaatcatcgtcctttccttggctgctcgcctgtgttgccacctggattctgcgcgggacgtccttctgctacgtcccttcggccctcaatccagcggaccttccttcccgcggcctgctgccggctctgcggcctcttccgcgtcttcgccttcgccctcagacgagtcggatctccctttgggccgcctccccgcgtcgactttaagaccaatgacggccgcaggaacccctagtgatggagttggccactccctctctgcgcgctcgctcgctcactgaggccgggcgaccaaaggtcgcccgacgcccgggctttgcccgggcggcctcagtgagcgagcgagcgcgcagctgcctgcaggggcgcctgatgcggtattttctccttacgcatctgtgcggtatttcacaccgcatacgtcaaagcaaccatagtacgcgccctgtagcggcgcattaagcgcggcgggtgtggtggttacgcgcagcgtgaccgctacacttgccagcgccttagcgcccgctcctttcgctttcttcccttcctttctcgccacgttcgccggctttccccgtcaagctctaaatcgggggctccctttagggttccgatttagtgctttacggcacctcgaccccaaaaaacttgatttgggtgatggttcacgtagtgggccatcgccctgatagacggtttttcgccctttgacgttggagtccacgttctttaatagtggactcttgttccaaactggaacaacactcaactctatctcgggctattcttttgatttataagggattttgccgatttcggtctattggttaaaaaatgagctgatttaacaaaaatttaacgcgaattttaacaaaatattaacgtttacaattttatggtgcactctcagtacaatctgctctgatgccgcatagttaagccagccccgacacccgccaacacccgctgacgcgccctgacgggcttgtctgctcccggcatccgcttacagacaagctgtgaccgtctccgggagctgcatgtgtcagaggttttcaccgtcatcaccgaaacgcgcgagacgaaagggcctcgtgatacgcctatttttataggttaatgtcatgataataatggtttcttagacgtcaggtggcacttttcggggaaatgtgcgcggaacccctatttgtttatttttctaaatacattcaaatatgtatccgctcatgagacaataaccctgataaatgcttcaataatattgaaaaaggaagagtatgagtattcaacatttccgtgtcgcccttattcccttttttgcggcattttgccttcctgtttttgctcacccagaaacgctggtgaaagtaaaagatgctgaagatcagttgggtgcacgagtgggttacatcgaactggatctcaacagcggtaagatccttgagagttttcgccccgaagaacgttttccaatgatgagcacttttaaagttctgctatgtggcgcggtattatcccgtattgacgccgggcaagagcaactcggtcgccgcatacactattctcagaatgacttggttgagtactcaccagtcacagaaaagcatcttacggatggcatgacagtaagagaattatgcagtgctgccataaccatgagtgataacactgcggccaacttacttctgacaacgatcggaggaccgaaggagctaaccgcttttttgcacaacatgggggatcatgtaactcgccttgatcgttgggaaccggagctgaatgaagccataccaaacgacgagcgtgacaccacgatgcctgtagcaatggcaacaacgttgcgcaaactattaactggcgaactacttactctagcttcccggcaacaattaatagactggatggaggcggataaagttgcaggaccacttctgcgctcggcccttccggctggctggtttattgctgataaatctggagccggtgagcgtggaagccgcggtatcattgcagcactggggccagatggtaagccctcccgtatcgtagttatctacacgacggggagtcaggcaactatggatgaacgaaatagacagatcgctgagataggtgcctcactgattaagcattggtaactgtcagaccaagtttactcatatatactttagattgatttaaaacttcatttttaatttaaaaggatctaggtgaagatcctttttgataatctcatgaccaaaatcccttaacgtgagttttcgttccactgagcgtcagaccccgtagaaaagatcaaaggatcttcttgagatcctttttttctgcgcgtaatctgctgcttgcaaacaaaaaaaccaccgctaccagcggtggtttgtttgccggatcaagagctaccaactctttttccgaaggtaactggcttcagcagagcgcagataccaaatactgttcttctagtgtagccgtagttaggccaccacttcaagaactctgtagcaccgcctacatacctcgctctgctaatcctgttaccagtggctgctgccagtggcgataagtcgtgtcttaccgggttggactcaagacgatagttaccggataaggcgcagcggtcgggctgaacggggggttcgtgcacacagcccagcttggagcgaacgacctacaccgaactgagatacctacagcgtgagctatgagaaagcgccacgcttcccgaagggagaaaggcggacaggtatccggtaagcggcagggtcggaacaggagagcgcacgagggagcttccagggggaaacgcctggtatctttatagtcctgtcgggtttcgccacctctgacttgagcgtcgatttttgtgatgctcgtcaggggggcggagcctatggaaaaacgccagcaacgcggcctttttacggttcctggccttttgctggccttttgctcacatgt

SEQ ID NO: 43 - DNA, 6757 bp, Artificial Sequence
  pGW113
cctgcaggcagctgcgcgctcgctcgctcactgaggccgcccgggcgtcgggcgacctttggtcgcccggcctcagtgagcgagcgagcgcgcagagagggagtggccaactccatcactaggggttcctgcggcctctagaaaggatctgcgatcgctccggtgcccgtcagtgggcagagcgcacatcgcccacagtccccgagaagttggggggaggggtcggcaattgaacgggtgcctagagaaggtggcgcggggtaaactgggaaagtgatgtcgtgtactggctccgcctttttcccgagggtgggggagaaccgtatataagtgcagtagtcgccgtgaacgttctttttcgcaacgggtttgccgccagaacacagctgaagcttcgaggggctcgcatctctccttcacgcgcccgccgccctacctgaggccgccatccacgccggttgagtcgcgttctgccgcctcccgcctgtggtgcctcctgaactgcgtccgccgtctaggtaagtttaaagctcaggtcgagaccgggcctttgtccggcgctcccttggagcctacctagactcagccggctctccacgctttgcctgaccctgcttgctcaactctacgtctttgtttcgttttctgttctgcgccgttacagatctggctaactaccggtgccaccatgtgtcctcagaagctaaccatctcctggtttgccatcgttttgctggtgtctccactcatggccatgtgggagctggagaaagacgtttatgttgtagaggtggactggactcccgatgcccctggagaaacagtgaacctcacctgtgacacgcctgaagaagatgacatcacctggacctcagaccagagacatggagtcataggctctggaaagaccctgaccatcactgtcaaagagtttctagatgctggccagtacacctgccacaaaggaggcgagactctgagccactcacatctgctgctccacaagaaggaaaatggaatttggtccactgaaattttaaaaaatttcaaaaacaagactttcctgaagtgtgaagcaccaaattactccggacggttcacgtgctcatggctggtgcaaagaaacatggacttgaagttcaacatcaagagcagtagcagttcccctgactctcgggcagtgacatgtggaatggcgtctctgtctgcagagaaggtcacactggaccaaagggactatgagaagtattcagtgtcctgccaggaggatgtcacctgcccaactgccgaggagaccctgcccattgaactggcgttggaagcacggcagcagaataaatatgagaactacagcaccagcttcttcatcagggacatcatcaaaccagacccgcccaagaacttgcagatgaagcctttgaagaactcacaggtggaggtcagctgggagtaccctgactcctggagcactccccattcctacttctccctcaagttctttgttcgaatccagcgcaagaaagaaaagatgaaggagacagaggaggggtgtaaccagaaaggtgcgttcctcgtagagaagacatctaccgaagtccaatgcaaaggcgggaatgtctgcgtgcaagctcaggatcgctattacaattcctcatgcagcaagtgggcatgtgttccctgcagggtccgatccggcagtggagagggcagaggaagtctgctaacatgcggtgacgtcgaggagaatcctggcccaatggagagtgtggtacagccttcagtgtttgtggtggatggacagacggacatcccattcaggcggctggaacagaaccaccggagacggcgctgtggcactgtccaggtcagcctggccctggtgctgctgctaagtgctgggctggccactcagggctggtttctcctgagactgcatcaacgtcttggagacatagtagctcatctgccagatggaggcaaaggctcctgggagaagctgatacaagatcaacgatctcaccaggccaacccagcagcacatcttacaggagccaacgccagcttgataggtattggtggacctctgttatgggagacacgacttggcctggccttcttgaggggcttgacgtatcatgatggggccctggtgaccatggagcccggttactactatgtgtactccaaagtgcagctgagcggcgtgggctgcccccaggggctggccaatggcctccccatcacccatggactatacaagcgcacatcccgctacccgaaggagttagaactgctggtcagtcggcggtcaccctgtggccgggccaacagctcccgagtctggtgggacagcagcttcctgggcggcgtggtacatctggaggctggggaagaggtggtggtccgcgtgcctggaaaccgcctggtcagaccacgtgacggcaccaggtcctatttcggagctttcatggtcactagtggatccggcgcaacaaacttctctctgctgaaacaagccggagatgtcgaagagaatcctggaccgatgaacccaagtgctgccgtcattttctgcctcatcctgctgggtctgagtgggactcaagggatccctctcgcaaggacggtccgctgcaactgcatccatatcgatgacgggccagtgagaatgagggccatagggaagcttgaaatcatccctgcgagcctatcctgcccacgtgttgagatcattgccacgatgaaaaagaatgatgagcagagatgtctgaatccggaatctaagaccatcaagaatttaatgaaagcgtttagccaaaaaaggtctaaaagggctcctagcggtacccagtgcaccaactacgccctgctgaagctggccggcgatgtggagagcaaccccgggcccgctagcatgaacgctacacactgcatcttggctttgcagctcttcctcatggctgtttctggctgttactgccacggcacagtcattgaaagcctagaaagtctgaataactattttaactcaagtggcatagatgtggaagaaaagagtctcttcttggatatctggaggaactggcaaaaggatggtgacatgaaaatcctgcagagccagattatctctttctacctcagactctttgaagtcttgaaagacaatcaggccatcagcaacaacataagcgtcattgaatcacacctgattactaccttcttcagcaacagcaaggcgaaaaaggatgcattcatgagtattgccaagtttgaggtcaacaacccacaggtccagcgccaagcattcaatgagctcatccgagtggtccaccagctgttgccggaatccagcctcaggaagcggaaaaggagtcgctgctgagaattcacgcgttaagtcgacaatcaacctctggattacaaaatttgtgaaagattgactggtattcttaactatgttgctccttttacgctatgtggatacgctgctttaatgcctttgtatcatgctattgcttcccgtatggctttcattttctcctccttgtataaatcctggttgctgtctctttatgaggagttgtggcccgttgtcaggcaacgtggcgtggtgtgcactgtgtttgctgacgcaacccccactggttggggcattgccaccacctgtcagctcctttccgggactttcgctttccccctccctattgccacggcggaactcatcgccgcctgccttgcccgctgctggacaggggctcggctgttgggcactgacaattccgtggtgttgtcggggaaatcatcgtcctttccttggctgctcgcctgtgttgccacctggattctgcgcgggacgtccttctgctacgtcccttcggccctcaatccagcggaccttccttcccgcggcctgctgccggctctgcggcctcttccgcgtcttcgccttcgccctcagacgagtcggatctccctttgggccgcctccccgcgtcgactttaagaccaatgacggccgcaggaacccctagtgatggagttggccactccctctctgcgcgctcgctcgctcactgaggccgggcgaccaaaggtcgcccgacgcccgggctttgcccgggcggcctcagtgagcgagcgagcgcgcagctgcctgcaggggcgcctgatgcggtattttctccttacgcatctgtgcggtatttcacaccgcatacgtcaaagcaaccatagtacgcgccctgtagcggcgcattaagcgcggcgggtgtggtggttacgcgcagcgtgaccgctacacttgccagcgccttagcgcccgctcctttcgctttcttcccttcctttctcgccacgttcgccggctttccccgtcaagctctaaatcgggggctccctttagggttccgatttagtgctttacggcacctcgaccccaaaaaacttgatttgggtgatggttcacgtagtgggccatcgccctgatagacggtttttcgccctttgacgttggagtccacgttctttaatagtggactcttgttccaaactggaacaacactcaactctatctcgggctattcttttgatttataagggattttgccgatttcggtctattggttaaaaaatgagctgatttaacaaaaatttaacgcgaattttaacaaaatattaacgtttacaattttatggtgcactctcagtacaatctgctctgatgccgcatagttaagccagccccgacacccgccaacacccgctgacgcgccctgacgggcttgtctgctcccggcatccgcttacagacaagctgtgaccgtctccgggagctgcatgtgtcagaggttttcaccgtcatcaccgaaacgcgcgagacgaaagggcctcgtgatacgcctatttttataggttaatgtcatgataataatggtttcttagacgtcaggtggcacttttcggggaaatgtgcgcggaacccctatttgtttatttttctaaatacattcaaatatgtatccgctcatgagacaataaccctgataaatgcttcaataatattgaaaaaggaagagtatgagtattcaacatttccgtgtcgcccttattcccttttttgcggcattttgccttcctgtttttgctcacccagaaacgctggtgaaagtaaaagatgctgaagatcagttgggtgcacgagtgggttacatcgaactggatctcaacagcggtaagatccttgagagttttcgccccgaagaacgttttccaatgatgagcacttttaaagttctgctatgtggcgcggtattatcccgtattgacgccgggcaagagcaactcggtcgccgcatacactattctcagaatgacttggttgagtactcaccagtcacagaaaagcatcttacggatggcatgacagtaagagaattatgcagtgctgccataaccatgagtgataacactgcggccaacttacttctgacaacgatcggaggaccgaaggagctaaccgcttttttgcacaacatgggggatcatgtaactcgccttgatcgttgggaaccggagctgaatgaagccataccaaacgacgagcgtgacaccacgatgcctgtagcaatggcaacaacgttgcgcaaactattaactggcgaactacttactctagcttcccggcaacaattaatagactggatggaggcggataaagttgcaggaccacttctgcgctcggcccttccggctggctggtttattgctgataaatctggagccggtgagcgtggaagccgcggtatcattgcagcactggggccagatggtaagccctcccgtatcgtagttatctacacgacggggagtcaggcaactatggatgaacgaaatagacagatcgctgagataggtgcctcactgattaagcattggtaactgtcagaccaagtttactcatatatactttagattgatttaaaacttcatttttaatttaaaaggatctaggtgaagatcctttttgataatctcatgaccaaaatcccttaacgtgagttttcgttccactgagcgtcagaccccgtagaaaagatcaaaggatcttcttgagatcctttttttctgcgcgtaatctgctgcttgcaaacaaaaaaaccaccgctaccagcggtggtttgtttgccggatcaagagctaccaactctttttccgaaggtaactggcttcagcagagcgcagataccaaatactgttcttctagtgtagccgtagttaggccaccacttcaagaactctgtagcaccgcctacatacctcgctctgctaatcctgttaccagtggctgctgccagtggcgataagtcgtgtcttaccgggttggactcaagacgatagttaccggataaggcgcagcggtcgggctgaacggggggttcgtgcacacagcccagcttggagcgaacgacctacaccgaactgagatacctacagcgtgagctatgagaaagcgccacgcttcccgaagggagaaaggcggacaggtatccggtaagcggcagggtcggaacaggagagcgcacgagggagcttccagggggaaacgcctggtatctttatagtcctgtcgggtttcgccacctctgacttgagcgtcgatttttgtgatgctcgtcaggggggcggagcctatggaaaaacgccagcaacgcggcctttttacggttcctggccttttgctggccttttgctcacatgt

SEQ ID NO: 44 - DNA, 7309 bp, Artificial Sequence
  pGW114
cctgcaggcagctgcgcgctcgctcgctcactgaggccgcccgggcgtcgggcgacctttggtcgcccggcctcagtgagcgagcgagcgcgcagagagggagtggccaactccatcactaggggttcctgcggcctctagaaaggatctgcgatcgctccggtgcccgtcagtgggcagagcgcacatcgcccacagtccccgagaagttggggggaggggtcggcaattgaacgggtgcctagagaaggtggcgcggggtaaactgggaaagtgatgtcgtgtactggctccgcctttttcccgagggtgggggagaaccgtatataagtgcagtagtcgccgtgaacgttctttttcgcaacgggtttgccgccagaacacagctgaagcttcgaggggctcgcatctctccttcacgcgcccgccgccctacctgaggccgccatccacgccggttgagtcgcgttctgccgcctcccgcctgtggtgcctcctgaactgcgtccgccgtctaggtaagtttaaagctcaggtcgagaccgggcctttgtccggcgctcccttggagcctacctagactcagccggctctccacgctttgcctgaccctgcttgctcaactctacgtctttgtttcgttttctgttctgcgccgttacagatctggctaactaccggtgccaccatggcttgcaattgtcagttgatgcaggatacaccactcctcaagtttccatgtccaaggctcattcttctctttgtgctgctgattcgtctttcacaagtgtcttcagatgttgatgaacaactgtccaagtcagtgaaagataaggtattgctgccttgccgttacaactctcctcatgaagatgagtctgaagaccgaatctactggcaaaaacatgacaaagtggtgctgtctgtcattgctgggaaactaaaagtgtggcccgagtataagaaccggactttatatgacaacactacctactctcttatcatcctgggcctggtcctttcagaccggggcacatacagctgtgtcgttcaaaagaaggaaagaggaacgtatgaagttaaacacttggctttagtaaagttgtccatcaaagctgacttctctacccccaacataactgagtctggaaacccatctgcagacactaaaaggattacctgctttgcttccgggggtttcccaaagcctcgcttctcttggttggaaaatggaagagaattacctggcatcaatacgacaatttcccaggatcctgaatctgaattgtacaccattagtagccaactagatttcaatacgactcgcaaccacaccattaagtgtctcattaaatatggagatgctcacgtgtcagaggacttcacctgggaaaaacccccagaagaccctcctgatagcaagaacacacttgtgctctttggggcaggattcggcgcagtaataacagtcgtcgtcatcgttgtcatcatcaaatgcttctgtaagcacagaagctgtttcagaagaaatgaggcaagcagagaaacaaacaacagccttaccttcgggcctgaagaagcattagctgaacagaccgtcttccttcgtacgggcagtggagagggcagaggaagtctgctaacatgcggtgacgtcgaggagaatcctggcccaatggagagtgtggtacagccttcagtgtttgtggtggatggacagacggacatcccattcaggcggctggaacagaaccaccggagacggcgctgtggcactgtccaggtcagcctggccctggtgctgctgctaagtgctgggctggccactcagggctggtttctcctgagactgcatcaacgtcttggagacatagtagctcatctgccagatggaggcaaaggctcctgggagaagctgatacaagatcaacgatctcaccaggccaacccagcagcacatcttacaggagccaacgccagcttgataggtattggtggacctctgttatgggagacacgacttggcctggccttcttgaggggcttgacgtatcatgatggggccctggtgaccatggagcccggttactactatgtgtactccaaagtgcagctgagcggcgtgggctgcccccaggggctggccaatggcctccccatcacccatggactatacaagcgcacatcccgctacccgaaggagttagaactgctggtcagtcggcggtcaccctgtggccgggccaacagctcccgagtctggtgggacagcagcttcctgggcggcgtggtacatctggaggctggggaagaggtggtggtccgcgtgcctggaaaccgcctggtcagaccacgtgacggcaccaggtcctatttcggagctttcatggtcactagtggatccggcgcaacaaacttctctctgctgaaacaagccggagatgtcgaagagaatcctggaccgatggaccagcacacacttgatgtggaggataccgcggatgccagacatccagcaggtacttcgtgcccctcggatgcggcgctcctcagagataccgggctcctcgcggacgctgcgctcctctcagatactgtgcgccccacaaatgccgcgctccccacggatgctgcctaccctgcggttaatgttcgggatcgcgaggccgcgtggccgcctgcactgaacttctgttcccgccacccaaagctctatggcctagtcgctttggttttgctgcttctgatcgccgcctgtgttcctatcttcacccgcaccgagcctcggccagcgctcacaatcaccacctcgcccaacctgggtacccgagagaataatgcagaccaggtcacccctgtttcccacattggctgccccaacactacacaacagggctctcctgtgttcgccaagctactggctaaaaaccaagcatcgttgtgcaatacaactctgaactggcacagccaagatggagctgggagctcatacctatctcaaggtctgaggtacgaagaagacaaaaaggagttggtggtagacagtcccgggctctactacgtatttttggaactgaagctcagtccaacattcacaaacacaggccacaaggtgcagggctgggtctctcttgttttgcaagcaaagcctcaggtagatgactttgacaacttggccctgacagtggaactgttcccttgctccatggagaacaagttagtggaccgttcctggagtcaactgttgctcctgaaggctggccaccgcctcagtgtgggtctgagggcttatctgcatggagcccaggatgcatacagagactgggagctgtcttatcccaacaccaccagctttggactctttcttgtgaaacccgacaacccatgggaaagcggtacccagtgcaccaactacgccctgctgaagctggccggcgatgtggagagcaaccccgggcccgctagcatgaacgctacacactgcatcttggctttgcagctcttcctcatggctgtttctggctgttactgccacggcacagtcattgaaagcctagaaagtctgaataactattttaactcaagtggcatagatgtggaagaaaagagtctcttcttggatatctggaggaactggcaaaaggatggtgacatgaaaatcctgcagagccagattatctctttctacctcagactctttgaagtcttgaaagacaatcaggccatcagcaacaacataagcgtcattgaatcacacctgattactaccttcttcagcaacagcaaggcgaaaaaggatgcattcatgagtattgccaagtttgaggtcaacaacccacaggtgcagcgccaagcattcaatgagctcatccgagtggtccaccagctgttgccggaatccagcctcaggaagcggaaaaggagtcgctgctgagaattcacgcgttaagtcgacaatcaacctctggattacaaaatttgtgaaagattgactggtattcttaactatgttgctccttttacgctatgtggatacgctgctttaatgcctttgtatcatgctattgcttcccgtatggctttcattttctcctccttgtataaatcctggttgctgtctctttatgaggagttgtggcccgttgtcaggcaacgtggcgtggtgtgcactgtgtttgctgacgcaacccccactggttggggcattgccaccacctgtcagctcctttccgggactttcgctttccccctccctattgccacggcggaactcatcgccgcctgccttgcccgctgctggacaggggctcggctgttgggcactgacaattccgtggtgttgtcggggaaatcatcgtcctttccttggctgctcgcctgtgttgccacctggattctgcgcgggacgtccttctgctacgtcccttcggccctcaatccagcggaccttccttcccgcggcctgctgccggctctgcggcctcttccgcgtcttcgccttcgccctcagacgagtcggatctccctttgggccgcctccccgcgtcgactttaagaccaatgacggccgcaggaacccctagtgatggagttggccactccctctctgcgcgctcgctcgctcactgaggccgggcgaccaaaggtcgcccgacgcccgggctttgcccgggcggcctcagtgagcgagcgagcgcgcagctgcctgcaggggcgcctgatgcggtattttctccttacgcatctgtgcggtatttcacaccgcatacgtcaaagcaaccatagtacgcgccctgtagcggcgcattaagcgcggcgggtgtggtggttacgcgcagcgtgaccgctacacttgccagcgccttagcgcccgctcctttcgctttcttcccttcctttctcgccacgttcgccggctttccccgtcaagctctaaatcgggggctccctttagggttccgatttagtgctttacggcacctcgaccccaaaaaacttgatttgggtgatggttcacgtagtgggccatcgccctgatagacggtttttcgccctttgacgttggagtccacgttctttaatagtggactcttgttccaaactggaacaacactcaactctatctcgggctattcttttgatttataagggattttgccgatttcggtctattggttaaaaaatgagctgatttaacaaaaatttaacgcgaattttaacaaaatattaacgtttacaattttatggtgcactctcagtacaatctgctctgatgccgcatagttaagccagccccgacacccgccaacacccgctgacgcgccctgacgggcttgtctgctcccggcatccgcttacagacaagctgtgaccgtctccgggagctgcatgtgtcagaggttttcaccgtcatcaccgaaacgcgcgagacgaaagggcctcgtgatacgcctatttttataggttaatgtcatgataataatggtttcttagacgtcaggtggcacttttcggggaaatgtgcgcggaacccctatttgtttatttttctaaatacattcaaatatgtatccgctcatgagacaataaccctgataaatgcttcaataatattgaaaaaggaagagtatgagtattcaacatttccgtgtcgcccttattcccttttttgcggcattttgccttcctgtttttgctcacccagaaacgctggtgaaagtaaaagatgctgaagatcagttgggtgcacgagtgggttacatcgaactggatctcaacagcggtaagatccttgagagttttcgccccgaagaacgttttccaatgatgagcacttttaaagttctgctatgtggcgcggtattatcccgtattgacgccgggcaagagcaactcggtcgccgcatacactattctcagaatgacttggttgagtactcaccagtcacagaaaagcatcttacggatggcatgacagtaagagaattatgcagtgctgccataaccatgagtgataacactgcggccaacttacttctgacaacgatcggaggaccgaaggagctaaccgcttttttgcacaacatgggggatcatgtaactcgccttgatcgttgggaaccggagctgaatgaagccataccaaacgacgagcgtgacaccacgatgcctgtagcaatggcaacaacgttgcgcaaactattaactggcgaactacttactctagcttcccggcaacaattaatagactggatggaggcggataaagttgcaggaccacttctgcgctcggcccttccggctggctggtttattgctgataaatctggagccggtgagcgtggaagccgcggtatcattgcagcactggggccagatggtaagccctcccgtatcgtagttatctacacgacggggagtcaggcaactatggatgaacgaaatagacagatcgctgagataggtgcctcactgattaagcattggtaactgtcagaccaagtttactcatatatactttagattgatttaaaacttcatttttaatttaaaaggatctaggtgaagatcctttttgataatctcatgaccaaaatcccttaacgtgagttttcgttccactgagcgtcagaccccgtagaaaagatcaaaggatcttcttgagatcctttttttctgcgcgtaatctgctgcttgcaaacaaaaaaaccaccgctaccagcggtggtttgtttgccggatcaagagctaccaactctttttccgaaggtaactggcttcagcagagcgcagataccaaatactgttcttctagtgtagccgtagttaggccaccacttcaagaactctgtagcaccgcctacatacctcgctctgctaatcctgttaccagtggctgctgccagtggcgataagtcgtgtcttaccgggttggactcaagacgatagttaccggataaggcgcagcggtcgggctgaacggggggttcgtgcacacagcccagcttggagcgaacgacctacaccgaactgagatacctacagcgtgagctatgagaaagcgccacgcttcccgaagggagaaaggcggacaggtatccggtaagcggcagggtcggaacaggagagcgcacgagggagcttccagggggaaacgcctggtatctttatagtcctgtcgggtttcgccacctctgacttgagcgtcgatttttgtgatgctcgtcaggggggcggagcctatggaaaaacgccagcaacgcggcctttttacggttcctggccttttgctggccttttgctcacatgt

SEQ ID NO: 45 - DNA, 7390 bp, Artificial Sequence
  pGW115
cctgcaggcagctgcgcgctcgctcgctcactgaggccgcccgggcgtcgggcgacctttggtcgcccggcctcagtgagcgagcgagcgcgcagagagggagtggccaactccatcactaggggttcctgcggcctctagaaaggatctgcgatcgctccggtgcccgtcagtgggcagagcgcacatcgcccacagtccccgagaagttggggggaggggtcggcaattgaacgggtgcctagagaaggtggcgcggggtaaactgggaaagtgatgtcgtgtactggctccgcctttttcccgagggtgggggagaaccgtatataagtgcagtagtcgccgtgaacgttctttttcgcaacgggtttgccgccagaacacagctgaagcttcgaggggctcgcatctctccttcacgcgcccgccgccctacctgaggccgccatccacgccggttgagtcgcgttctgccgcctcccgcctgtggtgcctcctgaactgcgtccgccgtctaggtaagtttaaagctcaggtcgagaccgggcctttgtccggcgctcccttggagcctacctagactcagccggctctccacgctttgcctgaccctgcttgctcaactctacgtctttgtttcgttttctgttctgcgccgttacagatctggctaactaccggtgccaccatgtgtcctcagaagctaaccatctcctggtttgccatcgttttgctggtgtctccactcatggccatgtgggagctggagaaagacgtttatgttgtagaggtggactggactcccgatgcccctggagaaacagtgaacctcacctgtgacacgcctgaagaagatgacatcacctggacctcagaccagagacatggagtcataggctctggaaagaccctgaccatcactgtcaaagagtttctagatgctggccagtacacctgccacaaaggaggcgagactctgagccactcacatctgctgctccacaagaaggaaaatggaatttggtccactgaaattttaaaaaatttcaaaaacaagactttcctgaagtgtgaagcaccaaattactccggacggttcacgtgctcatggctggtgcaaagaaacatggacttgaagttcaacatcaagagcagtagcagttcccctgactctcgggcagtgacatgtggaatggcgtctctgtctgcagagaaggtcacactggaccaaagggactatgagaagtattcagtgtcctgccaggaggatgtcacctgcccaactgccgaggagaccctgcccattgaactggcgttggaagcacggcagcagaataaatatgagaactacagcaccagcttcttcatcagggacatcatcaaaccagacccgcccaagaacttgcagatgaagcctttgaagaactcacaggtggaggtcagctgggagtaccctgactcctggagcactccccattcctacttctccctcaagttctttgttcgaatccagcgcaagaaagaaaagatgaaggagacagaggaggggtgtaaccagaaaggtgcgttcctcgtagagaagacatctaccgaagtccaatgcaaaggcgggaatgtctgcgtgcaagctcaggatcgctattacaattcctcatgcagcaagtgggcatgtgttccctgcagggtccgatccggcagtggagagggcagaggaagtctgctaacatgcggtgacgtcgaggagaatcctggcccaatggagagtgtggtacagccttcagtgtttgtggtggatggacagacggacatcccattcaggcggctggaacagaaccaccggagacggcgctgtggcactgtccaggtcagcctggccctggtgctgctgctaagtgctgggctggccactcagggctggtttctcctgagactgcatcaacgtcttggagacatagtagctcatctgccagatggaggcaaaggctcctgggagaagctgatacaagatcaacgatctcaccaggccaacccagcagcacatcttacaggagccaacgccagcttgataggtattggtggacctctgttatgggagacacgacttggcctggccttcttgaggggcttgacgtatcatgatggggccctggtgaccatggagcccggttactactatgtgtactccaaagtgcagctgagcggcgtgggctgcccccaggggctggccaatggcctccccatcacccatggactatacaagcgcacatcccgctacccgaaggagttagaactgctggtcagtcggcggtcaccctgtggccgggccaacagctcccgagtctggtgggacagcagcttcctgggcggcgtggtacatctggaggctggggaagaggtggtggtccgcgtgcctggaaaccgcctggtcagaccacgtgacggcaccaggtcctatttcggagctttcatggtcactagtggatccggcgcaacaaacttctctctgctgaaacaagccggagatgtcgaagagaatcctggaccgatggaccagcacacacttgatgtggaggataccgcggatgccagacatccagcaggtacttcgtgcccctcggatgcggcgctcctcagagataccgggctcctcgcggacgctgcgctcctctcagatactgtgcgccccacaaatgccgcgctccccacggatgctgcctaccctgcggttaatgttcgggatcgcgaggccgcgtggccgcctgcactgaacttctgttcccgccacccaaagctctatggcctagtcgctttggttttgctgcttctgatcgccgcctgtgttcctatcttcacccgcaccgagcctcggccagcgctcacaatcaccacctcgcccaacctgggtacccgagagaataatgcagaccaggtcacccctgtttcccacattggctgccccaacactacacaacagggctctcctgtgttcgccaagctactggctaaaaaccaagcatcgttgtgcaatacaactctgaactggcacagccaagatggagctgggagctcatacctatctcaaggtctgaggtacgaagaagacaaaaaggagttggtggtagacagtcccgggctctactacgtatttttggaactgaagctcagtccaacattcacaaacacaggccacaaggtgcagggctgggtctctcttgttttgcaagcaaagcctcaggtagatgactttgacaacttggccctgacagtggaactgttcccttgctccatggagaacaagttagtggaccgttcctggagtcaactgttgctcctgaaggctggccaccgcctcagtgtgggtctgagggcttatctgcatggagcccaggatgcatacagagactgggagctgtcttatcccaacaccaccagctttggactctttcttgtgaaacccgacaacccatgggaaagcggtacccagtgcaccaactacgccctgctgaagctggccggcgatgtggagagcaaccccgggcccgctagcatgaacgctacacactgcatcttggctttgcagctcttcctcatggctgtttctggctgttactgccacggcacagtcattgaaagcctagaaagtctgaataactattttaactcaagtggcatagatgtggaagaaaagagtctcttcttggatatctggaggaactggcaaaaggatggtgacatgaaaatcctgcagagccagattatctctttctacctcagactctttgaagtcttgaaagacaatcaggccatcagcaacaacataagcgtcattgaatcacacctgattactaccttcttcagcaacagcaaggcgaaaaaggatgcattcatgagtattgccaagtttgaggtcaacaacccacaggtccagcgccaagcattcaatgagctcatccgagtggtccaccagctgttgccggaatccagcctcaggaagcggaaaaggagtcgctgctgagaattcacgcgttaagtcgacaatcaacctctggattacaaaatttgtgaaagattgactggtattcttaactatgttgctccttttacgctatgtggatacgctgctttaatgcctttgtatcatgctattgcttcccgtatggctttcattttctcctccttgtataaatcctggttgctgtctctttatgaggagttgtggcccgttgtcaggcaacgtggcgtggtgtgcactgtgtttgctgacgcaacccccactggttggggcattgccaccacctgtcagctcctttccgggactttcgctttccccctccctattgccacggcggaactcatcgccgcctgccttgcccgctgctggacaggggctcggctgttgggcactgacaattccgtggtgttgtcggggaaatcatcgtcctttccttggctgctcgcctgtgttgccacctggattctgcgcgggacgtccttctgctacgtcccttcggccctcaatccagcggaccttccttcccgcggcctgctgccggctctgcggcctcttccgcgtcttcgccttcgccctcagacgagtcggatctccctttgggccgcctccccgcgtcgactttaagaccaatgacggccgcaggaacccctagtgatggagttggccactccctctctgcgcgctcgctcgctcactgaggccgggcgaccaaaggtcgcccgacgcccgggctttgcccgggcggcctcagtgagcgagcgagcgcgcagctgcctgcaggggcgcctgatgcggtattttctccttacgcatctgtgcggtatttcacaccgcatacgtcaaagcaaccatagtacgcgccctgtagcggcgcattaagcgcggcgggtgtggtggttacgcgcagcgtgaccgctacacttgccagcgccttagcgcccgctcctttcgctttcttcccttcctttctcgccacgttcgccggctttccccgtcaagctctaaatcgggggctccctttagggttccgatttagtgctttacggcacctcgaccccaaaaaacttgatttgggtgatggttcacgtagtgggccatcgccctgatagacggtttttcgccctttgacgttggagtccacgttctttaatagtggactcttgttccaaactggaacaacactcaactctatctcgggctattcttttgatttataagggattttgccgatttcggtctattggttaaaaaatgagctgatttaacaaaaatttaacgcgaattttaacaaaatattaacgtttacaattttatggtgcactctcagtacaatctgctctgatgccgcatagttaagccagccccgacacccgccaacacccgctgacgcgccctgacgggcttgtctgctcccggcatccgcttacagacaagctgtgaccgtctccgggagctgcatgtgtcagaggttttcaccgtcatcaccgaaacgcgcgagacgaaagggcctcgtgatacgcctatttttataggttaatgtcatgataataatggtttcttagacgtcaggtggcacttttcggggaaatgtgcgcggaacccctatttgtttatttttctaaatacattcaaatatgtatccgctcatgagacaataaccctgataaatgcttcaataatattgaaaaaggaagagtatgagtattcaacatttccgtgtcgcccttattcccttttttgcggcattttgccttcctgtttttgctcacccagaaacgctggtgaaagtaaaagatgctgaagatcagttgggtgcacgagtgggttacatcgaactggatctcaacagcggtaagatccttgagagttttcgccccgaagaacgttttccaatgatgagcacttttaaagttctgctatgtggcgcggtattatcccgtattgacgccgggcaagagcaactcggtcgccgcatacactattctcagaatgacttggttgagtactcaccagtcacagaaaagcatcttacggatggcatgacagtaagagaattatgcagtgctgccataaccatgagtgataacactgcggccaacttacttctgacaacgatcggaggaccgaaggagctaaccgcttttttgcacaacatgggggatcatgtaactcgccttgatcgttgggaaccggagctgaatgaagccataccaaacgacgagcgtgacaccacgatgcctgtagcaatggcaacaacgttgcgcaaactattaactggcgaactacttactctagcttcccggcaacaattaatagactggatggaggcggataaagttgcaggaccacttctgcgctcggcccttccggctggctggtttattgctgataaatctggagccggtgagcgtggaagccgcggtatcattgcagcactggggccagatggtaagccctcccgtatcgtagttatctacacgacggggagtcaggcaactatggatgaacgaaatagacagatcgctgagataggtgcctcactgattaagcattggtaactgtcagaccaagtttactcatatatactttagattgatttaaaacttcatttttaatttaaaaggatctaggtgaagatcctttttgataatctcatgaccaaaatcccttaacgtgagttttcgttccactgagcgtcagaccccgtagaaaagatcaaaggatcttcttgagatcctttttttctgcgcgtaatctgctgcttgcaaacaaaaaaaccaccgctaccagcggtggtttgtttgccggatcaagagctaccaactctttttccgaaggtaactggcttcagcagagcgcagataccaaatactgttcttctagtgtagccgtagttaggccaccacttcaagaactctgtagcaccgcctacatacctcgctctgctaatcctgttaccagtggctgctgccagtggcgataagtcgtgtcttaccgggttggactcaagacgatagttaccggataaggcgcagcggtcgggctgaacggggggttcgtgcacacagcccagcttggagcgaacgacctacaccgaactgagatacctacagcgtgagctatgagaaagcgccacgcttcccgaagggagaaaggcggacaggtatccggtaagcggcagggtcggaacaggagagcgcacgagggagcttccagggggaaacgcctggtatctttatagtcctgtcgggtttcgccacctctgacttgagcgtcgatttttgtgatgctcgtcaggggggcggagcctatggaaaaacgccagcaacgcggcctttttacggttcctggccttttgctggccttttgctcacatgt

SEQ ID NO: 46 - DNA, 6728 bp, Artificial Sequence; identical to SEQ ID NO: 35
  pGW118

SEQ ID NO: 47 - DNA, 6729 bp, Artificial Sequence
  pGW119
cctgcaggcagctgcgcgctcgctcgctcactgaggccgcccgggcgtcgggcgacctttggtcgcccggcctcagtgagcgagcgagcgcgcagagagggagtggccaactccatcactaggggttcctgcggcctctagaaaggatctgcgatcgctccggtgcccgtcagtgggcagagcgcacatcgcccacagtccccgagaagttggggggaggggtcggcaattgaacgggtgcctagagaaggtggcgcggggtaaactgggaaagtgatgtcgtgtactggctccgcctttttcccgagggtgggggagaaccgtatataagtgcagtagtcgccgtgaacgttctttttcgcaacgggtttgccgccagaacacagctgaagcttcgaggggctcgcatctctccttcacgcgcccgccgccctacctgaggccgccatccacgccggttgagtcgcgttctgccgcctcccgcctgtggtgcctcctgaactgcgtccgccgtctaggtaagtttaaagctcaggtcgagaccgggcctttgtccggcgctcccttggagcctacctagactcagccggctctccacgctttgcctgaccctgcttgctcaactctacgtctttgtttcgttttctgttctgcgccgttacagatctggctaactaccggtgccaccatgaacgctacacactgcatcttggctttgcagctcttcctcatggctgtttctggctgttactgccacggcacagtcattgaaagcctagaaagtctgaataactattttaactcaagtggcatagatgtggaagaaaagagtctcttcttggatatctggaggaactggcaaaaggatggtgacatgaaaatcctgcagagccagattatctctttctacctcagactctttgaagtcttgaaagacaatcaggccatcagcaacaacataagcgtcattgaatcacacctgattactaccttcttcagcaacagcaaggcgaaaaaggatgcattcatgagtattgccaagtttgaggtcaacaacccacaggtccagcgccaagcattcaatgagctcatccgagtggtccaccagctgttgccggaatccagcctcaggaagcggaaaaggagtcgctgctgaatccggcgcaacaaacttctctctgctgaaacaagccggagatgtcgaagagaatcctggaccgatggcttgcaattgtcagttgatgcaggatacaccactcctcaagtttccatgtccaaggctcattcttctctttgtgctgctgattcgtctttcacaagtgtcttcagatgttgatgaacaactgtccaagtcagtgaaagataaggtattgctgccttgccgttacaactctcctcatgaagatgagtctgaagaccgaatctactggcaaaaacatgacaaagtggtgctgtctgtcattgttgggaaactaaaagtgtggcccgagtataagaaccggactttatatgacaacactacctactctcttatcatcctgggcctggtcctttcagaccggggcacatacagctgtgtcgttcaaaagaaggaaagaggaacgtatgaagttaaacacttggctttagtaaagttgtccatcaaagctgacttctctacccccaacataactgagtctggaaacccatctgcagacactaaaaggattacctgctttgcttccgggggtttcccaaagcctcgcttctcttggttggaaaatggaagagaattacctggcatcaatacgacaatttcccaggatcctgaatctgaattgtacaccattagtagccaactagatttcaatacgactcgcaaccacaccattaagtgtctcattaaatatggagatgctcacgtgtcagaggacttcacctgggaaaaacccccagaagaccctcctgatagcaagaacacacttgtgctctttggggcaggattcggcgcagtaataacagtcgtcgtcatcgttgtcatcatcaaatgcttctgtaagcacagaagctgtttcagaagaaatgaggcaagcagagaaacaaacaacagccttaccttcgggcctgaagaagcattagctgaacagaccgtcttccttcgtacgggcagtggagagggcagaggaagtctgctaacatgcggtgacgtcgaggagaatcctggcccaatggagagtgtggtacagccttcagtgtttgtggtggatggacagacggacatcccattcaggcggctggaacagaaccaccggagacggcgctgtggcactgtccaggtcagcctggccctggtgctgctgctaggtgctgggctggccactcagggctggtttctcctgagactgcatcaacgtcttggagacatagtagctcatctgccagatggaggcaaaggctcctgggagaagctgatacaagatcaacgatctcaccaggccaacccagcagcacatcttacaggagccaacgccagcttgataggtattggtggacctctgttatgggagacacgacttggcctggccttcttgaggggcttgacgtatcatgatggggccctggtgaccatggagcccggttactactatgtgtactccaaagtgcagctgagcggcgtgggctgcccccaggggctggccaatggcctccccatcacccatggactatacaagcgcacatcccgctacccgaaggagttagaactgctggtcagtcggcggtcaccctgtggccgggccaacagctcccgagtctggtgggacagcagcttcctgggcggcgtggtacatctggaggctggggaagaggtggtggtccgcgtgcctggaaaccgcctggtcagaccacgtgacggcaccaggtcctatttcggagctttcatggtcactagcagcggtacccagtgcaccaactacgccctgctgaagctggccggcgatgtggagagcaaccccgggcccatggaccagcacacacttgatgtggaggataccgcggatgccagacatccagcaggtacttcgtgcccctcggatgcggcgctcctcagagataccgggctcctcgcggacgctgcgctcctctcagatactgtgcgccccacaaatgccgcgctccccacggatgctgcctaccctgcggttaatgttcgggatcgcgaggccgcgtggccgcctgcactgaacttctgttcccgccacccaaagctctatggcctagtcgctttggttttgctgcttctgatcgccgcctgtgttcctatcttcacccgcaccgagcctcggccagcgctcacaatcaccacctcgcccaacctgggtacccgagagaataatgcagaccaggtcacccctgtttcccacattggctgccccaacactacacaacagggctctcctgtgttcgccaagctactggctaaaaaccaagcatcgttgtgcaatacaactctgaactggcacagccaagatggagctgggagctcatacctatctcaaggtctgaggtacgaagaagacaaaaaggagttggtggtagacagtcccgggctctactacgtatttttggaactgaagctcagtccaacattcacaaacacaggccacaaggtgcagggctgggtctctcttgttttgcaagcaaagcctcaggtagatgactttgacaacttggccctgacagtggaactgttcccttgctccatggagaacaagttagtggaccgttcctggagtcaactgttgctcctgaaggctggccaccgcctcagtgtgggtctgagggcttatctgcatggagcccaggatgcatacagagactgggagctgtcttatcccaacaccaccagctttggactctttcttgtgaaacccgacaacccatgggaatgagaattcaataaaagatctttattttcattagatctgtgtgttggttttttgtgtgcggccgcaggaacccctagtgatggagttggccactccctctctgcgcgctcgctcgctcactgaggccgggcgaccaaaggtcgcccgacgcccgggctttgcccgggcggcctcagtgagcgagcgagcgcgcagctgcctgcaggggcgcctgatgcggtattttctccttacgcatctgtgcggtatttcacaccgcatacgtcaaagcaaccatagtacgcgccctgtagcggcgcattaagcgcggcgggtgtggtggttacgcgcagcgtgaccgctacacttgccagcgccttagcgcccgctcctttcgctttcttcccttcctttctcgccacgttcgccggctttccccgtcaagctctaaatcgggggctccctttagggttccgatttagtgctttacggcacctcgaccccaaaaaacttgatttgggtgatggttcacgtagtgggccatcgccctgatagacggtttttcgccctttgacgttggagtccacgttctttaatagtggactcttgttccaaactggaacaacactcaactctatctcgggctattcttttgatttataagggattttgccgatttcggtctattggttaaaaaatgagctgatttaacaaaaatttaacgcgaattttaacaaaatattaacgtttacaattttatggtgcactctcagtacaatctgctctgatgccgcatagttaagccagccccgacacccgccaacacccgctgacgcgccctgacgggcttgtctgctcccggcatccgcttacagacaagctgtgaccgtctccgggagctgcatgtgtcagaggttttcaccgtcatcaccgaaacgcgcgagacgaaagggcctcgtgatacgcctatttttataggttaatgtcatgataataatggtttcttagacgtcaggtggcacttttcggggaaatgtgcgcggaacccctatttgtttatttttctaaatacattcaaatatgtatccgctcatgagacaataaccctgataaatgcttcaataatattgaaaaaggaagagtatgagtattcaacatttccgtgtcgcccttattcccttttttgcggcattttgccttcctgtttttgctcacccagaaacgctggtgaaagtaaaagatgctgaagatcagttgggtgcacgagtgggttacatcgaactggatctcaacagcggtaagatccttgagagttttcgccccgaagaacgttttccaatgatgagcacttttaaagttctgctatgtggcgcggtattatcccgtattgacgccgggcaagagcaactcggtcgccgcatacactattctcagaatgacttggttgagtactcaccagtcacagaaaagcatcttacggatggcatgacagtaagagaattatgcagtgctgccataaccatgagtgataacactgcggccaacttacttctgacaacgatcggaggaccgaaggagctaaccgcttttttgcacaacatgggggatcatgtaactcgccttgatcgttgggaaccggagctgaatgaagccataccaaacgacgagcgtgacaccacgatgcctgtagcaatggcaacaacgttgcgcaaactattaactggcgaactacttactctagcttcccggcaacaattaatagactggatggaggcggataaagttgcaggaccacttctgcgctcggcccttccggctggctggtttattgctgataaatctggagccggtgagcgtggaagccgcggtatcattgcagcactggggccagatggtaagccctcccgtatcgtagttatctacacgacggggagtcaggcaactatggatgaacgaaatagacagatcgctgagataggtgcctcactgattaagcattggtaactgtcagaccaagtttactcatatatactttagattgatttaaaacttcatttttaatttaaaaggatctaggtgaagatcctttttgataatctcatgaccaaaatcccttaacgtgagttttcgttccactgagcgtcagaccccgtagaaaagatcaaaggatcttcttgagatcctttttttctgcgcgtaatctgctgcttgcaaacaaaaaaaccaccgctaccagcggtggtttgtttgccggatcaagagctaccaactctttttccgaaggtaactggcttcagcagagcgcagataccaaatactgttcttctagtgtagccgtagttaggccaccacttcaagaactctgtagcaccgcctacatacctcgctctgctaatcctgttaccagtggctgctgccagtggcgataagtcgtgtcttaccgggttggactcaagacgatagttaccggataaggcgcagcggtcgggctgaacggggggttcgtgcacacagcccagcttggagcgaacgacctacaccgaactgagatacctacagcgtgagctatgagaaagcgccacgcttcccgaagggagaaaggcggacaggtatccggtaagcggcagggtcggaacaggagagcgcacgagggagcttccagggggaaacgcctggtatctttatagtcctgtcgggtttcgccacctctgacttgagcgtcgatttttgtgatgctcgtcaggggggcggagcctatggaaaaacgccagcaacgcggcctttttacggttcctggccttttgctggccttttgctcacatgt

SEQ ID NO: 48 - DNA, 6598 bp, Artificial Sequence
  pGW122
cctgcaggcagctgcgcgctcgctcgctcactgaggccgcccgggcgtcgggcgacctttggtcgcccggcctcagtgagcgagcgagcgcgcagagagggagtggccaactccatcactaggggttcctgcggcctctagaaaggatctgcgatcgctccggtgcccgtcagtgggcagagcgcacatcgcccacagtccccgagaagttggggggaggggtcggcaattgaacgggtgcctagagaaggtggcgcggggtaaactgggaaagtgatgtcgtgtactggctccgcctttttcccgagggtgggggagaaccgtatataagtgcagtagtcgccgtgaacgttctttttcgcaacgggtttgccgccagaacacagctgaagcttcgaggggctcgcatctctccttcacgcgcccgccgccctacctgaggccgccatccacgccggttgagtcgcgttctgccgcctcccgcctgtggtgcctcctgaactgcgtccgccgtctaggtaagtttaaagctcaggtcgagaccgggcctttgtccggcgctcccttggagcctacctagactcagccggctctccacgctttgcctgaccctgcttgctcaactctacgtctttgtttcgttttctgttctgcgccgttacagatctggctaactaccggtgccaccatgtgtcctcagaagctaaccatctcctggtttgccatcgttttgctggtgtctccactcatggccatgtgggagctggagaaagacgtttatgttgtagaggtggactggactcccgatgcccctggagaaacagtgaacctcacctgtgacacgcctgaagaagatgacatcacctggacctcagaccagagacatggagtcataggctctggaaagaccctgaccatcactgtcaaagagtttctagatgctggccagtacacctgccacaaaggaggcgagactctgagccactcacatctgctgctccacaagaaggaaaatggaatttggtccactgaaattttaaaaaatttcaaaaacaagactttcctgaagtgtgaagcaccaaattactccggacggttcacgtgctcatggctggtgcaaagaaacatggacttgaagttcaacatcaagagcagtagcagttcccctgactctcgggcagtgacatgtggaatggcgtctctgtctgcagagaaggtcacactggaccaaagggactatgagaagtattcagtgtcctgccaggaggatgtcacctgcccaactgccgaggagaccctgcccattgaactggcgttggaagcacggcagcagaataaatatgagaactacagcaccagcttcttcatcagggacatcatcaaaccagacccgcccaagaacttgcagatgaagcctttgaagaactcacaggtggaggtcagctgggagtaccctgactcctggagcactccccattcctacttctccctcaagttctttgttcgaatccagcgcaagaaagaaaagatgaaggagacagaggaggggtgtaaccagaaaggtgcgttcctcgtagagaagacatctaccgaagtccaatgcaaaggcgggaatgtctgcgtgcaagctcaggatcgctattacaattcctcatgcagcaagtgggcatgtgttccctgcagggtccgatccggcagtggagagggcagaggaagtctgctaacatgcggtgacgtcgaggagaatcctggcccaatggaccagcacacacttgatgtggaggataccgcggatgccagacatccagcaggtacttcgtgcccctcggatgcggcgctcctcagagataccgggctcctcgcggacgctgcgctcctctcagatactgtgcgccccacaaatgccgcgctccccacggatgctgcctaccctgcggttaatgttcgggatcgcgaggccgcgtggccgcctgcactgaacttctgttcccgccacccaaagctctatggcctagtcgctttggttttgctgcttctgatcgccgcctgtgttcctatcttcacccgcaccgagcctcggccagcgctcacaatcaccacctcgcccaacctgggtacccgagagaataatgcagaccaggtcacccctgtttcccacattggctgccccaacactacacaacagggctctcctgtgttcgccaagctactggctaaaaaccaagcatcgttgtgcaatacaactctgaactggcacagccaagatggagctgggagctcatacctatctcaaggtctgaggtacgaagaagacaaaaaggagttggtggtagacagtcccgggctctactacgtatttttggaactgaagctcagtccaacattcacaaacacaggccacaaggtgcagggctgggtctctcttgttttgcaagcaaagcctcaggtagatgactttgacaacttggccctgacagtggaactgttcccttgctccatggagaacaagttagtggaccgttcctggagtcaactgttgctcctgaaggctggccaccgcctcagtgtgggtctgagggcttatctgcatggagcccaggatgcatacagagactgggagctgtcttatcccaacaccaccagctttggactctttcttgtgaaacccgacaacccatgggaaggatccggcgcaacaaacttctctctgctgaaacaagccggagatgtcgaagagaatcctggaccggctagcatgaacgctacacactgcatcttggctttgcagctcttcctcatggctgtttctggctgttactgccacggcacagtcattgaaagcctagaaagtctgaataactattttaactcaagtggcatagatgtggaagaaaagagtctcttcttggatatctggaggaactggcaaaaggatggtgacatgaaaatcctgcagagccagattatctctttctacctcagactctttgaagtcttgaaagacaatcaggccatcagcaacaacataagcgtcattgaatcacacctgattactaccttcttcagcaacagcaaggcgaaaaaggatgcattcatgagtattgccaagtttgaggtcaacaacccacaggtccagcgccaagcattcaatgagctcatccgagtggtccaccagctgttgccggaatccagcctcaggaagcggaaaaggagtcgctgctgagaattcacgcgttaagtcgacaatcaacctctggattacaaaatttgtgaaagattgactggtattcttaactatgttgctccttttacgctatgtggatacgctgctttaatgcctttgtatcatgctattgcttcccgtatggctttcattttctcctccttgtataaatcctggttgctgtctctttatgaggagttgtggcccgttgtcaggcaacgtggcgtggtgtgcactgtgtttgctgacgcaacccccactggttggggcattgccaccacctgtcagctcctttccgggactttcgctttccccctccctattgccacggcggaactcatcgccgcctgccttgcccgctgctggacaggggctcggctgttgggcactgacaattccgtggtgttgtcggggaaatcatcgtcctttccttggctgctcgcctgtgttgccacctggattctgcgcgggacgtccttctgctacgtcccttcggccctcaatccagcggaccttccttcccgcggcctgctgccggctctgcggcctcttccgcgtcttcgccttcgccctcagacgagtcggatctccctttgggccgcctccccgcgtcgactttaagaccaatgacggccgcaggaacccctagtgatggagttggccactccctctctgcgcgctcgctcgctcactgaggccgggcgaccaaaggtcgcccgacgcccgggctttgcccgggcggcctcagtgagcgagcgagcgcgcagctgcctgcaggggcgcctgatgcggtattttctccttacgcatctgtgcggtatttcacaccgcatacgtcaaagcaaccatagtacgcgccctgtagcggcgcattaagcgcggcgggtgtggtggttacgcgcagcgtgaccgctacacttgccagcgccttagcgcccgctcctttcgctttcttcccttcctttctcgccacgttcgccggctttccccgtcaagctctaaatcgggggctccctttagggttccgatttagtgctttacggcacctcgaccccaaaaaacttgatttgggtgatggttcacgtagtgggccatcgccctgatagacggtttttcgccctttgacgttggagtccacgttctttaatagtggactcttgttccaaactggaacaacactcaactctatctcgggctattcttttgatttataagggattttgccgatttcggtctattggttaaaaaatgagctgatttaacaaaaatttaacgcgaattttaacaaaatattaacgtttacaattttatggtgcactctcagtacaatctgctctgatgccgcatagttaagccagccccgacacccgccaacacccgctgacgcgccctgacgggcttgtctgctcccggcatccgcttacagacaagctgtgaccgtctccgggagctgcatgtgtcagaggttttcaccgtcatcaccgaaacgcgcgagacgaaagggcctcgtgatacgcctatttttataggttaatgtcatgataataatggtttcttagacgtcaggtggcacttttcggggaaatgtgcgcggaacccctatttgtttatttttctaaatacattcaaatatgtatccgctcatgagacaataaccctgataaatgcttcaataatattgaaaaaggaagagtatgagtattcaacatttccgtgtcgcccttattcccttttttgcggcattttgccttcctgtttttgctcacccagaaacgctggtgaaagtaaaagatgctgaagatcagttgggtgcacgagtgggttacatcgaactggatctcaacagcggtaagatccttgagagttttcgccccgaagaacgttttccaatgatgagcacttttaaagttctgctatgtggcgcggtattatcccgtattgacgccgggcaagagcaactcggtcgccgcatacactattctcagaatgacttggttgagtactcaccagtcacagaaaagcatcttacggatggcatgacagtaagagaattatgcagtgctgccataaccatgagtgataacactgcggccaacttacttctgacaacgatcggaggaccgaaggagctaaccgcttttttgcacaacatgggggatcatgtaactcgccttgatcgttgggaaccggagctgaatgaagccataccaaacgacgagcgtgacaccacgatgcctgtagcaatggcaacaacgttgcgcaaactattaactggcgaactacttactctagcttcccggcaacaattaatagactggatggaggcggataaagttgcaggaccacttctgcgctcggcccttccggctggctggtttattgctgataaatctggagccggtgagcgtggaagccgcggtatcattgcagcactggggccagatggtaagccctcccgtatcgtagttatctacacgacggggagtcaggcaactatggatgaacgaaatagacagatcgctgagataggtgcctcactgattaagcattggtaactgtcagaccaagtttactcatatatactttagattgatttaaaacttcatttttaatttaaaaggatctaggtgaagatcctttttgataatctcatgaccaaaatcccttaacgtgagttttcgttccactgagcgtcagaccccgtagaaaagatcaaaggatcttcttgagatcctttttttctgcgcgtaatctgctgcttgcaaacaaaaaaaccaccgctaccagcggtggtttgtttgccggatcaagagctaccaactctttttccgaaggtaactggcttcagcagagcgcagataccaaatactgttcttctagtgtagccgtagttaggccaccacttcaagaactctgtagcaccgcctacatacctcgctctgctaatcctgttaccagtggctgctgccagtggcgataagtcgtgtcttaccgggttggactcaagacgatagttaccggataaggcgcagcggtcgggctgaacggggggttcgtgcacacagcccagcttggagcgaacgacctacaccgaactgagatacctacagcgtgagctatgagaaagcgccacgcttcccgaagggagaaaggcggacaggtatccggtaagcggcagggtcggaacaggagagcgcacgagggagcttccagggggaaacgcctggtatctttatagtcctgtcgggtttcgccacctctgacttgagcgtcgatttttgtgatgctcgtcaggggggcggagcctatggaaaaacgccagcaacgcggcctttttacggttcctggccttttgctggccttttgctcacatgt

SEQ ID NO: 49 - DNA, 6448 bp, Artificial Sequence
  pGW127b
cctgcaggcagctgcgcgctcgctcgctcactgaggccgcccgggcgtcgggcgacctttggtcgcccggcctcagtgagcgagcgagcgcgcagagagggagtggccaactccatcactaggggttcctgcggcctctagaaaggatctgcgatcgctccggtgcccgtcagtgggcagagcgcacatcgcccacagtccccgagaagttggggggaggggtcggcaattgaacgggtgcctagagaaggtggcgcggggtaaactgggaaagtgatgtcgtgtactggctccgcctttttcccgagggtgggggagaaccgtatataagtgcagtagtcgccgtgaacgttctttttcgcaacgggtttgccgccagaacacagctgaagcttcgaggggctcgcatctctccttcacgcgcccgccgccctacctgaggccgccatccacgccggttgagtcgcgttctgccgcctcccgcctgtggtgcctcctgaactgcgtccgccgtctaggtaagtttaaagctcaggtcgagaccgggcctttgtccggcgctcccttggagcctacctagactcagccggctctccacgctttgcctgaccctgcttgctcaactctacgtctttgtttcgttttctgttctgcgccgttacagatctggctaactaccggtgccaccatgaaatatacaagttatatcttggcttttcagctctgcatcgttttgggttctcttggctgttactgccaggacccatatgtaaaagaagcagaaaaccttaagaaatattttaatgcaggtcattcagatgtagcggataatggaactcttttcttaggcattttgaagaattggaaagaggagagtgacagaaaaataatgcagagccaaattgtctccttttacttcaaactttttaaaaactttaaagatgaccagagcatccaaaagagtgtggagaccatcaaggaagacatgaatgtcaagtttttcaatagcaacaaaaagaaacgagatgacttcgaaaagctgactaattattcggtaactgacttgaatgtccaacgcaaagcaatacatgaactcatccaagtgatggctgaactgtcgccagcagctaaaacagggaagcgaaaaaggagtcagatgctgtttcgaggtcgaagagcatcccagggcggaggatccggcgcaacaaacttctctctgctgaaacaagccggagatgtcgaagagaatcctggaccgatgtgtcaccagcagttggtcatctcttggttttccctggtttttctggcatctcccctcgtggccatatgggaactgaagaaagatgtttatgtcgtagaattggattggtatccggatgcccctggagaaatggtggtcctcacctgtgacacccctgaagaagatggtatcacctggaccttggaccagagcagtgaggtcttaggctctggcaaaaccctgaccatccaagtcaaagagtttggagatgctggccagtacacctgtcacaaaggaggcgaggttctaagccattcgctcctgctgcttcacaaaaaggaagatggaatttggtccactgatattttaaaggaccagaaagaacccaaaaataagacctttctaagatgcgaggccaagaattattctggacgtttcacctgctggtggctgacgacaatcagtactgatttgacattcagtgtcaaaagcagcagaggctcttctgacccccaaggggtgacgtgcggagctgctacactctctgcagagagagtcagaggggacaacaaggagtatgagtactcagtggagtgccaggaggacagtgcctgcccagctgctgaggagagtctgcccattgaggtcatggtggatgccgttcacaagctcaagtatgaaaactacaccagcagcttcttcatcagggacatcatcaaacctgacccacccaagaacttgcagctgaagccattaaagaattctcggcaggtggaggtcagctgggagtaccctgacacctggagtactccacattcctacttctccctgacattctgcgttcaggtccagggcaagagcaagagagaaaagaaagatagagtcttcacggacaagacctcagccacggtcatctgccgcaaaaatgccagcattagcgtgcgggcccaggaccgctactatagctcatcttggagcgaatgggcatctgtgccctgcagtggcactagtggagagggcagaggaagtctgctaacatgcggtgacgtcgaggagaatcctggcccaatggaatacgcctctgacgcttcactggaccccgaagccccgtggcctcccgcgccccgcgctcgcgcctgccgcgtactgccttgggccctggtcgcggggctgctgctgctgctgctgctcgctgccgcctgcgccgtcttcctcgcctgcccctgggccgtgtccggggctcgcgcctcgcccggctccgcggccagcccgagactccgcgagggtcccgagctttcgcccgacgatcccgccggcctcttggacctgcggcagggcatgtttgcgcagctggtggcccaaaatgttctgctgatcgatgggcccctgagctggtacagtgacccaggcctggcaggcgtgtccctgacggggggcctgagctacaaagaggacacgaaggagctggtggtggccaaggctggagtctactatgtcttctttcaactagagctgcggcgcgtggtggccggcgagggctcaggctccgtttcacttgcgctgcacctgcagccactgcgctctgctgctggggccgccgccctggctttgaccgtggacctgccacccgcctcctccgaggctcggaactcggccttcggtttccagggccgcttgctgcacctgagtgccggccagcgcctgggcgtccatcttcacactgaggccagggcacgccatgcctggcagcttacccagggcgccacagtcttgggactcttccgggtgacccccgaaatcccagccggactcccttcaccgaggtcggaataagaattcacgcgttaagtcgacaatcaacctctggattacaaaatttgtgaaagattgactggtattcttaactatgttgctccttttacgctatgtggatacgctgctttaatgcctttgtatcatgctattgcttcccgtatggctttcattttctcctccttgtataaatcctggttgctgtctctttatgaggagttgtggcccgttgtcaggcaacgtggcgtggtgtgcactgtgtttgctgacgcaacccccactggttggggcattgccaccacctgtcagctcctttccgggactttcgctttccccctccctattgccacggcggaactcatcgccgcctgccttgcccgctgctggacaggggctcggctgttgggcactgacaattccgtggtgttgtcggggaaatcatcgtcctttccttggctgctcgcctgtgttgccacctggattctgcgcgggacgtccttctgctacgtcccttcggccctcaatccagcggaccttccttcccgcggcctgctgccggctctgcggcctcttccgcgtcttcgccttcgccctcagacgagtcggatctccctttgggccgcctccccgcgtcgactttaagaccaatgacggccgcaggaacccctagtgatggagttggccactccctctctgcgcgctcgctcgctcactgaggccgggcgaccaaaggtcgcccgacgcccgggctttgcccgggcggcctcagtgagcgagcgagcgcgcagctgcctgcaggggcgcctgatgcggtattttctccttacgcatctgtgcggtatttcacaccgcatacgtcaaagcaaccatagtacgcgccctgtagcggcgcattaagcgcggcgggtgtggtggttacgcgcagcgtgaccgctacacttgccagcgccttagcgcccgctcctttcgctttcttcccttcctttctcgccacgttcgccggctttccccgtcaagctctaaatcgggggctccctttagggttccgatttagtgctttacggcacctcgaccccaaaaaacttgatttgggtgatggttcacgtagtgggccatcgccctgatagacggtttttcgccctttgacgttggagtccacgttctttaatagtggactcttgttccaaactggaacaacactcaactctatctcgggctattcttttgatttataagggattttgccgatttcggtctattggttaaaaaatgagctgatttaacaaaaatttaacgcgaattttaacaaaatattaacgtttacaattttatggtgcactctcagtacaatctgctctgatgccgcatagttaagccagccccgacacccgccaacacccgctgacgcgccctgacgggcttgtctgctcccggcatccgcttacagacaagctgtgaccgtctccgggagctgcatgtgtcagaggttttcaccgtcatcaccgaaacgcgcgagacgaaagggcctcgtgatacgcctatttttataggttaatgtcatgataataatggtttcttagacgtcaggtggcacttttcggggaaatgtgcgcggaacccctatttgtttatttttctaaatacattcaaatatgtatccgctcatgagacaataaccctgataaatgcttcaataatattgaaaaaggaagagtatgagtattcaacatttccgtgtcgcccttattcccttttttgcggcattttgccttcctgtttttgctcacccagaaacgctggtgaaagtaaaagatgctgaagatcagttgggtgcacgagtgggttacatcgaactggatctcaacagcggtaagatccttgagagttttcgccccgaagaacgttttccaatgatgagcacttttaaagttctgctatgtggcgcggtattatcccgtattgacgccgggcaagagcaactcggtcgccgcatacactattctcagaatgacttggttgagtactcaccagtcacagaaaagcatcttacggatggcatgacagtaagagaattatgcagtgctgccataaccatgagtgataacactgcggccaacttacttctgacaacgatcggaggaccgaaggagctaaccgcttttttgcacaacatgggggatcatgtaactcgccttgatcgttgggaaccggagctgaatgaagccataccaaacgacgagcgtgacaccacgatgcctgtagcaatggcaacaacgttgcgcaaactattaactggcgaactacttactctagcttcccggcaacaattaatagactggatggaggcggataaagttgcaggaccacttctgcgctcggcccttccggctggctggtttattgctgataaatctggagccggtgagcgtggaagccgcggtatcattgcagcactggggccagatggtaagccctcccgtatcgtagttatctacacgacggggagtcaggcaactatggatgaacgaaatagacagatcgctgagataggtgcctcactgattaagcattggtaactgtcagaccaagtttactcatatatactttagattgatttaaaacttcatttttaatttaaaaggatctaggtgaagatcctttttgataatctcatgaccaaaatcccttaacgtgagttttcgttccactgagcgtcagaccccgtagaaaagatcaaaggatcttcttgagatcctttttttctgcgcgtaatctgctgcttgcaaacaaaaaaaccaccgctaccagcggtggtttgtttgccggatcaagagctaccaactctttttccgaaggtaactggcttcagcagagcgcagataccaaatactgttcttctagtgtagccgtagttaggccaccacttcaagaactctgtagcaccgcctacatacctcgctctgctaatcctgttaccagtggctgctgccagtggcgataagtcgtgtcttaccgggttggactcaagacgatagttaccggataaggcgcagcggtcgggctgaacggggggttcgtgcacacagcccagcttggagcgaacgacctacaccgaactgagatacctacagcgtgagctatgagaaagcgccacgcttcccgaagggagaaaggcggacaggtatccggtaagcggcagggtcggaacaggagagcgcacgagggagcttccagggggaaacgcctggtatctttatagtcctgtcgggtttcgccacctctgacttgagcgtcgatttttgtgatgctcgtcaggggggcggagcctatggaaaaacgccagcaacgcggcctttttacggttcctggccttttgctggccttttgctcacatgt

SEQ ID NO: 50 - DNA, 7267 bp, Artificial Sequence
  pGW128b
cctgcaggcagctgcgcgctcgctcgctcactgaggccgcccgggcgtcgggcgacctttggtcgcccggcctcagtgagcgagcgagcgcgcagagagggagtggccaactccatcactaggggttcctgcggcctctagaaaggatctgcgatcgctccggtgcccgtcagtgggcagagcgcacatcgcccacagtccccgagaagttggggggaggggtcggcaattgaacgggtgcctagagaaggtggcgcggggtaaactgggaaagtgatgtcgtgtactggctccgcctttttcccgagggtgggggagaaccgtatataagtgcagtagtcgccgtgaacgttctttttcgcaacgggtttgccgccagaacacagctgaagcttcgaggggctcgcatctctccttcacgcgcccgccgccctacctgaggccgccatccacgccggttgagtcgcgttctgccgcctcccgcctgtggtgcctcctgaactgcgtccgccgtctaggtaagtttaaagctcaggtcgagaccgggcctttgtccggcgctcccttggagcctacctagactcagccggctctccacgctttgcctgaccctgcttgctcaactctacgtctttgtttcgttttctgttctgcgccgttacagatctggctaactaccggtgccaccatgaaatatacaagttatatcttggcttttcagctctgcatcgttttgggttctcttggctgttactgccaggacccatatgtaaaagaagcagaaaaccttaagaaatattttaatgcaggtcattcagatgtagcggataatggaactcttttcttaggcattttgaagaattggaaagaggagagtgacagaaaaataatgcagagccaaattgtctccttttacttcaaactttttaaaaactttaaagatgaccagagcatccaaaagagtgtggagaccatcaaggaagacatgaatgtcaagtttttcaatagcaacaaaaagaaacgagatgacttcgaaaagctgactaattattcggtaactgacttgaatgtccaacgcaaagcaatacatgaactcatccaagtgatggctgaactgtcgccagcagctaaaacagggaagcgaaaaaggagtcagatgctgtttcgaggtcgaagagcatcccagggcggaggatccggcgcaacaaacttctctctgctgaaacaagccggagatgtcgaagagaatcctggaccgatgtgtcaccagcagttggtcatctcttggttttccctggtttttctggcatctcccctcgtggccatatgggaactgaagaaagatgtttatgtcgtagaattggattggtatccggatgcccctggagaaatggtggtcctcacctgtgacacccctgaagaagatggtatcacctggaccttggaccagagcagtgaggtcttaggctctggcaaaaccctgaccatccaagtcaaagagtttggagatgctggccagtacacctgtcacaaaggaggcgaggttctaagccattcgctcctgctgcttcacaaaaaggaagatggaatttggtccactgatattttaaaggaccagaaagaacccaaaaataagacctttctaagatgcgaggccaagaattattctggacgtttcacctgctggtggctgacgacaatcagtactgatttgacattcagtgtcaaaagcagcagaggctcttctgacccccaaggggtgacgtgcggagctgctacactctctgcagagagagtcagaggggacaacaaggagtatgagtactcagtggagtgccaggaggacagtgcctgcccagctgctgaggagagtctgcccattgaggtcatggtggatgccgttcacaagctcaagtatgaaaactacaccagcagcttcttcatcagggacatcatcaaacctgacccacccaagaacttgcagctgaagccattaaagaattctcggcaggtggaggtcagctgggagtaccctgacacctggagtactccacattcctacttctccctgacattctgcgttcaggtccagggcaagagcaagagagaaaagaaagatagagtcttcacggacaagacctcagccacggtcatctgccgcaaaaatgccagcattagcgtgcgggcccaggaccgctactatagctcatcttggagcgaatgggcatctgtgccctgcagtggcagtggagagggcagaggaagtctgctaacatgcggtgacgtcgaggagaatcctggcccaatggaatacgcctctgacgcttcactggaccccgaagccccgtggcctcccgcgccccgcgctcgcgcctgccgcgtactgccttgggccctggtcgcggggctgctgctgctgctgctgctcgctgccgcctgcgccgtcttcctcgcctgcccctgggccgtgtccggggctcgcgcctcgcccggctccgcggccagcccgagactccgcgagggtcccgagctttcgcccgacgatcccgccggcctcttggacctgcggcagggcatgtttgcgcagctggtggcccaaaatgttctgctgatcgatgggcccctgagctggtacagtgacccaggcctggcaggcgtgtccctgacggggggcctgagctacaaagaggacacgaaggagctggtggtggccaaggctggagtctactatgtcttctttcaactagagctgcggcgcgtggtggccggcgagggctcaggctccgtttcacttgcgctgcacctgcagccactgcgctctgctgctggggccgccgccctggctttgaccgtggacctgccacccgcctcctccgaggctcggaactcggccttcggtttccagggccgcttgctgcacctgagtgccggccagcgcctgggcgtccatcttcacactgaggccagggcacgccatgcctggcagcttacccagggcgccacagtcttgggactcttccgggtgacccccgaaatcccagccggactcccttcaccgaggtcggaaggtgctagcggtacccagtgcaccaactacgccctgctgaagctggccggcgatgtggagagcaaccccgggcccatggaggagagtgtcgtacggccctcagtgtttgtggtggatggacagaccgacatcccattcacgaggctgggacgaagccaccggagacagtcgtgcagtgtggcccgggtgggtctgggtctcttgctgttgctgatgggggccgggctggccgtccaaggctggttcctcctgcagctgcactggcgtctaggagagatggtcacccgcctgcctgacggacctgcaggctcctgggagcagctgatacaagagcgaaggtctcacgaggtcaacccagcagcgcatctcacaggggccaactccagcttgaccggcagcggggggccgctgttatgggagactcagctgggcctggccttcctgaggggcctcagctaccacgatggggcccttgtggtcaccaaagctggctactactacatctactccaaggtgcagctgggcggtgtgggctgcccgctgggcctggccagcaccatcacccacggcctctacaagcgcacaccccgctaccccgaggagctggagctgttggtcagccagcagtcaccctgcggacgggccaccagcagctcccgggtctggtgggacagcagcttcctgggtggtgtggtacacctggaggctggggagaaggtggtcgtccgtgtgctggatgaacgcctggttcgactgcgtgatggtacccggtcttacttcggggctttcatggtgggtggaggcggttgcggaaagcgtaagtgagaattcacgcgttaagtcgacaatcaacctctggattacaaaatttgtgaaagattgactggtattcttaactatgttgctccttttacgctatgtggatacgctgctttaatgcctttgtatcatgctattgcttcccgtatggctttcattttctcctccttgtataaatcctggttgctgtctctttatgaggagttgtggcccgttgtcaggcaacgtggcgtggtgtgcactgtgtttgctgacgcaacccccactggttggggcattgccaccacctgtcagctcctttccgggactttcgctttccccctccctattgccacggcggaactcatcgccgcctgccttgcccgctgctggacaggggctcggctgttgggcactgacaattccgtggtgttgtcggggaaatcatcgtcctttccttggctgctcgcctgtgttgccacctggattctgcgcgggacgtccttctgctacgtcccttcggccctcaatccagcggaccttccttcccgcggcctgctgccggctctgcggcctcttccgcgtcttcgccttcgccctcagacgagtcggatctccctttgggccgcctccccgcgtcgactttaagaccaatgacggccgcaggaacccctagtgatggagttggccactccctctctgcgcgctcgctcgctcactgaggccgggcgaccaaaggtcgcccgacgcccgggctttgcccgggcggcctcagtgagcgagcgagcgcgcagctgcctgcaggggcgcctgatgcggtattttctccttacgcatctgtgcggtatttcacaccgcatacgtcaaagcaaccatagtacgcgccctgtagcggcgcattaagcgcggcgggtgtggtggttacgcgcagcgtgaccgctacacttgccagcgccttagcgcccgctcctttcgctttcttcccttcctttctcgccacgttcgccggctttccccgtcaagctctaaatcgggggctccctttagggttccgatttagtgctttacggcacctcgaccccaaaaaacttgatttgggtgatggttcacgtagtgggccatcgccctgatagacggtttttcgccctttgacgttggagtccacgttctttaatagtggactcttgttccaaactggaacaacactcaactctatctcgggctattcttttgatttataagggattttgccgatttcggtctattggttaaaaaatgagctgatttaacaaaaatttaacgcgaattttaacaaaatattaacgtttacaattttatggtgcactctcagtacaatctgctctgatgccgcatagttaagccagccccgacacccgccaacacccgctgacgcgccctgacgggcttgtctgctcccggcatccgcttacagacaagctgtgaccgtctccgggagctgcatgtgtcagaggttttcaccgtcatcaccgaaacgcgcgagacgaaagggcctcgtgatacgcctatttttataggttaatgtcatgataataatggtttcttagacgtcaggtggcacttttcggggaaatgtgcgcggaacccctatttgtttatttttctaaatacattcaaatatgtatccgctcatgagacaataaccctgataaatgcttcaataatattgaaaaaggaagagtatgagtattcaacatttccgtgtcgcccttattcccttttttgcggcattttgccttcctgtttttgctcacccagaaacgctggtgaaagtaaaagatgctgaagatcagttgggtgcacgagtgggttacatcgaactggatctcaacagcggtaagatccttgagagttttcgccccgaagaacgttttccaatgatgagcacttttaaagttctgctatgtggcgcggtattatcccgtattgacgccgggcaagagcaactcggtcgccgcatacactattctcagaatgacttggttgagtactcaccagtcacagaaaagcatcttacggatggcatgacagtaagagaattatgcagtgctgccataaccatgagtgataacactgcggccaacttacttctgacaacgatcggaggaccgaaggagctaaccgcttttttgcacaacatgggggatcatgtaactcgccttgatcgttgggaaccggagctgaatgaagccataccaaacgacgagcgtgacaccacgatgcctgtagcaatggcaacaacgttgcgcaaactattaactggcgaactacttactctagcttcccggcaacaattaatagactggatggaggcggataaagttgcaggaccacttctgcgctcggcccttccggctggctggtttattgctgataaatctggagccggtgagcgtggaagccgcggtatcattgcagcactggggccagatggtaagccctcccgtatcgtagttatctacacgacggggagtcaggcaactatggatgaacgaaatagacagatcgctgagataggtgcctcactgattaagcattggtaactgtcagaccaagtttactcatatatactttagattgatttaaaacttcatttttaatttaaaaggatctaggtgaagatcctttttgataatctcatgaccaaaatcccttaacgtgagttttcgttccactgagcgtcagaccccgtagaaaagatcaaaggatcttcttgagatcctttttttctgcgcgtaatctgctgcttgcaaacaaaaaaaccaccgctaccagcggtggtttgtttgccggatcaagagctaccaactctttttccgaaggtaactggcttcagcagagcgcagataccaaatactgttcttctagtgtagccgtagttaggccaccacttcaagaactctgtagcaccgcctacatacctcgctctgctaatcctgttaccagtggctgctgccagtggcgataagtcgtgtcttaccgggttggactcaagacgatagttaccggataaggcgcagcggtcgggctgaacggggggttcgtgcacacagcccagcttggagcgaacgacctacaccgaactgagatacctacagcgtgagctatgagaaagcgccacgcttcccgaagggagaaaggcggacaggtatccggtaagcggcagggtcggaacaggagagcgcacgagggagcttccagggggaaacgcctggtatctttatagtcctgtcgggtttcgccacctctgacttgagcgtcgatttttgtgatgctcgtcaggggggcggagcctatggaaaaacgccagcaacgcggcctttttacggttcctggccttttgctggccttttgctcacatgt

SEQ ID NO: 51 - DNA, 4619 bp, Artificial Sequence
  pGW145
cctgcaggcagctgcgcgctcgctcgctcactgaggccgcccgggcgtcgggcgacctttggtcgcccggcctcagtgagcgagcgagcgcgcagagagggagtggccaactccatcactaggggttcctgcggcctctagaaaggatctgcgatcgctccggtgcccgtcagtgggcagagcgcacatcgcccacagtccccgagaagttggggggaggggtcggcaattgaacgggtgcctagagaaggtggcgcggggtaaactgggaaagtgatgtcgtgtactggctccgcctttttcccgagggtgggggagaaccgtatataagtgcagtagtcgccgtgaacgttctttttcgcaacgggtttgccgccagaacacagctgaagcttcgaggggctcgcatctctccttcacgcgcccgccgccctacctgaggccgccatccacgccggttgagtcgcgttctgccgcctcccgcctgtggtgcctcctgaactgcgtccgccgtctaggtaagtttaaagctcaggtcgagaccgggcctttgtccggcgctcccttggagcctacctagactcagccggctctccacgctttgcctgaccctgcttgctcaactctacgtctttgtttcgttttctgttctgcgccgttacagatctggctaactaccggtgccaccatgaaatatacaagttatatcttggcttttcagctctgcatcgttttgggttctcttggctgttactgccaggacccatatgtaaaagaagcagaaaaccttaagaaatattttaatgcaggtcattcagatgtagcggataatggaactcttttcttaggcattttgaagaattggaaagaggagagtgacagaaaaataatgcagagccaaattgtctccttttacttcaaactttttaaaaactttaaagatgaccagagcatccaaaagagtgtggagaccatcaaggaagacatgaatgtcaagtttttcaatagcaacaaaaagaaacgagatgacttcgaaaagctgactaattattcggtaactgacttgaatgtccaacgcaaagcaatacatgaactcatccaagtgatggctgaactgtcgccagcagctaaaacagggaagcgaaaaaggagtcagatgctgtttcgaggtcgaagagcatcccagtgagaattcacgcgttaagtcgacaatcaacctctggattacaaaatttgtgaaagattgactggtattcttaactatgttgctccttttacgctatgtggatacgctgctttaatgcctttgtatcatgctattgcttcccgtatggctttcattttctcctccttgtataaatcctggttgctgtctctttatgaggagttgtggcccgttgtcaggcaacgtggcgtggtgtgcactgtgtttgctgacgcaacccccactggttggggcattgccaccacctgtcagctcctttccgggactttcgctttccccctccctattgccacggcggaactcatcgccgcctgccttgcccgctgctggacaggggctcggctgttgggcactgacaattccgtggtgttgtcggggaaatcatcgtcctttccttggctgctcgcctgtgttgccacctggattctgcgcgggacgtccttctgctacgtcccttcggccctcaatccagcggaccttccttcccgcggcctgctgccggctctgcggcctcttccgcgtcttcgccttcgccctcagacgagtcggatctccctttgggccgcctccccgcgtcgactttaagaccaatgacggccgaataaaagatctttattttcattagatctgtgtgttggttttttgtgtgcggccgcaggaacccctagtgatggagttggccactccctctctgcgcgctcgctcgctcactgaggccgggcgaccaaaggtcgcccgacgcccgggctttgcccgggcggcctcagtgagcgagcgagcgcgcagctgcctgcaggggcgcctgatgcggtattttctccttacgcatctgtgcggtatttcacaccgcatacgtcaaagcaaccatagtacgcgccctgtagcggcgcattaagcgcggcgggtgtggtggttacgcgcagcgtgaccgctacacttgccagcgccttagcgcccgctcctttcgctttcttcccttcctttctcgccacgttcgccggctttccccgtcaagctctaaatcgggggctccctttagggttccgatttagtgctttacggcacctcgaccccaaaaaacttgatttgggtgatggttcacgtagtgggccatcgccctgatagacggtttttcgccctttgacgttggagtccacgttctttaatagtggactcttgttccaaactggaacaacactcaactctatctcgggctattcttttgatttataagggattttgccgatttcggtctattggttaaaaaatgagctgatttaacaaaaatttaacgcgaattttaacaaaatattaacgtttacaattttatggtgcactctcagtacaatctgctctgatgccgcatagttaagccagccccgacacccgccaacacccgctgacgcgccctgacgggcttgtctgctcccggcatccgcttacagacaagctgtgaccgtctccgggagctgcatgtgtcagaggttttcaccgtcatcaccgaaacgcgcgagacgaaagggcctcgtgatacgcctatttttataggttaatgtcatgataataatggtttcttagacgtcaggtggcacttttcggggaaatgtgcgcggaacccctatttgtttatttttctaaatacattcaaatatgtatccgctcatgagacaataaccctgataaatgcttcaataatattgaaaaaggaagagtatgagtattcaacatttccgtgtcgcccttattcccttttttgcggcattttgccttcctgtttttgctcacccagaaacgctggtgaaagtaaaagatgctgaagatcagttgggtgcacgagtgggttacatcgaactggatctcaacagcggtaagatccttgagagttttcgccccgaagaacgttttccaatgatgagcacttttaaagttctgctatgtggcgcggtattatcccgtattgacgccgggcaagagcaactcggtcgccgcatacactattctcagaatgacttggttgagtactcaccagtcacagaaaagcatcttacggatggcatgacagtaagagaattatgcagtgctgccataaccatgagtgataacactgcggccaacttacttctgacaacgatcggaggaccgaaggagctaaccgcttttttgcacaacatgggggatcatgtaactcgccttgatcgttgggaaccggagctgaatgaagccataccaaacgacgagcgtgacaccacgatgcctgtagcaatggcaacaacgttgcgcaaactattaactggcgaactacttactctagcttcccggcaacaattaatagactggatggaggcggataaagttgcaggaccacttctgcgctcggcccttccggctggctggtttattgctgataaatctggagccggtgagcgtggaagccgcggtatcattgcagcactggggccagatggtaagccctcccgtatcgtagttatctacacgacggggagtcaggcaactatggatgaacgaaatagacagatcgctgagataggtgcctcactgattaagcattggtaactgtcagaccaagtttactcatatatactttagattgatttaaaacttcatttttaatttaaaaggatctaggtgaagatcctttttgataatctcatgaccaaaatcccttaacgtgagttttcgttccactgagcgtcagaccccgtagaaaagatcaaaggatcttcttgagatcctttttttctgcgcgtaatctgctgcttgcaaacaaaaaaaccaccgctaccagcggtggtttgtttgccggatcaagagctaccaactctttttccgaaggtaactggcttcagcagagcgcagataccaaatactgttcttctagtgtagccgtagttaggccaccacttcaagaactctgtagcaccgcctacatacctcgctctgctaatcctgttaccagtggctgctgccagtggcgataagtcgtgtcttaccgggttggactcaagacgatagttaccggataaggcgcagcggtcgggctgaacggggggttcgtgcacacagcccagcttggagcgaacgacctacaccgaactgagatacctacagcgtgagctatgagaaagcgccacgcttcccgaagggagaaaggcggacaggtatccggtaagcggcagggtcggaacaggagagcgcacgagggagcttccagggggaaacgcctggtatctttatagtcctgtcgggtttcgccacctctgacttgagcgtcgatttttgtgatgctcgtcaggggggcggagcctatggaaaaacgccagcaacgcggcctttttacggttcctggccttttgctggccttttgctcacatgt

SEQ ID NO: 52 - DNA, 5105 bp, Artificial Sequence
  pGW146
cctgcaggcagctgcgcgctcgctcgctcactgaggccgcccgggcgtcgggcgacctttggtcgcccggcctcagtgagcgagcgagcgcgcagagagggagtggccaactccatcactaggggttcctgcggcctctagaaaggatctgcgatcgctccggtgcccgtcagtgggcagagcgcacatcgcccacagtccccgagaagttggggggaggggtcggcaattgaacgggtgcctagagaaggtggcgcggggtaaactgggaaagtgatgtcgtgtactggctccgcctttttcccgagggtgggggagaaccgtatataagtgcagtagtcgccgtgaacgttctttttcgcaacgggtttgccgccagaacacagctgaagcttcgaggggctcgcatctctccttcacgcgcccgccgccctacctgaggccgccatccacgccggttgagtcgcgttctgccgcctcccgcctgtggtgcctcctgaactgcgtccgccgtctaggtaagtttaaagctcaggtcgagaccgggcctttgtccggcgctcccttggagcctacctagactcagccggctctccacgctttgcctgaccctgcttgctcaactctacgtctttgtttcgttttctgttctgcgccgttacagatctggctaactaccggtgccaccatgtgtcaccagcagttggtcatctcttggttttccctggtttttctggcatctcccctcgtggccatatgggaactgaagaaagatgtttatgtcgtagaattggattggtatccggatgcccctggagaaatggtggtcctcacctgtgacacccctgaagaagatggtatcacctggaccttggaccagagcagtgaggtcttaggctctggcaaaaccctgaccatccaagtcaaagagtttggagatgctggccagtacacctgtcacaaaggaggcgaggttctaagccattcgctcctgctgcttcacaaaaaggaagatggaatttggtccactgatattttaaaggaccagaaagaacccaaaaataagacctttctaagatgcgaggccaagaattattctggacgtttcacctgctggtggctgacgacaatcagtactgatttgacattcagtgtcaaaagcagcagaggctcttctgacccccaaggggtgacgtgcggagctgctacactctctgcagagagagtcagaggggacaacaaggagtatgagtactcagtggagtgccaggaggacagtgcctgcccagctgctgaggagagtctgcccattgaggtcatggtggatgccgttcacaagctcaagtatgaaaactacaccagcagcttcttcatcagggacatcatcaaacctgacccacccaagaacttgcagctgaagccattaaagaattctcggcaggtggaggtcagctgggagtaccctgacacctggagtactccacattcctacttctccctgacattctgcgttcaggtccagggcaagagcaagagagaaaagaaagatagagtcttcacggacaagacctcagccacggtcatctgccgcaaaaatgccagcattagcgtgcgggcccaggaccgctactatagctcatcttggagcgaatgggcatctgtgccctgcagttgagaattcacgcgttaagtcgacaatcaacctctggattacaaaatttgtgaaagattgactggtattcttaactatgttgctccttttacgctatgtggatacgctgctttaatgcctttgtatcatgctattgcttcccgtatggctttcattttctcctccttgtataaatcctggttgctgtctctttatgaggagttgtggcccgttgtcaggcaacgtggcgtggtgtgcactgtgtttgctgacgcaacccccactggttggggcattgccaccacctgtcagctcctttccgggactttcgctttccccctccctattgccacggcggaactcatcgccgcctgccttgcccgctgctggacaggggctcggctgttgggcactgacaattccgtggtgttgtcggggaaatcatcgtcctttccttggctgctcgcctgtgttgccacctggattctgcgcgggacgtccttctgctacgtcccttcggccctcaatccagcggaccttccttcccgcggcctgctgccggctctgcggcctcttccgcgtcttcgccttcgccctcagacgagtcggatctccctttgggccgcctccccgcgtcgactttaagaccaatgacggccgaataaaagatctttattttcattagatctgtgtgttggttttttgtgtgcggccgcaggaacccctagtgatggagttggccactccctctctgcgcgctcgctcgctcactgaggccgggcgaccaaaggtcgcccgacgcccgggctttgcccgggcggcctcagtgagcgagcgagcgcgcagctgcctgcaggggcgcctgatgcggtattttctccttacgcatctgtgcggtatttcacaccgcatacgtcaaagcaaccatagtacgcgccctgtagcggcgcattaagcgcggcgggtgtggtggttacgcgcagcgtgaccgctacacttgccagcgccttagcgcccgctcctttcgctttcttcccttcctttctcgccacgttcgccggctttccccgtcaagctctaaatcgggggctccctttagggttccgatttagtgctttacggcacctcgaccccaaaaaacttgatttgggtgatggttcacgtagtgggccatcgccctgatagacggtttttcgccctttgacgttggagtccacgttctttaatagtggactcttgttccaaactggaacaacactcaactctatctcgggctattcttttgatttataagggattttgccgatttcggtctattggttaaaaaatgagctgatttaacaaaaatttaacgcgaattttaacaaaatattaacgtttacaattttatggtgcactctcagtacaatctgctctgatgccgcatagttaagccagccccgacacccgccaacacccgctgacgcgccctgacgggcttgtctgctcccggcatccgcttacagacaagctgtgaccgtctccgggagctgcatgtgtcagaggttttcaccgtcatcaccgaaacgcgcgagacgaaagggcctcgtgatacgcctatttttataggttaatgtcatgataataatggtttcttagacgtcaggtggcacttttcggggaaatgtgcgcggaacccctatttgtttatttttctaaatacattcaaatatgtatccgctcatgagacaataaccctgataaatgcttcaataatattgaaaaaggaagagtatgagtattcaacatttccgtgtcgcccttattcccttttttgcggcattttgccttcctgtttttgctcacccagaaacgctggtgaaagtaaaagatgctgaagatcagttgggtgcacgagtgggttacatcgaactggatctcaacagcggtaagatccttgagagttttcgccccgaagaacgttttccaatgatgagcacttttaaagttctgctatgtggcgcggtattatcccgtattgacgccgggcaagagcaactcggtcgccgcatacactattctcagaatgacttggttgagtactcaccagtcacagaaaagcatcttacggatggcatgacagtaagagaattatgcagtgctgccataaccatgagtgataacactgcggccaacttacttctgacaacgatcggaggaccgaaggagctaaccgcttttttgcacaacatgggggatcatgtaactcgccttgatcgttgggaaccggagctgaatgaagccataccaaacgacgagcgtgacaccacgatgcctgtagcaatggcaacaacgttgcgcaaactattaactggcgaactacttactctagcttcccggcaacaattaatagactggatggaggcggataaagttgcaggaccacttctgcgctcggcccttccggctggctggtttattgctgataaatctggagccggtgagcgtggaagccgcggtatcattgcagcactggggccagatggtaagccctcccgtatcgtagttatctacacgacggggagtcaggcaactatggatgaacgaaatagacagatcgctgagataggtgcctcactgattaagcattggtaactgtcagaccaagtttactcatatatactttagattgatttaaaacttcatttttaatttaaaaggatctaggtgaagatcctttttgataatctcatgaccaaaatcccttaacgtgagttttcgttccactgagcgtcagaccccgtagaaaagatcaaaggatcttcttgagatcctttttttctgcgcgtaatctgctgcttgcaaacaaaaaaaccaccgctaccagcggtggtttgtttgccggatcaagagctaccaactctttttccgaaggtaactggcttcagcagagcgcagataccaaatactgttcttctagtgtagccgtagttaggccaccacttcaagaactctgtagcaccgcctacatacctcgctctgctaatcctgttaccagtggctgctgccagtggcgataagtcgtgtcttaccgggttggactcaagacgatagttaccggataaggcgcagcggtcgggctgaacggggggttcgtgcacacagcccagcttggagcgaacgacctacaccgaactgagatacctacagcgtgagctatgagaaagcgccacgcttcccgaagggagaaaggcggacaggtatccggtaagcggcagggtcggaacaggagagcgcacgagggagcttccagggggaaacgcctggtatctttatagtcctgtcgggtttcgccacctctgacttgagcgtcgatttttgtgatgctcgtcaggggggcggagcctatggaaaaacgccagcaacgcggcctttttacggttcctggccttttgctggccttttgctcacatgt

SEQ ID NO: 53 - DNA, 4883 bp, Artificial Sequence
  pGW147
cctgcaggcagctgcgcgctcgctcgctcactgaggccgcccgggcgtcgggcgacctttggtcgcccggcctcagtgagcgagcgagcgcgcagagagggagtggccaactccatcactaggggttcctgcggcctctagaaaggatctgcgatcgctccggtgcccgtcagtgggcagagcgcacatcgcccacagtccccgagaagttggggggaggggtcggcaattgaacgggtgcctagagaaggtggcgcggggtaaactgggaaagtgatgtcgtgtactggctccgcctttttcccgagggtgggggagaaccgtatataagtgcagtagtcgccgtgaacgttctttttcgcaacgggtttgccgccagaacacagctgaagcttcgaggggctcgcatctctccttcacgcgcccgccgccctacctgaggccgccatccacgccggttgagtcgcgttctgccgcctcccgcctgtggtgcctcctgaactgcgtccgccgtctaggtaagtttaaagctcaggtcgagaccgggcctttgtccggcgctcccttggagcctacctagactcagccggctctccacgctttgcctgaccctgcttgctcaactctacgtctttgtttcgttttctgttctgcgccgttacagatctggctaactaccggtgccaccatggaatacgcctctgacgcttcactggaccccgaagccccgtggcctcccgcgccccgcgctcgcgcctgccgcgtactgccttgggccctggtcgcggggctgctgctgctgctgctgctcgctgccgcctgcgccgtcttcctcgcctgcccctgggccgtgtccggggctcgcgcctcgcccggctccgcggccagcccgagactccgcgagggtcccgagctttcgcccgacgatcccgccggcctcttggacctgcggcagggcatgtttgcgcagctggtggcccaaaatgttctgctgatcgatgggcccctgagctggtacagtgacccaggcctggcaggcgtgtccctgacggggggcctgagctacaaagaggacacgaaggagctggtggtggccaaggctggagtctactatgtcttctttcaactagagctgcggcgcgtggtggccggcgagggctcaggctccgtttcacttgcgctgcacctgcagccactgcgctctgctgctggggccgccgccctggctttgaccgtggacctgccacccgcctcctccgaggctcggaactcggccttcggtttccagggccgcttgctgcacctgagtgccggccagcgcctgggcgtccatcttcacactgaggccagggcacgccatgcctggcagcttacccagggcgccacagtcttgggactcttccgggtgacccccgaaatcccagccggactcccttcaccgaggtcggaatgagaattcacgcgttaagtcgacaatcaacctctggattacaaaatttgtgaaagattgactggtattcttaactatgttgctccttttacgctatgtggatacgctgctttaatgcctttgtatcatgctattgcttcccgtatggctttcattttctcctccttgtataaatcctggttgctgtctctttatgaggagttgtggcccgttgtcaggcaacgtggcgtggtgtgcactgtgtttgctgacgcaacccccactggttggggcattgccaccacctgtcagctcctttccgggactttcgctttccccctccctattgccacggcggaactcatcgccgcctgccttgcccgctgctggacaggggctcggctgttgggcactgacaattccgtggtgttgtcggggaaatcatcgtcctttccttggctgctcgcctgtgttgccacctggattctgcgcgggacgtccttctgctacgtcccttcggccctcaatccagcggaccttccttcccgcggcctgctgccggctctgcggcctcttccgcgtcttcgccttcgccctcagacgagtcggatctccctttgggccgcctccccgcgtcgactttaagaccaatgacggccgaataaaagatctttattttcattagatctgtgtgttggttttttgtgtgcggccgcaggaacccctagtgatggagttggccactccctctctgcgcgctcgctcgctcactgaggccgggcgaccaaaggtcgcccgacgcccgggctttgcccgggcggcctcagtgagcgagcgagcgcgcagctgcctgcaggggcgcctgatgcggtattttctccttacgcatctgtgcggtatttcacaccgcatacgtcaaagcaaccatagtacgcgccctgtagcggcgcattaagcgcggcgggtgtggtggttacgcgcagcgtgaccgctacacttgccagcgccttagcgcccgctcctttcgctttcttcccttcctttctcgccacgttcgccggctttccccgtcaagctctaaatcgggggctccctttagggttccgatttagtgctttacggcacctcgaccccaaaaaacttgatttgggtgatggttcacgtagtgggccatcgccctgatagacggtttttcgccctttgacgttggagtccacgttctttaatagtggactcttgttccaaactggaacaacactcaactctatctcgggctattcttttgatttataagggattttgccgatttcggtctattggttaaaaaatgagctgatttaacaaaaatttaacgcgaattttaacaaaatattaacgtttacaattttatggtgcactctcagtacaatctgctctgatgccgcatagttaagccagccccgacacccgccaacacccgctgacgcgccctgacgggcttgtctgctcccggcatccgcttacagacaagctgtgaccgtctccgggagctgcatgtgtcagaggttttcaccgtcatcaccgaaacgcgcgagacgaaagggcctcgtgatacgcctatttttataggttaatgtcatgataataatggtttcttagacgtcaggtggcacttttcggggaaatgtgcgcggaacccctatttgtttatttttctaaatacattcaaatatgtatccgctcatgagacaataaccctgataaatgcttcaataatattgaaaaaggaagagtatgagtattcaacatttccgtgtcgcccttattcccttttttgcggcattttgccttcctgtttttgctcacccagaaacgctggtgaaagtaaaagatgctgaagatcagttgggtgcacgagtgggttacatcgaactggatctcaacagcggtaagatccttgagagttttcgccccgaagaacgttttccaatgatgagcacttttaaagttctgctatgtggcgcggtattatcccgtattgacgccgggcaagagcaactcggtcgccgcatacactattctcagaatgacttggttgagtactcaccagtcacagaaaagcatcttacggatggcatgacagtaagagaattatgcagtgctgccataaccatgagtgataacactgcggccaacttacttctgacaacgatcggaggaccgaaggagctaaccgcttttttgcacaacatgggggatcatgtaactcgccttgatcgttgggaaccggagctgaatgaagccataccaaacgacgagcgtgacaccacgatgcctgtagcaatggcaacaacgttgcgcaaactattaactggcgaactacttactctagcttcccggcaacaattaatagactggatggaggcggataaagttgcaggaccacttctgcgctcggcccttccggctggctggtttattgctgataaatctggagccggtgagcgtggaagccgcggtatcattgcagcactggggccagatggtaagccctcccgtatcgtagttatctacacgacggggagtcaggcaactatggatgaacgaaatagacagatcgctgagataggtgcctcactgattaagcattggtaactgtcagaccaagtttactcatatatactttagattgatttaaaacttcatttttaatttaaaaggatctaggtgaagatcctttttgataatctcatgaccaaaatcccttaacgtgagttttcgttccactgagcgtcagaccccgtagaaaagatcaaaggatcttcttgagatcctttttttctgcgcgtaatctgctgcttgcaaacaaaaaaaccaccgctaccagcggtggtttgtttgccggatcaagagctaccaactctttttccgaaggtaactggcttcagcagagcgcagataccaaatactgttcttctagtgtagccgtagttaggccaccacttcaagaactctgtagcaccgcctacatacctcgctctgctaatcctgttaccagtggctgctgccagtggcgataagtcgtgtcttaccgggttggactcaagacgatagttaccggataaggcgcagcggtcgggctgaacggggggttcgtgcacacagcccagcttggagcgaacgacctacaccgaactgagatacctacagcgtgagctatgagaaagcgccacgcttcccgaagggagaaaggcggacaggtatccggtaagcggcagggtcggaacaggagagcgcacgagggagcttccagggggaaacgcctggtatctttatagtcctgtcgggtttcgccacctctgacttgagcgtcgatttttgtgatgctcgtcaggggggcggagcctatggaaaaacgccagcaacgcggcctttttacggttcctggccttttgctggccttttgctcacatgt

SEQ ID NO: 54 - DNA, 4856 bp, Artificial Sequence
  pGW149
cctgcaggcagctgcgcgctcgctcgctcactgaggccgcccgggcgtcgggcgacctttggtcgcccggcctcagtgagcgagcgagcgcgcagagagggagtggccaactccatcactaggggttcctgcggcctctagaaaggatctgcgatcgctccggtgcccgtcagtgggcagagcgcacatcgcccacagtccccgagaagttggggggaggggtcggcaattgaacgggtgcctagagaaggtggcgcggggtaaactgggaaagtgatgtcgtgtactggctccgcctttttcccgagggtgggggagaaccgtatataagtgcagtagtcgccgtgaacgttctttttcgcaacgggtttgccgccagaacacagctgaagcttcgaggggctcgcatctctccttcacgcgcccgccgccctacctgaggccgccatccacgccggttgagtcgcgttctgccgcctcccgcctgtggtgcctcctgaactgcgtccgccgtctaggtaagtttaaagctcaggtcgagaccgggcctttgtccggcgctcccttggagcctacctagactcagccggctctccacgctttgcctgaccctgcttgctcaactctacgtctttgtttcgttttctgttctgcgccgttacagatctggctaactaccggtgccaccatggaggagagtgtcgtacggccctcagtgtttgtggtggatggacagaccgacatcccattcacgaggctgggacgaagccaccggagacagtcgtgcagtgtggcccgggtgggtctgggtctcttgctgttgctgatgggggccgggctggccgtccaaggctggttcctcctgcagctgcactggcgtctaggagagatggtcacccgcctgcctgacggacctgcaggctcctggcaagagcgaaggtctcacgaggtcaacccagcagcgcatctcacaggggccaactccagcttgaccggcagcggggggccgctgttatgggagactcagctgggcctggccttcctgaggggcctcagctaccacgatggggcccttgtggtcaccaaagctggctactactacatctactccaaggtgcagctgggcggtgtgggctgcccgctgggcctggccagcaccatcacccacggcctctacaagcgcacaccccgctaccccgaggagctggagctgttggtcagccagcagtcaccctgcggacgggccaccagcagctcccgggtctggtgggacagcagcttcctgggtggtgtggtacacctggaggctggggagaaggtggtcgtccgtgtgctggatgaacgcctggttcgactgcgtgatggtacccggtcttacttcggggctttcatggtgggtggaggcggttgcggaaagcgtaagtgagaattcacgcgttaagtcgacaatcaacctctggattacaaaatttgtgaaagattgactggtattcttaactatgttgctccttttacgctatgtggatacgctgctttaatgcctttgtatcatgctattgcttcccgtatggctttcattttctcctccttgtataaatcctggttgctgtctctttatgaggagttgtggcccgttgtcaggcaacgtggcgtggtgtgcactgtgtttgctgacgcaacccccactggttggggcattgccaccacctgtcagctcctttccgggactttcgctttccccctccctattgccacggcggaactcatcgccgcctgccttgcccgctgctggacaggggctcggctgttgggcactgacaattccgtggtgttgtcggggaaatcatcgtcctttccttggctgctcgcctgtgttgccacctggattctgcgcgggacgtccttctgctacgtcccttcggccctcaatccagcggaccttccttcccgcggcctgctgccggctctgcggcctcttccgcgtcttcgccttcgccctcagacgagtcggatctccctttgggccgcctccccgcgtcgactttaagaccaatgacggccgaataaaagatctttattttcattagatctgtgtgttggttttttgtgtgcggccgcaggaacccctagtgatggagttggccactccctctctgcgcgctcgctcgctcactgaggccgggcgaccaaaggtcgcccgacgcccgggctttgcccgggcggcctcagtgagcgagcgagcgcgcagctgcctgcaggggcgcctgatgcggtattttctccttacgcatctgtgcggtatttcacaccgcatacgtcaaagcaaccatagtacgcgccctgtagcggcgcattaagcgcggcgggtgtggtggttacgcgcagcgtgaccgctacacttgccagcgccttagcgcccgctcctttcgctttcttcccttcctttctcgccacgttcgccggctttccccgtcaagctctaaatcgggggctccctttagggttccgatttagtgctttacggcacctcgaccccaaaaaacttgatttgggtgatggttcacgtagtgggccatcgccctgatagacggtttttcgccctttgacgttggagtccacgttctttaatagtggactcttgttccaaactggaacaacactcaactctatctcgggctattcttttgatttataagggattttgccgatttcggtctattggttaaaaaatgagctgatttaacaaaaatttaacgcgaattttaacaaaatattaacgtttacaattttatggtgcactctcagtacaatctgctctgatgccgcatagttaagccagccccgacacccgccaacacccgctgacgcgccctgacgggcttgtctgctcccggcatccgcttacagacaagctgtgaccgtctccgggagctgcatgtgtcagaggttttcaccgtcatcaccgaaacgcgcgagacgaaagggcctcgtgatacgcctatttttataggttaatgtcatgataataatggtttcttagacgtcaggtggcacttttcggggaaatgtgcgcggaacccctatttgtttatttttctaaatacattcaaatatgtatccgctcatgagacaataaccctgataaatgcttcaataatattgaaaaaggaagagtatgagtattcaacatttccgtgtcgcccttattcccttttttgcggcattttgccttcctgtttttgctcacccagaaacgctggtgaaagtaaaagatgctgaagatcagttgggtgcacgagtgggttacatcgaactggatctcaacagcggtaagatccttgagagttttcgccccgaagaacgttttccaatgatgagcacttttaaagttctgctatgtggcgcggtattatcccgtattgacgccgggcaagagcaactcggtcgccgcatacactattctcagaatgacttggttgagtactcaccagtcacagaaaagcatcttacggatggcatgacagtaagagaattatgcagtgctgccataaccatgagtgataacactgcggccaacttacttctgacaacgatcggaggaccgaaggagctaaccgcttttttgcacaacatgggggatcatgtaactcgccttgatcgttgggaaccggagctgaatgaagccataccaaacgacgagcgtgacaccacgatgcctgtagcaatggcaacaacgttgcgcaaactattaactggcgaactacttactctagcttcccggcaacaattaatagactggatggaggcggataaagttgcaggaccacttctgcgctcggcccttccggctggctggtttattgctgataaatctggagccggtgagcgtggaagccgcggtatcattgcagcactggggccagatggtaagccctcccgtatcgtagttatctacacgacggggagtcaggcaactatggatgaacgaaatagacagatcgctgagataggtgcctcactgattaagcattggtaactgtcagaccaagtttactcatatatactttagattgatttaaaacttcatttttaatttaaaaggatctaggtgaagatcctttttgataatctcatgaccaaaatcccttaacgtgagttttcgttccactgagcgtcagaccccgtagaaaagatcaaaggatcttcttgagatcctttttttctgcgcgtaatctgctgcttgcaaacaaaaaaaccaccgctaccagcggtggtttgtttgccggatcaagagctaccaactctttttccgaaggtaactggcttcagcagagcgcagataccaaatactgttcttctagtgtagccgtagttaggccaccacttcaagaactctgtagcaccgcctacatacctcgctctgctaatcctgttaccagtggctgctgccagtggcgataagtcgtgtcttaccgggttggactcaagacgatagttaccggataaggcgcagcggtcgggctgaacggggggttcgtgcacacagcccagcttggagcgaacgacctacaccgaactgagatacctacagcgtgagctatgagaaagcgccacgcttcccgaagggagaaaggcggacaggtatccggtaagcggcagggtcggaacaggagagcgcacgagggagcttccagggggaaacgcctggtatctttatagtcctgtcgggtttcgccacctctgacttgagcgtcgatttttgtgatgctcgtcaggggggcggagcctatggaaaaacgccagcaacgcggcctttttacggttcctggccttttgctggccttttgctcacatgt

SEQ ID NO: 55 - DNA, 6914 bp, Artificial Sequence
  pGW036
cctgcaggcagctgcgcgctcgctcgctcactgaggccgcccgggcgtcgggcgacctttggtcgcccggcctcagtgagcgagcgagcgcgcagagagggagtggccaactccatcactaggggttcctgcggcctctagaaaggatctgcgatcgctccggtgcccgtcagtgggcagagcgcacatcgcccacagtccccgagaagttggggggaggggtcggcaattgaacgggtgcctagagaaggtggcgcggggtaaactgggaaagtgatgtcgtgtactggctccgcctttttcccgagggtgggggagaaccgtatataagtgcagtagtcgccgtgaacgttctttttcgcaacgggtttgccgccagaacacagctgaagcttcgaggggctcgcatctctccttcacgcgcccgccgccctacctgaggccgccatccacgccggttgagtcgcgttctgccgcctcccgcctgtggtgcctcctgaactgcgtccgccgtctaggtaagtttaaagctcaggtcgagaccgggcctttgtccggcgctcccttggagcctacctagactcagccggctctccacgctttgcctgaccctgcttgctcaactctacgtctttgtttcgttttctgttctgcgccgttacagatctggctaactaccggtgccaccatggccccaaagaagaagcggaaggtcggtatccacggagtcccagcagccaagcggaactacatcctgggcctggccatcggcatcaccagcgtgggctacggcatcatcgactacgagacacgggacgtgatcgatgccggcgtgcggctgttcaaagaggccaacgtggaaaacaacgagggcaggcggagcaagagaggcgccagaaggctgaagcggcggaggcggcatagaatccagagagtgaagaagctgctgttcgactacaacctgctgaccgaccacagcgagctgagcggcatcaacccctacgaggccagagtgaagggcctgagccagaagctgagcgaggaagagttctctgccgccctgctgcacctggccaagagaagaggcgtgcacaacgtgaacgaggtggaagaggacaccggcaacgagctgtccaccaaagagcagatcagccggaacagcaaggccctggaagagaaatacgtggccgaactgcagctggaacggctgaagaaagacggcgaagtgcggggcagcatcaacagattcaagaccagcgactacgtgaaagaagccaaacagctgctgaaggtgcagaaggcctaccaccagctggaccagagcttcatcgacacctacatcgacctgctggaaacccggcggacctactatgagggacctggcgagggcagccccttcggctggaaggacatcaaagaatggtacgagatgctgatgggccactgcacctacttccccgaggaactgcggagcgtgaagtacgcctacaacgccgacctgtacaacgccctgaacgacctgaacaatctcgtgatcaccagggacgagaacgagaagctggaatattacgagaagttccagatcatcgagaacgtgttcaagcagaagaagaagcccaccctgaagcagatcgccaaagaaatcctcgtgaacgaagaggatattaagggctacagagtgaccagcaccggcaagcccgagttcaccaacctgaaggtgtaccacgacatcaaggacattaccgcccggaaagagattattgagaacgccgagctgctggatcagattgccaagatcctgaccatctaccagagcagcgaggacatccaggaagaactgaccaatctgaactccgagctgacccaggaagagatcgagcagatctctaatctgaagggctataccggcacccacaacctgagcctgaaggccatcaacctgatcctggacgagctgtggcacaccaacgacaaccagatcgctatcttcaaccggctgaagctggtgcccaagaaggtggacctgtcccagcagaaagagatccccaccaccctggtggacgacttcatcctgagccccgtcgtgaagagaagcttcatccagagcatcaaagtgatcaacgccatcatcaagaagtacggcctgcccaacgacatcattatcgagctggcccgcgagaagaactccaaggacgcccagaaaatgatcaacgagatgcagaagcggaaccggcagaccaacgagcggatcgaggaaatcatccggaccaccggcaaagagaacgccaagtacctgatcgagaagatcaagctgcacgacatgcaggaaggcaagtgcctgtacagcctggaagccatccctctggaagatctgctgaacaaccccttcaactatgaggtggaccacatcatccccagaagcgtgtccttcgacaacagcttcaacaacaaggtgctcgtgaagcaggaagaagccagcaagaagggcaaccggaccccattccagtacctgagcagcagcgacagcaagatcagctacgaaaccttcaagaagcacatcctgaatctggccaagggcaagggcagaatcagcaagaccaagaaagagtatctgctggaagaacgggacatcaacaggttctccgtgcagaaagacttcatcaaccggaacctggtggataccagatacgccaccagaggcctgatgaacctgctgcggagctacttcagagtgaacaacctggacgtgaaagtgaagtccatcaatggcggcttcaccagctttctgcggcggaagtggaagtttaagaaagagcggaacaaggggtacaagcaccacgccgaggacgccctgatcattgccaacgccgatttcatcttcaaagagtggaagaaactggacaaggccaaaaaagtgatggaaaaccagatgttcgaggaaaagcaggccgagagcatgcccgagatcgaaaccgagcaggagtacaaagagatcttcatcaccccccaccagatcaagcacattaaggacttcaaggactacaagtacagccaccgggtggacaagaagcctaatagagagctgattaacgacaccctgtactccacccggaaggacgacaagggcaacaccctgatcgtgaacaatctgaacggcctgtacgacaaggacaatgacaagctgaaaaagctgatcaacaagagccccgaaaagctgctgatgtaccaccacgacccccagacctaccagaaactgaagctgattatggaacagtacggcgacgagaagaatcccctgtacaagtactacgaggaaaccgggaactacctgaccaagtactccaaaaaggacaacggccccgtgatcaagaagattaagtattacggcaacaaactgaacgcccatctggacatcaccgacgactaccccaacagcagaaacaaggtcgtgaagctgtccctgaagccctacagattcgacgtgtacctggacaatggcgtgtacaagttcgtgaccgtgaagaatctggatgtgatcaaaaaagaaaactactacgaagtgaatagcaagtgctatgaggaagctaagaagctgaagaagatcagcaaccaggccgagtttatcgcctccttctacaacaacgatctgatcaagatcaacggcgagctgtatagagtgatcggcgtgaacaacgacctgctgaaccggatcgaagtgaacatgatcgacatcacctaccgcgagtacctggaaaacatgaacgacaagaggccccccaggatcattaagacaatcgcctccaagacccagagcattaagaagtacagcacagacattctgggcaacctgtatgaagtgaaatctaagaagcaccctcagatcatcaaaaagggcaaaaggccggcggccacgaaaaaggccggccaggcaaaaaagaaaaagggatccggacgggctgacgcattggacgattttgatctggatatgctgggaagtgacgccctcgatgattttgaccttgacatgcttggttcggatgcccttgatgactttgacctcgacatgctcggcagtgacgcccttgatgatttcgacctggacatgctgatttaagaattcaataaaagatctttattttcattagatctgtgtgttggttttttgtgtgcggccgcaggaacccctagtgatggagttggccactccctctctgcgcgctcgctcgctcactgaggccgggcgaccaaaggtcgcccgacgcccgggctttgcccgggcggcctcagtgagcgagcgagcgcgcagctgcctgcaggggcgcctgatgcggtattttctccttacgcatctgtgcggtatttcacaccgcatacgtcaaagcaaccatagtacgcgccctgtagcggcgcattaagcgcggcgggtgtggtggttacgcgcagcgtgaccgctacacttgccagcgccttagcgcccgctcctttcgctttcttcccttcctttctcgccacgttcgccggctttccccgtcaagctctaaatcgggggctccctttagggttccgatttagtgctttacggcacctcgaccccaaaaaacttgatttgggtgatggttcacgtagtgggccatcgccctgatagacggtttttcgccctttgacgttggagtccacgttctttaatagtggactcttgttccaaactggaacaacactcaactctatctcgggctattcttttgatttataagggattttgccgatttcggtctattggttaaaaaatgagctgatttaacaaaaatttaacgcgaattttaacaaaatattaacgtttacaattttatggtgcactctcagtacaatctgctctgatgccgcatagttaagccagccccgacacccgccaacacccgctgacgcgccctgacgggcttgtctgctcccggcatccgcttacagacaagctgtgaccgtctccgggagctgcatgtgtcagaggttttcaccgtcatcaccgaaacgcgcgagacgaaagggcctcgtgatacgcctatttttataggttaatgtcatgataataatggtttcttagacgtcaggtggcacttttcggggaaatgtgcgcggaacccctatttgtttatttttctaaatacattcaaatatgtatccgctcatgagacaataaccctgataaatgcttcaataatattgaaaaaggaagagtatgagtattcaacatttccgtgtcgcccttattcccttttttgcggcattttgccttcctgtttttgctcacccagaaacgctggtgaaagtaaaagatgctgaagatcagttgggtgcacgagtgggttacatcgaactggatctcaacagcggtaagatccttgagagttttcgccccgaagaacgttttccaatgatgagcacttttaaagttctgctatgtggcgcggtattatcccgtattgacgccgggcaagagcaactcggtcgccgcatacactattctcagaatgacttggttgagtactcaccagtcacagaaaagcatcttacggatggcatgacagtaagagaattatgcagtgctgccataaccatgagtgataacactgcggccaacttacttctgacaacgatcggaggaccgaaggagctaaccgcttttttgcacaacatgggggatcatgtaactcgccttgatcgttgggaaccggagctgaatgaagccataccaaacgacgagcgtgacaccacgatgcctgtagcaatggcaacaacgttgcgcaaactattaactggcgaactacttactctagcttcccggcaacaattaatagactggatggaggcggataaagttgcaggaccacttctgcgctcggcccttccggctggctggtttattgctgataaatctggagccggtgagcgtggaagccgcggtatcattgcagcactggggccagatggtaagccctcccgtatcgtagttatctacacgacggggagtcaggcaactatggatgaacgaaatagacagatcgctgagataggtgcctcactgattaagcattggtaactgtcagaccaagtttactcatatatactttagattgatttaaaacttcatttttaatttaaaaggatctaggtgaagatcctttttgataatctcatgaccaaaatcccttaacgtgagttttcgttccactgagcgtcagaccccgtagaaaagatcaaaggatcttcttgagatcctttttttctgcgcgtaatctgctgcttgcaaacaaaaaaaccaccgctaccagcggtggtttgtttgccggatcaagagctaccaactctttttccgaaggtaactggcttcagcagagcgcagataccaaatactgttcttctagtgtagccgtagttaggccaccacttcaagaactctgtagcaccgcctacatacctcgctctgctaatcctgttaccagtggctgctgccagtggcgataagtcgtgtcttaccgggttggactcaagacgatagttaccggataaggcgcagcggtcgggctgaacggggggttcgtgcacacagcccagcttggagcgaacgacctacaccgaactgagatacctacagcgtgagctatgagaaagcgccacgcttcccgaagggagaaaggcggacaggtatccggtaagcggcagggtcggaacaggagagcgcacgagggagcttccagggggaaacgcctggtatctttatagtcctgtcgggtttcgccacctctgacttgagcgtcgatttttgtgatgctcgtcaggggggcggagcctatggaaaaacgccagcaacgcggcctttttacggttcctggccttttgctggccttttgctcacatgt

SEQ ID NO: 56 - DNA, 7454 bp, Artificial Sequence
  pGW011b
cctgcaggcagctgcgcgctcgctcgctcactgaggccgcccgggcaaagcccgggcgtcgggcgacctttggtcgcccggcctcagtgagcgagcgagcgcgcagagagggagtggccaactccatcactaggggttcctgcggccgcacgcgttctaggtcttgaaaggagtgggaattggctccggtgcccgtcagtgggcagagcgcacatcgcccacagtccccgagaagttggggggaggggtcggcaattgatccggtgcctagagaaggtggcgcggggtaaactgggaaagtgatgtcgtgtactggctccgcctttttcccgagggtgggggagaaccgtatataagtgcagtagtcgccgtgaacgttctttttcgcaacgggtttgccgccagaacacaggtgtcgtgacgcgcgtacgtaatacgactcactatagggccgccaccatgaaaaggccggcggccacgaaaaaggccggccaggcaaaaaagaaaaaggacaagaagtacagcatcggcctggccatcggcaccaactctgtgggctgggccgtgatcaccgacgagtacaaggtgcccagcaagaaattcaaggtgctgggcaacaccgaccggcacagcatcaagaagaacctgatcggagccctgctgttcgacagcggcgaaacagccgaggccacccggctgaagagaaccgccagaagaagatacaccagacggaagaaccggatctgctatctgcaagagatcttcagcaacgagatggccaaggtggacgacagcttcttccacagactggaagagtccttcctggtggaagaggataagaagcacgagcggcaccccatcttcggcaacatcgtggacgaggtggcctaccacgagaagtaccccaccatctaccacctgagaaagaaactggtggacagcaccgacaaggccgacctgcggctgatctatctggccctggcccacatgatcaagttccggggccacttcctgatcgagggcgacctgaaccccgacaacagcgacgtggacaagctgttcatccagctggtgcagacctacaaccagctgttcgaggaaaaccccatcaacgccagcggcgtggacgccaaggccatcctgtctgccagactgagcaagagcagacggctggaaaatctgatcgcccagctgcccggcgagaagaagaatggcctgttcggcaacctgattgccctgagcctgggcctgacccccaacttcaagagcaacttcgacctggccgaggatgccaaactgcagctgagcaaggacacctacgacgacgacctggacaacctgctggcccagatcggcgaccagtacgccgacctgtttctggccgccaagaacctgtccgacgccatcctgctgagcgacatcctgagagtgaacaccgagatcaccaaggcccccctgagcgcctctatgatcaagagatacgacgagcaccaccaggacctgaccctgctgaaagctctcgtgcggcagcagctgcctgagaagtacaaagagattttcttcgaccagagcaagaacggctacgccggctacattgacggcggagccagccaggaagagttctacaagttcatcaagcccatcctggaaaagatggacggcaccgaggaactgctcgtgaagctgaacagagaggacctgctgcggaagcagcggaccttcgacaacggcagcatcccccaccagatccacctgggagagctgcacgccattctgcggcggcaggaagatttttacccattcctgaaggacaaccgggaaaagatcgagaagatcctgaccttccgcatcccctactacgtgggccctctggccaggggaaacagcagattcgcctggatgaccagaaagagcgaggaaaccatcaccccctggaacttcgaggaagtggtggacaagggcgcttccgcccagagcttcatcgagcggatgaccaacttcgataagaacctgcccaacgagaaggtgctgcccaagcacagcctgctgtacgagtacttcaccgtgtataacgagctgaccaaagtgaaatacgtgaccgagggaatgagaaagcccgccttcctgagcggcgagcagaaaaaggccatcgtggacctgctgttcaagaccaaccggaaagtgaccgtgaagcagctgaaagaggactacttcaagaaaatcgagtgcttcgactccgtggaaatctccggcgtggaagatcggttcaacgcctccctgggcacataccacgatctgctgaaaattatcaaggacaaggacttcctggacaatgaggaaaacgaggacattctggaagatatcgtgctgaccctgacactgtttgaggacagagagatgatcgaggaacggctgaaaacctatgcccacctgttcgacgacaaagtgatgaagcagctgaagcggcggagatacaccggctggggcaggctgagccggaagctgatcaacggcatccgggacaagcagtccggcaagacaatcctggatttcctgaagtccgacggcttcgccaacagaaacttcatgcagctgatccacgacgacagcctgacctttaaagaggacatccagaaagcccaggtgtccggccagggcgatagcctgcacgagcacattgccaatctggccggcagccccgccattaagaagggcatcctgcagacagtgaaggtggtggacgagctcgtgaaagtgatgggccggcacaagcccgagaacatcgtgatcgaaatggccagagagaaccagaccacccagaagggacagaagaacagccgcgagagaatgaagcggatcgaagagggcatcaaagagctgggcagccagatcctgaaagaacaccccgtggaaaacacccagctgcagaacgagaagctgtacctgtactacctgcagaatgggcgggatatgtacgtggaccaggaactggacatcaaccggctgtccgactacgatgtggaccacatcgtgcctcagagctttctgaaggacgactccatcgacaacaaggtgctgaccagaagcgacaaggcccggggcaagagcgacaacgtgccctccgaagaggtcgtgaagaagatgaagaactactggcggcagctgctgaacgccaagctgattacccagagaaagttcgacaatctgaccaaggccgagagaggcggcctgagcgaactggataaggccggcttcatcaagagacagctggtggaaacccggcagatcacaaagcacgtggcacagatcctggactcccggatgaacactaagtacgacgagaatgacaagctgatccgggaagtgaaagtgatcaccctgaagtccaagctggtgtccgatttccggaaggatttccagttttacaaagtgcgcgagatcaacaactaccaccacgcccacgacgcctacctgaacgccgtcgtgggaaccgccctgatcaaaaagtaccctaagctggaaagcgagttcgtgtacggcgactacaaggtgtacgacgtgcggaagatgatcgccaagagcgagcaggaaatcggcaaggctaccgccaagtacttcttctacagcaacatcatgaactttttcaagaccgagattaccctggccaacggcgagatccggaagcggcctctgatcgagacaaacggcgaaaccggggagatcgtgtgggataagggccgggattttgccaccgtgcggaaagtgctgagcatgccccaagtgaatatcgtgaaaaagaccgaggtgcagacaggcggcttcagcaaagagtctatcctgcccaagaggaacagcgataagctgatcgccagaaagaaggactgggaccctaagaagtacggcggcttcgacagccccaccgtggcctattctgtgctggtggtggccaaagtggaaaagggcaagtccaagaaactgaagagtgtgaaagagctgctggggatcaccatcatggaaagaagcagcttcgagaagaatcccatcgactttctggaagccaagggctacaaagaagtgaaaaaggacctgatcatcaagctgcctaagtactccctgttcgagctggaaaacggccggaagagaatgctggcctctgccggcgaactgcagaagggaaacgaactggccctgccctccaaatatgtgaacttcctgtacctggccagccactatgagaagctgaagggctcccccgaggataatgagcagaaacagctgtttgtggaacagcacaagcactacctggacgagatcatcgagcagatcagcgagttctccaagagagtgatcctggccgacgctaatctggacaaagtgctgtccgcctacaacaagcaccgggataagcccatcagagagcaggccgagaatatcatccacctgtttaccctgaccaatctgggagcccctgccgccttcaagtactttgacaccaccatcgaccggaagaggtacaccagcaccaaagaggtgctggacgccaccctgatccaccagagcatcaccggcctgtacgagacacggatcgacctgtctcagctgggaggcgacagccctaagaaaaagaggaaggtgagctgagaattcaataaataaaagatctttattttcattagatctgtgtgttggttttttgtgtgcggaccgagcggccgcaggaacccctagtgatggagttggccactccctctctgcgcgctcgctcgctcactgaggccgggcgaccaaaggtcgcccgacgcccgggctttgcccgggcggcctcagtgagcgagcgagcgcgcagctgcctgcaggggcgcctgatgcggtattttctccttacgcatctgtgcggtatttcacaccgcatacgtcaaagcaaccatagtacgcgccctgtagcggcgcattaagcgcggcgggtgtggtggttacgcgcagcgtgaccgctacacttgccagcgccctagcgcccgctcctttcgctttcttcccttcctttctcgccacgttcgccggctttccccgtcaagctctaaatcgggggctccctttagggttccgatttagtgctttacggcacctcgaccccaaaaaacttgatttgggtgatggttcacgtagtgggccatcgccctgatagacggtttttcgccctttgacgttggagtccacgttctttaatagtggactcttgttccaaactggaacaacactcaaccctatctcgggctattcttttgatttataagggattttgccgatttcggcctattggttaaaaaatgagctgatttaacaaaaatttaacgcgaattttaacaaaatattaacgtttacaattttatggtgcactctcagtacaatctgctctgatgccgcatagttaagccagccccgacacccgccaacacccgctgacgcgccctgacgggcttgtctgctcccggcatccgcttacagacaagctgtgaccgtctccgggagctgcatgtgtcagaggttttcaccgtcatcaccgaaacgcgcgagacgaaagggcctcgtgatacgcctatttttataggttaatgtcatgataataatggtttcttagacgtcaggtggcacttttcggggaaatgtgcgcggaacccctatttgtttatttttctaaatacattcaaatatgtatccgctcatgagacaataaccctgataaatgcttcaataatattgaaaaaggaagagtatgagtattcaacatttccgtgtcgcccttattcccttttttgcggcattttgccttcctgtttttgctcacccagaaacgctggtgaaagtaaaagatgctgaagatcagttgggtgcacgagtgggttacatcgaactggatctcaacagcggtaagatccttgagagttttcgccccgaagaacgttttccaatgatgagcacttttaaagttctgctatgtggcgcggtattatcccgtattgacgccgggcaagagcaactcggtcgccgcatacactattctcagaatgacttggttgagtactcaccagtcacagaaaagcatcttacggatggcatgacagtaagagaattatgcagtgctgccataaccatgagtgataacactgcggccaacttacttctgacaacgatcggaggaccgaaggagctaaccgcttttttgcacaacatgggggatcatgtaactcgccttgatcgttgggaaccggagctgaatgaagccataccaaacgacgagcgtgacaccacgatgcctgtagcaatggcaacaacgttgcgcaaactattaactggcgaactacttactctagcttcccggcaacaattaatagactggatggaggcggataaagttgcaggaccacttctgcgctcggcccttccggctggctggtttattgctgataaatctggagccggtgagcgtgggtctcgcggtatcattgcagcactggggccagatggtaagccctcccgtatcgtagttatctacacgacggggagtcaggcaactatggatgaacgaaatagacagatcgctgagataggtgcctcactgattaagcattggtaactgtcagaccaagtttactcatatatactttagattgatttaaaacttcatttttaatttaaaaggatctaggtgaagatcctttttgataatctcatgaccaaaatcccttaacgtgagttttcgttccactgagcgtcagaccccgtagaaaagatcaaaggatcttcttgagatcctttttttctgcgcgtaatctgctgcttgcaaacaaaaaaaccaccgctaccagcggtggtttgtttgccggatcaagagctaccaactctttttccgaaggtaactggcttcagcagagcgcagataccaaatactgtccttctagtgtagccgtagttaggccaccacttcaagaactctgtagcaccgcctacatacctcgctctgctaatcctgttaccagtggctgctgccagtggcgataagtcgtgtcttaccgggttggactcaagacgatagttaccggataaggcgcagcggtcgggctgaacggggggttcgtgcacacagcccagcttggagcgaacgacctacaccgaactgagatacctacagcgtgagctatgagaaagcgccacgcttcccgaagggagaaaggcggacaggtatccggtaagcggcagggtcggaacaggagagcgcacgagggagcttccagggggaaacgcctggtatctttatagtcctgtcgggtttcgccacctctgacttgagcgtcgatttttgtgatgctcgtcaggggggcggagcctatggaaaaacgccagcaacgcggcctttttacggttcctggccttttgctggccttttgctcacatgt

SEQ ID NO: 57 - DNA, 3997 bp, Artificial Sequence
  pGW089
cctgcaggcagctgcgcgctcgctcgctcactgaggccgcccgggcgtcgggcgacctttggtcgcccggcctcagtgagcgagcgagcgcgcagagagggagtggccaactccatcactaggggttcctgcggcctctagaaaggatctgcgatcgctccggtgcccgtcagtgggcagagcgcacatcgcccacagtccccgagaagttggggggaggggtcggcaattgaacgggtgcctagagaaggtggcgcggggtaaactgggaaagtgatgtcgtgtactggctccgcctttttcccgagggtgggggagaaccgtatataagtgcagtagtcgccgtgaacgttctttttcgcaacgggtttgccgccagaacacagctgaagcttcgaggggctcgcatctctccttcacgcgcccgccgccctacctgaggccgccatccacgccggttgagtcgcgttctgccgcctcccgcctgtggtgcctcctgaactgcgtccgccgtctaggtaagtttaaagctcaggtcgagaccgggcctttgtccggcgctcccttggagcctacctagactcagccggctctccacgctttgcctgaccctgcttgctcaactctacgtctttgtttcgttttctgttctgcgccgttacagatctggctaactaccggtgccacatgtacagcatgcagctcgcatcctgtgtcacattgacacttgtgctccttgtcaacagcgcacccacttcaagctccacttcaagctctacagcggaagcacagcagcagcagcagcagcagcagcagcagcagcagcacctggagcagctgttgatggacctacaggagctcctgagcaggatggagaattacaggaacctgaaactccccaggatgctcaccttcaaattttacttgcccaagcaggccacagaattgaaagatcttcagtgcctagaagatgaacttggacctctgcggcatgttctggatttgactcaaagcaaaagctttcaattggaagatgctgagaatttcatcagcaatatcagagtaactgttgtaaaactaaagggctctgacaacacatttgagtgccaattcgatgatgagtcagcaactgtggtggactttctgaggagatggatagccttctgtcaaagcatcatctcaacaagccctcaataagaattcaataaaagatctttattttcattagatctgtgtgttggttttttgtgtgcggccgcaggaacccctagtgatggagttggccactccctctctgcgcgctcgctcgctcactgaggccgggcgaccaaaggtcgcccgacgcccgggctttgcccgggcggcctcagtgagcgagcgagcgcgcagctgcctgcaggggcgcctgatgcggtattttctccttacgcatctgtgcggtatttcacaccgcatacgtcaaagcaaccatagtacgcgccctgtagcggcgcattaagcgcggcgggtgtggtggttacgcgcagcgtgaccgctacacttgccagcgccttagcgcccgctcctttcgctttcttcccttcctttctcgccacgttcgccggctttccccgtcaagctctaaatcgggggctccctttagggttccgatttagtgctttacggcacctcgaccccaaaaaacttgatttgggtgatggttcacgtagtgggccatcgccctgatagacggtttttcgccctttgacgttggagtccacgttctttaatagtggactcttgttccaaactggaacaacactcaactctatctcgggctattcttttgatttataagggattttgccgatttcggtctattggttaaaaaatgagctgatttaacaaaaatttaacgcgaattttaacaaaatattaacgtttacaattttatggtgcactctcagtacaatctgctctgatgccgcatagttaagccagccccgacacccgccaacacccgctgacgcgccctgacgggcttgtctgctcccggcatccgcttacagacaagctgtgaccgtctccgggagctgcatgtgtcagaggttttcaccgtcatcaccgaaacgcgcgagacgaaagggcctcgtgatacgcctatttttataggttaatgtcatgataataatggtttcttagacgtcaggtggcacttttcggggaaatgtgcgcggaacccctatttgtttatttttctaaatacattcaaatatgtatccgctcatgagacaataaccctgataaatgcttcaataatattgaaaaaggaagagtatgagtattcaacatttccgtgtcgcccttattcccttttttgcggcattttgccttcctgtttttgctcacccagaaacgctggtgaaagtaaaagatgctgaagatcagttgggtgcacgagtgggttacatcgaactggatctcaacagcggtaagatccttgagagttttcgccccgaagaacgttttccaatgatgagcacttttaaagttctgctatgtggcgcggtattatcccgtattgacgccgggcaagagcaactcggtcgccgcatacactattctcagaatgacttggttgagtactcaccagtcacagaaaagcatcttacggatggcatgacagtaagagaattatgcagtgctgccataaccatgagtgataacactgcggccaacttacttctgacaacgatcggaggaccgaaggagctaaccgcttttttgcacaacatgggggatcatgtaactcgccttgatcgttgggaaccggagctgaatgaagccataccaaacgacgagcgtgacaccacgatgcctgtagcaatggcaacaacgttgcgcaaactattaactggcgaactacttactctagcttcccggcaacaattaatagactggatggaggcggataaagttgcaggaccacttctgcgctcggcccttccggctggctggtttattgctgataaatctggagccggtgagcgtggaagccgcggtatcattgcagcactggggccagatggtaagccctcccgtatcgtagttatctacacgacggggagtcaggcaactatggatgaacgaaatagacagatcgctgagataggtgcctcactgattaagcattggtaactgtcagaccaagtttactcatatatactttagattgatttaaaacttcatttttaatttaaaaggatctaggtgaagatcctttttgataatctcatgaccaaaatcccttaacgtgagttttcgttccactgagcgtcagaccccgtagaaaagatcaaaggatcttcttgagatcctttttttctgcgcgtaatctgctgcttgcaaacaaaaaaaccaccgctaccagcggtggtttgtttgccggatcaagagctaccaactctttttccgaaggtaactggcttcagcagagcgcagataccaaatactgttcttctagtgtagccgtagttaggccaccacttcaagaactctgtagcaccgcctacatacctcgctctgctaatcctgttaccagtggctgctgccagtggcgataagtcgtgtcttaccgggttggactcaagacgatagttaccggataaggcgcagcggtcgggctgaacggggggttcgtgcacacagcccagcttggagcgaacgacctacaccgaactgagatacctacagcgtgagctatgagaaagcgccacgcttcccgaagggagaaaggcggacaggtatccggtaagcggcagggtcggaacaggagagcgcacgagggagcttccagggggaaacgcctggtatctttatagtcctgtcgggtttcgccacctctgacttgagcgtcgatttttgtgatgctcgtcaggggggcggagcctatggaaaaacgccagcaacgcggcctttttacggttcctggccttttgctggccttttgctcacatgt

SEQ ID NO: 58 - DNA, 7319 bp, Artificial Sequence
  pGW094
cctgcaggcagctgcgcgctcgctcgctcactgaggccgcccgggcgtcgggcgacctttggtcgcccggcctcagtgagcgagcgagcgcgcagagagggagtggccaactccatcactaggggttcctgcggcctctagaaaggatctgcgatcgctccggtgcccgtcagtgggcagagcgcacatcgcccacagtccccgagaagttggggggaggggtcggcaattgaacgggtgcctagagaaggtggcgcggggtaaactgggaaagtgatgtcgtgtactggctccgcctttttcccgagggtgggggagaaccgtatataagtgcagtagtcgccgtgaacgttctttttcgcaacgggtttgccgccagaacacagctgaagcttcgaggggctcgcatctctccttcacgcgcccgccgccctacctgaggccgccatccacgccggttgagtcgcgttctgccgcctcccgcctgtggtgcctcctgaactgcgtccgccgtctaggtaagtttaaagctcaggtcgagaccgggcctttgtccggcgctcccttggagcctacctagactcagccggctctccacgctttgcctgaccctgcttgctcaactctacgtctttgtttcgttttctgttctgcgccgttacagatctggctaactaccggtgccaccatgaacgctacacactgcatcttggctttgcagctcttcctcatggctgtttctggctgttactgccacggcacagtcattgaaagcctagaaagtctgaataactattttaactcaagtggcatagatgtggaagaaaagagtctcttcttggatatctggaggaactggcaaaaggatggtgacatgaaaatcctgcagagccagattatctctttctacctcagactctttgaagtcttgaaagacaatcaggccatcagcaacaacataagcgtcattgaatcacacctgattactaccttcttcagcaacagcaaggcgaaaaaggatgcattcatgagtattgccaagtttgaggtcaacaacccacaggtccagcgccaagcattcaatgagctcatccgagtggtccaccagctgttgccggaatccagcctcaggaagcggaaaaggagtcgctgcggatccggcgcaacaaacttctctctgctgaaacaagccggagatgtcgaagagaatcctggaccgatggcttgcaattgtcagttgatgcaggatacaccactcctcaagtttccatgtccaaggctcattcttctctttgtgctgctgattcgtctttcacaagtgtcttcagatgttgatgaacaactgtccaagtcagtgaaagataaggtattgctgccttgccgttacaactctcctcatgaagatgagtctgaagaccgaatctactggcaaaaacatgacaaagtggtgctgtctgtcattgttgggaaactaaaagtgtggcccgagtataagaaccggactttatatgacaacactacctactctcttatcatcctgggcctggtcctttcagaccggggcacatacagctgtgtcgttcaaaagaaggaaagaggaacgtatgaagttaaacacttggctttagtaaagttgtccatcaaagctgacttctctacccccaacataactgagtctggaaacccatctgcagacactaaaaggattacctgctttgcttccgggggtttcccaaagcctcgcttctcttggttggaaaatggaagagaattacctggcatcaatacgacaatttcccaggatcctgaatctgaattgtacaccattagtagccaactagatttcaatacgactcgcaaccacaccattaagtgtctcattaaatatggagatgctcacgtgtcagaggacttcacctgggaaaaacccccagaagaccctcctgatagcaagaacacacttgtgctctttggggcaggattcggcgcagtaataacagtcgtcgtcatcgttgtcatcatcaaatgcttctgtaagcacagaagctgtttcagaagaaatgaggcaagcagagaaacaaacaacagccttaccttcgggcctgaagaagcattagctgaacagaccgtcttccttcgtacgggcagtggagagggcagaggaagtctgctaacatgcggtgacgtcgaggagaatcctggcccaatggagagtgtggtacagccttcagtgtttgtggtggatggacagacggacatcccattcaggcggctggaacagaaccaccggagacggcgctgtggcactgtccaggtcagcctggccctggtgctgctgctaggtgctgggctggccactcagggctggtttctcctgagactgcatcaacgtcttggagacatagtagctcatctgccagatggaggcaaaggctcctgggagaagctgatacaagatcaacgatctcaccaggccaacccagcagcacatcttacaggagccaacgccagcttgataggtattggtggacctctgttatgggagacacgacttggcctggccttcttgaggggcttgacgtatcatgatggggccctggtgaccatggagcccggttactactatgtgtactccaaagtgcagctgagcggcgtgggctgcccccaggggctggccaatggcctccccatcacccatggactatacaagcgcacatcccgctacccgaaggagttagaactgctggtcagtcggcggtcaccctgtggccgggccaacagctcccgagtctggtgggacagcagcttcctgggcggcgtggtacatctggaggctggggaagaggtggtggtccgcgtgcctggaaaccgcctggtcagaccacgtgacggcaccaggtcctatttcggagctttcatggtcactagtggatccggcgcaacaaacttctctctgctgaaacaagccggagatgtcgaagagaatcctggaccgatggaggaaatgcctttgagagagtcaagtcctcaaagggcagagaggtgcaagaagtcatggctcttgtgcatagtggctctgttactgatgctgctctgttctttgggtacactgatctatacttcactcaagccaactgccatcgagtcctgcatggttaagtttgaactatcatcctcaaaatggcacatgacatctcccaaacctcactgtgtgaatacgacatctgatgggaagctgaagatactgcagagtggcacatatttaatctacggccaagtgattcctgtggataagaaatacataaaagacaatgcccccttcgtagtacagatatataaaaagaatgatgtcctacaaactctaatgaatgattttcaaatcttgcctataggaggggtttatgaactgcatgctggagataacatatatctgaagttcaactctaaagaccatattcagaaaaataacacatactgggggatcatcttaatgcctgatctaccattcatctctgctagcagcggtacccagtgcaccaactacgccctgctgaagctggccggcgatgtggagagcaaccccgggcccatggaccagcacacacttgatgtggaggataccgcggatgccagacatccagcaggtacttcgtgcccctcggatgcggcgctcctcagagataccgggctcctcgcggacgctgcgctcctctcagatactgtgcgccccacaaatgccgcgctccccacggatgctgcctaccctgcggttaatgttcgggatcgcgaggccgcgtggccgcctgcactgaacttctgttcccgccacccaaagctctatggcctagtcgctttggttttgctgcttctgatcgccgcctgtgttcctatcttcacccgcaccgagcctcggccagcgctcacaatcaccacctcgcccaacctgggtacccgagagaataatgcagaccaggtcacccctgtttcccacattggctgccccaacactacacaacagggctctcctgtgttcgccaagctactggctaaaaaccaagcatcgttgtgcaatacaactctgaactggcacagccaagatggagctgggagctcatacctatctcaaggtctgaggtacgaagaagacaaaaaggagttggtggtagacagtcccgggctctactacgtatttttggaactgaagctcagtccaacattcacaaacacaggccacaaggtgcagggctgggtctctcttgttttgcaagcaaagcctcaggtagatgactttgacaacttggccctgacagtggaactgttcccttgctccatggagaacaagttagtggaccgttcctggagtcaactgttgctcctgaaggctggccaccgcctcagtgtgggtctgagggcttatctgcatggagcccaggatgcatacagagactgggagctgtcttatcccaacaccaccagctttggactctttcttgtgaaacccgacaacccatgggaatgagaattcaataaaagatctttattttcattagatctgtgtgttggttttttgtgtgcggccgcaggaacccctagtgatggagttggccactccctctctgcgcgctcgctcgctcactgaggccgggcgaccaaaggtcgcccgacgcccgggctttgcccgggcggcctcagtgagcgagcgagcgcgcagctgcctgcaggggcgcctgatgcggtattttctccttacgcatctgtgcggtatttcacaccgcatacgtcaaagcaaccatagtacgcgccctgtagcggcgcattaagcgcggcgggtgtggtggttacgcgcagcgtgaccgctacacttgccagcgccttagcgcccgctcctttcgctttcttcccttcctttctcgccacgttcgccggctttccccgtcaagctctaaatcgggggctccctttagggttccgatttagtgctttacggcacctcgaccccaaaaaacttgatttgggtgatggttcacgtagtgggccatcgccctgatagacggtttttcgccctttgacgttggagtccacgttctttaatagtggactcttgttccaaactggaacaacactcaactctatctcgggctattcttttgatttataagggattttgccgatttcggtctattggttaaaaaatgagctgatttaacaaaaatttaacgcgaattttaacaaaatattaacgtttacaattttatggtgcactctcagtacaatctgctctgatgccgcatagttaagccagccccgacacccgccaacacccgctgacgcgccctgacgggcttgtctgctcccggcatccgcttacagacaagctgtgaccgtctccgggagctgcatgtgtcagaggttttcaccgtcatcaccgaaacgcgcgagacgaaagggcctcgtgatacgcctatttttataggttaatgtcatgataataatggtttcttagacgtcaggtggcacttttcggggaaatgtgcgcggaacccctatttgtttatttttctaaatacattcaaatatgtatccgctcatgagacaataaccctgataaatgcttcaataatattgaaaaaggaagagtatgagtattcaacatttccgtgtcgcccttattcccttttttgcggcattttgccttcctgtttttgctcacccagaaacgctggtgaaagtaaaagatgctgaagatcagttgggtgcacgagtgggttacatcgaactggatctcaacagcggtaagatccttgagagttttcgccccgaagaacgttttccaatgatgagcacttttaaagttctgctatgtggcgcggtattatcccgtattgacgccgggcaagagcaactcggtcgccgcatacactattctcagaatgacttggttgagtactcaccagtcacagaaaagcatcttacggatggcatgacagtaagagaattatgcagtgctgccataaccatgagtgataacactgcggccaacttacttctgacaacgatcggaggaccgaaggagctaaccgcttttttgcacaacatgggggatcatgtaactcgccttgatcgttgggaaccggagctgaatgaagccataccaaacgacgagcgtgacaccacgatgcctgtagcaatggcaacaacgttgcgcaaactattaactggcgaactacttactctagcttcccggcaacaattaatagactggatggaggcggataaagttgcaggaccacttctgcgctcggcccttccggctggctggtttattgctgataaatctggagccggtgagcgtggaagccgcggtatcattgcagcactggggccagatggtaagccctcccgtatcgtagttatctacacgacggggagtcaggcaactatggatgaacgaaatagacagatcgctgagataggtgcctcactgattaagcattggtaactgtcagaccaagtttactcatatatactttagattgatttaaaacttcatttttaatttaaaaggatctaggtgaagatcctttttgataatctcatgaccaaaatcccttaacgtgagttttcgttccactgagcgtcagaccccgtagaaaagatcaaaggatcttcttgagatcctttttttctgcgcgtaatctgctgcttgcaaacaaaaaaaccaccgctaccagcggtggtttgtttgccggatcaagagctaccaactctttttccgaaggtaactggcttcagcagagcgcagataccaaatactgttcttctagtgtagccgtagttaggccaccacttcaagaactctgtagcaccgcctacatacctcgctctgctaatcctgttaccagtggctgctgccagtggcgataagtcgtgtcttaccgggttggactcaagacgatagttaccggataaggcgcagcggtcgggctgaacggggggttcgtgcacacagcccagcttggagcgaacgacctacaccgaactgagatacctacagcgtgagctatgagaaagcgccacgcttcccgaagggagaaaggcggacaggtatccggtaagcggcagggtcggaacaggagagcgcacgagggagcttccagggggaaacgcctggtatctttatagtcctgtcgggtttcgccacctctgacttgagcgtcgatttttgtgatgctcgtcaggggggcggagcctatggaaaaacgccagcaacgcggcctttttacggttcctggccttttgctggccttttgctcacatgt

SEQ ID NO: 59 - DNA, 589 bp, Artificial Sequence
  Ori
ttgagatcctttttttctgcgcgtaatctgctgcttgcaaacaaaaaaaccaccgctaccagcggtggtttgtttgccggatcaagagctaccaactctttttccgaaggtaactggcttcagcagagcgcagataccaaatactgttcttctagtgtagccgtagttaggccaccacttcaagaactctgtagcaccgcctacatacctcgctctgctaatcctgttaccagtggctgctgccagtggcgataagtcgtgtcttaccgggttggactcaagacgatagttaccggataaggcgcagcggtcgggctgaacggggggttcgtgcacacagcccagcttggagcgaacgacctacaccgaactgagatacctacagcgtgagctatgagaaagcgccacgcttcccgaagggagaaaggcggacaggtatccggtaagcggcagggtcggaacaggagagcgcacgagggagcttccagggggaaacgcctggtatctttatagtcctgtcgggtttcgccacctctgacttgagcgtcgatttttgtgatgctcgtcaggggggcggagcctatggaaa

SEQ ID NO: 60 - DNA, 456 bp, Artificial Sequence
  f1Ori
acgcgccctgtagcggcgcattaagcgcggcgggtgtggtggttacgcgcagcgtgaccgctacacttgccagcgccttagcgcccgctcctttcgctttcttcccttcctttctcgccacgttcgccggctttccccgtcaagctctaaatcgggggctccctttagggttccgatttagtgctttacggcacctcgaccccaaaaaacttgatttgggtgatggttcacgtagtgggccatcgccctgatagacggtttttcgccctttgacgttggagtccacgttctttaatagtggactcttgttccaaactggaacaacactcaactctatctcgggctattcttttgatttataagggattttgccgatttcggtctattggttaaaaaatgagctgatttaacaaaaatttaacgcgaattttaacaaaatattaacgtttacaattt

SEQ ID NO: 61 - DNA, 105 bp, Artificial Sequence
  AmpR Promoter
cgcggaacccctatttgtttatttttctaaatacattcaaatatgtatccgctcatgagacaataaccctgataaatgcttcaataatattgaaaaaggaagagt

SEQ ID NO: 62 - DNA, 861 bp, Artificial Sequence
  AmpR
atgagtattcaacatttccgtgtcgcccttattcccttttttgcggcattttgccttcctgtttttgctcacccagaaacgctggtgaaagtaaaagatgctgaagatcagttgggtgcacgagtgggttacatcgaactggatctcaacagcggtaagatccttgagagttttcgccccgaagaacgttttccaatgatgagcacttttaaagttctgctatgtggcgcggtattatcccgtattgacgccgggcaagagcaactcggtcgccgcatacactattctcagaatgacttggttgagtactcaccagtcacagaaaagcatcttacggatggcatgacagtaagagaattatgcagtgctgccataaccatgagtgataacactgcggccaacttacttctgacaacgatcggaggaccgaaggagctaaccgcttttttgcacaacatgggggatcatgtaactcgccttgatcgttgggaaccggagctgaatgaagccataccaaacgacgagcgtgacaccacgatgcctgtagcaatggcaacaacgttgcgcaaactattaactggcgaactacttactctagcttcccggcaacaattaatagactggatggaggcggataaagttgcaggaccacttctgcgctcggcccttccggctggctggtttattgctgataaatctggagccggtgagcgtggaagccgcggtatcattgcagcactggggccagatggtaagccctcccgtatcgtagttatctacacgacggggagtcaggcaactatggatgaacgaaatagacagatcgctgagataggtgcctcactgattaagcattggtaa

SEQ ID NO: 63 - DNA, 141 bp, Artificial Sequence
  AAV ITR
aggaacccctagtgatggagttggccactccctctctgcgcgctcgctcgctcactgaggccgggcgaccaaaggtcgcccgacgcccgggctttgcccgggcggcctcagtgagcgagcgagcgcgcagctgcctgcagg

SEQ ID NO: 64 - DNA, 212 bp, Artificial Sequence
  EFS core promoter
gggcagagcgcacatcgcccacagtccccgagaagttggggggaggggtcggcaattgaacgggtgcctagagaaggtggcgcggggtaaactgggaaagtgatgtcgtgtactggctccgcctttttcccgagggtgggggagaaccgtatataagtgcagtagtcgccgtgaacgttctttttcgcaacgggtttgccgccagaacacag

SEQ ID NO: 65 - DNA, 269 bp, Artificial Sequence
  LTR promoter
ggggctcgcatctctccttcacgcgcccgccgccctacctgaggccgccatccacgccggttgagtcgcgttctgccgcctcccgcctgtggtgcctcctgaactgcgtccgccgtctaggtaagtttaaagctcaggtcgagaccgggcctttgtccggcgctcccttggagcctacctagactcagccggctctccacgctttgcctgaccctgcttgctcaactctacgtctttgtttcgttttctgttctgcgccgttacagatc

SEQ ID NO: 66 - DNA, 493 bp, Artificial Sequence
  EFS LTR promoter
gggcagagcgcacatcgcccacagtccccgagaagttggggggaggggtcggcaattgaacgggtgcctagagaaggtggcgcggggtaaactgggaaagtgatgtcgtgtactggctccgcctttttcccgagggtgggggagaaccgtatataagtgcagtagtcgccgtgaacgttctttttcgcaacgggtttgccgccagaacacagctgaagcttcgaggggctcgcatctctccttcacgcgcccgccgccctacctgaggccgccatccacgccggttgagtcgcgttctgccgcctcccgcctgtggtgcctcctgaactgcgtccgccgtctaggtaagtttaaagctcaggtcgagaccgggcctttgtccggcgctcccttggagcctacctagactcagccggctctccacgctttgcctgaccctgcttgctcaactctacgtctttgtttcgttttctgttctgcgccgttacagatc

SEQ ID NO: 67 - DNA, 68 bp, Artificial Sequence
  T2A
gaggaagtctgctaacatgcggtgacgtcgaggagaatcctggcccaatggagagtgtggtacagcct

SEQ ID NO: 68 - DNA, 72 bp, Artificial Sequence
  P2A
actagtggatccggcgcaacaaacttctctctgctgaaacaagccggagatgtcgaagagaatcctggaccg

SEQ ID NO: 69 - DNA, 75 bp, Artificial Sequence
  E2A
gctagcagcggtacccagtgcaccaactacgccctgctgaagctggccggcgatgtggagagcaaccccgggccc

SEQ ID NO: 70 - DNA, 81 bp, Artificial Sequence
  F2A
ggcatatgcggtaccgtgaagcagaccctgaacttcgatctgctgaagctggccggcgatgtggagagcaaccccgggccc

SEQ ID NO: 71 - DNA, 589 bp, Artificial Sequence
  WPRE
aatcaacctctggattacaaaatttgtgaaagattgactggtattcttaactatgttgctccttttacgctatgtggatacgctgctttaatgcctttgtatcatgctattgcttcccgtatggctttcattttctcctccttgtataaatcctggttgctgtctctttatgaggagttgtggcccgttgtcaggcaacgtggcgtggtgtgcactgtgtttgctgacgcaacccccactggttggggcattgccaccacctgtcagctcctttccgggactttcgctttccccctccctattgccacggcggaactcatcgccgcctgccttgcccgctgctggacaggggctcggctgttgggcactgacaattccgtggtgttgtcggggaaatcatcgtcctttccttggctgctcgcctgtgttgccacctggattctgcgcgggacgtccttctgctacgtcccttcggccctcaatccagcggaccttccttcccgcggcctgctgccggctctgcggcctcttccgcgtcttcgccttcgccctcagacgagtcggatctccctttgggccgcctccccgc

SEQ ID NO: 72 - DNA, 49 bp, Artificial Sequence
  short PolyA
aataaaagatctttattttcattagatctgtgtgttggttttttgtgtg

SEQ ID NO: 73 - DNA, 918 bp, Artificial Sequence
  ORF Cd80
atggcttgcaattgtcagttgatgcaggatacaccactcctcaagtttccatgtccaaggctcattcttctctttgtgctgctgattcgtctttcacaagtgtcttcagatgttgatgaacaactgtccaagtcagtgaaagataaggtattgctgccttgccgttacaactctcctcatgaagatgagtctgaagaccgaatctactggcaaaaacatgacaaagtggtgctgtctgtcattgctgggaaactaaaagtgtggcccgagtataagaaccggactttatatgacaacactacctactctcttatcatcctgggcctggtcctttcagaccggggcacatacagctgtgtcgttcaaaagaaggaaagaggaacgtatgaagttaaacacttggctttagtaaagttgtccatcaaagctgacttctctacccccaacataactgagtctggaaacccatctgcagacactaaaaggattacctgctttgcttccgggggtttcccaaagcctcgcttctcttggttggaaaatggaagagaattacctggcatcaatacgacaatttcccaggatcctgaatctgaattgtacaccattagtagccaactagatttcaatacgactcgcaaccacaccattaagtgtctcattaaatatggagatgctcacgtgtcagaggacttcacctgggaaaaacccccagaagaccctcctgatagcaagaacacacttgtgctctttggggcaggattcggcgcagtaataacagtcgtcgtcatcgttgtcatcatcaaatgcttctgtaagcacagaagctgtttcagaagaaatgaggcaagcagagaaacaaacaacagccttaccttcgggcctgaagaagcattagctgaacagaccgtcttcctt

SEQ ID NO: 74 - DNA, 717 bp, Artificial Sequence
  ORF Light
atggagagtgtggtacagccttcagtgtttgtggtggatggacagacggacatcccattcaggcggctggaacagaaccaccggagacggcgctgtggcactgtccaggtcagcctggccctggtgctgctgctaggtgctgggctggccactcagggctggtttctcctgagactgcatcaacgtcttggagacatagtagctcatctgccagatggaggcaaaggctcctgggagaagctgatacaagatcaacgatctcaccaggccaacccagcagcacatcttacaggagccaacgccagcttgataggtattggtggacctctgttatgggagacacgacttggcctggccttcttgaggggcttgacgtatcatgatggggccctggtgaccatggagcccggttactactatgtgtactccaaagtgcagctgagcggcgtgggctgcccccaggggctggccaatggcctccccatcacccatggactatacaagcgcacatcccgctacccgaaggagttagaactgctggtcagtcggcggtcaccctgtggccgggccaacagctcccgagtctggtgggacagcagcttcctgggcggcgtggtacatctggaggctggggaagaggtggtggtccgcgtgcctggaaaccgcctggtcagaccacgtgacggcaccaggtcctatttcggagctttcatggtc

SEQ ID NO: 75 - DNA, 294 bp, Artificial Sequence
  ORF Cxcl10
atgaacccaagtgctgccgtcattttctgcctcatcctgctgggtctgagtgggactcaagggatccctctcgcaaggacggtccgctgcaactgcatccatatcgatgacgggccagtgagaatgagggccatagggaagcttgaaatcatccctgcgagcctatcctgcccacgtgttgagatcattgccacgatgaaaaagaatgatgagcagagatgtctgaatccggaatctaagaccatcaagaatttaatgaaagcgtttagccaaaaaaggtctaaaagggctcct

SEQ ID NO: 76 - DNA, 927 bp, Artificial Sequence
  ORF 41BBL
atggaccagcacacacttgatgtggaggataccgcggatgccagacatccagcaggtacttcgtgcccctcggatgcggcgctcctcagagataccgggctcctcgcggacgctgcgctcctctcagatactgtgcgccccacaaatgccgcgctccccacggatgctgcctaccctgcggttaatgttcgggatcgcgaggccgcgtggccgcctgcactgaacttctgttcccgccacccaaagctctatggcctagtcgctttggttttgctgcttctgatcgccgcctgtgttcctatcttcacccgcaccgagcctcggccagcgctcacaatcaccacctcgcccaacctgggtacccgagagaataatgcagaccaggtcacccctgtttcccacattggctgccccaacactacacaacagggctctcctgtgttcgccaagctactggctaaaaaccaagcatcgttgtgcaatacaactctgaactggcacagccaagatggagctgggagctcatacctatctcaaggtctgaggtacgaagaagacaaaaaggagttggtggtagacagtcccgggctctactacgtatttttggaactgaagctcagtccaacattcacaaacacaggccacaaggtgcagggctgggtctctcttgttttgcaagcaaagcctcaggtagatgactttgacaacttggccctgacagtggaactgttcccttgctccatggagaacaagttagtggaccgttcctggagtcaactgttgctcctgaaggctggccaccgcctcagtgtgggtctgagggcttatctgcatggagcccaggatgcatacagagactgggagctgtcttatcccaacaccaccagctttggactctttcttatgaaacccgacaacccatgggaa

SEQ ID NO: 77 - DNA, 468 bp, Artificial Sequence
  ORF IFNg
atgaacgctacacactgcatcttggctttgcagctcttcctcatggctgtttctggctgttactgccacggcacagtcattgaaagcctagaaagtctgaataactattttaactcaagtggcatagatgtggaagaaaagagtctcttcttggatatctggaggaactggcaaaaggatggtgacatgaaaatcctgcagagccagattatctctttctacctcagactctttgaagtcttgaaagacaatcaggccatcagcaacaacataagcgtcattgaatcacacctgattactaccttcttcagcaacagcaaggcgaaaaaggatgcattcatgagtattgccaagtttgaggtcaacaacccacaggtccagcgccaagcattcaatgagctcatccgagtggtccaccagctgttgccggaatccagcctcaggaagcggaaaaggagtcgctgctga

SEQ ID NO: 78 - DNA, 516 bp, Artificial Sequence
  ORF Il2
atgtacagcatgcagctcgcatcctgtgtcacattgacacttgtgctccttgtcaacagcgcacccacttcaagctccacttcaagctctacagcggaagcacagcagcagcagcagcagcagcagcagcagcagcagcacctggagcagctgttgatggacctacaggagctcctgagcaggatggagaattacaggaacctgaaactccccaggatgctcaccttcaaattttacttgcccaagcaggccacagaattgaaagatcttcagtgcctagaagatgaacttggacctctgcggcatgttctggatttgactcaaagcaaaagctttcaattggaagatgctgagaatttcatcagcaatatcagagtaactgttgtaaaactaaagggctctgacaacacatttgagtgccaattcgatgatgagtcagcaactgtggtggactttctgaggagatggatagccttctgtcaaagcatcatctcaacaagccctcaataagaattc

SEQ ID NO: 79 - DNA, 519 bp, Artificial Sequence
  ORF Gitrl
atggaggaaatgcctttgagagagtcaagtcctcaaagggcagagaggtgcaagaagtcatggctcttgtgcatagtggctctgttactgatgctgctctgttctttgggtacactgatctatacttcactcaagccaactgccatcgagtcctgcatggttaagtttgaactatcatcctcaaaatggcacatgacatctcccaaacctcactgtgtgaatacgacatctgatgggaagctgaagatactgcagagtggcacatatttaatctacggccaagtgattcctgtggataagaaatacataaaagacaatgcccccttcgtagtacagatatataaaaagaatgatgtcctacaaactctaatgaatgattttcaaatcttgcctataggaggggtttatgaactgcatgctggagataacatatatctgaagttcaactctaaagaccatattcagaaaaataacacatactgggggatcatcttaatgcctgatctaccattcatctct

SEQ ID NO: 80 - DNA, 1008 bp, Artificial Sequence
  ORF Il23
atgtgtcctcagaagctaaccatctcctggtttgccatcgttttgctggtgtctccactcatggccatgtgggagctggagaaagacgtttatgttgtagaggtggactggactcccgatgcccctggagaaacagtgaacctcacctgtgacacgcctgaagaagatgacatcacctggacctcagaccagagacatggagtcataggctctggaaagaccctgaccatcactgtcaaagagtttctagatgctggccagtacacctgccacaaaggaggcgagactctgagccactcacatctgctgctccacaagaaggaaaatggaatttggtccactgaaattttaaaaaatttcaaaaacaagactttcctgaagtgtgaagcaccaaattactccggacggttcacgtgctcatggctggtgcaaagaaacatggacttgaagttcaacatcaagagcagtagcagttcccctgactctcgggcagtgacatgtggaatggcgtctctgtctgcagagaaggtcacactggaccaaagggactatgagaagtattcagtgtcctgccaggaggatgtcacctgcccaactgccgaggagaccctgcccattgaactggcgttggaagcacggcagcagaataaatatgagaactacagcaccagcttcttcatcagggacatcatcaaaccagacccgcccaagaacttgcagatgaagcctttgaagaactcacaggtggaggtcagctgggagtaccctgactcctggagcactccccattcctacttctccctcaagttctttgttcgaatccagcgcaagaaagaaaagatgaaggagacagaggaggggtgtaaccagaaaggtgcgttcctcgtagagaagacatctaccgaagtccaatgcaaaggcgggaatgtctgcgtgcaagctcaggatcgctattacaattcctcatgcagcaagtgggcatgtgttccctgcagggtccgatcctag

SEQ ID NO: 81 - DNA, 498 bp, Artificial Sequence
  ORF hIFNg
atgaaatatacaagttatatcttggcttttcagctctgcatcgttttgggttctcttggctgttactgccaggacccatatgtaaaagaagcagaaaaccttaagaaatattttaatgcaggtcattcagatgtagcggataatggaactcttttcttaggcattttgaagaattggaaagaggagagtgacagaaaaataatgcagagccaaattgtctccttttacttcaaactttttaaaaactttaaagatgaccagagcatccaaaagagtgtggagaccatcaaggaagacatgaatgtcaagtttttcaatagcaacaaaaagaaacgagatgacttcgaaaagctgactaattattcggtaactgacttgaatgtccaacgcaaagcaatacatgaactcatccaagtgatggctgaactgtcgccagcagctaaaacagggaagcgaaaaaggagtcagatgctgtttcgaggtcgaagagcatcccag

SEQ ID NO: 82 - DNA, 983 bp, Artificial Sequence
  ORF hIL23
tgtgtcaccagcagttggtcatctcttggttttccctggtttttctggcatctcccctcgtggccatatgggaactgaagaaagatgtttatgtcgtagaattggattggtatccggatgcccctggagaaatggtggtcctcacctgtgacacccctgaagaagatggtatcacctggaccttggaccagagcagtgaggtcttaggctctggcaaaaccctgaccatccaagtcaaagagtttggagatgctggccagtacacctgtcacaaaggaggcgaggttctaagccattcgctcctgctgcttcacaaaaaggaagatggaatttggtccactgatattttaaaggaccagaaagaacccaaaaataagacctttctaagatgcgaggccaagaattattctggacgtttcacctgctggtggctgacgacaatcagtactgatttgacattcagtgtcaaaagcagcagaggctcttctgacccccaaggggtgacgtgcggagctgctacactctctgcagagagagtcagaggggacaacaaggagtatgagtactcagtggagtgccaggaggacagtgcctgcccagctgctgaggagagtctgcccattgaggtcatggtggatgccgttcacaagctcaagtatgaaaactacaccagcagcttcttcatcagggacatcatcaaacctgacccacccaagaacttgcagctgaagccattaaagaattctcggcaggtggaggtcagctgggagtaccctgacacctggagtactccacattcctacttctccctgacattctgcgttcaggtccagggcaagagcaagagagaaaagaaagatagagtcttcacggacaagacctcagccacggtcatctgccgcaaaaatgccagcattagcgtgcgggcccaggaccgctactatagctcatcttggagcgaatgggcatctgtgccctgcagt

SEQ ID NO: 83 - DNA, 762 bp, Artificial Sequence
  ORF h41BBL
atggaatacgcctctgacgcttcactggaccccgaagccccgtggcctcccgcgccccgcgctcgcgcctgccgcgtactgccttgggccctggtcgcggggctgctgctgctgctgctgctcgctgccgcctgcgccgtcttcctcgcctgcccctgggccgtgtccggggctcgcgcctcgcccggctccgcggccagcccgagactccgcgagggtcccgagctttcgcccgacgatcccgccggcctcttggacctgcggcagggcatgtttgcgcagctggtggcccaaaatgttctgctgatcgatgggcccctgagctggtacagtgacccaggcctggcaggcgtgtccctgacggggggcctgagctacaaagaggacacgaaggagctggtggtggccaaggctggagtctactatgtcttctttcaactagagctgcggcgcgtggtggccggcgagggctcaggctccgtttcacttgcgctgcacctgcagccactgcgctctgctgctggggccgccgccctggctttgaccgtggacctgccacccgcctcctccgaggctcggaactcggccttcggtttccagggccgcttgctgcacctgagtgccggccagcgcctgggcgtccatcttcacactgaggccagggcacgccatgcctggcagcttacccagggcgccacagtcttgggactcttccgggtgacccccgaaatcccagccggactcccttcaccgaggtcggaa

SEQ ID NO: 84 - DNA, 708 bp, Artificial Sequence
  ORF hLIGHT
atggaggagagtgtcgtacggccctcagtgtttgtggtggatggacagaccgacatcccattcacgaggctgggacgaagccaccggagacagtcgtgcagtgtggcccgggtgggtctgggtctcttgctgttgctgatgggggccgggctggccgtccaaggctggttcctcctgcagctgcactggcgtctaggagagatggtcacccgcctgcctgacggacctgcaggctcctggcaagagcgaaggtctcacgaggtcaacccagcagcgcatctcacaggggccaactccagcttgaccggcagcggggggccgctgttatgggagactcagctgggcctggccttcctgaggggcctcagctaccacgatggggcccttgtggtcaccaaagctggctactactacatctactccaaggtgcagctgggcggtgtgggctgcccgctgggcctggccagcaccatcacccacggcctctacaagcgcacaccccgctaccccgaggagctggagctgttggtcagccagcagtcaccctgcggacgggccaccagcagctcccgggtctggtgggacagcagcttcctgggtggtgtggtacacctggaggctggggagaaggtggtcgtccgtgtgctggatgaacgcctggttcgactgcgtgatggtacccggtcttacttcggggctttcatggtg

SEQ ID NO: 85 - DNA, 15 bp, Artificial Sequence
  CGKRK
tgcggaaagcgtaag

SEQ ID NO: 86 - DNA, 20 bp, Artificial Sequence
  sgRNA
gcttcagtttgtctgtggga

SEQ ID NO: 87 - DNA, 20 bp, Artificial Sequence
  sgRNA
attcactgagcatctattag

SEQ ID NO: 88 - DNA, 20 bp, Artificial Sequence
  sgRNA
atcaggaagcatccgcatcc

SEQ ID NO: 89 - DNA, 20 bp, Artificial Sequence
  sgRNA
gagagttctgaatcagggtg

SEQ ID NO: 90 - DNA, 20 bp, Artificial Sequence
  sgRNA
tccaggcctgttctgagcac

SEQ ID NO: 91 - DNA, 20 bp, Artificial Sequence
  sgRNA
ggacctttgagttgccctca

SEQ ID NO: 92 - DNA, 20 bp, Artificial Sequence
  sgRNA
ccaagtccgcgttgctgctg

SEQ ID NO: 93 - DNA, 20 bp, Artificial Sequence
  sgRNA
atctgcatgacccactcgat

SEQ ID NO: 94 - DNA, 20 bp, Artificial Sequence
  sgRNA
gtttgagggtcatctagctg

SEQ ID NO: 95 - DNA, 20 bp, Artificial Sequence
  sgRNA
gcaggcaggagtgggtgggt

SEQ ID NO: 96 - DNA, 20 bp, Artificial Sequence
  sgRNA
ctttgtagattattcgagtt

SEQ ID NO: 97 - DNA, 20 bp, Artificial Sequence
  sgRNA
gagttcggtttcagtcttga

SEQ ID NO: 98 - DNA, 20 bp, Artificial Sequence
  sgRNA
aaagagaattggaaagcaag

SEQ ID NO: 99 - DNA, 20 bp, Artificial Sequence
  sgRNA
tgtgtacatctctcttaaat

SEQ ID NO: 100 - DNA, 20 bp, Artificial Sequence
  sgRNA
caggctctcagagaacctgt

SEQ ID NO: 101 - DNA, 20 bp, Artificial Sequence
  sgRNA
gaaattcctctgaggcagaa

SEQ ID NO: 102 - DNA, 20 bp, Artificial Sequence
  sgRNA
cctgtgctatttataaggga

SEQ ID NO: 103 - DNA, 20 bp, Artificial Sequence
  sgRNA
gtgagaatgatcttccttca

SEQ ID NO: 104 - DNA, 20 bp, Artificial Sequence
  sgRNA
agagtttcctttcgactcct

SEQ ID NO: 105 - DNA, 20 bp, Artificial Sequence
  sgRNA
ttaagatggtgacagatagg

SEQ ID NO: 106 - DNA, 20 bp, Artificial Sequence
  sgRNA
atacctgatcgaaggctcct

SEQ ID NO: 107 - DNA, 20 bp, Artificial Sequence
  sgRNA
aaaccctactctcagatccc

SEQ ID NO: 108 - DNA, 20 bp, Artificial Sequence
  sgRNA
tagttcttctaggtcagctg

SEQ ID NO: 109 - DNA, 20 bp, Artificial Sequence
  sgRNA
taaccacaaattgatcgtcc

SEQ ID NO: 110 - DNA, 20 bp, Artificial Sequence
  sgRNA
actttggagatgactcagca

SEQ ID NO: 111 - DNA, 20 bp, Artificial Sequence
  sgRNA
tttattgtgacccatgaact

SEQ ID NO: 112 - DNA, 20 bp, Artificial Sequence
  sgRNA
gcaatgccctcggtttacag

SEQ ID NO: 113 - DNA, 20 bp, Artificial Sequence
  sgRNA
tttcaaagagtctacctgtg

SEQ ID NO: 114 - DNA, 20 bp, Artificial Sequence
  sgRNA
gcaatttatactgttaatgc

SEQ ID NO: 115 - DNA, 20 bp, Artificial Sequence
  sgRNA
tccattcagtcagtgtatgg

SEQ ID NO: 116 - DNA, 20 bp, Artificial Sequence
  sgRNA
cacactcatcaagagcccgg

SEQ ID NO: 117 - DNA, 20 bp, Artificial Sequence
  sgRNA
gtgggcaagaagcgaaggaa

SEQ ID NO: 118 - DNA, 20 bp, Artificial Sequence
  sgRNA
agaggacacacgtgtgctac

SEQ ID NO: 119 - DNA, 20 bp, Artificial Sequence
  sgRNA
aggcagagtcatacttccaa

SEQ ID NO: 120 - DNA, 20 bp, Artificial Sequence
  sgRNA
ctaccctggctccctataaa

SEQ ID NO: 121 - DNA, 20 bp, Artificial Sequence
  sgRNA
ttatgacagcaacaagtgtt

SEQ ID NO: 122 - DNA, 20 bp, Artificial Sequence
  sgRNA
tggtgtcttctgaccaagaa

SEQ ID NO: 123 - DNA, 20 bp, Artificial Sequence
  sgRNA
tcgtcgcaacccacacttcc

SEQ ID NO: 124 - DNA, 20 bp, Artificial Sequence
  sgRNA
ttaactaatcctgagtaagg

SEQ ID NO: 125 - DNA, 20 bp, Artificial Sequence
  sgRNA
aagtcactcaattcataact

SEQ ID NO: 126 - DNA, 20 bp, Artificial Sequence
  sgRNA
caactccctgttagcccgga

SEQ ID NO: 127 - DNA, 20 bp, Artificial Sequence
  sgRNA
agtgcttagcagtgttccaa

SEQ ID NO: 128 - DNA, 20 bp, Artificial Sequence
  sgRNA
gcaccaggccaaacatacaa

SEQ ID NO: 129 - DNA, 20 bp, Artificial Sequence
  sgRNA
cactacaagggaagttcaga

SEQ ID NO: 130 - DNA, 20 bp, Artificial Sequence
  sgRNA
cgccacctagtggtaacaag

SEQ ID NO: 131 - DNA, 20 bp, Artificial Sequence
  sgRNA
gggccctgaaaggatagcga

SEQ ID NO: 132 - DNA, 20 bp, Artificial Sequence
  sgRNA
ttctacatacacttcgaagc

SEQ ID NO: 133 - DNA, 20 bp, Artificial Sequence
  sgRNA
tgtgactcaggtgggatgga

SEQ ID NO: 134 - DNA, 20 bp, Artificial Sequence
  sgRNA
gaggaggtacgtgaggaaag

SEQ ID NO: 135 - DNA, 20 bp, Artificial Sequence
  sgRNA
cagtgagagtgatcgaccgg

SEQ ID NO: 136 - DNA, 20 bp, Artificial Sequence
  sgRNA
gagacttgggcatgagttac

SEQ ID NO: 137 - DNA, 20 bp, Artificial Sequence
  sgRNA
aacccaatcggctgctgagc

SEQ ID NO: 138 - DNA, 20 bp, Artificial Sequence
  sgRNA
ccgcctgtgcccaattagcc

SEQ ID NO: 139 - DNA, 20 bp, Artificial Sequence
  sgRNA
ccctccctcccttccctccc

SEQ ID NO: 140 - DNA, 20 bp, Artificial Sequence
  sgRNA
acagggcctggacagggaag

SEQ ID NO: 141 - DNA, 20 bp, Artificial Sequence
  sgRNA
agaaagttccgggagtcgag

SEQ ID NO: 142 - DNA, 20 bp, Artificial Sequence
  sgRNA
cagagggctgtcagagggag

SEQ ID NO: 143 - DNA, 20 bp, Artificial Sequence
  sgRNA
aacttggtttctgttgtagg

SEQ ID NO: 144 - DNA, 20 bp, Artificial Sequence
  sgRNA
attccctagccgggcagggc

SEQ ID NO: 145 - DNA, 20 bp, Artificial Sequence
  sgRNA
aattgtagcgagatagacga

SEQ ID NO: 146 - DNA, 20 bp, Artificial Sequence
  sgRNA
gtggttggtgtacactcacg

SEQ ID NO: 147 - DNA, 20 bp, Artificial Sequence
  sgRNA
cgttctgtggctgagcctaa

SEQ ID NO: 148 - DNA, 20 bp, Artificial Sequence
  sgRNA
tgcaggcaacttgcagactg

SEQ ID NO: 149 - DNA, 20 bp, Artificial Sequence
  sgRNA
ttcacgcaagcaagttaagg

SEQ ID NO: 150 - DNA, 20 bp, Artificial Sequence
  sgRNA
cgtgccgttctaccagcatt

SEQ ID NO: 151 - DNA, 20 bp, Artificial Sequence
  sgRNA
acgacctccggatctgagtc

SEQ ID NO: 152 - DNA, 20 bp, Artificial Sequence
  sgRNA
ccgtgatatttcaaacagcc

SEQ ID NO: 153 - DNA, 20 bp, Artificial Sequence
  sgRNA
agcatcaacagctaggagac

SEQ ID NO: 154 - DNA, 20 bp, Artificial Sequence
  sgRNA
gcggagtctaggctgataaa

SEQ ID NO: 155 - DNA, 20 bp, Artificial Sequence
  sgRNA
ggtctgggaacgcgggagtg

SEQ ID NO: 156 - DNA, 20 bp, Artificial Sequence
  sgRNA
tatttattggtcacttcact

SEQ ID NO: 157 - DNA, 20 bp, Artificial Sequence
  sgRNA
ctccagccctctcatagttg

SEQ ID NO: 158 - DNA, 20 bp, Artificial Sequence
  sgRNA
aggatttaacatggactgaa

SEQ ID NO: 159 - DNA, 20 bp, Artificial Sequence
  sgRNA
ctgtgatcgaacagacgaga

SEQ ID NO: 160 - DNA, 20 bp, Artificial Sequence
  sgRNA
gcagtgtggcagccgccgat

SEQ ID NO: 161 - DNA, 20 bp, Artificial Sequence
  sgRNA
aacagctggtaactgccgat

SEQ ID NO: 162 - DNA, 20 bp, Artificial Sequence
  sgRNA
ctgcgtcacgcagcgtcggg

SEQ ID NO: 163 - DNA, 20 bp, Artificial Sequence
  sgRNA
ggtcgcactatgggccaatg

SEQ ID NO: 164 - DNA, 20 bp, Artificial Sequence
  sgRNA
gtaggtctaaaccagtcaaa

SEQ ID NO: 165 - DNA, 20 bp, Artificial Sequence
  sgRNA
gggtcgaccacgcgttgtgg

SEQ ID NO: 166 - DNA, 20 bp, Artificial Sequence
  sgRNA
tgatagggaatgcattctcc

SEQ ID NO: 167 - DNA, 20 bp, Artificial Sequence
  sgRNA
actttgagttcccgaagccc

SEQ ID NO: 168 - DNA, 20 bp, Artificial Sequence
  sgRNA
caagcctaagggatctagcc

SEQ ID NO: 169 - DNA, 20 bp, Artificial Sequence
  sgRNA
agctggccgtgcagagagga

SEQ ID NO: 170 - DNA, 20 bp, Artificial Sequence
  sgRNA
tcatctgggagatgagcctc

SEQ ID NO: 171 - DNA, 20 bp, Artificial Sequence
  sgRNA
ttcggttggcattcggctaa

SEQ ID NO: 172 - DNA, 20 bp, Artificial Sequence
  sgRNA
gggtctgagatgctttgaaa

SEQ ID NO: 173 - DNA, 20 bp, Artificial Sequence
  sgRNA
ggcgcctgtcaatttgcggg

SEQ ID NO: 174 - DNA, 20 bp, Artificial Sequence
  sgRNA
ttgctagtagcggccttgga

SEQ ID NO: 175 - DNA, 20 bp, Artificial Sequence
  sgRNA
ctagtctgttcttgccttgt

SEQ ID NO: 176 - DNA, 20 bp, Artificial Sequence
  sgRNA
gggagggtggccgccggaaa

SEQ ID NO: 177 - DNA, 20 bp, Artificial Sequence
  sgRNA
gaatctggcagctctttaag

SEQ ID NO: 178 - DNA, 20 bp, Artificial Sequence
  sgRNA
ggacgctaagaagggtttgg

SEQ ID NO: 179 - DNA, 20 bp, Artificial Sequence
  sgRNA
ctgtcaccaccctccgttcc

SEQ ID NO: 180 - DNA, 20 bp, Artificial Sequence
  sgRNA
cttcacgtcctttccctgaa

SEQ ID NO: 181 - DNA, 20 bp, Artificial Sequence
  sgRNA
tgggaaggcgcttcgagcga

SEQ ID NO: 182 - DNA, 20 bp, Artificial Sequence
  sgRNA
ttcttagatcttgcgcaaag

SEQ ID NO: 183 - DNA, 20 bp, Artificial Sequence
  sgRNA
ccacgaagaatagccctagg

SEQ ID NO: 184 - DNA, 20 bp, Artificial Sequence
  sgRNA
agcggccggtggcccatccc

SEQ ID NO: 185 - DNA, 20 bp, Artificial Sequence
  sgRNA
gctgtcgggaagacgactgt

SEQ ID NO: 186 - DNA, 20 bp, Artificial Sequence
  sgRNA
gcacacgcccagttccggtg

SEQ ID NO: 187 - DNA, 20 bp, Artificial Sequence
  sgRNA
tcgcagactcttggatgact

SEQ ID NO: 188 - DNA, 20 bp, Artificial Sequence
  sgRNA
aatctttacaggcatatctc

SEQ ID NO: 189 - DNA, 20 bp, Artificial Sequence
  sgRNA
tcacacggcccagttgttgt

SEQ ID NO: 190 - DNA, 20 bp, Artificial Sequence
  sgRNA
gtacatctaattcctcattg

SEQ ID NO: 191 - DNA, 20 bp, Artificial Sequence
  sgRNA
ttcaaactattctccattcc

SEQ ID NO: 192 - DNA, 20 bp, Artificial Sequence
  sgRNA
gactttctgcttattattca

SEQ ID NO: 193 - DNA, 20 bp, Artificial Sequence
  sgRNA
cccacctcactcacacactc

SEQ ID NO: 194 - DNA, 20 bp, Artificial Sequence
  sgRNA
gggaccctcggctgctcccc

SEQ ID NO: 195 - DNA, 20 bp, Artificial Sequence
  sgRNA
gagaactcgcccctcccatc

SEQ ID NO: 196 - DNA, 20 bp, Artificial Sequence
  sgRNA
tcccccttctacaggaaacc

SEQ ID NO: 197 - DNA, 20 bp, Artificial Sequence
  sgRNA
gtggactggaatggtgcagg

SEQ ID NO: 198 - DNA, 20 bp, Artificial Sequence
  sgRNA
acccacagggcccctttatt

SEQ ID NO: 199 - DNA, 20 bp, Artificial Sequence
  sgRNA
aaacacagatggactttggg

SEQ ID NO: 200 - DNA, 20 bp, Artificial Sequence
  sgRNA
aaaaatgtcagtcagcgccc

SEQ ID NO: 201 - DNA, 20 bp, Artificial Sequence
  sgRNA
tttatgttctgagtttgtgt

SEQ ID NO: 202 - DNA, 20 bp, Artificial Sequence
  sgRNA
aaagcacaagggaagttcag

SEQ ID NO: 203 - DNA, 20 bp, Artificial Sequence
  sgRNA
ttttctaacacagtgacaga

SEQ ID NO: 204 - DNA, 20 bp, Artificial Sequence
  sgRNA
cttaagtgctgactctcatt

SEQ ID NO: 205 - DNA, 20 bp, Artificial Sequence
  sgRNA
accagatcaaatacaacaaa

SEQ ID NO: 206 - DNA, 20 bp, Artificial Sequence
  sgRNA
agcaatatggtaattagtag

SEQ ID NO: 207 - DNA, 20 bp, Artificial Sequence
  sgRNA
tttttttcctctgggctaac

SEQ ID NO: 208 - DNA, 20 bp, Artificial Sequence
  sgRNA
acagtcactcaaatcagaac

SEQ ID NO: 209 - DNA, 20 bp, Artificial Sequence
  sgRNA
tttaacgctgcaacttttgc

SEQ ID NO: 210 - DNA, 20 bp, Artificial Sequence
  sgRNA
agagtttcctttagactcct

SEQ ID NO: 211 - DNA, 20 bp, Artificial Sequence
  sgRNA
taaataccagcagccagagg

SEQ ID NO: 212 - DNA, 20 bp, Artificial Sequence
  sgRNA
atcctcaggagacttcaatt

SEQ ID NO: 213 - DNA, 20 bp, Artificial Sequence
  sgRNA
aactaaggttttgtggcatt

SEQ ID NO: 214 - DNA, 20 bp, Artificial Sequence
  sgRNA
aagatgagatggtgacagat

SEQ ID NO: 215 - DNA, 20 bp, Artificial Sequence
  sgRNA
cggagcgcggggcggggccg

SEQ ID NO: 216 - DNA, 20 bp, Artificial Sequence
  sgRNA
gctgtgtggcagccgctgat

SEQ ID NO: 217 - DNA, 20 bp, Artificial Sequence
  sgRNA
caggggctagggccgggtcc

SEQ ID NO: 218 - DNA, 20 bp, Artificial Sequence
  sgRNA
cccaggtttcggctcacccc

SEQ ID NO: 219 - DNA, 20 bp, Artificial Sequence
  sgRNA
ggctgcgcgtcgccttcgtc

SEQ ID NO: 220 - DNA, 20 bp, Artificial Sequence
  sgRNA
ggcgagtgtctgggcgagcg

SEQ ID NO: 221 - DNA, 20 bp, Artificial Sequence
  sgRNA
ggctgggcccggtcctgggc

SEQ ID NO: 222 - DNA, 20 bp, Artificial Sequence
  sgRNA
accaactcgttaccgccgag

SEQ ID NO: 223 - DNA, 20 bp, Artificial Sequence
  sgRNA
aagaaaaggaaactgaaaac

SEQ ID NO: 224 - DNA, 20 bp, Artificial Sequence
  sgRNA
agacaggtgacggtccctgc

SEQ ID NO: 225 - DNA, 20 bp, Artificial Sequence
  sgRNA
gtgcccagccaatcaggaca

SEQ ID NO: 226 - DNA, 20 bp, Artificial Sequence
  sgRNA
gaaagtccctctctctaacc

SEQ ID NO: 227 - DNA, 20 bp, Artificial Sequence
  sgRNA
caagccagcgacgcagtgcc

SEQ ID NO: 228 - DNA, 20 bp, Artificial Sequence
  sgRNA
gagtctcgtgatgtttaaga

SEQ ID NO: 229 - DNA, 20 bp, Artificial Sequence
  sgRNA
tgagtttgctgtctgtacat

SEQ ID NO: 230 - DNA, 20 bp, Artificial Sequence
  sgRNA
caggggcaagggctggtgcc

SEQ ID NO: 231 - DNA, 20 bp, Artificial Sequence
  sgRNA
ccactattccagactccaaa

SEQ ID NO: 232 - DNA, 20 bp, Artificial Sequence
  sgRNA
ggagttggggggactgtgtc

SEQ ID NO: 233 - DNA, 20 bp, Artificial Sequence
  sgRNA
ttctcagatgtgtctccggc

SEQ ID NO: 234 - DNA, 20 bp, Artificial Sequence
  sgRNA
gaagaacaaggtctagcgga

SEQ ID NO: 235 - DNA, 20 bp, Artificial Sequence
  sgRNA
gacacaaggagctgcagtcg

SEQ ID NO: 236 - DNA, 20 bp, Artificial Sequence
  sgRNA
tctagatgagagagcagtga

SEQ ID NO: 237 - DNA, 20 bp, Artificial Sequence
  sgRNA
gagacagagactcgaatttc

SEQ ID NO: 238 - DNA, 20 bp, Artificial Sequence
  sgRNA
aagaaaactgaaatagcctc

SEQ ID NO: 239 - DNA, 20 bp, Artificial Sequence
  sgRNA
attttggaaactccccttag

SEQ ID NO: 240 - DNA, 20 bp, Artificial Sequence
  sgRNA
gccctttatagggccagttg

SEQ ID NO: 241 - DNA, 20 bp, Artificial Sequence
  sgRNA
ttatgataccggccaatgct

SEQ ID NO: 242 - DNA, 20 bp, Artificial Sequence
  sgRNA
tggccgcgggcggaggggcg

SEQ ID NO: 243 - DNA, 20 bp, Artificial Sequence
  sgRNA
gggcgtggccgcgggcggag

SEQ ID NO: 244 - DNA, 20 bp, Artificial Sequence
  sgRNA
gaaaggctctgggctgggaa

SEQ ID NO: 245 - DNA, 20 bp, Artificial Sequence
  sgRNA
cgcagagtcacggggacgag

SEQ ID NO: 246 - DNA, 20 bp, Artificial Sequence
  sgRNA
aaagcggagagagatccgag

SEQ ID NO: 247 - DNA, 20 bp, Artificial Sequence
  sgRNA
agagaaacaacaccacagcc

SEQ ID NO: 248 - DNA, 20 bp, Artificial Sequence
  sgRNA
ctttgtcatgtttgtggatg

SEQ ID NO: 249 - DNA, 20 bp, Artificial Sequence
  sgRNA
ccaagcaagagcactgtccc

SEQ ID NO: 250 - DNA, 20 bp, Artificial Sequence
  sgRNA
tccaaataacttctgccggc

SEQ ID NO: 251 - DNA, 20 bp, Artificial Sequence
  sgRNA
tttgtagtcattctcatcag

SEQ ID NO: 252 - DNA, 20 bp, Artificial Sequence
  sgRNA
gctttacactcatgctccga

SEQ ID NO: 253 - DNA, 20 bp, Artificial Sequence
  sgRNA
cccggcgggccccgcgcgcc

SEQ ID NO: 254 - DNA, 20 bp, Artificial Sequence
  sgRNA
gcgcggcgaagcgcggcggc

SEQ ID NO: 255 - DNA, 20 bp, Artificial Sequence
  sgRNA
gccccttcccgacaggcccc

SEQ ID NO: 256 - DNA, 20 bp, Artificial Sequence
  sgRNA
ccggcatgcagcggggctcc

SEQ ID NO: 257 - DNA, 20 bp, Artificial Sequence
  sgRNA
gaggtctcggcgaagcggcg

SEQ ID NO: 258 - DNA, 20 bp, Artificial Sequence
  sgRNA
ggtgtgcggctgcgcagact

SEQ ID NO: 259 - DNA, 20 bp, Artificial Sequence
  sgRNA
taacgcgagagcgcgcgggg

SEQ ID NO: 260 - DNA, 20 bp, Artificial Sequence
  sgRNA
gaaggcgacggccccgcccc

SEQ ID NO: 261 - DNA, 20 bp, Artificial Sequence
  sgRNA
cccgtatccgactccacccc

SEQ ID NO: 262 - DNA, 20 bp, Artificial Sequence
  sgRNA
ggtggactcactgcctctcc

SEQ ID NO: 263 - DNA, 20 bp, Artificial Sequence
  sgRNA
cattttctgccccaaattcc

SEQ ID NO: 264 - DNA, 20 bp, Artificial Sequence
  sgRNA
tgcacgggggttactctgga

SEQ ID NO: 265 - DNA, 20 bp, Artificial Sequence
  sgRNA
gaggcgtaggcgtcaccagt

SEQ ID NO: 266 - DNA, 20 bp, Artificial Sequence
  sgRNA
agatcgatccggagtcccga

SEQ ID NO: 267 - DNA, 20 bp, Artificial Sequence
  sgRNA
tgttctctaaagaatttctc

SEQ ID NO: 268 - DNA, 20 bp, Artificial Sequence
  sgRNA
gaccacaaacttgattgtgc

SEQ ID NO: 269 - DNA, 20 bp, Artificial Sequence
  sgRNA
aaaccctagtctcagatcca

SEQ ID NO: 270 - DNA, 20 bp, Artificial Sequence
  sgRNA
tttctctcctaaactctgat

SEQ ID NO: 271 - DNA, 20 bp, Artificial Sequence
  sgRNA
tccctctgctcctctttttt

SEQ ID NO: 272 - DNA, 20 bp, Artificial Sequence
  sgRNA
ctgcaacatgggacttcccc

SEQ ID NO: 273 - DNA, 20 bp, Artificial Sequence
  sgRNA
ttattgtagcctccaagtta

SEQ ID NO: 274 - DNA, 20 bp, Artificial Sequence
  sgRNA
gttgacttagcaaaacctgc

SEQ ID NO: 275 - DNA, 20 bp, Artificial Sequence
  sgRNA
tcggtccccaacttgagcac

SEQ ID NO: 276 - DNA, 20 bp, Artificial Sequence
  sgRNA
gggttaggggcatgcaggaa

SEQ ID NO: 277 - DNA, 20 bp, Artificial Sequence
  sgRNA
tggacttgtcagcgcctgcc

SEQ ID NO: 278 - DNA, 20 bp, Artificial Sequence
  sgRNA
tttcactgtttagcgttgcg

SEQ ID NO: 279 - DNA, 20 bp, Artificial Sequence
  sgRNA
tttctctcacactaaaagaa

SEQ ID NO: 280 - DNA, 20 bp, Artificial Sequence
  sgRNA
ctggaacaatgatgtgagct

SEQ ID NO: 281 - DNA, 20 bp, Artificial Sequence
  sgRNA
ttccgttcctcattgactat

SEQ ID NO: 282 - DNA, 20 bp, Artificial Sequence
  sgRNA
tagttccttgccatatccta

SEQ ID NO: 283 - DNA, 20 bp, Artificial Sequence
  sgRNA
aaacagtcagcaaaacactg

SEQ ID NO: 284 - DNA, 20 bp, Artificial Sequence
  sgRNA
tcggtccccaacttgagcac

SEQ ID NO: 285 - DNA, 20 bp, Artificial Sequence
  sgRNA
gggttaggggcatgcaggaa

SEQ ID NO: 286 - DNA, 20 bp, Artificial Sequence
  sgRNA
tggacttgtcagcgcctgcc

SEQ ID NO: 287 - DNA, 20 bp, Artificial Sequence
  sgRNA
tttcactgtttagcgttgcg

SEQ ID NO: 288 - DNA, 20 bp, Artificial Sequence
  sgRNA
gccgggagtgaggcaggaag

SEQ ID NO: 289 - DNA, 20 bp, Artificial Sequence
  sgRNA
gctactcaggggccaggggc

SEQ ID NO: 290 - DNA, 20 bp, Artificial Sequence
  sgRNA
gcgggacttggcgccggctg

SEQ ID NO: 291 - DNA, 20 bp, Artificial Sequence
  sgRNA
tgttggttgggcgggaggtg

SEQ ID NO: 292 - DNA, 20 bp, Artificial Sequence
  sgRNA
cgatgcccacgccggccaac

SEQ ID NO: 293 - DNA, 20 bp, Artificial Sequence
  sgRNA
tcttcgtggagtgtgaagat

SEQ ID NO: 294 - DNA, 20 bp, Artificial Sequence
  sgRNA
accgtcccatacgcccccta

SEQ ID NO: 295 - DNA, 20 bp, Artificial Sequence
  sgRNA
atgtcggggcttgcgcggga

SEQ ID NO: 296 - DNA, 20 bp, Artificial Sequence
  sgRNA
acttggctccctgccttccc

SEQ ID NO: 297 - DNA, 20 bp, Artificial Sequence
  sgRNA
gtactgactgataacctccc

SEQ ID NO: 298 - DNA, 20 bp, Artificial Sequence
  sgRNA
acacgcatacacaacatttt

SEQ ID NO: 299 - DNA, 20 bp, Artificial Sequence
  sgRNA
tacagacttgtatgtttcca

SEQ ID NO: 300 - DNA, 20 bp, Artificial Sequence
  sgRNA
taataggagacactctcctt

SEQ ID NO: 301 - DNA, 20 bp, Artificial Sequence
  sgRNA
agctgcttggctacaaaagg

SEQ ID NO: 302 - DNA, 20 bp, Artificial Sequence
  sgRNA
ttggaaggccggaaacggaa

SEQ ID NO: 303 - DNA, 20 bp, Artificial Sequence
  sgRNA
ggcggggaggggttgggggc

SEQ ID NO: 304 - DNA, 20 bp, Artificial Sequence
  sgRNA
atgtctcctgcctgaaggtc

SEQ ID NO: 305 - DNA, 20 bp, Artificial Sequence
  sgRNA
caggatgcaggcagtggccc

SEQ ID NO: 306 - DNA, 20 bp, Artificial Sequence
  sgRNA
caactgcctccacccacttt

SEQ ID NO: 307 - DNA, 20 bp, Artificial Sequence
  sgRNA
atgtccggccggtcgagggg

SEQ ID NO: 308 - DNA, 20 bp, Artificial Sequence
  sgRNA
tcagactggcagcggttgga

SEQ ID NO: 309 - DNA, 20 bp, Artificial Sequence
  sgRNA
ggcaactctgaggctcaccc

SEQ ID NO: 310 - DNA, 20 bp, Artificial Sequence
  sgRNA
gggacttgagcaattggcga

SEQ ID NO: 311 - DNA, 20 bp, Artificial Sequence
  sgRNA
caggggcgggcccaagggct

SEQ ID NO: 312 - DNA, 20 bp, Artificial Sequence
  sgRNA
gtcaggttggtttgagaggc

SEQ ID NO: 313 - DNA, 20 bp, Artificial Sequence
  sgRNA
cggaacgctgggttcccaga

SEQ ID NO: 314 - DNA, 20 bp, Artificial Sequence
  sgRNA
gtggtgaggccaatagaaat

SEQ ID NO: 315 - DNA, 20 bp, Artificial Sequence
  sgRNA
ggcatagaccaatgacaaag

SEQ ID NO: 316 - DNA, 20 bp, Artificial Sequence
  sgRNA
caatggaaaaagacggccat

SEQ ID NO: 317 - DNA, 20 bp, Artificial Sequence
  sgRNA
tgggtataaaagtgcaaggc

SEQ ID NO: 318 - DNA, 20 bp, Artificial Sequence
  sgRNA
cttcgtcggttcactatgtt

SEQ ID NO: 319 - DNA, 20 bp, Artificial Sequence
  sgRNA
gcggggagaggcaggggagg

SEQ ID NO: 320 - DNA, 20 bp, Artificial Sequence
  sgRNA
ggggagaggcaggggaggcg

SEQ ID NO: 321 - DNA, 20 bp, Artificial Sequence
  sgRNA
gagggagaagggaggtggga

SEQ ID NO: 322 - DNA, 20 bp, Artificial Sequence
  sgRNA
gggagggaaggggatggatg

SEQ ID NO: 323 - DNA, 20 bp, Artificial Sequence
  sgRNA
gcaggggaggctgggatggg

SEQ ID NO: 324 - DNA, 20 bp, Artificial Sequence
  sgRNA
gaggccgggaggggctggga

SEQ ID NO: 325 - DNA, 20 bp, Artificial Sequence
  sgRNA
aaggacagggaagcctggag

SEQ ID NO: 326 - DNA, 20 bp, Artificial Sequence
  sgRNA
actgatagggagggacctgg

SEQ ID NO: 327 - DNA, 20 bp, Artificial Sequence
  sgRNA
gcggggcgcggggcggggcg

SEQ ID NO: 328 - DNA, 20 bp, Artificial Sequence
  sgRNA
gggaggaggcactttggctt

SEQ ID NO: 329 - DNA, 20 bp, Artificial Sequence
  sgRNA
gggagggagcgcccccctcc

SEQ ID NO: 330 - DNA, 20 bp, Artificial Sequence
  sgRNA
tgggtctccgcgcccagcgc

SEQ ID NO: 331 - DNA, 20 bp, Artificial Sequence
  sgRNA
agtcccctgcggggtcgcgg

SEQ ID NO: 332 - DNA, 20 bp, Artificial Sequence
  sgRNA
gccccgcaagaagggacgcg

SEQ ID NO: 333 - DNA, 20 bp, Artificial Sequence
  sgRNA
ggaaagacgataccagcccc

SEQ ID NO: 334 - DNA, 20 bp, Artificial Sequence
  sgRNA
acctggccaccactcgccgc

SEQ ID NO: 335 - DNA, 20 bp, Artificial Sequence
  sgRNA
gggcggggcggggacggggc

SEQ ID NO: 336 - DNA, 20 bp, Artificial Sequence
  sgRNA
ggggcgctgcgcggcggctc

SEQ ID NO: 337 - DNA, 20 bp, Artificial Sequence
  sgRNA
cggcgcccaggtccgcgtcc

SEQ ID NO: 338 - DNA, 20 bp, Artificial Sequence
  sgRNA
cgagaccgccccgggacagg

SEQ ID NO: 339 - DNA, 20 bp, Artificial Sequence
  sgRNA
tcgccagaggagccaggccg

SEQ ID NO: 340 - DNA, 20 bp, Artificial Sequence
  sgRNA
gtgtgcccgtcggccggagg

SEQ ID NO: 341 - DNA, 20 bp, Artificial Sequence
  sgRNA
ggcaggtcggcctgtccgcc

SEQ ID NO: 342 - DNA, 20 bp, Artificial Sequence
  sgRNA
ctgggcagagccgaactttc

SEQ ID NO: 343 - DNA, 20 bp, Artificial Sequence
  sgRNA
ttctcctcccctaggccgcc

SEQ ID NO: 344 - DNA, 20 bp, Artificial Sequence
  sgRNA
gcctccctcaccaccgtgca

SEQ ID NO: 345 - DNA, 20 bp, Artificial Sequence
  sgRNA
gcttttgtagaggctgtggc

SEQ ID NO: 346 - DNA, 20 bp, Artificial Sequence
  sgRNA
caaacaccctgtccaactcc

SEQ ID NO: 347 - DNA, 20 bp, Artificial Sequence
  sgRNA
tagaagaagacggcagcaga

SEQ ID NO: 348 - DNA, 20 bp, Artificial Sequence
  sgRNA
aatggtgcccgagaagagtg

SEQ ID NO: 349 - DNA, 20 bp, Artificial Sequence
  sgRNA
catgaaacaccacgagcacc

SEQ ID NO: 350 - DNA, 20 bp, Artificial Sequence
  sgRNA
ttaaagaaagttagctgggt

SEQ ID NO: 351 - DNA, 20 bp, Artificial Sequence
  sgRNA
gagtttaaactgcaaggaaa

SEQ ID NO: 352 - DNA, 20 bp, Artificial Sequence
  sgRNA
tcaaaatctgtagagaaaag

SEQ ID NO: 353 - DNA, 20 bp, Artificial Sequence
  sgRNA
ttaaatttcttcctcaagtg

SEQ ID NO: 354 - DNA, 20 bp, Artificial Sequence
  sgRNA
gctcatcttaacgtcatgtc

SEQ ID NO: 355 - DNA, 20 bp, Artificial Sequence
  sgRNA
ctccctttgggggtttccca

SEQ ID NO: 356 - DNA, 20 bp, Artificial Sequence
  sgRNA
gacgggggcggggacggggg

SEQ ID NO: 357 - DNA, 20 bp, Artificial Sequence
  sgRNA
ccgcccccgcgcgcccgggc

SEQ ID NO: 358 - DNA, 20 bp, Artificial Sequence
  sgRNA
gcgcacgcggcgagggcggc

SEQ ID NO: 359 - DNA, 20 bp, Artificial Sequence
  sgRNA
ccccgcgtgacgcccagcgc

SEQ ID NO: 360 - DNA, 20 bp, Artificial Sequence
  sgRNA
cgacgcgaactcggggcgcc

SEQ ID NO: 361 - DNA, 20 bp, Artificial Sequence
  sgRNA
gggtctcgcgcgccccctcc

SEQ ID NO: 362 - DNA, 20 bp, Artificial Sequence
  sgRNA
cgctttcgcttccccagcca

SEQ ID NO: 363 - DNA, 20 bp, Artificial Sequence
  sgRNA
aggcgagtgagactcattgc

SEQ ID NO: 364 - DNA, 20 bp, Artificial Sequence
  sgRNA
ggctccagttccgctgtctg

SEQ ID NO: 365 - DNA, 20 bp, Artificial Sequence
  sgRNA
ttcattctgggctgggccgc

SEQ ID NO: 366 - DNA, 20 bp, Artificial Sequence
  sgRNA
tacagtgcgaaccagagttc

SEQ ID NO: 367 - DNA, 20 bp, Artificial Sequence
  sgRNA
tctcgcgcgccccctcccgg

SEQ ID NO: 368 - DNA, 20 bp, Artificial Sequence
  sgRNA
agtaaaatacagttgtctca

SEQ ID NO: 369 - DNA, 20 bp, Artificial Sequence
  sgRNA
aggcgagtgagactcattgc

SEQ ID NO: 370 - DNA, 20 bp, Artificial Sequence
  sgRNA
gctccagttccgctgtctgc

SEQ ID NO: 371 - DNA, 20 bp, Artificial Sequence
  sgRNA
tacagtgcgaaccagagttc

SEQ ID NO: 372 - DNA, 20 bp, Artificial Sequence
  sgRNA
cggcgccgccaggaggcgcc

SEQ ID NO: 373 - DNA, 20 bp, Artificial Sequence
  sgRNA
ggaggcagggagaggcgaga

SEQ ID NO: 374 - DNA, 20 bp, Artificial Sequence
  sgRNA
ttcccaccccagcctcaggg

SEQ ID NO: 375 - DNA, 20 bp, Artificial Sequence
  sgRNA
aaagcagccccgcagcaccc

SEQ ID NO: 376 - DNA, 20 bp, Artificial Sequence
  sgRNA
ggctgcctcgtcacttgtct

SEQ ID NO: 377 - DNA, 20 bp, Artificial Sequence
  sgRNA
actggtgcaagtggaaaggc

SEQ ID NO: 378 - DNA, 20 bp, Artificial Sequence
  sgRNA
gcgcggcgctaacgtgtgta

SEQ ID NO: 379 - DNA, 20 bp, Artificial Sequence
  sgRNA
agcgcagcgcgacgtgcgcc

SEQ ID NO: 380 - DNA, 20 bp, Artificial Sequence
  sgRNA
ctcttccaggaagcgtggcc

SEQ ID NO: 381 - DNA, 20 bp, Artificial Sequence
  sgRNA
cgcccactcctccgtcctat

SEQ ID NO: 382 - DNA, 20 bp, Artificial Sequence
  sgRNA
tagactcacactcctaagga

SEQ ID NO: 383 - DNA, 20 bp, Artificial Sequence
  sgRNA
gcgcactgaggtttcgcgta

SEQ ID NO: 384 - DNA, 20 bp, Artificial Sequence
  sgRNA
gcattgcggagctcgctagt

SEQ ID NO: 385 - DNA, 20 bp, Artificial Sequence
  sgRNA
cgttatcccttttttccggc

SEQ ID NO: 386 - DNA, 20 bp, Artificial Sequence
  sgRNA
tgaaagggagaagtgaaagt

SEQ ID NO: 387 - DNA, 20 bp, Artificial Sequence
  sgRNA
atggtcctctctctattcag

SEQ ID NO: 388 - DNA, 20 bp, Artificial Sequence
  sgRNA
gaagactttgctctgtgcat

SEQ ID NO: 389 - DNA, 20 bp, Artificial Sequence
  sgRNA
tatttttcacctgcactcaa

SEQ ID NO: 390 - DNA, 20 bp, Artificial Sequence
  sgRNA
caactagggaatttagaaaa

SEQ ID NO: 391 - DNA, 20 bp, Artificial Sequence
  sgRNA
actgactcaggccccgcccc

SEQ ID NO: 392 - DNA, 20 bp, Artificial Sequence
  sgRNA
atccaaaggaaggaggccgg

SEQ ID NO: 393 - DNA, 20 bp, Artificial Sequence
  sgRNA
agacgacccaggcgtccctg

SEQ ID NO: 394 - DNA, 20 bp, Artificial Sequence
  sgRNA
aggaccttgcctgcaagtcc

SEQ ID NO: 395 - DNA, 20 bp, Artificial Sequence
  sgRNA
gtctctacttcccatacagc

SEQ ID NO: 396 - DNA, 20 bp, Artificial Sequence
  sgRNA
gtagggattggactttctga

SEQ ID NO: 397 - DNA, 20 bp, Artificial Sequence
  sgRNA
gtctgtagcagactgtctac

SEQ ID NO: 398 - DNA, 20 bp, Artificial Sequence
  sgRNA
ttccaatccaaaatcctgca

SEQ ID NO: 399 - DNA, 20 bp, Artificial Sequence
  sgRNA
acccgcagcaagcaccacca

SEQ ID NO: 400 - DNA, 20 bp, Artificial Sequence
  sgRNA
taaacttgcccaaagccatg

SEQ ID NO: 401 - DNA, 20 bp, Artificial Sequence
  sgRNA
gtggcactggaccaagctgg

SEQ ID NO: 402 - DNA, 20 bp, Artificial Sequence
  sgRNA
tcttgaacacaaatgaatct

SEQ ID NO: 403 - DNA, 20 bp, Artificial Sequence
  sgRNA
caaggtttctctcctatcat

SEQ ID NO: 404 - DNA, 20 bp, Artificial Sequence
  sgRNA
tgtgctcttgaagaggggag

SEQ ID NO: 405 - DNA, 20 bp, Artificial Sequence
  sgRNA
ctccttccttcgtttacaga

SEQ ID NO: 406 - DNA, 20 bp, Artificial Sequence
  sgRNA
gtgcattctctagcagggta

SEQ ID NO: 407 - DNA, 20 bp, Artificial Sequence
  sgRNA
aacttggtttctgttgtagg

SEQ ID NO: 408 - DNA, 20 bp, Artificial Sequence
  sgRNA
ggggaggtcttctgagccac

SEQ ID NO: 409 - DNA, 20 bp, Artificial Sequence
  sgRNA
agctgcaccttctttcagcg

SEQ ID NO: 410 - DNA, 20 bp, Artificial Sequence
  sgRNA
cccagcaaggactcattatc

SEQ ID NO: 411 - DNA, 20 bp, Artificial Sequence
  sgRNA
ttgaacaggaaggcgttttg